European Patent Application EP 4 119 569 A1, published January 18, 2023. Title: CONJUGATED ANTISENSE COMPOUNDS FOR USE IN THERAPY. Applicant: Ionis Pharmaceuticals, Inc. The sequence listing filed with the application follows.

SEQUENCE LISTING (13 sequences)

SEQ ID NO: 1 - DNA, 6489 bp, Homo sapiens
aggtacctttggggctggctttctcaaggaagcccagctccctgtgattgagaatgaagtgtgcaatcgctatgactgggattgggacacactttctgggcactgctggccagtcccaaaatggaacataaggaagtggttcttctacttcttttatttctgaaatcagcagcacctgagcaaagccatgtggtccaggattgctaccatggtgatggacagagttatcgaggcacgtactccaccactgtcacaggaaggacctgccaagcttggtcatctatgacaccacatcaacataataggaccacagaaaactacccaaatgctggcttgatcatgaactactgcaggaatccagatgctgtggcagctccttattgttatacgagggatcccggtgtcaggtgggagtactgcaacctgacgcaatgctcagacgcagaagggactgccgtcgcgcctccgactgttaccccggttccaagcctagaggctccttccgaacaagcaccgactgagcaaaggcctggggtgcaggagtgctaccatggtaatggacagagttatcgaggcacatactccaccactgtcacaggaagaacctgccaagcttggtcatctatgacaccacactcgcatagtcggaccccagaatactacccaaatgctggcttgatcatgaactactgcaggaatccagatgctgtggcagctccttattgttatacgagggatcccggtgtcaggtgggagtactgcaacctgacgcaatgctcagacgcagaagggactgccgtcgcgcctccgactgttaccccggttccaagcctagaggctccttccgaacaagcaccgactgagcaaaggcctggggtgcaggagtgctaccatggtaatggacagagttatcgaggcacatactccaccactgtcacaggaagaacctgccaagcttggtcatctatgacaccacactcgcatagtcggaccccagaatactacccaaatgctggcttgatcatgaactactgcaggaatccagatgctgtggcagctccttattgttatacgagggatcccggtgtcaggtgggagtactgcaacctgacgcaatgctcagacgcagaagggactgccgtcgcgcctccgactgttaccccggttccaagcctagaggctccttccgaacaagcaccgactgagcagaggcctggggtgcaggagtgctaccacggtaatggacagagttatcgaggcacatactccaccactgtcactggaagaacctgccaagcttggtcatctatgacaccacactcgcatagtcggaccccagaatactacccaaatgctggcttgatcatgaactactgcaggaatccagatgctgtggcagctccttattgttatacgagggatcccggtgtcaggtgggagtactgcaacctgacgcaatgctcagacgcagaagggactgccgtcgcgcctccgactgttaccccggttccaagcctagaggctccttccgaacaagcaccgactgagcaaaggcctggggtgcaggagtgctaccatggtaatggacagagttatcgaggcacatactccaccactgtcacaggaagaacctgccaagcttggtcatctatgacaccacactcgcatagtcggaccccagaatactacccaaatgctggcttgatcatgaactactgcaggaatccagatgctgtggcagctccttattgttatacgagggatcccggtgtcaggtgggagtactgcaacctgacgcaatgctcagacgcagaagggactgccgtcgcgcctccgactgttaccccggttccaagcctagaggctccttccgaacaagcaccgactgagcaaaggcctggggtgcaggagtgctaccatggtaatggacagagttatcgaggcacatactccaccactgtcacaggaagaacctgccaagcttggtcatctatgacaccacactcgcatagtcggaccccagaatactacccaaatgctggcttgatcatgaactactgcaggaatccagatgctgtggcagctccttattgttatacgagggatcccggtgtcaggtgggagtactgcaacctgacgcaatgctcagacgcagaagggactgccgtcgcgcctccgactgttaccccggttccaagcctagaggctccttccgaacaagcaccgactgagcaaaggcctggggtgcaggagtgctaccatggtaatggacagagttatcgaggcacatactccaccactgtcacaggaagaacctgccaagcttggtcatctatgacaccacactcgcatagtcggaccccagaatactacccaaatgctggcttgatcatgaactactgcaggaatccagatgctgtggcagctccttattgttatacgagggatcccggtgtcaggtgggagtactgcaacctgacgcaatgctcagacgcagaagggactgccgtcgcgcctccgactgttaccccggttccaagcctagaggctccttccgaacaagcaccgactgagcagaggcctggggtgcaggagtgctaccacggtaatggacagagttatcgaggcacatactccaccactgtcactggaagaacctgccaagcttggtcatctatgacaccacactcgcatagtcggaccccagaatactacccaaatgctggcttgatcatgaactactgcaggaatccagatcctgtggcagccccttattgttatacgagggatcccagtgtcaggtgggagtactgcaacctgacacaatgctcagacgcagaagggactgccgtcgcgcctccaactattaccccgattccaagcctagaggctccttctgaacaagcaccaactgagcaaaggcctggggtgcaggagtgctaccacggaaatggacagagttatcaaggcacatacttcattactgtcacaggaagaacctgccaagcttggtcatctatgacaccacactcgcatagtcggaccccagcatactacccaaatgctggcttgatcaagaactactgccgaaatccagatcctgtggcagccccttggtgttatacaacagatcccagtgtcaggtgggagtactgcaacctgacacgatgctcagatgcagaatggactgccttcgtccctccgaatgttattctggctccaagcctagaggctttttttgaacaagcactgactgaggaaacccccggggtacaggactgctactaccattatggacagagttaccgaggcacatactccaccactgtcacaggaagaacttgccaagcttggtcatctatgacaccacaccagcatagtcggaccccagaaaactacccaaatgctggcctgaccaggaactactgcaggaatccagatgctgagattcgcccttggtgttacaccatggatcccagtgtcaggtgggagtactgcaacctgacacaatgcctggtgacagaatcaagtgtccttgcaactctcacggtggtcccagatccaagcacagaggcttcttctgaagaagcaccaacggagcaaagccccggggtccaggattgctaccatggtgatggacagagttatcgaggctcattctctaccactgtcacaggaaggacatgtcagtcttggtcctctatgacaccacactggcatcagaggacaacagaatattatccaaatggtggcctgaccaggaactactgcaggaatccagatgctgagattagtccttggtgttataccatggatcccaatgtcagatgggagtactgcaacctgacacaatgtccagtgacagaatcaagtgtccttgcgacgtccacggctgtttctgaacaagcaccaacggagcaaagccccacagtccaggactgctaccatggtgatggacagagttatcgaggctcattctccaccactgttacaggaaggacatgtcagtcttggtcctctatgacaccacactggcatcagagaaccacagaatactacccaaatggtggcctgaccaggaactactgcaggaatccagatgctgagattcgcccttggtgttataccatggatcccagtgtcagatgggagtactgcaacctgacgcaatgtccagtgatggaatcaactctcctcacaactcccacggtggtcccagttccaagcacagagcttccttctgaagaagcaccaactgaaaacagcactggggtccaggactgctaccgaggtgatggacagagttatcgaggcacactctccaccactatcacaggaagaacatgtcagtcttggtcgtctatgacaccacattggcatcggaggatcccattatactatccaaatgctggcctgaccaggaactactgcaggaatccagatgctgagattcgcccttggtgttacaccatggatcccagtgtcaggtgggagtactgcaacctgacacgatgtccagtgacagaatcgagtgtcctcacaactcccacagtggccccggttccaagcacagaggctccttctgaacaagcaccacctgagaaaagccctgtggtccaggattgctaccatggtgatggacggagttatcgaggcatatcctccaccactgtcacaggaaggacctgtcaatcttggtcatctatgataccacactggcatcagaggaccccagaaaactacccaaatgctggcctgaccgagaactactgcaggaatccagattctgggaaacaaccctggtgttacacaaccgatccgtgtgtgaggtgggagtactgcaatctgacacaatgctcagaaacagaatcaggtgtcctagagactcccactgttgttccagttccaagcatggaggctcattctgaagcagcaccaactgagcaaacccctgtggtccggcagtgctaccatggtaatggccagagttatcgaggcacattctccaccactgtcacaggaaggacatgtcaatcttggtcatccatgacaccacaccggcatcagaggaccccagaaaactacccaaatgatggcctgacaatgaactactgcaggaatccagatgccgatacaggcccttggtgttttaccatggaccccagcatcaggtgggagtactgcaacctgacgcgatgctcagacacagaagggactgtggtcgctcctccgactgtcatccaggttccaagcctagggcctccttctgaacaagactgtatgtttgggaatgggaaaggataccggggcaagaaggcaaccactgttactgggacgccatgccaggaatgggctgcccaggagccccatagacacagcacgttcattccagggacaaataaatgggcaggtctggaaaaaaattactgccgtaaccctgatggtgacatcaatggtccctggtgctacacaatgaatccaagaaaactttttgactactgtgatatccctctctgtgcatcctcttcatttgattgtgggaagcctcaagtggagccgaagaaatgtcctggaagcattgtaggggggtgtgtggcccacccacattcctggccctggcaagtcagtctcagaacaaggtttggaaagcacttctgtggaggcaccttaatatccccagagtgggtgctgactgctgctcactgcttgaagaagtcctcaaggccttcatcctacaaggtcatcctgggtgcacaccaagaagtgaacctcgaatctcatgttcaggaaatagaagtgtctaggctgttcttggagcccacacaagcagatattgccttgctaaagctaagcaggcctgccgtcatcactgacaaagtaatgccagcttgtctgccatccccagactacatggtcaccgccaggactgaatgttacatcactggctggggagaaacccaaggtacctttgggactggccttctcaaggaagcccagctccttgttattgagaatgaagtgtgcaatcactataagtatatttgtgctgagcatttggccagaggcactgacagttgccagggtgacagtggagggcctctggtttgcttcgagaaggacaaatacattttacaaggagtcacttcttggggtcttggctgtgcacgccccaataagcctggtgtctatgctcgtgtttcaaggtttgttacttggattgagggaatgatgagaaataattaattggacgggagacagagtgaagcatcaacctacttagaagctgaaacgtgggtaaggatttagcatgctggaaataatagacagcaatcaaacgaagacactgttcccagctaccagctatgccaaaccttggcatttttggtatttttgtgtataagcttttaaggtctgactgacaaattctgtattaaggtgtcatagctatgacatttgttaaaaataaactctgcacttattttgatttga

SEQ ID NO: 2 - DNA, 150001 bp, Homo sapiens
atctttcagcctctatattattttattgtgatttttaatttccttgaattggattttgccattgtgctaaatcttgatgatcttcatttgtatccgtagtctgaattatatttctgtcatttgagttagctcagtcttgttaagaacccttgttggaaaactggtgcagttgtttggaggacatatgaccttctggccatttgatttattggagttcttacgttggttctttctcatgtctctgtgtgggtgtttctttaactgcagtgtagattgagtacagccaatagacttcttctttggaggttttcacagggccaaggccttgtacagggtctttatttgtagctgacttcttgtctttggtttcatagtggggcatgttagcaaaatagttttgctgttgaagttttggggtgtgatccattttttattttaatgattgtgtatttcctttatacctaaaacaagcagaaaaccagtaaaggtctttgagtctctgaattcataactccagcattcatattgcttcctcaggtaagtggggttttcacccagcccttaagggtgttagattattttttatgtgaaattagccagattgtatttctaaacatgatgtaaaacaataatgacaaaagttataataaactagccttcttaccaaatccacatgtctaatgtgtgtgggagggtgttaggcaggggacctgcagctaagggagaggcagacaggccccatggccccaaatctaggatagtatttggtattggttgatgggtgagagaaagagagggaacatctgtgcaggatgtggtatcagcacctggactacatcttagggattccttcttcatttttcagtatgccctgacaataattatatctatcagacttacccccttgaccactggaacactaagactgttttgggatctctgcctgactttctcagaggtgctggtgaggacattatgagtctggaacctagaaaagcgttctgactctgctgactttctcagaggtgctggtgaggacattatgagtctggagccctagaaaagcgttctgactctgccactagccagacagacctggactaggcacgttaactctttgtatgacttgactccaacccctcatttgtaaaaccagcattttcaagtggtgttttccacatcagccttttgcataagctgtcatttgaagaaaggtttttgtttgtttgttttttgtttaacaaaaaggttaaaaaccactggtctagataattgcaaagtttgctttcctttttctgtgctttttctactatttttaaaatgtcatcctccttggtttcttgatccccctttctgcactcctgagtctgggaacactgaggccaactaaaaggaaacttggcaaaagaggaacacctttgggtgtgccaggctgctcccagtgttttgcacttataaaaatttaaatgctgcaaacctctaagacttagatattattgttcctattttacaagtgaggaacctgaggctcagagaaggtgcaggatggcacagggagacctgaattggaaccctggttcccacttactggctgtcgggacttagaaaagtcatgaactctcattgattgttttcttatatgaaatgggggctgcagggttgtcgggggagaaacaataagaatgtgcatcaagtgtcgagcacgtgctacgcactccatcatggcagctcctactaatatacagaatagagttgtatctaacatgactctttcttgcaagtgacagaaaatccaacttaagatggattaagcaaaaaaggggaattcttgttgagctgaaaagtctttaggctcacatgatggccccagggcccaggccctgtccagccatgcagtaggcatcatccttgggcacaaaggtgagattcttgtggtggcagatgctgtggcagctcttgctttgccaggaaagactgaggaaggccactgtccccattaagtgaacaatagttggccaggtctgagaggttgaacttgggtcacaggcctgtccctgaacccatcactgattggctccaacctgcatcagctattacatgctagaggtggaggcaggaccccactcatacccagaagggcaaagggtggatccctcaacaggattatgggatgtagggtgatagactgctgggcagccagaaagcaaacagatcctctccaatacctcaactgatgaaagcaccaagctaaaatcataaggatctgggtgtgaattctggctctaccatcttccatgtgacattgggcagttatttaatctcttttagccttggctttcttacctgtactaacatataaggtgattgtgatgagcatcatcatcgtcaacatcatcatcaccatccacattgccaccaccactcccattatcatcttcatcaacatcatcaccaccgccaccatcaccattatcattaccaccaccgctatcactattatcatcaccctcaacatcatcaccatcatcactatcatcaccaccaccatcatcgttactaccactaccaccaccatcatcaccacagccaccaccaccatcaccatcattactactcagcaccaccatcatcattccaccaccatcaccatcattccaccatcaccattatcattaccaccaccactgtcactattatcatcaccctcaacatcatcaccaccaccatcatcattactaccaccaccaccaccatcaccatcatcatcattctaccaccatcaccattatcatcaccatcaccatcaccaccgctatcatcatgataatcattatcattaccaccaccattagcattatcattaccaccaccatcactatcactatcaccatcaccacgaccactaccaccatcaccaacaccatcattactacccaccaccaccatcatcatcattccaccaccatcacaattattaccaccaccaccatcaccaccaccaccaccatcactatcatcatcagtagacatcatataaccagtttgtagctggcccagagcctacttgctgtttcttctgccccacaaccatccacacatttctaaccaccatcccccactaggcttctgcctcgcctggtctcacctgcaggtccactgagaaaatgattctcagaacactaactagaccatgaggtgccacaaaacataactcaggcctgttcatcaattttctacatgtcaataatgacatcaggtcaattggcgttctcagcctctgagagggaggtcaaagttttcctgctctccccttcatgtttccaggtgttccctgacttggatcaaatgcagagtttggaggtgttgaggccaaggggattttccaggtcagtcgtcatccacaatcaatggactgatcctgccgctggacttaccctgctgccctctccccaaggccccatcagggagggcttcaatcctcttgtcacctgtggcctacctgccctcagagatgacatctctatgtcggccactggatggcagcacctactcgcagaccacatcaactttcctggcaacttgcggtaggttttcaccattatcaggatgtttgccttgctcaaatagcagattctagagaacggtgctccctcacacaactatgtagtccaggtgatgcaccctctgcccgatgcttggtagtcagaaacttccatcatgcagctctgcccagattgagctgagctggcctctggagtgaggtgctgggacaaacatcttccatgctgctcatgtcaactccagatgcagtcaggtttctgaaccaaagtcaatgatctaagtgcagtcaaaggctctgggggaagaaagagagagtgcctcatctcttgcctgtgccatgctcgcaaagcaaggatttttgcaaaattctaatgaaagctgggcttgcaaaattagaaaactggattatttgtgagaacactgaaacatccctgggtgtgtccatctggaaaaacagcatttcctctggcaattttgcaaccgttctatttgaatttggcaaagaaaataaagcagtttttcacaaaagaataaacacaaccaggagaatcttcactctcccaaattgtcaaagaagtataaattagaaaatgaatcaggacaatttcaacctgttagattagctaatatttaaaaattgaacactcatacaagtgtggtgaagtgattgttttctagtgacattttacactgtcataaccttctagaaaataaattggcagtgttattgggagacagaaatatgtctatataatttatgggaacttaggctcagaaaatattaaggaataagaatgaactttatgaacaaagatgtggagggttggaagcaagaggggggccaacgcgcacggggaggaagcatttgggcagtgactccgcagacccaggctcaggttgaactagacaacctccttacacctcagtttccttaactgtagagcaggagtgatggaactgcctgtttcataggactgttgtgaggatgaagtgagatacaccacattataagcttgtgcctggaaaggataatgcttagtaaatgatgactattcttttttattgcaataaaatgtacacagcgtaagagttactattttaaccatttttgcagggtaccaccaagtggcatttagtacattcacagtggtgtgcaaccatcatcatatttccagaatattttcctcatccccaaaggaaacctcatgctcattaatcagtagctctcctttaaaatattagttatgaagatcatagcactatacaaaactcattatgtaatgttgagtgaaaaaatcagggtgtgaaattttgtgatatgatgtaattagtgaaagaagcatacaaaaagtctgaaaatataaaaacaatagcaattgcatttctcagactctacatttaaacattattctttatggttttaaaagcaaagaaaaaggtaaagaaacaacaaccaaccgcaaagcaccatgacaaagctcagattgttaaatccaggtttttggaacatagactcttatatgacgtttacactctccagggttcagagagtctggcagcattgggagctgccttgtgttctacagcctcacggacagacaggaggtccatcaccactgctctgttcttctggagtttccttgtgaacatgttgtggacgtagttaccatttctttcatctttttaaacacaggtacctttggggctggctttctcaaggaagcccagctccctgtgattgagaatgaagtgtgcaatcgctatgagtttctgaatggaagagtcaaatccactgagctctgtgctgggcatttggctggaggcattgacagttgcaaggtaagaaaagatcaagagaccaaagttagtcttgtgctctcctgtctcagtctcagtcccttagacttgagtcccaaagtagcgaattcaagtaggatttaatcaatggaagaccccagtctaagtgttgctcagaaactccctagatctgtcccaaatgtatattcagatcatccaaggggacttcttggggcttgagttccagatcagcagcaagggagccataagtgccataactacctcagaccactcaccctcctggggtgtcccggtggccagggactaaagtggtgatttttctggtagggaaggaggtagagggtacaggacagagactaactgcacacaatatctgagactggagctcagatattgctgatgatcagagttggcgtgtctccccaattgatttacaactggggcttggatactgttttaaacgggaggagcctcctaaccatcttgacacaaccactgacgtgactacactagagatagactctttccacttaattctaccactcttgctttacttcatgagaacgaaaatgtaagattgcaccatgaattcatttgcggaaagattgatactatgcttttattttattttattttattttattttattttattttattttattgagactctcaccccggttgaagtgcactgacgtgattttggctcactgcaacttccacctcctgggttcaagtgaatactccagcctccctagtagctgggattacaggtgcccaccaccacgcctggctaatttttgtatttttagtagagatggggtttcaccacattggcctggctggtctcaaactcctgaccttgtgatccacctgtcttggcctcccaaagtgctgggattacagagttgagccaccgcactcgaccctatgttttatttttaaaaatatttatttatttatttaagccacaactactagaataggaaggattgatattttattaattttatttggtatttattatttttttttctttcctgagacattcttgctctgtcacccaggctggagtgcagtggcacattcttggctcactgcaacctccatctcctgtgttcaagcaattctagtgcctcagcctacttagtagctgggatgactggcatgtgcctccacacccagctaatttttgtattttttgtagagacagggttttggcatgttgcccaggcttgtctcaaactcctggcctcaggtgatccatctgccgtggcctcccaaaatgctgggattataggcatgagccaccaccccctcctggaaggattgatatcttataacataatttataattacagaaaacatgtgagttcactaggaataaataaattttgaagataataaaagattttcacttatgttgtcatttcggcacagtttggtataggatgtggagatgttaacatttatacctagcttgctcgtaaactaagacctgaaagggttgtgtctatcagctgcacccctgggtagcgacacaacctcgggaaggcctcagccccctcctcgtacagcactgcctgttggaaagcttgagggaggctatggatgtgcagcacttggcagagggtctggtcatggaagttaccagcaaatatgagctacttttatgattttattttatccaaaagaaagagaatgaaagaagaggggaggaaacaagactaatcaggaaagatgaaggtctaggggtgagggaaggagtaaggagacataaaggcaatgtggagcagctgaggggggaaatggctttcaccacttcccagcatctattgacattgcactctcaaatattttataagactctatattcaaggtaatgtttgaaccctgctgagccagtggcatgggtctctgagagaatcattaacttaatttgactatctggtttgtgggtgcgtttactctcatgtaagtcaacaatgtcctgggattgggacacactttctgggcactgctggccagtcccaaaatggaacataaggaagtggttcttctacttcttttatttctgaaatcaggtaagacatagtttttttaaattataagaattattttttctcccacaatgtagtaaaaatacatatgccatggctttatgtgcaattcatttaatttttgattcatgaaattcccagttcaaaatcttgtatatgattgaaaaattcttaaaaaaataagtttaatttccccgtgaagactgtcacggtgctggaatgaatgggcagaaaaaataatggttgatttttctaatctaaaagagtgtgcctacatgatggccagtctggctgaaaaataaatagccattgtagctaactatgcaaaggatggctaagctcttcgcttggttctcagtttcattaatttatatcatctctgttcaggtgccatgctcccctcactagcaagttgaaacaatgaaataactctttgaatatgtttggttccttgacctgttcatggagtgggactcagcatttctctctttgttatggcctgagtaaggctttccatcggtatacatttgcttcttatccctggagaaattatacacatccatttgccagatgatatacgcatataatgattcaacaaatactcagggtatttgttgagtgggttaggtccccacatttttatacatacatacacacatacacaccgtgtgtgattgtgaatgtaagtgtgtgtcctttacaaatactagcttatttagctcatggtataggtagggtagcatagtcatccccattttataaacaaagaaatctagacttaggaaaatcatgttatttgtctcgtgaccaaattcccaaatcaaggaaataaagaaacctggatttaagccagatttccaagaaaaaatctagggctcttctcactttttcatctttgttccaacatttgaaaaaataaatctaaacacattccaatgtaactgaagagcaggttaattgtttgccacttgcagaatccaattaagaagagagaagtctggtataaagaaagtgatttgcttccaaagctagcttaggggaagaaatgcagcagtcctgccgtactacttcactttaggagcagaaagtggcacttttaaaaggcaacagaggaggcgagcaaggattcaggggtccatgctagcttgggcaccttatccaccaggtagttgagcagttgcctgctggtgcctttgtgagcagggtgttgtcccttgaggcaaatctctggagggtgagagttttgtagtgggcatgctttggtttataaatcacctgtgaactcaggagttccatcttgaagcacatacatagttagatgaacttgccctgcagggagagtctgatgaaagggaggtagatgcttgcaatttaatctataaattaccagataaaattttacaagttgactttaaagtcaaacacatttgaatttagtggaagccattcaagaaaatatcaaagaaaatacagagcaggagaagattaagcaaagagttttttggggaaattggtgtctatgtctgtgtgtgtagggagtgcaggggatatgaatattctatttcagcccatggaaactaggatgtagatcactgtgaacttattcagcaggctacacccaaaggctagaacaaacttctctgccacaggattaacatatgttttaatcgacctggggggcacattctctgataagctcttttggaaagccaggctttctgtggacgtgttatctttccaatgtgtgctggaatgcccggggagaggaaaaagtttcttttacagccatgctcagtgagaagcggagaaacatcttctattcacaaattgctaagtcttttacacatgcaaatatgcatacacattcacacaccacagtgaggaagaaattctcacaccattaataaaatacatttacttcagtagcaatatacatctacattttgcctataatataaaagtatttttcctattaaaagatttgtttaatgtttcttcaccaacaaataaaccctattaaatccccattgccatatgagccctggaggtgaatcagagaaacaaaaggattgtggaaaaatcatcaggttaaaaaaagaaaaattgattctgttttgggatatttcctagcaacatgagctggggaggggatctcagcagtgatgctctatgaagcataataaaatgacacagttacaggtaacttagttaaagggggaaataaatggaagtttcctctttttgaatatcaattgtagcctgctctgctacatttcaaaaacactcttcaaaatgtttaactgaactcactgtaggaagcaccttattaatttattgtgtgttttgaagtcacactgtgagctatagaatttacccaagcacaactcttcctggaaaagagagttcaaatgagaaacagtgcggggtgaagacatggatatgggcctaaaatatctatttctcaatgatattttgatatatctatcaagtgctttttagtggattaggttcagaatgcatcagccaatgcctgttcaataatccagttttccagcatagagcatattaaattgaggaaggacaaagtcacagaggtggggagcaggtggactgtggccaaggactttgcatgaaacagtgagcgtgcatcctcctccttgccctgccctcatggtctgtgtactctcaggaggtcaggacaggcctttctgagaatgagaatctgttcatctgcctttctactggatacttgtcatcggcatacaaacacatgttctctgcagtgtgtcatctttcagaacctcccctgaccctgtattccctagaagtctcgctgctttcagagccaggcttctctcctgctgccacccccactgctcttctagtcactctttaacccactccatctgcatgtggcccccaccacacccctcaaagtggtcaaggttgtcctgttgcttaattccatggaagcttggctatcttcattttattagcctcttttggcctctcaccctgtgaaaatcactacattttgtgccagagatggagctggcatctccaggcttggaagagggctgctgaagctcagccaggtgtcctaaggagcctcaggacaggggatgctcagtagccttgcaatgggaacacagctgagccccacttggccaccctttgccacaaccaggcagaaagcagcttttgaacagatttgttgcctcagatttgatctcaaagaaaaatcgtgggcagtattggtcccaggttctgcttttttacaatttcctctgaaatctggatgcctatcaacaccttggaaaaactgaattctccccaactaatagtggtgtgtcactgtagtaagcctagtacaaaaatggccttctttgtggaggagcttcatatcctccattttttttttgcttaatttttgcccaagatgagaacataatttagttcactttttatttattcccaacatcatccatgcaccaacatttttgtaactaaaggagggaccattcagaagatgcttatcaactgtcaaagtgacagtgttacaaccaatgcacatattgtaagaaatcaaacaatggcctccaaggttcatttctacacagggattagcagatcaacatcaatcttggcaacacagttgccactgatggtgtcttattttttttatcatgacatggcaatcaagagcaaacatgatttattcttatttaagattttatggttagactaggcagatagctagatatgagcaggaggtggaagcccctgagagaatggaggtctggagaatctgaaaccccagagattacccaagtcctgcatgctagacatgagtggaggagggggaatacctaggtagaaaagaatgccccttaagatgcccagcagtcgctcactgtgcagttaacttttcagaatgctgctagatacatgctgatagggagggaagagggcaaaggagaaattcctaagagatacacggttgcagttagtatacatctgagtgctatacaaccttctttgggtggtggcaagaagcaatgcagccattacgtagaattcatatcaaacacctgtatcacaggtgttaaagaaacaagaaacattgtacttcttgtattcttaataatgatttgcaatattgtctttagtatcactgcaaacctctataaatatgatttttaaaaagtatttctttaggttggaattacttctacgcattgacttatcttcctgggtttcattagccgtacccgttgtactttcttccttaccactgtttatctcaaactcttgagattaaagtatgggctcaggagggagcgaggagcttcaggactctcacggacctccagcacagtgtagctgccttatggaaaagtggccacactgttttctgcactggtccctgcccctactattcctcactgggcagagcacagccaccctggccctgcctgaacattttagtcagtgttggctctgtgcttctctggggaggaaatccaagagacaacccacagcccctctgccatttcagctgcagcagtaccaccgttaatgcccttgggcttgagaaagaagggacctggccacttccctgacacctccagcacacagcagggaaagaattccagtttctctttcttgtgagctttcacctgctactcttcaccaggcaaggctcctggcttgggcccacagtgcaggcacctcgaactcagttgaacatttccactggctgcactctgtgtttttgtggggtgaagctcccagaggtgactgaaagtccttctgccactaacactgcagtcatactgcccttgctgtacttggactagggaaggaaaaaagatcctgagtgctttactcacaccccagtgtgccccagccaccctatggaaaagaggccagtgtgtcatccctgcaagcaccctgaggcccctgcccctgctgcccccaagctgtagagccagaatataaagctggcagaaaaatgtaaaaaggctagactggcttagcctcccagcctacatctttctcctgtgctggatccttcctgctcttgaacatcggactccaagttcttcagctgtgggacttggactgtcttccttgctcctcagattgcaggtggcctattatgggaccttgtaatcttgtgagttaataccacttaataagctcccctttgtgtgagtatatctatatctatagatagatataggtatactcactatatatacacatatatacatatactctctctctctctctctcatatatatatatatataatctcctattagttctgtccctctagagaaccccgactaatacagattttcataccagaagtggttcttgaggaacagaatattaaggatggaattctttcattggttttgggacttctggtgttggctgattaatatgattagaccaaaaaatgctaaggactctacttctaatagtatggagaacactgatagtacttggcctgaattgtttagagagttatgcaaaataaatgcatttgacactactgattcatcacttatgagaggcaaggagtttagtgactctatacataatacctttgactatatgtggagaaccaaggaacataatgaagttggttgattgctcctaagttctctggagaaagagatgaaagaaaatgatgatctcaggggatctgtctcccaccttcagaagcagatactgagccacaaatctgctaagattgccctgaatgagagttttaactcctgtagagaaagagttgaaattgtgaaaaaacagagacaagctgttatcatgcgagtagctgatctgcaacaagaggtgcatgcacagccttgccaggtgtttactgttaaagtgagggcattgactggaaaaaaatgggaccctggaacttggagtggggatgtgtgggagaaccctgatgaagctgaggacactgagtttgtgaactctgatgaaacttttttgccagaagaaacagtttccccatccccagtagtggtaacatcccctccctgacccgtgctgccattagcctttccacctttgtctgaggatgtaaaccctgcactgcttgaggcaacagtgatggccttccctgaggcagctgccaggcaagataatgttgattctcctcaagaggcacccctaatgcccctgaatgcttctagacctataactaggctaaattccttgcgggccccagaggtgaggttcagagtgtgacccatgaggaggtgcattatactctaaaagaactgcttaagctttctaatttatattggcagaaatctggagaacaggcatgggaatggatattaagggtaagggataatggtggaagggacatagagttggatcaagctgaatttattggtttggccctactaagtagggattctgcatttaatgttgcagctcggggacttagaaaaggttctgatagggccgggagcagtggctcacgcctgtaatcccagcaccttgggaggcgggggcgggcagatcacgagatcaggagattgagacaattctggctaaaatggtgaaaccccatctctgctaaaaatacaaaaattagctgggcatggtgatgcgtaactgtaatctcatctacttgggaggctgaggcaagagaactgcttgaacctgtgaggcagagattgcagtgagccaagatcgccccactgcattccagcctggtaacagagcaagactccatttccaaaaaaaaaaaaaaaaaagttataatagtttatttgcttggttagctgaaatatggattaaaagatggtccaatgttagtgagctggaaatgccttggtttaatgtagaggaagtgatccaaaggcttagggagattaggatggtggagtggattagtcactttagacctactcatcccagctgggagggtccagaagatacacccttggccgaagctttgtgaaatagatttgtgagagcagcacctgtatttttgaagagcccgtaattgctcttctctgtatgtcagatctaacagtaggaaccacagtcactcaactacaaaatttaaatacaatgggaataattggatcctgaggtggcaggggccaagtgttggcactgaaccatcaaaggcaaggtgggcataactaccataatagacagcagaggcaaagcagccatcagaatagtctgactcatgtagagctctggcattggctaattaatcatggtgttcctagaagtgaaattgatgggaaacctactgtattcctacttgatttatataaacaaaaaactgccaggtagaatggactaaagactaatctgaattataaaaacagagaatcatgggccctcaatcaatttccagactcgaacctgttacagttccagaacccactgaatgaaggggaggctggatccccttgaggaaggacaccactaggctactgacaacttatgctgttactctttctcccatccttccctaaggagacctctggccttttaccagggtaactgtgtgtactggagaaagggaagtaatgagacatttcagaaagtactggacactggctctgagctgacgttgattccagggtacccaaaacgttattgtggttccccagttaaagtaggggcttatggaggttaggtaattaatggagttttagctcatttctgacttacagtggttccagtgggtccctggacttatcctctggtcattttcccagtgccaaaatgcataatttgtatagacatacttattagctggcagaaatgccacattggctccctgactggtaggatgagggctattatggtgggaaaggccaaacagaagccattagagctgtctctacctagaaaaataaaaaaatcaaaaacaatatcccatccctggagggactgaagtgattagtgtcaccatcaaggacttgaaagacgcaggggtggtgattcccaccacatccctgttcaactctcccatttgacctgtgcagaggacagatggatcttggaaaatgatggtggattattttaagcttaaccaagtggtgactccaattgcagctgctctaccagttgtggttttgttgcttgagcaaattaacacatctcctggtgcctggtatgcagccattggcttggcaagtggctttttctccattcctgtccataagacccaccagaagcaatttgccttcagctgacaaggccagcattatacctttaccaccctacctcaggggtgtatcaactctccagctttgtgtcataatcttatttggagagaccttgctcgcttttcacttccacgagatataacactggtccattacattcatgacattatgatgattggatacagtgagcaagaagtagcaaacacactgaacttattggtgagacatttgtatgccagaggatgggaaataaatccagctaaaatttagggactttctacctcggtaaaatttctagggttccagtggcatgagacctatggagatattccttctaaggtgaagcataacttgctgcgtttggcccctcttacaaccaagaaagaggcacaatgcctggtgggcctatttggattttggaggcaacacattcctcgtttgggtgtgttactctggcccatttatcgagtgacctgaaaggctgccagatttaagtgcagtctagaacaaaagaaggctctgaaacaggtccaggctgctgtgaaagctgctctgccatttgggccacatgaccccgcagatccaatggtgcttgaggtgtcagtggcagatagggatgctgtttggagcctttggcaggcccccataggtgaatcacagtggagacctctaggattttggagcaaggccctgccacttctgcagataactactctccttttgagagacagctattggtctgttattgggctttggtggtaactgaacgtttgactgtgggtcataaagtcaccatgctacctgaacctgcctatcatgaactggttgctttctgacccatctagccatgaagtgggtcagcacagcggcatttcatcatcaaattgaagtggtgtgtatgtgatcgggcttgagcaggtcctgaaggcacaagtaagttacataaggaagtggctcaaatgcccatgttctccactcatgccaccctgccttccctcccccagcctgcaccaatggcctcatggggagttccctatgatcagttgacagaggaagggaagactaaggactggttcatagatggttctgcacgatatgcaggcaccacccgaaagtggacagctgcagcactatatccactttctaaatgcatgtgtacacttgtgctaagaaaatatctttattttatttcctttatttttcctttatcatgtgaccttagatttatggacttcacatcagcatttaagcatttaagtgttgttcatatcagcatttaaatattgttaaccttatgtaataacttttggtttggggattggtgcgtttctggttgtatgaggatagttgtattatattaggcataattatgaccttattattgtctttatttgaagattatgtatgatttcaggatgtgtgtatgggttcaagttgacaaggagttggacttgtgatggttaatactgtcaacttgattggattgaaagatgcaaagtattaatctcggttatgtctgtgagggtgtggcaaaaggagattaacatttgagtcagtgggctgggaaggcagacccacccttaatctgggtacacaccatctaatcaagttccagtgtggccagattgtaaagcagggagaaaaatgtgaaaagactagactgaattagcttcccagcctacatctttctcctgtgccaaatgcttcctgctcttgaacatcggactccaagttcttcagcgttgggagttggactggctttcttgctcctcagcttgcagagggcctgttgtggaaccttgtgatccgctgagttaatactacttaataagatcccctttatatacatataatatattatattatatataatatatataatatatattatatataatatatataatatattatatattatatataatatatattatatattatatataatatatattatatataatatatattatatattatatattatatataatatatattatatataatatatataaaatatatatatatcctattagttctgtccctctagagaaccctgactaatacaatttatgtcattaatctcatttattgatttgtatacattgaaccaaccttatatcccaggaataaaacctacttgattgtggtggattagctttttgatgtactcttggattcaattgctggtattttattgagaatttttgcatctgtgttcatcaaggatattggcttgaagttttctttttttgttgttccatatcagaatgatgacgacctcatagaatgagttagtctgtcctcttttatcttttggaattgtttcaggaggcttgatatcagctcttctttatatgactggtatactttggctaggaatctctctggtccaggggtttttctggtgtaggtttttaattactgattcaacttcagaactcattactcattattgagttctaaaactcactttcatgtactcttcaaaagactgtcttcttctgttgttgagcggggtgttctctcaaggtcgtttaggtgaaggtggttgctggtgttcttctgtatccttactgcttgtctttctctttttttattgactactgaggattaatggtgatgtgtccaactttaactctagattagtctatttctcttttagattgtaactctgttttatatattttgaagctctgttgttaggcatgtgtatttggattgttaggtcttcttgatgatgacctttatcattatgtaatgtttcttcttatctctggaagtattcgttgttctgaagtctatttgtgctgatatgaatacagccttcacagctctattttcactagtatttgtatatctttttctcagcttttaaattgagatgttcagaccatttgcattaaagtagttgttaataggattaaatttaaatctaccattaagttggttatttctctttgtcccatttaaactttgttccttttttcatatttttctgccttcatttatattgagtttatctccacgacttacttattaaattaatttttaatggttttagtattttccacaatgtttataatatatactttgattttttcacattccaccttcaaatgacagaattatactggatatatagaaatcttacatcattgcacttctccttcctccctctcaaaatgttgtgctattgctctttgtaatagaggcttacttctattatgttatagctctcataatacattgacactatttttaccctgaataatcagttgttttttaaagtgattatgactacaaatattttgaataatttctttattttaccatttctggtgctccttatcttttacagtagatcccaatttccatctggagtcacattctttctgtgaaaaacaacctttagcatttcttatagcacgggactgctgttgctgttgtctttcagcttttctttgtctgaagaagtctttattttgccttcagtttttaaaagtgattttgctgagtatagatactgggttgagagtttcattccttgtatcattttaacaatgatgttccattatattccgttttgaatagtttctgactagaaatctgatctttgtttctttgtattcaatagttcctttttctctgactgcctttaagatattctcatctttgtttttcaacagtttgactataatttgtttattattaactttttgtatttattctgcttgaggtttcctgagctccttggatttgcagattgttgatttttattgtttttgtaaaattcatagccattatctattctactgttttgttttttttttcacttctctctctctgtattcttctttttggactgtaagtattcaaatgttagatcattcatattgcttcataaaccttatatgcttcttctgcttttttttttttgtcaggaactctttttttgtatctgtgttggtttggataagttctagtagactatgttcaagtttatggattattttgttagttgtgtctaattgactcctcagtgcattcagagaattcttcatctctgatattataaatctcttcctagcattttcatgttactcttttctatagtttccatctctttgctgaaattctccccctatccatggatattgtccacctttaccacaagattctttaacatattaacataggtatcatacaaacccaaactgatagtttccagatggtgtcttttctgagtctgtctgtcttgattgctttattatttaacagtgacttatcttccctcttcagcttttggtgtgtcttgtaattgtttaatcaaacactgggtatcataaatggaggaacagtagagattgcagtaaatattatttatgctttgaaatgggcacccatcttctgttgaaaatatgttttgtggtcaattgagtcaacctagtaactggttgaactgaatttggcatttgtgcttgttgcttttatcttaaatgcaccacaggtttaaattcctccagtgatgggttgctgctatcttttgcttagagtggggcctggggtgtggaagaattttctcagtgttcctatctattattagattttagcagtcactgcatgcctgcactacagaggggatatcttcatacacataatctaaccccattgaaactgctgtttcttcttaatgaatgctcaatctttggtggaaataaacaaatgctgtatctcctggagccacttcagtcttagtcaggttctgcagggctttgaagggaatgcattctcagtattcttgtgccttatttggatggaacttgaacctgtggtgggtttggagagaaagagtagcagacgtctgctatgttgcaatgcaggatgctgggcacaagaaaatttccagtctctcctccaaggaaataagatttgatcatctacctatccctgagaagtgaagggctttgcctgcggtgctagatgcaaaaccatttttctccccccattgcccagaaacttaaggctttggcttttctgagcagtggtctagggaattgtgcaaggttttcatatttgaccctgacagcccatcaccacctacagcttgcagtgccaaatgtatctccctctgatctctcctgtcctgtggtcctcatgaacattaagaagagatttctaaaaaagagcttgcacatgagcatagtttctggtgagaagaattctgatatgttaacttcctctaaacttttaaataaaatatttctaagaattaaataaagttctagaatgatatgaatctattcctttggttttttgcacgtctgtctgcctgctaatcaagagaagagaatggtcgtaattctcagagactttttcctgtttgtgtcataaatgacttcacatttttttctgttctaagaactattcagcttgatttcttctgttttaattttagcagcacctgagcaaagccatgtggtccaggattgctaccatggtgatggacagagttatcgaggcacgtactccaccactgtcacaggaaggacctgccaagcttggtcatctatgacaccacatcaacataataggaccacagaaaactacccaaatgcgtatgtcattaatcttacagtaagcaaaacaaggtccaagtaaaatttgtcttagaaaaggtgtgcgtcaagctaacttcttatgattaaatttttctcacacatagaatgcatggcaaaatgtctgagaaacattactttgagcaaagagtatgatagaagagaaatgttaagctggctctctttcctgagagtttgataaaatcaggagaatatctggcggtggtgaggccacaataatggaaaatcagaatgtttagacagagtcagcttcaacaacactcactaaaggtcaatgtgatctttaccccttgaaattctataattctaatctccaattcctgaagtgaaggttgtgttggccttttctgtcttggctcacaagtaaatgatatgtgcatatctatggaaaggcgaatctatctttttctatatctatgtctattccaacgggtagaaacaccctgggtcctgagcaccagtggtctgaaggaatacgggttgccaggaagagagaagcaaaggcaggaaggcagatgaaagtaagaaatgagacagatgctaaacaataaaaagtgcgggaagatagacagaagctggggtctgaccacaccatggccagtctttcacacataagtgactaccaaagacaagaaaaaatgatttccgcttgttggacaatagatggtagaggaccaagggaattgcgagagagagaacaatgagatcaactcaacagatgcactggttttcttcctggagacccttcctgcactgaagggcaggagatggagcccaaaaaaaactgtagccatcttgctgaacagaggagggacattggagtttgggattattcaggtggctaggattttctaggcctgctaacaatgagaacagatttgtggaggaaaggagttctagaaatatgcatagaaatctcctcgagtcattggctaaacatgaagctgcatgtacacagaaaatagatccacaagaaagtagggcaaagaacatctacggaagagcagcaactacaatggaacagtgagctcaataaacatgacagagctcaaatagcactaagggatattggagtttggaccacacagaggagagagacttcactgaacatcttgggcattcagtagagacccaggaaaagccatactttaggagtagaattagtatattcttagaataaaggcagctccacacaaacaatagcaaaactgaaaaggaagtctccaagcatcagaatgatgtccaagtcaatgaactgcctctgagaggaaaactcaaccatctttagaggtaaacatcaaagtcaagtggctcagctatgcagtatccacagtgtgaggcctaaatataaaacttgactacacatagaaaccttttagtgtgacccacaagcaggaggaaaatcagccaatacaaacagacccagaagagacagaaatgattagaatggcataaaaatttgacatatcactatataataattgagttctaggatttaagaaaacatgaatatagaatgcaacagacaccttatccagagacagtaagagtataaagagccaaatcgaagaactactaagagatatgtcttaaatgaaaaaattactagatggcctccccatctagttagacatttcagaagaaaataccaaatgaaaaataattgcatagaacctacagaaccagatacacacatacaaaacacacgcatgcatacacacacactcaaacatgtataagcttacaaacacacacacacatccacaaatgctgaaaaatgaaatcaaccgagccacacagacataaaggaaaacataaaaagatttcctacatgtgggaagcaagtcacagaaagggggaaggagattggaacagaaatatatactgaaagcaaggatggctgaaaattttccaaatataaagaagattaaaaaatcacggactcaagaagctcaatggatcagaaaaataatttctaaaatgacaattataggatgccactgggtacatagcagttcaactgtcagagggcaaagacataatacacagaaaaatctcgtaaggaacgggaaaaacaaaaagctgtgtcttgctagaggaacagtgatacaagtgactaatgtgttcccatcagaaacactgcaacctggacacaaaagaataacattaaagtaataaacgtaagaaagaagagctcaactgagaaggctacatccagcaataaaatgccttgaagttcatccatgttggaggaatgcacattgtgcactcccctaaacaaagaaaccggaaactgtaagactttggaatcagcaggcttatgtaacaaaagaggtgaccctaaggaattaaggagaagaagaatagaacaagaagggaactttctgcagcctatataatgaagaacctagcaattggcaaatgtagatgaaaatgctacatgttttcttgatcaaacgtttatatctttttaaatgagagttgacgagttgaagcaaaatgataccaatatatttaactttaccatatgtagaagtaaaaatttgaacatgtagcataaatcatgtagggattaattggaagtgtaccactgtaagtttcttacctcatgcacgatagtatgtaatactaataaaaggttaatgtgtgggttcaaagggatattgcaaatcctagagcaatcacaaagtttttaactctgaggtttgttgtataataacaatattttatgtattcaaaagagggaagccaaggaagaaaaaaaagtctttaaagagctctggctcttagtacatccagttgctcattgaatgagcttcctggaatggagggtctgggactgagactaggccacatgtgtagagccactagagacacaatgttggatccccatggcccataatacatttcccattttctcaggcagccacaggtcatgaatgtgaggatactgagaggttggagcaacgttcttgggaggcataaggaagagcgaatgcttcaagatccccgcagcccaaactcctcagctgctttgcctcctaattcattgttttttgctcctccatagctgtccgacctcttcagatctcttagtcttcctgccatcttcctttatgccatgggacccactgttctttcaactcatcccccagttctggagtggctgtggacagcagaggatagactgagagcaggagagaaggtcctgcccaggaacccattctagagatactgcattctgcctgggagcaagttttccagggcagctttgagaagtcttgcagaaacaaacctacttgaccgacatgatatgggaatgacagacagtaatactatttgcacaatgcttttccatgggaaaggtagagccttttcactaggttttgagtacatggagtgtgagagttgacctggaaaggttatcctccttgatgccatgttttctctgaagaactacatgttcgttgcaactcccacattagaatatgaagtcctaccgagagagatacggagactagacagatacagatgcatttgcatgtgaatacacaatcccacaatacagacgtcaaaacccataccagttattccagagagatggattgggcagaaggcagaaggagaatactctgatcgtttttcggccacgtgtgtgtgttatctcagtgtttctaagaagcgtttgctactttagattttttatttaaaaaaaatagtaataatctattaagtatgagagatgtgcagagaggattagtgatcgagagccatttttgctggtggcaatcatatggtacttttaatgggaatattagaaaggcaccggtaatgaccttgttgcagcacaaaggagagagtgtggggtgcccctgcatgttgtcccacctcttgtgacgtgtatcgttttggaatttccagtggcttgatcatgaactactgcaggaatccagatgctgtggcagctccttattgttatacgagggatcccggtgtcaggtgggagtactgcaacctgacgcaatgctcagacgcagaagggactgccgtcgcgcctccgactgttaccccggttccaagcctagaggctccttccgaacaaggtaaggagtctgtggccagacatctacacgcttcgatgctgggatgaaaagccatggaaattcccactgatgcagccgccttcaatggtaaacggatgctcgagtgttgcctgagttctaccatgtaggaggaagcctccgtgcactctctgggggagccagcggagtgatttctggtgcaacgtggttgggctttgtctttaggatgggcacaaaccctccagggggatcgacttcaaaattcaccttgttgtaaaacgggctacctcagtgtcccagccaaaatttttattgtaacatgctgtcaggtgtgtcactctttccaagccagtaagcttttccggggatttcttcaagtagccagcattcagagcaatcttcagcattgcagattctgagaaatgtggctctggagcctgtcaccctcgagaaacctaagagggctgcattgattccatgtggccctgggtctatggagcagtacatgagctcccagtgctctaaggctcttcagccctaggctttgaagggagtgatttctcagtattcttaaacctctttctgatgacacttgtacctgtgaggggtctagagagaaagagtagtagactcctactttactacaattcaggatgcagggcatgagaggattccctctctcctccaagggaagaagcttttggcgtgcacacatccctgagaagcaaagtgtctttgtcttcagtcagatacataggaccgttttctgccccatggcccggaagccaaaggccttggctttcatgatcaacggtctagggaaacatgcaaaatttccatgtctgtcccaaactctgcccccgacagccaattaccacctgcagcccgcattgccaaatgcggtgccgtttgcatgaagattcagtagagtttcctagaaaggtgctacctcgtgagctcactttccaatgaggaatctgatctgttgtgtttctctaaggtgtcaggtgaaatatttccaagaacttactacagttctagaatgggaggaatctgttgctttggtgtttgtttgttggtcggttttctcacatccatctgcctatggataaggaaaagagaacggtcgtaattctcatagactcctttctggttgtgtcacaaatggcttcacatgtttctctatgctcagagatactcagcttgatttcccgtgttttcatttcagcaccgactgagcaaaggcctggggtgcaggagtgctaccatggtaatggacagagttatcgaggcacatactccaccactgtcacaggaagaacctgccaagcttggtcatctatgacaccacactcgcatagtcggaccccagaatactacccaaatgcgtatgtctttgttctttaccataagagaagaaagggccaagtgaagtttctgttacaagagatgtgtctcaagctgagttctccgaactcaacttgtgacagatgcagatggcgtagcaaaatgtctcaggatgattgccttggagctaagggtctgagagaagggaaatgttaagctccctctccttcctcctagttctattgagcagaagggaaatctggaggtgaggagatcacattatgaagaaagtcagaatgacaaaggaccagacacttagattacccttccacaacaccaactaaacgtcaatggagactttccagttggaattccgttattctggcttccacttcctgaagggaaggttgcgtttgccttttctctctgggttcaagaggaaagaataggtgcttatttatggacaggtgaattgatctgtttctatatctacgtatattccgattgtcagaaaaacactcgttcctaagtaccagtggcctgaagggatacaggttcccagcaagagaagatccaaggaaggaaggcagatgagagtcagcacagagagggatgctgaaaagtaaaagggatgggtggatggagagaagcccgggtctgaccacccaatggccaatattttggccacaagcgactaccagagacatggaaaaatggtttctacatgtgggacaacagatggtagaggacctagagaattgagagaggggcaatgatgggctccactccgcagatgccttggctttcttcctggatacccttcctgcactgaatagcaaggagatggagcccaagcagactgtagccatcttgctgaatggaggagagggattggagtttgggatgactgtggtagctgaaatttttctaggtctgctagaaataagaactggtttgtgtggaggaaaagagctctacaaatacgcatagaagtctcctccagtcgttggcctgacatgacgctgcctgtgcacaggaaatggttccacgagaaagtgtggcaaagaacatttactgagaaacagcaagtacaagagcacaggaagctcaataaagaagagagagatcacatagcactctgggatactggagttcttcccagctagaccagagagtcctcacggagcacattgccaattcagtggagaccccagaacagccgtaatttaaaggtacacttagtatattactagaataaagtcagctgcagacaaccccttgcacagctggaaagcaagtgtccaagcatcaaatcggtttccaatcaatgaagtgcctgtgagaggaaatctcaactctctttagaagtaaacaacaaagtcgattgcctcagctatgcggtatccgcagagtgagtcctaaatttaaaatctgactacatgtagaaaagcgtttcgtgtgacccatgaccaggaaataaatcgggtaatacaaacaggctcaggaatgagagaaatgattagaattgcgtgaaaatttgacatatcagtatgataactgatttcaaatatttaaaaaaacaacatgcaagaaagcagatatcatatcaagagaaattaacagtacagaatagccaaattaaattaaagaggtagtataaaaaaagtatgtcttaattgaaaaaaattactgtatggccggctgatcaatttagacgtttcagaggaaaacattacccaacacacaattctagagaacctacagaatgagctacacacacacacacacacacacacacacacactgaaaacacacccatactcacacacacgcagaaactcacaagttctaacacacacagacacgcgcacccctgaagaaacagtgaaatataaaattaagcgagcctcacagacatgtaggaaaatatgaaaagatttcctgcatgtgggaagcaagtcacagtaaagagcaagggagtttataatagaaacaaataccagaatcaaggatggctgataacttttcaattacgaagaacattaaaaaaaatcacagaatcgtgaaactcaagggatcatatagggaatttcggaaaaaaaacccaacctgtatgatgtacttttgtacatcacagttcgaaggtaacaaggcaaagatgtaataagaagaaacctgtcacgagaaactggaggaaaaagagctgtgtcttcctacaagtacactgatacaaattgccaatgtgttcacctcagaaacactggaagccagataccagggaatattgttaaaatgataatcaggaacaaaaagagatcaaccgggaatgctgaatccagcaataaaatgccttgaaggtcatccatgtcggataaatgcatattgtgcactgccccaaagaaagaaaccggaaactgtaagaattggaaatcagcaggcttatgtaacaagagaggtgacccgaaggaattaggtagaagaagaattgaacaagaaaggaactttctgcagcccacgtaatgaagaatccagcaattggcaaatgtagatagatgtaaatgcaaaatattttcttgatcaaatttctatatctttgtaaatgagagttgactacttgaaacaaaatgatagcaagatatttaacttcagcatatgtagaggtaagaatttgaaatggtagcataaatcacgaagggattaattcgaagtgtaccgttgtaagtttctttacctcatgcacgatggtgtgtcatattaataaaagggtactgtgcgggttcgaagggatattgcaaatcctagagcaatcacaaaggtttgaactctgaggtttttggtataataagaatagtccatgcattcaaaagagggaagccaaggaagaactagaagtctttcaagagctcaggctcttatacatccagttgctcattgaaccagcttcctggaatggagggtctggggttgagactaggccacaagtctagagtctctagagagacagtgttggaaccccatggcccataatacatttcccattttctcaggcagccagaggtcatgaatgtgaggatactgggaggttggagcaacgttcttgggaggcataaggaagagcgaatgcttcaagatccccgcagcccaaactactcgcctgctttgccccctaatgcatttttctctgctgctccgtagctgtccgacctcttcagatctcttagtccaccctgccgtcttcctttatgccatgggtcccactgttctttcaactcatccccctttccctcagtcccggagtagctgcggccagcagagggtagactgagagcaggagagaaggacctgcctaggaaccccttctagagatactgcatcctgcctgggagcaagttttccagggcagctttgagaagtcttggagaaacaaacctactaaacctgacagacagtaatactatttgcacaatgcttttctgtgggaaaggtagagccttttcactacgtattgagtacatagagtgtgagggttgacctggaacggctatcctcctggatgacgtgtgttttctgaagaactacatgttcgttgcaactcccacattagaatatgaagtcctaccgagagagatacggagactagacagatacagatgcatttgcatgtgaatacacaatcccacaatacagacgtcaaaacccataccagttattccagagagatggattgggcagaaggcagaaggagaatactctgatcgtttttcggccacgtgtgtgtgttatctcagtgtttctaagaagcgtttgctactttagattttttatttaaaaaaatagtaataatctattaagtatgagagatgtgcagagaggattagtgatcgagagccatttttgctggtggcaatcatatggtacttttaatgggaatattagaaaggcaccggtaatgaccttgttgcagcacaaaggagagagtgtggggtgcccctgcatgttgtcccacctcttgtgacgtgtatcgttttggaatttccagtggcttgatcatgaactactgcaggaatccagatgctgtggcagctccttattgttatacgagggatcccggtgtcaggtgggagtactgcaacctgacgcaatgctcagacgcagaagggactgccgtcgcgcctccgactgttaccccggttccaagcctagaggctccttccgaacaaggtaaggagtctgtggccagacatctacacgcttcgatgctgggatgaaaagccatggaaattcccactgatgcagccgccttcaatggtaaacggatgctcgagtgttgcctgagttctaccatgtaggaggaagcctccgtgcactctctgggggagccagcggagtgatttctggtgcaacgtggttgggctttgtctttaggatgggcacaaaccctccagggggatcgacttcaaaattcaccttgttgtaaaacgggctacctcagtgtcccagccaaaatttttattgtaacatgctgtcaggtgtgtcactctttccaagccagtaagcttttccggggatttcttcaagtagccagcattcagagcaatcttcagcattgcagattctgagaaatgtggctctggagcctgtcaccctcgagaaacctaagagggctgcattgattccatgtggccctgggtctatggagcagtacatgagctcccagtgctctaaggctcttcagccctaggctttgaagggagtgatttctcagtattcttaaacctctttctgatgacacttgtacctgtgaggggtctagagagaaagagtagtagactcctactttactacaattcaggatgcagggcatgagaggattccctctctcctccaagggaagaagcttttggcgtgcacacatccctgagaagcaaagtgtctttgtcttcagtcagatacataggaccgttttctgccccatggcccggaagccaaaggccttggctttcatgatcaacggtctagggaaacatgcaaaatttccatgtctgtcccaaactctgcccccgacagccaattaccacctgcagcccgcattgccaaatgcggtgccgtttgcatgaagattcagtagagtttcctagaaaggtgctacctcgtgagctcactttccaatgaggaatctgatctgttgtgtttctctaaggtgtcaggtgaaatatttccaagaacttactacagttctagaatgggaggaatctgttgctttggtgtttgtttgttggtcggttttctcacatccatctgcctatggataaggaaaagagaacggtcgtaattctcatagactcctttctggttgtgtcacaaatggcttcacatgtttctctatgctcagagatactcagcttgatttcccgtgttttcatttcagcaccgactgagcaaaggcctggggtgcaggagtgctaccatggtaatggacagagttatcgaggcacatactccaccactgtcacaggaagaacctgccaagcttggtcatctatgacaccacactcgcatagtcggaccccagaatactacccaaatgcgtatgtctttgttctttaccataagagaagaaagggccaagtgaagtttctgttacaagagatgtgtctcaagctgagttctccgaactcaacttgtgacagatgcagatggcgtagcaaaatgtctcaggatgattgccttggagctaagggtctgagagaagggaaatgttaagctccctctccttcctcctagttctattgagcagaagggaaatctggaggtgaggagatcacattatgaagaaagtcagaatgacaaaggaccagacacttagattacccttccacaacaccaactaaacgtcaatggagactttccagttggaattccgttattctggcttccacttcctgaagggaaggttgcgtttgccttttctctctgggttcaagaggaaagaataggtgcttatttatggacaggtgaattgatctgtttctatatctacgtatattccgattgtcagaaaaacactcgttcctaagtaccagtggcctgaagggatacaggttcccagcaagagaagatccaaggaaggaaggcagatgagagtcagcacagagagggatgctgaaaagtaaaagggatgggtggatggagagaagcccgggtctgaccacccaatggccaatattttggccacaagcgactaccagagacatggaaaaatggtttctacatgtgggacaacagatggtagaggacctagagaattgagagaggggcaatgatgggctccactccgcagatgccttggctttcttcctggatacccttcctgcactgaatagcaaggagatggagcccaagcagactgtagccatcttgctgaatggaggagagggattggagtttgggatgactgtggtagctgaaatttttctaggtctgctagaaataagaactggtttgtggaggaaaagagctctacaaatacgcatagaagtctcctccagtcgttggcctgacatgacgctgcctgtgcacaggaaatggttccacgagaaagtgtggcaaagaacatttactgagaaacagcaagtacaagagcacaggaagctcaataaagaagagagagatcacatagcactctgggatactggagttcttcccagctagaccagagagtcctcacggagcacattgccaattcagtggagaccccagaacagccgtaatttaaaggtacacttagtatattactagaataaagtcagctgcagacaaccccttgcacagctggaaagcaagtgtccaagcatcaaatcggtttccaatcaatgaagtgcctgtgagaggaaatctcaactctctttagaagtaaacaacaaagtcgattgcctcagctatgcggtatccgcagagtgagtcctaaatttaaaatctgactacatgtagaaaagcgtttcgtgtgacccatgaccaggaaataaatcgggtaatacaaacaggctcaggaatgagagaaatgattagaattgcgtgaaaatttgacatatcagtatgataactgatttcaaatatttaaaaaaacaacatgcaagaaagcagatatcatatcaagagaaattaacagtacagaatagccaaattaaattaaagagctagtataaaaaaagtatgtcttaattgaaaaaaattactgtatggccggctgatcaatttagacgtttcagaggaaaacattacccaacacacaattctagagaacctacagaatgagctacacacacacacacacacacacacacaaactgaaaacacacccatactcacacacacgcagaaactcacaagttctaacacacacagacacgcgcacccctgaagaaacagtgaaatataaaattaagcgagcctcacagacatgtaggaaaatatgaaaagatttcctgcatgtgggaagcaagtcacagtaaagagcaagggagtttggaatagaaacaaataccggaatcaaggatggctgataacttttcaattacgaagaacattaaaaaaaatcacagaatcgtgaaactcaagggatcacatagggaatttcggaaaaaaaacccaacctgtatgatgtacttttgtacatcacagttcgaaggtaacaaggcaaagatataataagaagaaacctgtcacgagaaactggaggaaaaagagctgtgtcttcctacaagtacactgatacaaattgccaatgtgttcacctcagaaacactggaagccagataccagggaatattgttaaaatgataatcaggaacaaaaagagatcaaccgggaatgctgaatccagcaataaaatgccttgaagatcatccatgtcggataaatgcatattgtgcactgccccaaagaaagaaaccggaaactgtaagaattggaaatcagcaggcttatgtaacaagagaggtgacccgaaggaattaggtagaagaagaattgaacaagaaaggaactttctgcagcccacgtaatgaagaatccagcaattggcaaatgtagatagatgtaaatgcaaaatattttcttgatcaaatttctatatctttgtaaatgagagttgactacttgaaacaaaatgatagcaagatatttaacttcagcatatgtagaggtaagaatttgaaatggtagcataaatcacgaagggattaattcgaagtgtaccgttgtaagtttctttacctcatgcacgatggtgtgtcatattaataaaagggtactgtgcgggttcgaagggatattgcaaatcctagagcaatcacaaaggtttgaactctgaggtttttggtataataagaatagtccatgcattcaaaagagggaagccaaggaagaactagaagtctttcaagagctcaggctcttatacatccagttgctcattgaaccagcttcctggaatggagggtctggggttgagactaggccacaagtctagagtctctagagagacagtgttggaaccccatggcccataatacatttcccattttctcaggcagccagaggtcatgaatgtgaggatactgggaggttggagcaacgttcttgggaggcataaggaagagcgaatgcttcaagatccccgcagcccaaactactcgcctgctttgccccctaatgcatttttctctgctgctccgtagctgtccgacctcttcagatctcttagtccaccctgccgtcttcctttatgccatgggtcccactgttctttcaactcatccccctttccctcagtcccggagtagctgcggccagcagagggtagactgagagcaggagagaaggacctgcctaggaaccccttctagagatactgcatcctgcctgggagcaagttttccagggcagctttgagaagtcttggagaaacaaacctactaaacctgacagacagtaatactatttgcacaatgcttttctgtgggaaaggtagagccttttcactacgtattgagtacatagagtgtgagggttgacctggaacggctatcctcctggatgacgtgtgttttctgaagaactacatgttcgttgcaactcccacattagaatatgaagtcctaccgagagagatacggagactagacagatacagatgcatttgcatgtgaatacacaatcccacaatacagacgtcaaaacccataccagttattccagagagatggattgggtaggaggcagaaggagaatactctgatcgtttttcggccacgtgtgtgtgttatctcagtgtttctaagaagcgtttgctactttagattttttatttaaaaaaaatagtaataatctattaagtatgagagatgtgcagagaggattagtgatcgagagccatttttgctggtggcaatcatatggtacttttaatgggaatattagaaaggcaccggtaatgaccttgttgcagcacaaaggagagagtgtggggtgcccctgcatgttgtcccacctcttgtgacgtgtatcgttttggaatttccagtggcttgatcatgaactactgcaggaatccagatgctgtggcagctccttattgttatacgagggatcccggtgtcaggtgggagtactgcaacctgacgcaatgctcagacgcagaagggactgccgtcgcgcctccgactgttaccccggttccaagcctagaggctccttccgaacaaggtaaggagtctgtggccagacatctacacgcttcgatgctgggatgaaaagccatggaaattcccactgatgcagccgccttcaatggtaaacggatgctcgagtgttgccggagttctgccatgttgggggaagcctccgtgtactctctgggggagccagcggagtgatttctggtgcaacttgggtgggctttgtctttagaatgggcacaaaccttccagggtgatgggcttcacaactcacctccttctaaaatgggctatctcagtgtcttagccaaaatttttattgtaacgtgctgtcaggtgtgtgattctttctgtcgcagtaagcttttctggggatttcttcaagtagccagcagtcagtgcaatcttcagcattgcagatttcaaaaaatgtggctctggagcctgtcatcctcgagaaacctaacagggctgcattaattccatatggtcctgggtctatggagcagtatatgagctcccaatgctctaaggctcttcagtcctaggctttgaagggagtgatttctcagtgttcttaaacctctttctgatggcacttgtacctgtgaggggtctagagagaaaggttagtagacttctcctttactgcaattcaggatgcagggcatgagaagattccctccctcctccaagggaagaaggttttggcgtgcacacatccttgagaagcaaagtgtctttgccttcagtcagatatataggatcgttttctgccccatggcctggaagccagaggccttggctttcatgatcaacgatctagggaaacatgcaaaatttccatgtctttcccctcctctgccctcgacagccaattaccacctgcatcctgcattgccaaatgcagtgccctttgtatgaacattcagtagagtttcatagaaaggtgctacttcgtgagcgcactttgcagtgagaaggagtctgttctgttctgtttttctaaggatttcaggtgaaatatttcctagaacttactacagttctagattggtaggaatctgtaggtttgctgtatgttttttggttggttttctcccatccatctgcctacaggtaagggaaagataacgttcgtaattctcatagactcctttctggttgtgtcataaatggcttcacatatttcgttattctcagagatactcagtttatttcttgtgttttcatttcagcaccgactgagcagaggcctggggtgcaggagtgctaccacggtaatggacagagttatcgaggcacatactccaccactgtcactggaagaacctgccaagcttggtcatctatgacaccacactcgcatagtcggaccccagaatactacccaaatgcgtatgtctttgttctttaccataagagaagaaagggccaagtgaagtttctgttacaagagatgtgtctcaagctgagttctccgaactcaacttgtgacagatgcagatggcgtagcaaaatgtctcaggatgattgccttggagctaagggtctgagagaagggaaatgttaagctccctctccttcctcctagttctattgagcagaagggaaatctggaggtgaggagatcacattatgaagaaagtcagaatgacaaaggaccagacacttagattacccttccacaacaccaactaaacgtcaatggagactttccagttggaattccgttattctggcttccacttcctgaagggaaggttgcgtttgccttttctctctgggttcaagaggaaagaataggtgcttatttatggacaggtgaattgatctgtttctatatctacgtatattccgattgtcagaaaaacactcgttcctaagtaccagtggcctgaagggatacaggttcccagcaagagaagatccaaggaaggaaggcagatgagagccagcacagagagggatgctgaaaagtaaaagggatgggtggatggagagaagcccgggtctgaccacccaatggccaatattttggccacaagcgactaccagagacatggaaaaatggtttctacatgtgggacaacagatggtagaggacctagagaattgagagaggggcaatgatgggctccactccgcagatgccttggctttcttcctggatacccttcctgcactgaatagcaaggagatggagcccaagcagactgtagccatcttgctgaatggaggagagggattggagtttgggatgactgtggtagctgaaatttttctaggtctgctagaaataagaactggtttgtggaggaaaagagctctacaaatacgcatagaagtctcctccagtcgttggcctgacatgacgctgcctgtgcacaggaaatggttccacgagaaagtgtggcaaagaacatttactgagaaacagcaagtacaagagcacaggaagctcaataaagaagagagagatcacatagcactctgggatactggagttcttcccagctagaccagagagtcctcacggagcacattgccaattcagtggagaccccagaacagccgtaatttaaaggtacacttagtatattactagaataaagtcagctgcagacaaccccttgcacagctggaaagcaagtgtccaagcatcaaatcggtttccaatcaatgaagtgcctgtgggaggaaatctcaactctctttagaagtaaacaacaaagtcgattgcctcagctatgcggtatccgcagagtgagtcctaaatttaaaatctgactacatgtagaaaagcgtttcgtgtgacccatgaccaggaaataaatcgggtaatacaaacaggctcaggaatgagagaaatgattagaattgcgtgaaaatttgacatatcagtatgataactgatttcaaatatttaaaaaaacaacatgcaagaaagcagatatcatatcaagagaaattaacagtacagaatagccaaattaaattaaagagctagtataaaaaaagtatgtcttaattgaaaaaaattactgtatggccggctgatcaaattagacgtttcagaggaaaacattacccaacacacaattctagagaacctacagaatgagctacacacacacacacacacacacacacacacactgaaaacacacccatactcacacacacgcagaaactcacaagttctaacacacacagacacgcgcacccctgaagaaacagtgaaatataaaattaagcgagcctcacagacatgtaggaaaatatgaaaagatttcctgcatgtgggaagcaagtcacagtaaagagcaagggagtttggaatagaaacaaataccggaatcaaggatggctgataacttttcaattacgaagaacattaaaaaaaatcacagaatcgtgaaactcaagggatcatatagggaatttcggaaaaaaaacccaacctgtatgatgtacttttgtacatcacagttcgaaggtaacaaggcaaagatataataagaagaaacctgtcacgagaaactggaggaaaaagagctgtgtcttcctacaagtacactgatacaaattgccaatgtgttcacctcagaaacactggaagccagataccagggaatattgttaaaatgataatcaggaacaaaaagagatcaaccgggaatgctgaatccagcaataaaatgccttgaagatcatccatgtcggataaatgcatattgtgcactgccccaaagaaagaaaccggaaactgtcagaattggaaatcagcaggcttatgtaacaagagaggtgacccgaaggaattaggtagaagaagaattgaacaagaaaggaactttctgcagcccacgtaatgaagaatccagcaattggcaaatgtagatagatgtaaatgcaaaatattttcttgatcaaatttctatatctttgtaaatgagagttgactacttgaaacaaaatgatagcaagatatttaacttcagcatatgtagaggtaagaatttgaaatggtagcataaatcacgaagggattaattcgaagtgtaccgttgtaagtttctttacctcatgcacgatggtgtgtcatattaataaaagggtactgtgcgggttcgaagggatattgcaaatcctagagcaatcacaaaggtttgaactctgaggtttttggtataataagaatagtccatgcattcaaaagagggaagccaaggaagaactagaagtctttcaagagctcaggctcttatacatccagttgctcattgaaccagcttcctggaatggagggtctggggttgagactaggccacaagtctagagtctctagagagacagtgttggaaccccatggcccataatacatttcccattttctcaggcagccagaggtcatgaatgtgaggatactgggaggttggagcaacgttcttgggaggcataaggaagagcgaatgcttcaagatccccgcagcccaaactactcgcctgctttgccccctaatgcatttttctctgctgctccgtagctgtccgacctcttcagatctcttagtccaccctgccgtcttcctttatgccatgggtcccattgttctttcaactcatccccctttccctcagtcccggagtagctgcggccagcagagggtagactgagagcaggagagaaggacctgcctaggaaccccttctagagatactgcatcctgcctgggagcaagttttccagggcagctttgagaagtcttggagaaacaaacctactaaacctgacagacagtaatactatttgcacaatgcttttctgtgggaaaggtagagccttttcactacgtattgagtacatagagtgtgagggttgacctggaacggctatcctcctggatgacgtgcgttttctgaagaactacatgttcgttgcaactcccacattagaatatgaagtcctaccgagagagatacggagactagacagatacagatgcatttgcatgtgaatacacaatcccacaatacagacgtcaaaacccataccagttattccagagagatggattgggcagaaggcagaaggagaatactctgatcgtttttcggccacgtgtgtgtgttatctcagtgtttctaagaagcgtttgctactttagattttttatttaaaaaaaatagtaataatctattaagtatgagagatgtgcagagaggattagtgatcgagagccatttttgctggtggcaatcatatggtacttttaatgggaatattagaaaggcaccggtaatgaccttgttgcagcacaaaggagagagtgtggggtgcccctgcatgttgtcccacctcttgtgacgtgtatcgttttggaatttccagtggcttgatcatgaactactgcaggaatccagatgctgtggcagctccttattgttatacgagggatcccggtgtcaggtgggagtactgcaacctgacgcaatgctcagacgcagaagggactgccgtcgcgcctccgactgttaccccggttccaagcctagaggctccttccgaacaaggtaaggagtctgtggccagacatctacacgcttcgatgctgggatgaaaagccatggaaattcccactgatgcagccgccttcaatggtaaacggatgctcgagtgttgcctgagttctaccatgtaggaggaagcctccgtgcactctctgggggagccagcggagtgatttctggtgcaacgtggttgggctttgtctttaggatgggcacaaaccctccagggggatcgacttcaaaattcaccttgttgtaaaacgggctacctcagtgtcccagccaaaatttttattgtaacatgctgtcaggtgtgtcactctttccaagccagtaagcttttccggggatttcttcaagtagccagcattcagagcaatcttcagcattgcagattctgagaaatgtggctctggagcctgtcaccctcgagaaacctaagagggctgcattgattccatgtggccctgggtctatggagcagtacatgagctcccagtgctctaaggctcttcagccctaggctttgaagggagtgatttctcagtattcttaaacctctttctgatgacacttgtacctgtgaggggtctagagagaaagagtagtagactcctactttactacaattcaggatgcagggcatgagaggattccctctctcctccaagggaagaagcttttggcgtgcacacatccctgagaagcaaagtgtctttgtcttcagtcagatacataggaccgttttctgccccatggcccggaagccaaaggccttggctttcatgatcaacggtctagggaaacatgcaaaatttccatgtctgtcccaaactctgcccccgacagccaattaccacctgcagcccgcattgccaaatgcggtgccgtttgcatgaagattcagtagagtttcctagaaaggtgctacctcgtgagctcactttccaatgaggaatctgatctgttgtgtttctctaaggtgtcaggtgaaatatttccaagaacttactacagttctagaatgggaggaatctgttgctttggtgtttgtttgttggtcggttttctcacatccatctgcctatggataaggaaaagagaacggtcgtaattctcatagactcctttctggttgtgtcacaaatggcttcacatgtttctctatgctcagagatactcagcttgatttcccgtgttttcatttcagcaccgactgagcaaaggcctggggtgcaggagtgctaccatggtaatggacagagttatcgaggcacatactccaccactgtcacaggaagaacctgccaagcttggtcatctatgacaccacactcgcatagtcggaccccagaatactacccaaatgcgtatgtctttgttctttaccataagagaagaaagggccaagtgaagtttctgttacaagagatgtgtctcaagctgagttctccgaactcaacttgtgacagatgcagatggcgtagcaaaatgtctcaggatgattgccttggagctaagggtctgagagaagggaaatgttaagctccctctccttcctcctagttctattgagcagaagggaaatctggaggtgaggagatcacattatgaagaaagtcagaatgacaaaggaccagacacttagattacccttccacaacaccaactaaacgtcaatggagactttccagttggaattccgttattctggcttccacttcctgaagggaaggttgcgtttgccttttctctctgggttcaagaggaaagaataggtgcttatttatggacaggtgaattgatctgtttctatatctacgtatattccgattgtcagaaaaacactcgttcctaagtaccagtggcctgaagggatacaggttcccagcaagagaagatccaaggaaggaaggcagatgagagtcagcacagagagggatgctgaaaagtaaaagggatgggtggatggagagaagcccgggtctgaccacccaatggccaatattttggccacaagcgactaccagagacatggaaaaatggtttctacatgtgggacaacagatggtagaggacctagagaattgagagaggggcaatgatgggctccactccgcagatgccttggctttcttcctggatacccttcctgcactgaatagcaaggagatggagcccaagcagactgtagccatcttgctgaatggaggagagggattggagtttgggatgactgtggtagctgaaatttttctaggtctgctagaaataagaactggtttgtggaggaaaagagctctacaaatacgcatagaagtctcctccagtcgttggcctgacatgacgctgcctgtgcacaggaaatggttccacgagaaagtgtggcaaagaacatttactgagaaacagcaagtacaagagcacaggaagctcaataaagaagagagagatcacatagcactctgggatactggagttcttcccagctagaccagagagtcctcacggagcacattgccaattcagtggagaccccagaacagccgtaatttaaaggtacacttagtatattactagaataaagtcagctgcagacaaccccttgcacagctggaaagcaagtgtccaagcatcaaatcggtttccaatcaatgaagtgcctgtgagaggaaatctcaactctctttagaagtaaacaacaaagtcgattgcctcagctatgcggtatccgcagagtgagtcctaaatttaaaatctgactacatgtagaaaagcgtttcgtgtgacccatgaccaggaaataaatcgggtaatacaaacaggctcaggaatgagagaaatgattagaattgcgtgaaaatttgaaatatcagtatgataactgatttcaaatatttaaaaaaacaacatgcaagaaagcagatatcatatcaagagaaattaacagtacagaatagccaaattaaattaaagagctagtataaaaaaagtatgtcttaattgaaaaaaattactgtatggccggctgatcaatttagacgtttcagaggaaaacattacccaacacacaattctagagaacctacagaatgagctacacacacacacacacacacacacacaaactgaaaacacacccatactcacacacacgcagaaactcacaagttctaacacacacagacacgcgcacccctgaagaaacagtgaaatataaaattaagcgagcctcacagacatgtaggaaaatatgaaaagatttcctgcatgtgggaagcaagtcacagtaaagagcaagggagtttggaatagaaacaaataccagaatcaaggatggctgataacttttcaattacgaagaacattaaaaaaaatcacagaatcgtgaaactcaagggatcacatagggaatttcggaaaaaaaacccaacctgtatgatgtacttttgtacatcacagttcgaaggtaacaaggcaaagatataataagaagaaacctgtcacgagaaactggaggaaaaagagctgtgtcttcctacaagtacactgatacaaattgccaatgtgttcacctcagaaacactggaagccagataccagggaatattgttaaaatgataatcaggaacaaaaagagatcaaccgggaatgctgaatccagcaataaaatgccttgaagatcatccatgtcggataaatgcatattgtgcactgccccaaagaaagaaaccggaaactgtaagaattggaaatcagcaggcttatgtaacaagagaggtgacccgaaggaattaggtagaagaagaattgaacaagaaaggaactttctgcagcccacgtaatgaagaatccagcaattggcaaatgtagatagatgtaaatgcaaaatattttcttgatcaaatttctatatctttgtaaatgagagttgactacttgaaacaaaatgatagcaagatatttaacttcagcatatgtagaggtaagaatttgaaatggtagcataaatcacgaagggattaattcgaagtgtaccgttgtaagtttctttacctcatgcacgatggtgtgtcatattaataaaagggtactgtgcgggttcgaagggatattgcaaatcctagagcaatcacaaaggtttgaactctgaggtttttggtataataagaatagtccatgcattcaaaagagggaagccaaggaagaactagaagtctttcaagagctcaggctcttatacatccagttgctcattgaaccagcttcctggaatggagggtctggggttgagactaggccacaagtctagagtctctagagagacagtgttggaaccccatggcccataatacatttcccattttctcaggcagccagaggtcatgaatgtgaggatactgggaggttggagcaacgttcttgggaggcataaggaagagcgaatgcttcaagatccccgcagcccaaactactcgcctgctttgccccctaatgcatttttctctgctgctccgtagctgtccgacctcttcagatctcttagtccaccctgccgtcttcctttatgccatgggtcccactgttctttcaactcatccccctttccctcagtcccggagtagctgcggccagcagagggtagactgagagcaggagagaaggacctgcctaggaaccccttctagagatactgcatcctgcctgggagcaagttttccagggcagctttgagaagtcttggagaaacaaacctactaaacctgacagacagtaatactatttgcacaatgcttttctgtgggaaaggtagagccttttcactacgtattgagtacatagagtgtgagggttgacctggaacggctatcctcctggatgacgtgtgttttctgaagaactacatgttcgttgcaactcccacattagaatatgaagtcctaccgagagagatacggagactagacagatacagatgcatttgcatgtgaatacacaatcccacaatacagacgtcaaaacccataccagttattccagagagatggattgggcagaaggcagaaggagaatactctgatcgtttttcggccacgtgtgtgtgttatctcagtgtttctaagaagcgtttgctactttagattttttatttaaaaaaaatagtaataatctattaagtatgagagatgtgcagagaggattagtgatcgagagccatttttgctggtggcaatcatatggtacttttaatgggaatattagaaaggcaccggtaatgaccttgttgcagcacaaaggagagagtgtggggtgcccctgcatgttgtcccacctcttgtgacgtgtatcgttttggaatttccagtggcttgatcatgaactactgcaggaatccagatgctgtggcagctccttattgttatacgagggatcccggtgtcaggtgggagtactgcaacctgacgcaatgctcagacgcagaagggactgccgtcgcgcctccgactgttaccccggttccaagcctagaggctccttccgaacaaggtaaggagtctgtggccagacatctacacgcttcgatgctgggatgaaaagccatggaaattcccactgatgcagccgccttcaatggtaaacggatgctcgagtgttgcctgagttctaccatgtaggaggaagcctccgtgcactctctgggggagccagcggagtgatttctggtgcaacgtggttgggctttgtctttaggatgggcacaaaccctccagggggatcgacttcaaaattcaccttgttgtaaaacgggctacctcagtgtcccagccaaaatttttattgtaacatgctgtcaggtgtgtcactctttccaagccagtaagcttttccggggatttcttcaagtagccagcattcagagcaatcttcagcattgcagattctgagaaatgtggctctggagcctgtcaccctcgagaaacctaagagggctgcattgattccatgtggccctgggtctatggagcagtacatgagctcccagtgctctaaggctcttcagccctaggctttgaagggagtgatttctcagtattcttaaacctctttctgatgacacttgtacctgtgaggggtctagagagaaagagtagtagactcctactttactacaattcaggatgcagggcatgagaggattccctctctcctccaagggaagaagcttttggcgtgcacacatccctgagaagcaaagtgtctttgtcttcagtcagatacataggaccgttttctgccccatggcccggaagccaaaggccttggctttcatgatcaacggtctagggaaacatgcaaaatttccatgtctgtcccaaactcttcccccgacagccaattaccacctgcagcccgcattgccaaatgcggtgccgtttgcatgaagattcagtagagtttcctagaaaggtgctacctcgtgagctcactttccaatgaggaatctgatctgttgtgtttctctaaggtgtcaggtgaaatatttccaagaacttactacagttctagaatgggaggaatctgttgctttggtgtttgtttgttggtcggttttctcacatccatctgcctatggataaggaaaagagaacggtcgtaattctcatagactcctttctggttgtgtcacaaatggcttcacatgtttctctatgctcagagatactcagcttgatttcccgtgttttcatttcagcaccgactgagcaaaggcctggggtgcaggagtgctaccatggtaatggacagagttatcgaggcacatactccaccactgtcacaggaagaacctgccaagcttggtcatctatgacaccacactcgcatagtcggaccccagaatactacccaaatgcgtatgtctttgttctttaccataagagaagaaagggccaagtgaagtttctgttacaagagatgtgtctcaagctgagttctccgaactcaacttgtgacagatgcagatggcgtagcaaaatgtctcaggatgattgccttggagctaagggtctgagagaagggaaatgttaagctccctctccttcctcctagttctattgagcagaagggaaatctggaggtgagaagatcacattatgaagaaagtcagaatgacaaaggaccagacacttagattacccttccacaacaccaactaaacgtcaatggagactttccagttggaattccgttattctggcttccacttcctgaagggaaggttgcgtttgccttttctctctgggttcaagaggaaagaataggtgcttatttatggacaggtgaattgatctgtttctatatctacgtatattccgattgtcagaaaaacactcgttcctaagtaccagtggcctgaagggatacaggttcccagcaagagaagatccaaggaaggaaggcagatgagagtcagcacagagagggatgctgaaaagtaaaagggatgggtggatggagagaagcccgggtctgaccacccaatggccaatattttggccacaagcgactaccagagacatggaaaaatggtttctacatgtgggacaacagatggtagaggacctagagaattgagagaggggcaatgatgggctccactccgcagatgccttggctttcttcctggatacccttcctgcactgaatagcaaggagatggagcccaagcagactgtagccatcttgctgaatggaggagagggattggagtttgggatgactgtggtagctgaaatttttctaggtctgctagaaataagaactggtttgtgtggaggaaaagagctctacaaatacgcatagaagtctcctccagtcgttggcctgacatgacgctgcctgtgcacaggaaatggttccacgagaaagtgtggcaaagaacatttactgagaaacagcaagtacaagagcacaggaagctcaataaagaagagagagatcacatagcactctgggatactggagttcttcccagctagaccagagagtcctcacggagcacattgccaattcagtggagaccccagaacagccgtaatttaaaggtacacttagtatattactagaataaagtcagctgcagacaaccccttgcacagctggaaagcaagtgtccaagcatcaaatcggtttccaatcaatgaagtgcctgtgagaggaaatctcaactctctttagaagtaaacaacaaagtcgattgcctcagctatgcggtatccgcagagtgagtcctaaatttaaaatctgactacatgtagaaaagcgtttcgtgtgacccatgaccaggaaataaatcgggtaatacaaacaggctcaggaatgagagaaatgattagaattgcgtgaaaatttgacatatcagtatgataactgatttcaaatatttaaaaaaacaacatgcaagaaagcagatatcatatcaagagaaattaacagtacagaatagccaaattaaattaaagaggtagtataaaaaaagtatgtcttaattgaaaaaaattactgtatggccggctgatcaatttagacgtttcagaggaaaacattacccaacacacaattctagagaacctacagaatgagctacacacacacacacacacacacacacaaactgaaaacacacccatactcacacacacgcagaaactcacaagttctaacacacacagacacgcgcacccctgaagaaacagtgaaatataaaattaagcgagcctcacagacatgtaggaaaatatgaaaagatttcctgcatgtgggaagcaagtcacagtaaagagcaagggagtttggaatagaaacaaataccggaatcaaggatggctgataacttttcaattacgaagaacattaaaaaaaatcacagaatcgtgaaactcaagggatcacatagggaatttcggaaaaaaaacccaacctgtatgatgtacttttgtacatcacagttcgaaggtaacaaggcaaagatataataagaagaaacctgtcacgagaaactggaggaaaaagagctgtgtcttcctacaagtacactgatacaaattgccaatgtgttcacctcagaaacactggaagccagataccagggaatattgttaaaatgataatcaggaacaaaaagagatcaaccgggaatgctgaatccagcaataaaatgccttgaaggtcatccatgtcggataaatgcatattgtgcactgccccaaagaaagaaaccggaaactgtaagaattggaaatcagcaggcttatgtaacaagagaggtgacccgaaggaattaggtagaagaagaattgaacaagaaaggaactttctgcagcccacgtaatgaagaatccagcaattggcaaatgtagatagatgtaaatgcaaaatattttcttgatcaaatttctatatctttgtaaatgagagttgactacttgaaacaaaatgatagcaagatatttaacttcagcatatgtagaggtaagaatttgaaatggtagcataaatcacgaagggattaattcgaagtgtaccgttgtaagtttctttacctcatgcacgatggtgtgtcatattaataaaagggtactgtgcgggttcgaagggatattgcaaatcctagagcaatcacaaaggtttgaactctgaggtttttggtataataagaatagtccatgcattcaaaagagggaagccaaggaagaactagaagtctttcaagagctcaggctcttatacatccagttgctcattgaaccagcttcctggaatggagggtctggggttgagactaggccacaagtctagagtctctagagagacagtgttggaaccccatggcccataatacatttcccattttctcaggcagccagaggtcatgaatgtgaggatactgggaggttggagcaacgttcttgggaggcataaggaagagcgaatgcttcaagatccccgcagcccaaactactcgcctgctttgccccctaatgcatttttctctgctgctccgtagctgtccgacctcttcagatctcttagtccaccctgccgtcttcctttatgccatgggtcccactgttctttcaactcatccccctttccctcagtcccggagtagctgcggccagcagagggtagactgagagcaggagagaaggacctgcctaggaaccccttctagagatactgcatcctgcctgggagcaagttttccagggcagctttgagaagtcttggagaaacaaacctactaaacctgacagacagtaatactatttgcacaatgcttttctgtgggaaaggtagagccttttcactacgtattgagtacatagagtgtgagggttgacctggaacggctatcctcctggatgacgtgcgttttctgaagaactacatgttcgttgcaactcccacattagaatatgaagtcctaccgagagagatacggagactagacagatacagatgcatttgcatgtgaatacacaatcccacaatacagacgtcaaaacccataccagttattccagagagatggattgggcagaaggcagaaggagaatactctgatcgtttttcggccacgtgtgtgtgttatctcagtgtttctaagaagcgtttgctactttagattttttatttaaaaaaaatagtaataatctattaagtatgagagatgtgcagagaggattagtgatcgagagccatttttgctggtggcaatcatatggtacttttaatgggaatattagaaaggcaccggtaatgaccttgttgcagcacaaaggagagagtgtggggtgcccctgcatgttgtcccacctcttgtgacgtgtatcgttttggaatttccagtggcttgatcatgaactactgcaggaatccagatgctgtggcagctccttattgttatacgagggatcccggtgtcaggtgggagtactgcaacctgacgcaatgctcagacgcagaagggactgccgtcgcgcctccgactgttaccccggttccaagcctagaggctccttccgaacaaggtaaggagtctgtggccagacatctacacgcttcgatgctgggatgaaaagccatggaaattcccactgatgcagccgccttcaatggtaaacggatgctcgagtgttgcctgagttctaccatgtaggaggaagcctccgtgcactctctgggggagccagcggagtgatttctggtgcaacgtggttgggctttgtctttaggatgggcacaaaccctccagggggatcgacttcaaaattcaccttgttgtaaaacgggctacctcagtgtcccagccaaaatttttattgtaacatgctgtcaggtgtgtcactctttccaagccagtaagcttttccggggatttcttcaagtagccagcattcagagcaatcttcagcattgcagattctgagaaatgtggctctggagcctgtcaccctcgagaaacctaagagggctgcattgattccatgtggccctgggtctatggagcagtacatgagctcccagtgctctaaggctcttcagccctaggctttgaagggagtgatttctcagtattcttaaacctctttctgatgacacttgtacctgtgaggggtctagagagaaagagtagtagactcctactttactacaattcaggatgcagggcatgagaggattccctctctcctccaagggaagaagcttttggcgtgcacacatccctgagaagcaaagtgtctttgtcttcagtcagatacataggaccgttttctgccccatggcccggaagccaaaggccttggctttcatgatcaacggtctagggaaacatgcaaaatttccatgtctgtcccaaactctgcccccgacagccaattaccacctgcagcccgcattgccaaatgcggtgccgtttgcatgaagattcagtagagtttcctagaaaggtgctacctcgtgagctcactttccaatgaggaatctgatctgttgtgtttctctaaggtgtcaggtgaaatatttccaagaacttactacagttctagaatgggaggaatctgttgctttggtgtttgtttgttggtcggttttctcacatccatctgcctatggataaggaaaagagaacggtcgtaattctcatagactcctttctggttgtgtcacaaatggcttcacatgtttctctatgctcagagatactcagcttgatttcccgtgttttcatttcagcaccgactgagcaaaggcctggggtgcaggagtgctaccatggtaatggacagagttatcgaggcacatactccaccactgtcacaggaagaacctgccaagcttggtcatctatgacaccacactcgcatagtcggaccccagaatactacccaaatgcgtatgtctttgttctttaccataagagaagaaagggccaagtgaagtttctgttacaagagatgtgtctcaagctgagttctccgaactcaacttgtgacagatgcagatggcgtagcaaaatgtctcaggatgattgccttggagctaagggtctgagagaagggaaatgttaagctccctctccttcctcctagttctattgagcagaagggaaatctggaggtgaggagatcacattatgaagaaagtcagaatgacaaaggaccagacacttagattacccttccacaacaccaactaaacgtcaatggagactttccagttggaattccgttattctggcttccacttcctgaagggaaggttgcgtttgccttttctctctgggttcaagaggaaagaataggtgcttatttatggacaggtgaattgatctgtttctatatctacgtatattccgattgtcagaaaaacactcgttcctaagtaccagtggcctgaagggatacaggttcccagcaagagaagatccaaggaaggaaggcagatgagagtcagcacagagagggatgctgaaaagtaaaagggatgggtggatggagagaagcccgggtctgaccacccaatggccaatattttggccacaagcgactaccagagacatggaaaaatggtttctacatgtgggacaacagatggtagaggacctagagaattgagagaggggcaatgatgggctccactccgcagatgccttggctttcttcctggatacccttcctgcactgaatagcaaggagatggagcccaagcagactgtagccatcttgctgaatggaggagagggattggagtttgggatgactgtggtagctgaaatttttctaggtctgctagaaataagaactggtttgtgtggaggaaaagagctctacaaatacgcatagaagtctcctccagtcgttggcctgacatgacgctgcctgtgcacaggaaatggttccacgagaaagtgtggcaaagaacatttactgagaaacagcaagtacaagagcacaggaagctcaataaagaagagagagatcacatagcactctgggatactggagttcttcccagctagaccagagagtcctcacggagcacattgccaattcagtggagaccccagaacagccgtaatttaaaggtacacttagaatattactagaataaagtcagctgcagacaaccccttgcacagctggaaagcaagtgtccaagcatcaaatcggtttccaatcaatgaagtgcctgtgagaggaaatctcaactctctttagaagtaaacaacaaagtcgattgcctcagctatgcggtatccgcagagtgagtcctaaatttaaaatctgactacatgtagaaaagcgtttcgtgtgacccatgaccaggaaataaatcgggtaatacaaacaggctcaggaatgagagaaatgattagaattgcgtgaaaatttgacatatcagtatgataactgatttcaaatatttaaaaaaacaacatgcaagaaagcagatatcatatcaagagaaattaacagtacagaatagccaaattaaattaaagagctagtataaaaaaagtatgtcttaattgaaaaaaattactgtatggccggctgatcaaattagacgtttcagaggaaaacattacccaacacacaattttagagaacctacagaatgagctacacacacacacacacacacacacacacacacaaactgaaaacacacccatactcacacacacgcagaaactcacaagttctaacacacacagacacgcgcacccctgaagaaacagtgaaatataaaattaagcgagcctcacagacatgtaggaaaatatgaaaagatttcctgcatgtgggaagcaagtcacagtaaagagcaagggagtttataatagaaacaaataccagaatcaaggatggctgataacttttcaattacgaagaacattaaaaaaaatcacagaatcgtgaaactcaagggatcatatagggaatttcggaaaaaaaacccaacctgtatgatgtacttttgtacatcacagttcgaaggtaacaaggcaaagatgtaataagaagaaacctgtcacgagaaactggaggaaaaagagctgtgtcttcctacaagtacactgatacaaattgccaatgtgttcacctcagaaacactggaagccagataccagggaatattgttaaaatgataatcaggaacaaaaagagatcaaccgggaatgctgaatccagcaataaaatgccttgaaggtcatccatgtcggataaatgcatattgtgcactgccccaaagaaagaaaccggaaactgtaagaattggaaatcagcaggcttatgtaacaagagaggtgacccgaaggaattaggtagaagaagaattgaacaagaaaggaactttctgcagcccacgtaatgaagaatccagcaattggcaaatgtagatagatgtaaatgcaaaatattttcttgatcaaatttctatatctttgtaaatgagagttgactacttgaaacaaaatgatagcaagatatttaacttcagcatatgtagaggtaagaatttgaaatggtagcataaatcacgaagggattaattcgaagtgtaccgttgtaagtttctttacctcatgcacgatggtgtgtcatattaataaaagggtactgtgcgggttcgaagggatattgcaaatcctagagcaatcacaaaggtttgaactctgaggtttttggtataataagaatagtccatgcattcaaaagagggaagccaaggaagaactagaagtctttcaagagctcaggctcttatacatccagttgctcattgaaccagcttcctggaatggagggtctggggttgagactaggccacaagtctagagtctctagagagacagtgttggaaccccatggcccataatacatttcccattttctcaggcagccagaggtcatgaatgtgaggatactgggaggttggagcaacgttcttgggaggcataaggaagagcgaatgcttcaagatccccgcagcccaaactactcgcctgctttgccccctaatgcatttttctctgctgctccgtagctgtccgacctcttcagatctcttagtccaccctgccgtcttcctttatgccatgggtcccactgttctttcaactcatccccctttccctcagtcccggagtagctgcggccagcagagggtagactgagagcaggagagaaggacctgcctaggaaccccttctagagatactgcatcctgcctgggagcaagttttccagggcagctttgagaagtcttggagaaacaaacctactaaacctgacagacagtaatactatttgcacaatgcttttctgtgggaaaggtagagccttttcactacgtattgagtacatagagtgtgagggttgacctggaacggctatcctcctggatgacgtgcgttttctgaagaactacatgttcgttgcaactcccacattagaatatgaagtcctaccgagagagatacggagactagacagatacagatgcatttgcatgtgaatacacaatcccacaatacagacgtcaaaacccataccagttattccagagagatggattgggcagaaggcagaaggagaatactctgatcgtttttcggccacgtgtgtgtgttatctcagtgtttctaagaagcgtttgctactttagattttttatttaaaaaaaatagtaataatctattaagtatgagagatgtgcagagacgattagtgatcgagagccatttttgctggtggcaatcatatggtacttttaatgggaatattagaaaggcaccggtaatgaccttgttgcagcacaaaggagagagtgtggggtgcccctgcatgttgtcccacctcttgtgacgtgtatcgttttggaatttccagtggcttgatcatgaactactgcaggaatccagatgctgtggcagctccttattgttatacgagggatcccggtgtcaggtgggagtactgcaacctgacgcaatgctcagacgcagaagggactgccgtcgcgcctccgactgttaccccggttccaagcctagaggctccttccgaacaaggtaaggagtctgtggccagacatctacacgcttcgatgctgggatgaaaagccatggaaattcccactgatgcagccgccttcaatggtaaacggatgctcgagtgttgcctgagttctaccatgtaggaggaagcctccgtgcactctctgggggagccagcggagtgatttctggtgcaacgtggttgggctttgtctttaggatgggcacaaaccctccagggggatcgacttcaaaattcaccttgttgtaaaacgggctacctcagtgtcccagccaaaatttttattgtaacatgctgtcaggtgtgtcactctttccaagccagtaagcttttccggggatttcttcaagtagccagcattcagagcaatcttcagcattgcagattctgagaaatgtggctctggagcctgtcatcctcgagaaacctaacagggctgcattaattccatatggtcctgggtctatggagcagtatatgagctcccaatgctctaaggctcttcagtcctaggctttgaagggagtgatttctcagtgttcttaaacctctttctgatggcacttgtacctgtgaggggtctagagagaaaggttagtagacttctcctttactgcaattcaggatgcagggcatgagaagattccctccctcctccaagggaagaaggttttggcgtgcacacatccttgagaagcaaagtgtctttgccttcagtcagatatataggatcgttttctgccccatggcctggaagccagaggccttggctttcatgatcaacgatctagggaaacatgcaaaatttccatgtctttcccctcctctgccctcgacagccaattaccacctgcatcctgcattgccaaatgcagtgccctttgtatgaacattcagtagagtttcatagaaaggtgctacttcgtgagcgcactttgcagtgagaaggagtctgttctgttctgtttttctaaggatttcaggtgaaatatttcctagaacttactacagttctagattggtaggaatctgtaggtttgctgtatgttttttggttggttttctcccatccatctgcctacaggtaagggaaagataacgttcataattctcatagactcctttctggttgtgtcataaatggcttcacatatttcgttattctcagagatactcagtttatttcttgtgttttcatttcagcaccgactgagcagaggcctggggtgcaggagtgctaccacggtaatggacagagttatcgaggcacatactccaccactgtcactggaagaacctgccaagcttggtcatctatgacaccacactcgcatagtcggaccccagaatactacccaaatgcgtatgtctttgttctttaccataagagaataaagggccaactgaagtttctgtgacaagagacatgcttcaagctgagttctccgaactcaacttgtgtcagattcagatggtgtagcaaaatgtctcaggatgatttccttggagctaagggtctgagagaagagaaatgttaagctgcctcaccttcctcctagttttgtggagcagaagggaaatgaggaggcgaggagatcaccttatgaagaaagtcagaatgacgaaccaccaaacacttagattacccttgcccaacacccactaagcgtcaatgaagactttccagttggaattccgttattctgacttccaattcctgaagggaagattgtgtttgccttttctgtctgggctcatgaggaaagtttatgtgcttacttatggacaggtgaattgatctgtttctatttctacctgtattccaatagggagaaaatctcttggtcctaagtaccagtggcctgaaaggatagaggttcccagcaagagaagatccaaggaaggaaggcagatgagagtcagcacagagagggatgctgaaaagtaaaagggatgggtagatggatagaagccctggtctgaccaccccatggccaatcatttggccataatcaacaaccaaagacatggaaaaatggtttctacatgtgggacaacagatggtagaggacctagagaattgagagagggccaatgatgagctcaactccatagatgccttggctttcttcctggatacccttcctgcactgaatagcaaggagatggagctcaagcagcctgtagccatctagctgagcagaggagagggattggagtttgggatgactctggtattttctaggtccgctacaaataagaactggtttgtggaggaaaggagctctacaaatacgcatagaagtctcctccagtagttggcctcacatgacactgcatgtgcacagaaaatggttctacagaaagtgtggcaaagaacatttactgagaaacagcaactacaagagaacagcaagctcaattaagaagatagagatcacatagcactctgtgttattggagttcttaccagctagatgagagagtgctcacggaacacattgccaattcagtggagaccccagaacagccataatttcaaagtacaattagtatattactagaataaaggcagctgcagacaaccccttgcacagctgaaaagcaagtgtccaagcatcaaatgggtttccaatcaatgaagtgcctgtgagaggaaatctcaactctcttcagaagtaaacaacaaagtcaattgcctcagctatgcggtatccccagagtgagtcctaaattaaaaatttgactacgtgtagaaaagaatttcgtgtgatccatgaccagaaaataaatcaggcaatacaaacaggctcagaaatgacatcgataattagaattgcatgaaaatttgacatatcagtatgataactgatttcagatatttaaaaaaagtgcaacaaagcaggtatcatatcaagacaaattaatagtatagaatagccaaatcaaattaaagaactattatacaaaaagtatgtcttaaatgaagaaattactgtatgtccgcctgaaaaatttagatgtttcagaagaaaaaattaaccaaaaacaattctgcagaacctacagaatgagccacacacacacacattcaaaacacacccatacacacacacatgcaaaaactcacaagttctaacacacacacaaacacacacacacatgcacatccctaaagaaatagggaaatataaaattaaccgaccctcagagacatgcaggaaaatataagaagatttcctgcatgtgggaagcaagtcacagtaaagagcaagggagtttggagtagatacaaataccggaatcacggatggctgataacttttcaattatgaagaacgttagaaaaatcacagattcatgaaactaaagggatcaaataggaaatttcgagaaaaaaaactacatgatgcacttctctacatcacagttcaaaggtaacaaggcaaggatataagaagaagaaacatctcacgagaaactggagaaaaaagagctgtgtcttcctagagtacagtgatacaaattgctaatgcgttcacctcagaaacactggaagccagataccagggaatattattaaaatgataatgaggaacaagaagagatcaaccgagaatgctgaatccagcaataaaatgccttgaagatcatccatgttggataaatgcatattgtgcactgcccaaaacaaagaaactggaaagtgtaagactttggaatcagcaggcttatgtagcaacagaggtgacccgaaagaattaggtataagaagaatagaagaattgcatgaaaatttgacatatgactaagataactatttcaaatatttaaaaaaagatgaatatgtaataaaacagataaaatatcaaaagaaagtaacagtattgactagccaaatcaaattaaagacttagtgtaaaaagctatgtcttaaaagaaaaaattactggatggctgcctgatcaatttagacatttctgaataggaaactaaccaaaaatcaattctacagaaccaactacacacatatatacacatacaacacacccatacacacccacgcaaaaactcacaagttcacacacacacacacacacacacaaccctcaagaaatagtgaaatagaaaaccaaccgaacctcacagacatgttgcaaaataggaaaagatttcctgcatatgggaagcaagtcacagaaaagagaacgggagattggaaacagaaacaaataccggaatcaaggatggccgaaaacttttcattgatcaagaatattaacaaaatcgcaaaaacacgaaattcaatgcatcaaataggcgtttcgaaaaaaagaaaaaatctggtatgatgcacttttgtacttcacattttcacggtaagaagacaaagatataataacaagaaacttcttatgagaaactggggaaaaacaagctgtttcttgctagaagaacagtgatacaaattgctaatgcattctcgtcaaaaacactggaagccagataccgggaatgttattaatgtggtaaacaggaacaagaagagatcaaccaagaatgctaaatccagcaataaaatgccttgaagatcatccatgctgcataaatgtatgttgtgcactgccccaaacaaagaaaccggaaactgtaagaatttggaatcagcaggctgatgtaacaagagaggtgacccaaaggaattaggtagaagaagaatagtacaagaagggaactttctgcagcccatgtaatgaagaacccagcaattggcaaatgtagatgtaaatgcaaaatattttcttgaccaaatttctatatatttttaaatgagcgttgactactggaaacaaaatgatagcaatatatttaattttagcatatgtagaggtaagaatttgaacaagtagcgtaaatcatgtagggaataattagaagtgtaccattgtaagtttcttacctcatgcacaatggtatgtaatattaataaaatgttactgtgtgggttcaaggagatattgcaaatcctagagcaatcacaaagttttgaactctgaggtatattgtataataagaatattccatgtattcaaaagagagaagccaaggaagaaagaaatttgtcacgagtttgggctcttagtacatcctgtagctcattgaaccagcttcctggaatggagggtctgggattgacactaggccacatgtatagagtctctagagagacagtgtttcatccccatggcccgtaatacatttcccattttctcaggcagccacaggtcatgaatgtgaggatagagagaggttggagcaacgttcttgggaggcataaggaagagcaaatgcttcaagatccccgcagcccaaactcctacctgctttgccccctaatgcagtgttcctccgtagctgtccgacctcttcagatctcttagtctaccctgccatcttcctttatgccatgggtcccactgttctttcaactcatccccctttccctcagtgcagagtagctgcggccagcagagggtagactgagagcaggagagaaggtcctgcccaggaacccattctagagatgctgcattctgcctgggagcaagttttccagggcagctttgagaagtcttgcagaaacaaacctatttgacccacatgatatgggaatgacagaaagtaatacaatttgcacagtgcttttccatgggaaaagtagagccttttcgcgaggttttgagtacatagagagtgaaggttgacctggaaaggttatcctcctggatcccatgttttttctgaagaactacctgttagttgcaacttgcacattagaatatgaagtcctaccgagagagatacggagaactagataaatacagatacttttgtatgtgaataaacgattccacaatacacacatcaaaatccataccagttattccagagagatggattgggcagaaggcagaaggagaatactctgatcgttttttgcccacgtgtatgtattatctcagtgtttctaagaagcgtttgctactttagatttttttttataataataatcttttaagtatgagaaatgtgcagacaggattagtgattgagagccatttgtgcttgtggcaatcatatggtacttttatgggaatattagaaaggcactggtaatgaccttgttgcagcacaaaggagagggtgtggggtgcccctgcatattgtcccacctcttgtgacgtgtatcgttttggaatttccagtggcttgatcatgaactactgcaggaatccagatcctgtggcagccccttattgttatacgagggatcccagtgtcaggtgggagtactgcaacctgacacaatgctcagacgcagaagggactgccgtcgcgcctccaactattaccccgattccaagcctagaggctccttctgaacaaggtaaggagcctgtggccagaaacctacacgtttcgatgctgggatgaaaagccatggaaattcccactgatgcagcagcctccaatggtaaacggatgctcgagtgttgactgagttctgtcatgtaggaggaagcctccgtgcactctctgggggagccagcggattgatttctggtacaacgttgggtgggctgtgtctttagaattggcacaaaccctccagggtgatcgacttcacaactcacctcgttgaaaaatgggctatctcagtgtcttagccaaaatttttattgtaacatgctgtcagatgtgtgactctttccaagccagtaagcttttcctgggacttcttcaattagccagcattcagtgcaatcttcagcattgcagattcagagaaatgtggctctggagcctgtcacccttgagaaacagggctaacagggttgcattaattccaaatcaccctggttctatggagcagtacatgaactcccaatgatctatgtttcaggacttcctcagtcataggtgggctctgcagccctaggtttttaagtgagtgactgccccgtgttctggtggcagttgtacctgtgagcggtctggatagaaagagtcggagacttctgtattattgcaactcaggatgtgggtcatgagaggatttcatctctcctgcaggggagtaagctgttcgcctccacccatccctgataactgaagtgtctttgtctgcagtcctagacgaaggactgttgtctctcccatggcccagaagctgaagaccttgccttttgttatgaaacgttcattgttttcatgtctgtccgtttctctgcccctaacacccaatcaccatgtatggcctgtacccccaaatgcatcgtgctttgctgtttgctgccccatagtcctcatgaacattcagtagaaattcccataaatgtgcttgcacgtgagcacagtttccattgagaagccctctcatttgtcctttttttctaagcttttatgtgaaatatttctaagaacttactacagttctaaagtgttaggaatttgtttctttggtgtttttgtttgttggttggttgttgcttttctcaagtccatctgcctacaaataaagaaacaagaatgttacttgtcatattctcctgaggtcataattctcagagacttttttctggtttgtgccataagtggcttcacatgtttgtctcttcttggaaacactcagtttgatttcttttcttttcatttcagcaccaactgagcaaaggcctggggtgcaggagtgctaccacggaaatggacagagttatcaaggcacatacttcattactgtcacaggaagaacctgccaagcttggtcatctatgacaccacactcgcatagtcggaccccagcatactacccaaatgcgtatgtctattttctttaccataagtgaaggaagggtcagtggaaatttctgttagtagagtcatgcttcaagctgagtgttcaggactcaagttgtctcagatgaacagtgcatagcaaaatgtctcaggaacattgtctttgagcaaagagtctaagagaagacaaatgttaatctggctctccttcctcctagtttaatggagcagaaaggtatctggaggcaaggatatcacattaagaaacaagtcaagatgacaaatgatgaaactcttagagtacccttccacaacacccactaaggttcaatgcagccttttctccttggaattctattaaactaaactccaattcctgaagtgaaggttctgttggggttttctgttttggcttacaaggaaagtatatatgtatatctatggagaggcaaatctatctctttctatatctacgtctattccaatatgtagaaacacagtcggttctgaccaccagtggtctgaagggatactggttgttagagaataaaaatggcaggaaggcagatgagagtcagcaaagagagagatcctgtaaagtaaaagggtggatagatggacagaagcccaggtctgaccagcccatggccaggctttaggccataagtgacaccaaagacatggaaaaatggtttctacatgttggacaacagacagtagtggaccaaaagaatagtgacagggggaacaatgagatcaactccatagataccttggctttcttcctggaggcccttcttgcactgaagagcaaggtgatggagcccagatggactgtagccatcttcctgaatgcaggagagagattggaatttgggactactgtggtagctaggattttataggcctgctgagaatgagaatggatttgtggatgaaaggagctccaggggcacgcatagtagtctcctcgaatctttggctaaacatgacgttgcatgtgcccagaaaaaggttccacaagaaagtagagaaaagaatatatcctgaggaatagcaactgcgattgaacagtgagctcaataaagaggacagagccctcatagcattctgggatactggagttctgaccagctggaggagagacctcactgaacctcttgggaatacagtagagactccagaaaagtcatactttaggagtagaattagtaaatttctagaaaaaaaggcagctctagacaaaccctggcaaaactgaaaagcaagtctccaagcattaaaatcatttccaagtcaattaactgcctgggagaggaaaaccctctttagaggtaaacaacaaagtcaagtggctcagctatgtggtgttcacagtgtgagttctaaatttaaaacttgactacacatagagaagcttttagtatgaaccatgaccaggtgaaaaatcagtcaatacaaatagacctagaaatgacagaaatgattagaatggcaaaaaatttgacatatcaatatgtcaactgagttttaggttttaagaaaacatgaatacggaatgaagcagataccatatcaagagacagtaacagtatagaagagccaaattaaattaaagaactagtataagaaggtatgtcttaaatgaaaaaattactggatgtattcccaatggagtgagatgtttcagaagtaaaaactaactgaaaaacaattttataccacctacagaaccagctacacatacacaaatgacacacacatatacacacatactcacacatgcacaggcttagaaacatgcacgcacacacacacacacacacacacacacctccacaaatactaaaaaatgaaatccactgatcctcacagacaggcgggaaaatataaaaagatttcctgcatgtgggtaggaagtcacagaaggagaggaaggagagattgctacaggaacaaatactggaagcaaggatagctaaaaacttttcaaataagaagaatattaaaaaccacagattcaagaagctgaatgaatcagacagggaatttccaaaaaaaaaaaaaaaaaaactgtatgattcacttttgtacatcaccgttcaacagtcagaaggcaaagatataataacaagaaacatctcatgagaaactggaggaaaaagagctgtgtcttgctagaagaacagtgatacaaattgctaatgcattctcatcagaaacactggaacccagttaacaggggatatcattaaaatgataaactagaaaaaaaagagatcaaatgagaatgctacatccagcaataaaatgccttgaagatcatccatgttggataaatgcatattgtgcactgccccaaataaataaaccaaaaactaataatttggaatcagcaggcttgtgtaacaagagatgttgcccaaagaaaattagctagaagaagaatagttcaagaggagaactttctgcagcccacgtaatgaagaacccagcaaatggcaaatgtagatgtaaatgcaaaatattttcttgatcaaatttctatatctttttaaatgagagttgactacttgaagcaaaatgatagcaatatatttaactttagcatatgtagaggtaaaaatttgaacatatagactaaatcatgtggggaataattggaagtgtaccattgtaagtttcttaccttatccacgatggtatgtaatattaatgaaaggttgaatttgtgggtccaaagggatattgtaaatcctaaagcaatcataaaattttgaattctgagggatattatataataagaattttccatgtatccaaaagagggaagccaaggaagaaaaagaagtctttcaagtactcaagctctgagcacatccagttgctcattgaaccagcttcctggaatggagggtctgggcttgagactaggtcacatgtgtagagtctctagagagacagtgttggatccccatggcccataatacatttcccgttttcccaggcagccacaggtcacgaatgggaggattctgagaggttggagcaatgttcttaggaggcataaggaggagtgaatgctctgagatttccccagcctgaggtcctccatagctgcccgacctcttcagacctcatagtctgcccagctgtctccctttatgccatgagtgccactgttctttcaactcatcccccattccctcagtcccggaattgctgtggccagcagaggatggactgagagcaggagaggaagtcctgaccaggaacccatcctagagatactgcatcctgcctgaaagctaggtttccagggcagctttgagaagtcttgcagaaagaaacccacttgacccacctgatacggtatcgacagacaggaatactttttgtgcaatggttttacatgctgaacatagagccttttggctacattttgagtacattgaatgagactgctggcctgggaaggatatcatgctggatgccatttttttctctggagaactatgtgttagttccaactcgcacattactatatgaagtcctacacagagagatacggagagctagacagatagagatacttttgtatgtgcataaccaattccacaatacacacgtcaaaatccataccagttattccagagagatggattgggcagaaggcagaaggaggatattctgatccctttttggccacatgtatgtataatctcagtgtttctaggaagtgtgtgctgcattagattttttttctttaaaaaaagtgataatatattaagtatgagaaatgtgcagagaggattagagattgagagccatttgtcattgtggcaattgtatggtatctcttttgggaatatttcaaaggcaccagtaatgaccttgttgtagcaaaatatacagtgttcctgcatatgtacccattttttgtgatgtgtattcttttggaatttccagtggcttgatcaagaactactgccgaaatccagatcctgtggcagccccttggtgttatacaacagatcccagtgtcaggtgggagtactgcaacctgacacgatgctcagatgcagaatggactgccttcgtccctccgaatgttattctggctccaagcctagaggctttttttgaacaaggtaagaagttgtgccagacatttacctgcttggatgctgggatgaaaagccatggatacccccactgacgcacaacccttcagtgctacactggttctcgtgtgttggttctgggtctgccatgtgggaggaagccttagcgcactctctgggggagccagaggtgtgatttttggtgcaacctgtgcgagctgtgtctttaggatgggcggaaaccattctgggtgctcgacttcaccactcccctcattgtaaaaggggctatctcattgtcctagacaaaattcttattgtaatatgctgtcagatgtgtgtgtctttccaagccagtaaacttttccagggatttcttcaagtagacagcattcagtgcaatcttcagcattgcagattccgagaaatgtggctctagatcctgttatccttgagaaacctaactgggttgcattaattccatatctccctgggtctgtggagtagtacatgagctcccgaagctctatctctcaggtctttttcagtccgaggcaggttgtgcagttcttagctttgaagggagtgattttttcgtgtgcttttgcctctttctgatggaacttgtacctgcggggggtctggagaaaaagagtagtagacttttgctttattgcaatgcattatgctgggcacgagaggattccctatcttattgtaggtgataagcttttggcctccactcatccctgagaagtgaagtgttgttgcctacagttttagctgcaggactgttgtctgccccatcaccaggagtttaatgctttcttttttgagcaatcatctagggacacatgcaaggtttttatatgtccttgcctcctccccaaaaaaccattttaatgcttggagacttgcttttcagctttgccaaatgcatcaccctttcttctatgctgttccatgtcgtcatgaacactctgtagagattcctagaaatgagcttccatgttagtggagtttccgatgagaagcaatctgatatttcttttccactaagttttacatgaaatatttctaagaacttactacagttctagaatggtaggcatctcttactttcgtgtttgtttgtgtgttttctcatgtccatttgcctattaataaagaatagagaatggttgtaaatctcagtgactcttttttggtttatgtcataaatggcttcctgtatttttctgttctaggaaataataagcttgatgtcttctgttttaatttcagcactgactgaggaaacccccggggtacaggactgctactaccattatggacagagttaccgaggcacatactccaccactgtcacaggaagaacttgccaagcttggtcatctatgacaccacaccagcatagtcggaccccagaaaactacccaaatgcgtacgtctttgttctttaccataagcgaaggaagggccaatggaagtttctgttagaagagtcatgcttcaaggtgactgctcaggactcaacttggctcagatgcagaggaacatttcctgtgagcaaaagttcttagagaagactttgtttttttgagacagagtcttgctttgttgcccaggctggagtgcagtggcatgatctcggctcactgcaagctccgcctcccgggttcacaccattctcctgcttcagcctctctagcagctgggactacaggcacccaccaccacacccggctaattttttgtatttttagtagagacagggtttcactgttctagccaggatggtcttggtctcctgacctcgtgatccgcctgcctcagcctcccaaagtgctgggattacaggcgtgagccaccgtgcctggctgagaagacattttttaagctggctctccttcctcctagttttatggaagcagaaggatatatggagttgagaagatcttattaataaaacagccgggatgacaaatgaccaaagagttagagtatccttctacaacatcggctgagggttaatacaaccttttcaccttggaattctatcattctaagctctagtccctgaagtgaatgttgtgttggccttttgcatcttgggtcacagggaattgatacttgcacatctatggagaggcaaatctttttctatctacttctttttcaatgggtacaaacacacttggtcctgagcaccagtggtctgaagagatacggtctgcccagaggagaagaacaaaggcaggaaagcagatgagagtcagcaaaggggcgatgctgaaaagtaaaaggggcgggtagatggacagaagccatgatctggccattctatggccagtctttcggccataagtgactaccaaagacacggcaaaacggtttccacatgttgaacaacagatgctagaggaccaagagtattgcaagagggagaaaatgagatcaacccatcaatgccttggctttcttcaaggagacccttcctgcactgaagagcaaggagatggagcccaagctgactgtagccatgttgctgaacagaggagagtgattggactttgggattactcaggtagttaggattttctagccatgctaagagtaagaatggacttgtggaggataggagctccaggcatagaagtctcctcaagtgttagtctaaacataaagcagcacttgcatagaagattttccacaagaaaatatggcaaaaaaacaccatatattgaggaacaacaactacaagggaacagtgagcttaataaaggtgacagagctcacatagtgctctggaatattggagttttgaccagctagagagaagagacctcattgaaaatcttgggcattcagtagagacctcagaaaagtcagactttatgagtagactttgtatattcctagaataaaggcagctccagaaaaaacctagcaaagctgaaaagcaaatctccaagcattaaaatggtgtcctagtcaattaactgccttctagaagaaaactcaacactctttacaggtgaacaacaaagttaagttgctgagctatgcaatatccacagtgtgagtcctaaatttataactttactacacataaaaaagcatttagtgtgaaccataaccaggaaaataatcagtcaataaaaatagaaccaggaatgatagaaatgatttaaatggcatgagaatttgacatattagtatcataactgcattgctggatttaagaaaacataaacatggaacgtaacagatatcatatcaagggaaagtaaaaggataaaagagtcaaatcaaattaaaggactattaaaaggtatatcttaaatgaaaaattcactggatggtctcccaatcaggttagttgtttccagggaaaaaattaactgaaaaataattcaatagaatctacagaaatagctgcacatatatacacacaatggcacacgtgcacacacccacacccacacaggtgtgaatcctagagccacacgagcattgaaacatagagaagtaaaaattgttcattgaggaatatgtagcaatgctcaatgtgttttaccctaataagagcttttgtgatgtatgattgaaaaactgacacaactgaagagagaaatagataagcccacactctgagttagagatttccttgattctctcactatggttataaatctttcccaaacacaacaggctagaacaaatatgcagaaaattagacatagtatctttgttctcaataaaaacgtcgacctatttaacattataccgaactaccgagtacacattaaagtgtgcatggagcattcactgaggtgtactctacacatgaccttccagcaagtctccatagatttaaaagaattaaagtcatacagagtgtgtcactttattctcccagaataaagtgagatatgaataatgagaagtttgccagcttctcaaatatttgggagtcatacggtgcatttcaaaatactctttgggacaaagaaaacatcactaaggaatttagaaaagttttgaactgagtaagaatataacacaatttatccaaacttaggagatgcagtgaatgtctttaggcttttacataattttagatgctcttagggaaaaacagaagcatgtaataatcaagatttcaaactgcaattctcaaagtgtagtctagagaaacctgaggacctttgagtaccttcagagacagtccatgaggttaaaggactttgctacgtgaaaagtaagatgctattggccctttttactttcattttccaacaagagaagaggggagttttccagcagttacataatatgtaatggcatcatgtctctgatggctaagaaaatgggcaattgttgactttgtgtgttaaaaaaattctcagtgttggtttcttatactataaatattcatcttgtgttttgaaaaagaaaagctctttggaatcccctatgaacaaagactttgacagttgttgatctaagaccacagcttaaatatctacacaagaaaaaaaaaaaaagcaaataagagccaaggaaagcagatggaaggaagtagtccaaaccagtgacattcagtgaacaagaaaagagaccaacaagggagtaaactcttgaaacagaaagttgattctttgaaaagatccatatgattgaacacagtctggctaaacaaatgacagaccaatgagggtgcacaaccatcaccatctggagtaacagaggagaggtgccattactatagcatcttccagttctgaaagctgaaaagaagattttgagaacaattgtatgtgaataaattcaggaatgttaatcatgtgggccaattcctgaggaagacaacaaatcagcaaaccagatgctgaatagttagtgtagtcctgtagagagacatacagagaggctgacagagaaatatttgtatgtgcataaaacaatctacaagacacacttcaaaatcaatctcagttaatctggaggaacatatttcacagaaggtggaaggagggtattctgatcctcttgtacattgtacaacattgtacaatgtacagagtataattgtacaagtacaattgaagttgtacaagtacaagtgcaacttgcacaatgtacagagtaaacattgatgtttactctcaattttcttatggagcacagatgactttggatgtgttacaatatgaatgataatttgtctttgagatgttcgcagttgtttagaagttgaggaccatttgtgcatattatgggacctttagtgaaaatatttcaaagtctctttttacactttgttacagcaaaatgtagagggcgctaagtgcccttgaatcttctcccatctctggtgacctgtgttgttttgaaatttgcagtggcctgaccaggaactactgcaggaatccagatgctgagattcgcccttggtgttacaccatggatcccagtgtcaggtgggagtactgcaacctgacacaatgcctggtgacagaatcaagtgtccttgcaactctcacggtggtcccagatccaagcacagaggcttcttctgaagaaggtaggaagtctatggccagacaaccacaccctaggacgttgggatgaaaagagttgcaaaatcttagtgatatagaagccttccatgctcacacaattccaagtagaatgtggactcagggtcagccactgggaaggaacactcagcgccttctctgggagaaccagagctgtgatgtttggtaccctgtgaaagggtggtatctataggaagggtgcagaccctctagggcactggacttaccactcccctggttattcaaaggatcattttagtgtcttagccagaagaatattctaacattttgccaaatttgtgaagatttaccaagctcatgataagcctttcatggtatttcttcaagtagtcagtgttcattgcatctttggctttgcggtttcggaggaatgcggtttttgagtctgtcatccttgagaaacctaatatgacttttcttagttccatatacttctgggtccaggtagcagtacatagccaacaaatgctccatcgttctggcctatctccatcttaagccagtcctgcacaactaggctttgatgggagggatctctcagtgttcttgcccctccttctcatggaacatatatctgtgttggtctctgagaagaagagtagtggatatctactttgttgcaatgcagaatcctgggccaaagataccagccatccctccaagggaataaaattttggccagtagccctctctgagagacaatttgtctttgcctacgagtcctagatgcaggaccgcttcctgccccatcttcaagaagctgaaggctttggctttggaggatcagcagtctagggaaatgtgtgacggtttcatgtctgtccccactgacagtcaatcaccacctacaacctgcacagcctgatgcatagcagtctagtttcctgccttattctcaggaacacccagaagatgtctatattaaagagcatgcacatgagtgcaattttgactgataggcactctgatctttcctttggtgcctgtgttttaaaggaaatctttctaagaactcgttaaagttctagaatgctatgaatctttgggttttattattggtatgtccatctgcctgctagtacagaacagagcatggtagtctttctcagagacaatgatcctgtttcagtcacagatttcttctgatgcttctgtgttctagaaattactcagcttgatttctcctctttgaatttcagcaccaacggagcaaagccccggggtccaggattgctaccatggtgatggacagagttatcgaggctcattctctaccactgtcacaggaaggacatgtcagtcttggtcctctatgacaccacactggcatcagaggacaacagaatattatccaaatgggtacaaccttgagttttcttcaaagacagacagcagcccccttacatttctcttggaagggccatgcttccaactaacttcttatgacaaatttatctcagatctggaatgttgggtagaatgtctcaggcttctttcttcaggcacagtgtctgaaaggagagaaatgtcaggccagctctcttttctcatagttgacagaagcaggaggatatttgaaggtggtgagttctcatgaatagaaagctcaggacacatggccacgtgcttagaaatagcaccattccacaatgcccactaaagaccaatgcaatagttcaaccagggatttctgtcattctaatctccaagtcctgaagtgaaggttgtattagccatgttcatcttgggcaacaaataaaggatatctatgttgacatccagatcttccaatcactttctcctctaacctgtacctgggttctgagaacaaggtatctgaagagctatgtgttgccagcacatgaggggcaaaagtaggaaggcagctgagagtcaggaagtataaagattctgaagagttacacatgcaggaagatggacagaaacccagttcagaccacgtcagcgtttctgccatgaaggactatcaaatacataggaaaagtgttttcataggttggacaacagacatgacaggcctgagaaaattcagaaagggaatcaaaggagatcaaccttatcatgtccctggcatccttccttgagacccttgaagggcaagcagatggagcccagctgaccacagcagtcttgcttaactgaggagagagactggagtttgtgatgcctcaggcatctgacgtattctaggctggctaagaatgagaggggatttgtggaggaaaggagctccaagaatacacaccgaagtcttctcaaggctttggctaaatacaaagctgcgtatgcacaaggagagttttcacaaagaaagaacaataaagaaaagctactggggaaagaacaactgcaagggaacagtgagctcaatggagatgctagagctcacatagcactgggggatatttgagttctgaccactcagaggagagacacctcactgaacatcttgggcattcagtagaggtcaaagaaagccataatttgggagtaggatcttcggattcctagaaataaggtgactccagaaacactccagcaacccttcttccaagccagtctaaaaggatccaaatgatttccaagtaaattaactgccttccagaaaaaagtaaactcaaccctccttagaggtaaggaacgaatacaagtttctcagttatatgacatccccagagtgcaacttgcatttaaaaatttactagacacaaaagaagttttcactgtgatccataactgggagaaaaatcactcaacacaaataggcccagaaataatagaaattatggcattggcaagaacatttaaaatgcacctctgagaactgtgtttcaggaaaatgtcagcaaaagctgaccatgagagaaatgaatgcataatatcagaaaagaaaagaattgaagagccaaatggaaatttaaaaactgagaaaagttatatctgtaatgaggaattcactggatggccttataaccagtttagatattatggtaggaaaaggtgaacgagaaaatgattcaattaaagctagacaaaccacaagacagacagacagacacaaatacacatacacacaatgactgaaccaattaatcaacagagcctcaaggacatctaggaaaacatccacacatttaatatatgtgttaggcaagtcacagaaagagaggaaaaagataatgtgacagaagttatacttgaagccatgacggctgacaaatttccaaacatacagaaaatgagaaattcatagtcatgaagctcaatgactcaggtatagatttttaaagagcaaaactctgatttactggggtacatcatagttaaattgtctgatttcaaagctaagaagaaaaaaagggggttcctatgaacaaacattttgacagttgatctaagaccacagcttaaatatctaggcaaggaaaagcaaataagacacaaggaaaggggatggatggaaatagtccaaaccaatgacattcagtgaacaagaaaatagaccaacaaaggagtaaatccatgaaacagaaagttggttctttgaaaagattcatgtgattgaccacagtctggctgaacagatgacagaccaaggagggagtacaaccatcaccatttgaagtaacaggggagaggagccattgctataccatactccaggtctgaaagctgacaagaagatatcaagaaaaactgtatgtgaataaattcatgaatgtagatcatgtggatcaattccttaggtaaacaacaaatcagcaaaccagatactgaatagattgggtactcctatagaaagacatacagatagccagacagagaaacatttgtacgtgcataaaacaatctacaagactcacttcaaaatctctcagttaatccaaagtaacatatttggcagaaggtggaaggagggtattctgatcctttcttgtacacattgatgttttctctcggttttcttatggagtatagacgagtttggatgtgttacaataagaatgataatctgtctttgaaatgttcacagttgtttagaagttgaggacgatttgtgattgttacaggacctttagtgagaatatttcaaagtcactttttaccactttgttacaacaaaatgtagaggatgtctggtgcccttgtatcttctcccatctctggtgaactgtattgttttgtaatttgcagtggcctgaccaggaactactgcaggaatccagatgctgagattagtccttggtgttataccatggatcccaatgtcagatgggagtactgcaacctgacacaatgtccagtgacagaatcaagtgtccttgcgacgtccacggctgtttctgaacaaggtaagaagtctctggccagacaaccacacccttggacgttgggataaaaagagttgcaaaatcttagtgatacagaagccttccatgctgcacgggaatctgaatgtggactcagggtcagccaatgggaaggaagcctcagcgccttctctgggggaaccagggctgagatttttggcaccccgtgacagggtggtgtctttaggaagcgtgcagaccttctagggcactggatttaccactcccctggttattcaatagattatttcagtgtcctagtgaaaatggatattctaacatcctgccaaatttgtgatgatttaccaagctcatcatgagcctttcctggtatttcttcaagtagacagtactcattgcaaacttcagctttacagtttcagaggaatgtggtttttgagtctgtcatccttgagaaacctgatatgactttacttagttccatatcctcctgggtctaggtaacagtacatagccagcaaatgctctatctccctgtctaccttaatcttaggcaggtgctgcacacctaggctttgatggaagggatttcttagtgttcttgcccctccttctcatggaacacgtatctgtgttgctgtttgtgaagaagagtagtggatgtctactttgttgcaatgcaggatcctgggcccaagatttcccgccgtccctccaagggaataaaattttggccagtacccctctctgagagacaatgtgtctttgcctggaagtcctagatggaggaccacttcctgccccatcttccagaaacttaaggctttggctttggaggatcagtgctctggagaaatgtgtgacggtttcatgtctgcccccactgacaaccaccacctacagcctgcaccgcctgatgcatggcactctggtctcctgccttgttctcaggaacacccaaaagagatctttgccaaagaacaggcacatgagtgcaattttgactgataggcactctgatctgtcctttggtgcccaggttttaaagaaaatctttctaaaaactcattgaagttccagaatgctatgaatctttgagctttgttattggcatgtccatctgcctactaatgtagaacagagcatggtcgtcattttcagagatgatgtcctgtttctatcatggattttttttctcatgcttctgtgttctggaaattactcagtttgttttctcctctttgaatttcagcaccaacggagcaaagccccacagtccaggactgctaccatggtgatggacagagttatcgaggctcattctccaccactgttacaggaaggacatgtcagtcttggtcctctatgacaccacactggcatcagagaaccacagaatactacccaaatgggtatgtctttgagttttctcccaagagaaacagccacccacttaaatttctcctggaagagccatgcttccagctaacttcttatgacccaatttctctcagacccagaatgttggacagaatgtctcaggcttcttgctttgggcacagggtctgagaggagagaaatgtcaggccagctctcttttctcatagttgatagaagtaggaggatacttggaggtggtgaggtctcatgaatagaaagctcagaagaacatatgaccatgtgcttagaaatagcaccattccacaatgcccactaaagaccagtgaaatagttcaaccagggaattctgtcattctaatctccaagccctggagtgaaggttgtgtttgccatgtttgtcttgggtaacaagtgaaggatatctatattgacttcgagatcttccgatcactttctcctctaacctgtataaacacattgggttctgagaacaaggtgtctgaaaagctatgtgttgccagcccatgaggggcaaaaggaggaaggcagctgagagtcaggaagtatagagatgctgaagagttacacattcaggaagatggacagaaacccatgtctggctatgccagcctttctgccatgaaggactatcaaatacatgagaaaacagttttcacaggttggacaacagatatggtaggcttgagagaactgagaaagggaatcaaaggagatcaacttcatcattaacctgtcttccttcctggacacagtgttggattgaaggacaagcagatggagcccagctgaccacagcagtcttgcttaactgaggagagagactggagtctgcgatgcctcaggcagctgatgtgttctaggctggctaagaatgagaagggatttgtggaagaaaggagctccaggaatacacacagaagtctcctcaaggctttggctaaatacaaagctgcgtatgcacagggagagttttcataaagaaagaacaacaaagaaaagctacttgggaaagaacaactgcaggggaacagtaagctcaatggagatgccagagctcacatagcactgggggatatttgaattctgaccactcagaggagaaacacctcactacattttgggcattcagtagagaccaaagaaagctgtattttgggattgggatcatcttattcctagaatcaaggtgactccagaaaaactccaacaacccttcttccaagccagtctaaaaggatccaaatgatctccaagtaaattaactgcattccacaagaaaaaaaaaactcaaccccccttagaggcaagggacaaatacaagttgctcagttatatggcattcctattgcgttacttctatttaaaaatttaatagagacacaagaagctttcactgtgatacataactgggagaaaaaatcactcaacacaaacaggcccagaaattatagaattgatgacattggtgagaacatttaaaatgcacctctgagaactgtgtttcaggaaaatgtcagcaaaagctgaccatgagagaaacaaaagcagaatagcaagagaaaagaaaagaaccggagagccaaatgaaaattaaagaactgagaaaaggtacatctctaatgaagaactcactggatggccttatcatcactttagacattacggtaggaaaggtgacctagaaaataattcaataggagctacacaaatcacaggacagacagacagaccaacagacagaaacacacacacacacacacacacacacacacacacacacacacacacacaaagactgaacctattaatcaacagagcctcaagggcatctaggaaaaatccacacatttaatatatgtgttaggcaagtcacagaaggagaagaaaaagatatcatgacagacattatacttgaagcgatgatggctcgcaacacgccaaatatacagaaaacaagaaactcatagtcaagaagctaaatgactcaggtatagaattttaaagagcaaaactctatgatttactgggatatatcatagttaagttgcctcaattcaaagctaaaaagaaaaaaagggggttcctatgaacaacagctttgacagctgttgatctaagaccacagcttaaatatctaggcaaggaaaagcaaataaggcacaaggaaagaggatggaaggaaatagtccaaaccaatgacattcagtggaaaagaaaatagaccaacaaaggagtaaatccatgaaacagaaagttaggttctttgaaaagtctatatgattggccaaagtctggctaaacagatgacagaccaaggagggagcatatccatcaccatcatgagtaacaggagagagatgccattgctatagcatcctccaggtgtgaaagctgagaagtagatattgagatcaactgtatgtaaataaattcatgaatgtagatcatgtggatggattgcttaggtaaataacaaatcagcaaatcaaacactgaatagatcatgcagttttatagagacttacagacagcctgacagataaacatttgtatgtacgtgaaacaatctccaagacacacttcaaaatccctctcggttaatccaaaggaatgtatttggcagaaggtagaaggagggtattctgatcctttctggtacacattgatgttttctctcagttttcttataaagcatagattactttgaatgtgttacaataagaatcataagctgtctttgaaatgttgacagttgtttagaagttgaggaccatttgtgagtgttatgggactttagtgagaatatttcaaatttgcttgtttacactttgttacaagaaaacatagagggtgccaggtggtgctgtatcttctccaatctctggtgacctgtattgttttggaatttgcagtggcctgaccaggaactactgcaggaatccagatgctgagattcgcccttggtgttataccatggatcccagtgtcagatgggagtactgcaacctgacgcaatgtccagtgatggaatcaactctcctcacaactcccacggtggtcccagttccaagcacagagcttccttctgaagaaggtaagaagcctgcagtcagacaaccataccctcggacattgggataaaaagatttgcaaaatctttgtgatgcagaaaacttccatgctgcacaggaagtcgaaggtgaagtcatggacagccaatgggaaggaagcttcagtgccttctctggggggaccagagctgggatgttgagtgccttgtgagggatggtgtctttaaaaggggcacagaccctctaggacactggatttatcacttccctgttatcaaacgaatcatattagtgtcctagccaagatggatattctaacatcctgccaaacttgtgaagatataccaagctcctaagcctgtccagccctttcttcaagtaggcagtgtttattgcagtcttcagctttaccattttgaaggaatgccatttttgaggctgttgttcttgagaaacctaacatgtcttcattagatccgtattgtcctgagactttgaagcagtacatagccaccaaattgtttatctccccagcctaccttcatcttgggcatgccttccacacctaggatttgagggaagggatttctcagtgttctcatccctgcttctcatggaacatttatctccgttgttttttgagaagaagagtagtggatgtcagctttcttgtaatgagggatcctgggcccaagattccctgtctcccctcctaggctataaaattttggcctgtactccttctccctgagaggcaatgtgtctttacctacaagtcctagatgcaagatccttttctgccccacaccccagaatctgaaggcttttgctttggaggagcagtggtctagtgtgcaagggtttcatgtataccccccactaacagccaatcaccacctatagcctgaacagcttgatgcatggcaccctggtctcctgccttgttctcatgaacacccagaagaggtgtaagcaaaagaccattcacatgagtgtaattttgaagtataggcactctgatctgttttttgtttgtttctttgtttgtttgttttccagggttgaattaaaatatttatgactacttattaaatttctagaatcctataagtctatttgtatttttattctacatttcaatttgcatgctaatatagaagagtgtaaattgttaatcctcagattattccactttgtgtgtcataatttttttcacatttcccttttctaggcaatactgagcttgattttctcttttaatttcagcaccaactgaaaacagcactggggtccaggactgctaccgaggtgatggacagagttatcgaggcacactctccaccactatcacaggaagaacatgtcagtcttggtcgtctatgacaccacattggcatcggaggatcccattatactatccaaatgcgtatgtctatcatgttagccataaaaggaacaatagtcaactaaaatttctcttagctggcccatgctacaagctcacttcctaggtccaaatttctcatagactcagagtttgtagcaaaatgtctcaggaaacttacttttgagcaaaaggtctgaatgaagagaagttttaggattgctatctttcataacaatttgatggaagcagcaggatatatggaggtggtgaagtctcattaatgtaaagctaaggagatcaaatgaccaaatgctgagacaaagtatcattccacaatgcccactaaaggtccatgcagtctttcaaccatgcaattctatcattctatcctccattccctgaagtgaaatttgtgtttgccatttttgacacgaatcagaagtaacaaattcaggctgggtgcagtggctcaggcctgtgatcccaacactttgggaggacaagacgggcagatcaccagaggtcaggagttcaagaccagcctggctaacatggcaaaaccccatctctacgaaaaattaaaaaattagccggtcatggtggtgggtacctgtaattccaactacttgggaggctgaggcaggagaaacacttgagcctgggattcagagtttgctgtgagccgagaacatgccactgcactccagcctgggtgacagagcaagactcaatctcaaaaaaaaaaaaaaagaagaagaagaagaaaagaagaagaggaagaagaagaagaggaagaagaagaagaagaagaagaggaagaggaagaggaggaggaggaggaggaggaagaagaagaagaagaagaagaagaagaagaagaagaagaagaagaagaagaagaagaagaagaagaaaatagaaatgagtgcatatatttatatatgagtactagcctgtatgaacacactgggttctaagcaccagttttctgaagggatatgggttgtcaggcagagtaaaagcaggaatgcagatgagagtcaggaagtaaacagatgtggtgattaaaatgggcaggtacatggacaaaaaaatgcatgtctgacaaaaactggcctcttgccataagtgagtatgaataatatggaaaaactgtttgcacatgttgaacagcagacagtacaacctgagatagtttagaaagggaaacaaataagatcaaccccataattacccttcctagacttaagggcaaagagttttaaccaaagcattccacagcagtcttgctaaactggggagagagactggagttttgtttactaataaaaccgagattttctaggttaggtaataatgagaaagtatttgtggagaaaaggagctccaggaatacacacagaagtctcttcaagtctctggctgaacagaaagctgtgtatgcacagaaagagtttccagagagaaaggagaacaaagaacagctactggggaaagaacaactgctggggaacagtgagctcaatgaagatgccagagctcacatagcactgggaggtatttgagctctgaccagcctgaggagagacacttcattgaacatcttgggcattcagcaaagaccccaaaaaaccatacttcaggagtagaattaatgcattcctagaataaagtctactccagaaacaccctagaaaagcttagaaaccaagtctaaaaagatccaaatgatctccaagtaaattaattgcctgtcagaagaaaacaacctcttcagaggtaaacaacaaaattaaattgctcaattatatagtatgcacaatgtgtggcatacatttaaaaatttgctaaacatacaaaaagcatttagtgtgacccataaccaggagaaaaatcagtcaatacaaatagacccaaaaatgataaaaataacagaattggcaaggagatttaaaatgtatgtatcataattgtgttcaaggatttaaagaaagcgtggacaagaaataaataaatggataatatcaacagaaagaaaaattgtaaaaggaccaaatggagagtcaagaactgaaaaaaaagacatctctttaatgagaaaatcactacatggccttataatcatattagatagtacagatgataaagctaactagaaaatattagggtggtgcaaaccatagcacgcttatacaaagcctgagaagataaacagagcctcaaggacatctatgaaaatatcaaaatatttaatatttgtttaaagcaagtcacagaggaagggaaagagatattggaacagaaaaaatacttgaagcagtgatggctgatgactttctaaatatggaaaaaatgataaactcacatagtcaagaagctcaatggatcagatataggattttaaaaagtaaagctgtatgatttatttggacacatcataattaaattgtccataatcaaagatagaaagtaaaatcttatttgaagcccaagggaaaaaacatacctttacatagagtaacagtgacacaaatgactgatgccttctcatcagaaacaacacaaatcagaaacaatagaataacacctttagagtggtaagaagaaaaaaagatcaaatcagaaacaacaaaataacacgtttagagtggtaaggaggaaaacaagatcaaatcagaaacaatggaataacacctttagagtgtaagaaagaaaaaaagatcaaatcaggaacaacagaataacgccttcagagtggtaagaaggaaaacaagataaaatcagaaacaatgaaataacacctttagagtagtaagaagaagaaaagatcaggtcagaaaaaatggaataatatgctaagaagaaaaaaaaagatcaagtcagaaacaatggaataacacctttagagtgaaaagaaggaaaaaaacccagcaagcttaaacgctatgcacagcaaacaattccactgaaaatgaatgttacgtaagtacatattctgtcctcctaaaaacaaagaacaaataaaagaatgtttcatcagcaggattatgtaataaaagatgtgaaagaatgctatgtaagtagaagaaaaataataccatatgggaattggcatcaaaaccacaaaatactatcaaaacaaaaaaactttattgataaatttaacacaatatgcaaaagaactataccatgtatactacataacattggtgagaagaaaattagaagatctaaataaagacacatcatgcttatagattaaaaaatccaatgtcacttttcacaaaactgatctttagtttcaacccacacccaagcagaattcctgcagtcttttcttgaaaacctaacagaatgtatatgctagaatcaccaagacaatctttaaaaagaataaaaaacttggaataaaatcacaagtttgtgggatagatgcatatggtaatatggaaattctcataaagacacagtaatcaagacatgtggtattggctgggacgcttggctgtaatcctaacactttgggaggccaagatgagaggattgcctgagatgaggagttgcagacaagcctgggcaacatagcaagaccctcatctctacaaatatttaaaaaaattagccaggtttggtgccatgtgcctgtagtcccagctattcaggaagctgaggtgggaggatcactggagcccatgaggtggaggctgaaatgagccatgattgtgctactgaactttagcctgggagacagattaaaaccttccctctctctctcaaacaaacaaacaaaaaatacatagtattgggcaaaacatatgcaaacaaaaacagaaaagggtcagcataaatttacatatatggtcaatttattttcaatacaggtagcaaagcaatttaatgaggaaatttttttccaaaattggtctgaaacaactggatagccatagaaaaaaactataacaaatgtgacgcttgaatcctactgtatgactcaaattaaattaatttgagatagctcttagacctcaatgtaacagctaattctgaggctgaaatataagactgctatgaaaaagtatagtatcttataaccttggagaaggaaaaattttttgagggaagaaccagaaaacactaactgtaaaagaaaacaaatgataatgtggacattcattgaataaaaacttatgctcaccaaatatgactgttaagaaaataaataagtaagtaacacactggaagaaaaacactctcatccatatatctgacaaatggcctgtatccagagtatagaaacatttctcccactcactaatcagaggacaaacaacctaatcaaaatgggcaacaggcttgaatagtcatttcttaggagaagatgcacacagagccaacaatcacctgaaaaagtgcacaacatcttagccatcaaaaatcaagagttataaccctcataagatgacactgaacatccagtgtacatggatatcattaagaagacacaataataagtggtgtcaccgatttggagctagaatgtgccactctctcatatgctggtggaagttcaaaatcatacaacaaattaaaaaatcagtctgatgctttcttataaagttcgataaatatgcatctatcctacaaacctgtaattctattcttgaatatttaccccccaaaatgaaaacataagtccacaaaaatctatataaatattcatagcagctttatgttttataaactcaaaataaaaactatttcaatgttttcatcaaaagaaaatgaaaactatttaaatggtttcatcaaaagaaaatgaaaaaagaatttccagtatatttatacaaaggaatactattcatcaacaaggaacaagttactgatagtctcagaagcatgaacaaacctcaaaaatatattaaggaaagaagccagacgtcaaagtgtatagtctgtatgagtccattcatgtgagtttatagaaaacacaatttatggtgaaagaaaccaatagcatttgacactggccgtgggaagagggtagcagagattgattgagcagccacacaagggagtttctggggtggtgaaaatgttctgcattgtgagggcagtgtgggctacacaagtatatgtatttatcaaatctcatccagctacatttaagatctgtgcatctcactctatgtgaaaatatactcaactgaaaaacagagcaggtatctgtttcaggtgctacatcacttgatacgtccagttgtgttaaaaaccactgcctaacatcctcaaatgggggatctgggcttgagactaggtcacatgtgtagagtctctacagagaccgtgttggattcccatgctccataatacgttccaagttttctcagacagccacaggtcatgaatgtgaggattctgagaggttggagcaacgttcttgggaggcataatggggaaggcattctccaagattcctccagcctggggtcttcacctgctgtgcctcttactgcattgttttctgactcatccatagccacttgaccccttcagatcccatagtctacctagccgtctccctttatgccttgggtcccgctgttctttcaactcatcacccattccttcagtcccagagtggctgcagccagcagaggatggactgagagcaggagaggaggtcgtgcccatgaacccatcctagagaagcagcatcctgcctgggagctagttttccagggaagcttttataagtcctgtagacccaaacccacttgctctaccagatacagtatttatagtaatactattttcatgattattttatattgcaaatgtagagcatttatgctacactatgagtaaatagagtaagggggctggcatgggaattatataatcttggatgccacttcttccttggggaaatgtatttgagttccaacttacatattactatatagtcttatagagagagagacaaagagctagacagacagagatatctttgtatgtgcattaaaaaatctaagatacatatttcaaaatctgtgtcatttattctggaggaaagtatttggcagaaggtgaaaggaagatattctgatcctttcttgtacagacatgtattatctcagttttcatagagagcatatactacttttgatgttttaaaacaaaaattataatctgtgatgtgtccacagttgtttaaaagttgaagctgaagaccatttgtgcttgtggcaatattattgtggtataatgggaatatttcaaaggcacttgttaacactttgttacagcaaaatgtagagggcgctaagtgcccttgaatattctcccatctctggtgacctgtgttgttttgaaatttgcagtggcctgaccaggaactactgcaggaatccagatgctgagattcgcccttggtgttacaccatggatcccagtgtcaggtgggagtactgcaacctgacacgatgtccagtgacagaatcgagtgtcctcacaactcccacagtggccccggttccaagcacagaggctccttctgaacaaggtaagaaatttgtggttagacatctatatactgggatgaaaaaccatggaaaatcttactgatgcagaagccttcagtggtacactggagggttggttgagggtctgcaatgtggaggaaagcctcagcgccctctctgggggatccagaactgtgatttttggcacgctgtgaggaggcagtgtctttaggaagggcacggtgtctttaggaagggcacagacccgccagggcactggacttaccactcccctggttattaaatgggtcatttcagtgtcctagccaaaatggatattctaacagcctgccaaatatgtgaagatttccaagccaataagcctttccagtgatttaaagtagacttttttcattgcaatctacagtttgcagtttcttaagaacatggcctttgagtatgatatcctagagaaacctaaggagactgcattatttttctattgtcctggggctgcatagcaggaggtaaccaacgaatgctgtctctccctggcctatctcagtctttcacaggctctgttcacctcagctttgaagttagaaatttctaggtgttcttgcctcttcttctcatgaaacctgcattggcagtgagtctacagaagaagaggaagagaattctgctttgttacaattcaggactctgggcactagaagattccctatctctcctccaagggaataagttgtttgtctctaaccctccttgagaaacaatgagtctttgcctgcactcctaaatgtaggatgatttcctgcccaaattttcaaaagattaagccttttgccttggtatgagcaatggtctagggaaatgcgcaagggtcttgtgtcggcccctgactgaccaccagtcacctcctacagcctgcaccaaggaatgcattgcattctggtcttctgccctgtggttctcatgaaaaccagcagagattcatatgatggagctgcacatgaatgtaatttccaatgtccagcattctcctctgttctttatctttagatttaaaaataatgtttctatgaacttattaaaattctagaatactatgaatctactgggtcttttcacatccttttgctactagtagaaaaaagaatagtaataattttcagaggctactgtccagtatgtgacataaattgtctcccatgtttctctgctcatgcaattactgagtatgatttattttattttaatttcagcaccacctgagaaaagccctgtggtccaggattgctaccatggtgatggacggagttatcgaggcatatcctccaccactgtcacaggaaggacctgtcaatcttggtcatctatgataccacactggcatcagaggaccccagaaaactacccaaatgcgtatgtatttgattaaaaccataagaggagcaacagccaactcaaatattggttagaagacccatgctttaagctcacttcctagggacaaatttctcttagactcacattttggcaaaatgtctcaggacctttgcttttgagcaaagagtctaagagaagagaaattttaggcctgctatttttcctaatagttttatggaaggagtagaatatacggaagtggcgaagtcatattaatgtaaagctcagaagataaatgaccaaagcttaaacacagcaccattccacaatgcccactaaaaatcaatgtcatctttcactcgtgcaattctgtcattctaaatttcaattcccgaaggtttgtttgccatttttgtcatgggtaataagtaaaaaaaaaaaaattaagatgtgtatatatatatatatatatatatatatacacacacacacacacacacaaacatctgaatatttatatatatgtctgaatatttatatacttgtgtataaaacttatatttaaatttttgcataaatttatatatttttaatatttcattaaaaattatattgtttcactatgtatgtctgagtatttttatatattttaatataacattttaaatatttatatataaatattcaggtatgtaactgaatattcatttacacacacaaatatatgtgtgcatgtgtgtatatatatatatacccatatatatatatatatatatatatacatatatatatatatatatatatgtatatatatatatatatatatatatacacacacacacacacacacatacatacaggtataaacacactgggcctgaagcaccagtggtctgaaaggacatgtgttgccaggacttgaagagcaaaagcaggaaggcggatgagagtcaggaggtacacaaacgctgaaaagtaaaatggacaagtacatggacaaaaagcaggtataagcataacagccttttggaagtaaatgactataaaatatatgaaaatactgttttcacaagttgcacaacagatagtagtgtattgagataatttagaacagaaaacaaatgtgatcaaccccataagtgtgctgtatttcatcatggattgaaggaaaaagagatggagcccaagaagaccacagcagtcttgatgaactgagagacaccagagtttgggattacaaaggcagctgggattttctacacttggtaataatgagaaagaatttgtggagataaagagctacagtcatgtacctagaagtcacctcagtgtaatataaatctgcatatgcacagggagtgattccacaatgaaagtaggacaaagaacagctactggggaaagaataactacaagggaacaatgagttcaatggagatggcagagctcacaaagcactgggggatatttgagttcttaccagctagaaaagagacctcattgcaaatcttgggcattcagtagagaccccagaaaagccactctttggaaacagagttgatgtattttaagagcaaaatctactccacaaaaatcctagcaaaattgaaaagcaagtcagaaagaccaaaatcctctcaacataaattagttgcccatcagaagaaagcttaacctcttcataggtaaacaataaaatcaaattgctcagttatctggcatccacaatatgtgacataaatttaaaaatttactagacatacaagaagcatttagtgtgatccataaccaggagaaaaatcattcaatacaaatagacccagaaatgacagaaatgatagaattagcaaaaacatttaaaatatacatatgatcatttgatcttgtgatcagatatcacaagagaagaaagagatacttgaacagaaaaaatgcctgaagcaatgatggctgaaaactttccaaatatgaagaaaaaaaagctcacagattcaagaaaactaatcaatcagaaatatgattttgaaaagtaaaaatgtatgatttactttggcaaatcttcttggttaaattgtctaaaatcaaagaaagctaggaaaattttataagccagaggaaaaaagattgtttatataaaggaacagttacacaaatgactgatgccttctcatcagaaacaatgaaagtcagaaacaataaagtaacatctttaaagtaatagaagaaaaacccaagaggtgagggatcgtggcagacaggaggcaggactagattgcagctctggacagagcagcatgcagaggctcatattgtgaattttagccccatattgactgcaagaacagaccagcaatcctgagaggacccacagaccgtgtgaaggaagcagactgctcctgcaggataagggagacaccccaaatactgtgagttccccaactgcagaagtggaaaagggaggccttactccctcaaacacaccccacaactggagaagctgaaagtctgtttgcaggagaagttcccaactttacctgggcctcagtaaatttagagagctgagccaagcaaaatataggggtagaggaagcagcagagaagacctcagagcttgctggatccccaagcagctcattcctgcctggcaccacagagatccatcagaagtgtggccaaaggaacagagggtaaaactccacatggaggactgctctacctgaactttctaacaatttgaacagggggagaagcctcctggccagaacttgggggagggcatgaatctggtttgcagacttcacaggtgggggaaggactaaagcccttttctttcacagctgggaggtggaaagcctcaggcaagttttcaagcctgactttccccccacctggaaacagacttggagctgttgcggggttgggggcatggtgggagtaagaccagcccttcagtttgcatgggtgctgggtgaggcctgtgactgacagcttccctccacttccccgacaactcagatgactcagcagaggcagccataatcctcctaggtacacaactccagtgacctgggaacttcacccccacaccatacagaagcttcagtaagacgtgcccaaggaaagtctgagctcagacacgcctagtcccacccccaactgatggtccttccctacccaccctggtagcagaagacaaagagcatataatctttggagttctagggcccacccacctctagtccctctccacactagtatagctgatgcaggaggccaaccagcacaaaaatagagcattaaaccaccaaagctaggaacccctatggagtccattgcaccctcctccacctccaccagaacaggcactggtatccacagctgagagacccatagatggttcacatcacaggactctgtacagacagtccccagtaccagcccagagctgggtagacttgctaggtggcaagacccagaagacaggcaataatcactgcagttcagctcacaggaagccacatccataggaaaagagggagagtactacatcaagggaacaccccatgggataaaaacatctgaacaacagccttcagccctaccttccctctgacacagtctacccaaatgagaaggaaccagaaaaccaaccctggtaatatgacaaaacaaggctcatcacactcccagttcaccagcaatggatccaaaccaagaagaaatccctgatttacctgaaagagaattcaggaggttagttattaagctaatcagggagggaccagagaaaggcaaagcccaatgcaaggaaatccaaaaaaaaaaaggtataagaagtaaaaggtgaaatattcaacaaaatagatagcttaataaaaaaacaataaaaaattcagtagactttggacacacctttggaaatgtgacatgctctggaaagtctcagcaatagaactgaacaagtagaaaaaataaattcagagctcaaagacaaggacttcaaattaacccaatccaacaaagacaaagaataaaggataagaaaatatgaacaaagccttcaagatgtctgggattatgttaaatgaccaaatataagaataatcgtggctcctgaggaaaaagacaatactaaaagcttggaaaacatatttgggggaataactggggaaaacttacctggccttgctggacacctagacatgcaaatacaagaaacacaaagaacatgtaaatacaagcagcacaaagaacacctgggaaattcatcacaaaaagatcttagcctaggcacattctcatcaggttatgcaaagttaagacgaaggcaagaatcttaagagctgtgagacagaagcaccaggtaatgtataaaggaaaccctatcagattaacagccagtttttcagcaggaactgtacaagctataaaggattggagccctatcatagcctcctcaaacaaaacaattatcagtcaagaattttgtatccagcgaaagtaagcatcatatatgaaggaaagatacagtcgtttttggacaaacaaatgctaagagaattcaccattaccaagtcaccactagaagaactgctaaaaggagctctaaatcttgaaacaaatcctagaaacacatgaaaacagaatctctttaaagcataaatcacacaggacctataaaacaaaagtacaagttaaaaaacaaaaacaaaaaacaaaaccaaagtacggaggcaataaagaatatgatgaatgcagtggcacctcacatttcaatgctaaaattgaatctaaatggcctaaatgctccacttaaaggatacaaaaagagttggtggctggcaagatggctgaataggaacagctccagtctgccgctccccgtgagatcaacacatagggtgggtcatttctgcatttccaaccaaggtacccggctcatctcattgggactggttagacagtgggtgcagcccacagagggtgacctgaagcagggtggggtgtcacctcacctgggaagtggaaggggtcagggaactccctcccctagccaaaggaagccgtgagggactgtgccgtgaagaccagtgcattctggcacaaatactatgcttttcccacggtctttgcaacctgaagaccaggagattcccttgggtgcctacaccaccagggccctggatttcaagcccaaaactgggctggcatttgggcagacactaagctagctgcaggagttttttttcataccccagtggtccctggaatgccagcaagacagaaccattcacccccgtgaagaaagggctgaagccagggagctaagtggtctttctcagtggatcccacccccatggagcccagcaagctaagctccactggcttgaaattcttgctgccagcacagcagtctgaagttgacctgggacgctcaagcttggtgggaggaggggtatccacaaatactggggcttgagtaggaggttttcccctcacagtgtaagcaaaaccgctaggaagtttgaactgggcagggtgcactgcagcttggcaaagccattgtagcaagagtgcctctctagattcctcctctctgggcagggcatctctgaaagaaaggcagcagccccagtcagaagcttatagataaaactcccatctccctgggacagagcaactggaggaaggggtggctgtgagtgcagctccagcagacttagtttcctgcctgccagctctgaaaagagcaccagatcccccaacacagcactagagctctgataagggacagactgcctcctcaagtgggtcctggtttcagaagataataagaaactcctctgagctaaaggagcatgttctaacacaatgcaaggaagctaagaaccttgaaaaaggtcagaggaattgctaactacagtaagcagtttagagaagaacataaatgaccttagggagctgaaaaacacagcacgagaacttcatgacacatacacaagtatcaatagcaaaatcgatcaagtggaagaaaggatatcagagattgaaaatcaacttaatgaagtaaagcgtgaaaacaagattaaggaataaagaatgaaaaggaatgaacaaatcctccaagtatgggactatgtgaaaagattgaacctacgtttgattggtgtacctgaaagtgatgggagaatggaaccaagttggaaaacactcttcaggatattatccaggagaacttccccaacctagcaagacaggccaacattcaaattaaggaaatacagagaataccacattcaaattcaggaaatacagagaacaccacaaagatactcctcaagaagagcaacctgaagacacataatcgtcagattcaccaaggttgaaatgaaggaaaaaaatgttgagggcagccagagagaaagtttgggttacccacaaagggaaccccatcagactaacagtggatcttcctgcagaaactctacaagccagaagagagtgggaggccaatattcaacattcttttttactattattatactttaagttctagggtacatgtgcacaaggtgcaggtttgttacatatgtatacatgtgccatgttggtgtgctgcacccattaactcttcatttacattaggtatatctcctaatactatccctccccactccccccatcccatgacaggccccggtgtgtgatgttccccactctgtgtccatgtactctcattgttcaattcccacctatgagtgagaacattcggtgtttggatttctgtccttgtgatagtttgctgagaatgatggtttccagcttcatccacatccctacaaaggacatgaagtcatccttctttatggctgcatagtattccatggtgtatatgtgccacattttcttaatccagtctaccattgatggacgtttgtgttggttccaagtctttgctattgtgaatagtgccgcaataaacatatgtgtgcatgtgtctttatagcagcatgatttataatcctttagatatatatccagtaattgtatggctgtgtcaaatggtatttctagttctaaatccttgaggaatcaccgcactgtcttccacaatggttgaactagtttacagtcccaccaccagtgtaaaaatgttcctatttctccacatcctctctagcatctgttgtttcctgactttttaatgatcaccattctaactggtatgagatggtatctcattgtggttttgatttgcatttctctgatggccagtgatggtgagcactttttcatgtgtctcttgactgcataaaagttttcttttgagaattgtctgttaatatcctttgccaactttttgatggggttgtttgattttttttcttgtaaatttgtttatgttctttgtagattctggatattagccctttgtcagatgggtagattgtaaaaattttctcccattctgtagcttgcctgttcattctgagggtagtttcttttgctgtgcagaagctctttagtttaattagatcccattggtcaattttggcttttgttgctattgcttttggtgatttagtcatgaagtccttgcccatgcctatgtcctgaatggtattgcttaggttttcttctagggtttatatggttttaggtctaacatttaagtctttaatccatcttgaattaatttttatataaggtgtaaggaagggatccagtttcagctttctacatatggctaggcagttttcccagcaccatgtattaaatagggaaacctttccctatttcttgtttttgtcaggtttgtcatagatcagatggttgtagatgtgtggtattatttctgagggctctgttctgttccattggtctatatctctgttttggtaccagtaccatgctgttttggttactgtagccttgtaatgtagtttgaagtcaggcagagtgatgcctccagctttgcttttttggcttaggattgtcttggcaatgcatgctcttttttgttccatatgaactttaaagtagttttttccaattctgtgaagaaagtcattggtagcttgatggggatggcattgaatctataaattaccttaggcagtatggccattttcacaatattgattcttcctatccatgagcatggaatgttcttccatttgtttgtgtcctcttttatttcattaagcagtggtttgtagttctccttgaagaggtccttcccatcccttgtaagttggattcctaggtattttattctctttgaagcaattgtgaatgggagttcatccatgtccctacaaaggacatgaagtcatgtatgggaatgcttgtgatttttgcacattgattttgtatcttgagactttgctgaagttgcttatcagcttaaggagattttggtctgagaagatggggttttctaaatatacaatcatgtcatctgcaaacagggacaatttaacttcctcttttcctaactgaataccctttatttccttctcctgcctaattgccctggccagaacttccaacactatgttgaataggagtggtgagagagggcatccctgtcttgtgccagttttcaaagggaatgcttccagtttttgcccattcagtatgatattggctatgggtttgtcataaatagctcttattattttgagatatgtcccatcaatacatagtttattgagagttcagcatggagagctgttgaattttgtcaaaggccttttctgcatctattgagataatcatgtggtttttgtctttggttctgtttatatgatggattacatttattgatttgcatatgttgaaccagccttgcatcccagggataaagccaacttgatcatggtggataagctttttgatgtgctgctggattcggtttgccagtattttattgaggatttttgcatcaatgttcatcatggatgttggtctaaaattctcatttttgttgtgtctctgccaggatttggtatcaggatgatgctggcctcataaaatgagttagggaggattccctctttttctatgattggaatagtttcagaagaattggtaccagctcctctttgtatctgtggtagaattcggctatgaatctctcctggactttttttggttggtaggctcttaattattgcctcaatttcagagcctgttattggtctattcaaggattcaatttctttctggtttagtcttggtagggtgtatgtgtccaggaatttttccatttcttctagattttctagtttatttgcacagaggtgtttataatattctctgatggtagtttgtatttctgtgggattggtagtgatatcccctttatcattttttattgcatctatttgattcttctctcttttcttctttattagtcttgctagtggtctatcaattttgttgatcttttcaaaaaaccagctcctggattcattgatgttttgaaggtttttttgtgtctctatctccttcagttctgctctggtcttagttatttcttgccttctgctagctttttaatgtgtttgctcttgcttctctagttcttttaatggtgatgttagggtgtcaattttagatctttcctgctttctcttgtgggcatttagtgctgtaaatctccccctacacactgctttaaatgtgtcccagagattctggtatgttgtgtctttgttgtcattggtttcaaagaatatctttatttctgccttcatttcgttacatacccagtagtcactcaggtgcaggttgttcagtttccatatagttgagcagtttttaatgagtttcttaatcctgagtcctagtttgattgcactgtggtctgagagacagtttgttataatttctgttcttttacatttgctgaggaatgcctcacttccaactatctggtcaatttcagaataagtgcgatgtggtgctgagaagaatgtatattctgttgatttggggtggagagttctgtagatgtctattaggtctgcttggtgcagagctgagttcaattcctggatatccatgttaactttctgtctcattgatctgtctaatgttgacagtggggtgttaaagtctcccattattattgtgtgggagtctaagtctctttgtaggtctctaaggacttgctttatgaatctaggtgctcctgtattgggtgcatatatatttaggatagttagctcttcttgttaaattggtccctttaccattatgtaatggccttctttgtctcttttgatctttgttagtttaaagtctgttttatcagagactaggattgcaacccctgctttttttgttgttttccatttgcttggtagatcttcctccatccctttattttgagcctatgtgtgtctctgcacgtgagatgtgtcttcagaatacagcacactgatggatcttgactctttatccaattttccagtctgtgtcttttaattggagcatttagcccatttacatttaaggttaatatttttatgtgtgaatttgatcctgtcatcatgatgttcgctggttattttgctcattagttgatgcagtttcttcctagcatcgatggtttttacaatttggcatgtttgtgcagtggctgataccgattgtttctttccatgtttagtgcttccttcaggagctcttgtaaggcaggcctggtggtgacaaaatctctcagcatttgcttgtctgtaaaggattttatttctccttcacttatgaagcttagtttggctggatatgatattctcagttgaaaattcttttctttaagaatgttgaatattggctgccactctcttctggcttgtagagtttctgctgagagatctgctgttagtctgatgggcttccctttgtgggtaacccgacctttctggtgaatctgacaattatgtgtcttggagttactcttctcgaggagtatttttgtggcattctctgtatttcctgaatttgaatgttggcctgcctttgtaggttggggaagttctcctggataatatcctgaagagtgttttccaacttggttccattctcctcgtcactttcaggtacaccaagcagatgtagatttggtcttttcacatagtcccatatttattggaggctttgttcatttctttttactcctttttttctctaaacttctcttctcgcttcatttcattcatttgatctttaatcactgataccctttcttccacttgattgaatcaactactgaaacttgttcatgtgtcacgtagttctcgtgccatggttttcagctccattagatcatttaaggtcttctctatgctgtttattttagtctgccattcatctaaactttttcaaggtttttagcttctttgcaatgggttcgaacatccttctttagctcggagaaatttgttattacagatcgtctgaagccttcttctctcaactcatcaaagtcattctctgtccagctttgttctgttgctcgtgaggagctgcgttccttcggaggagaagaggcaccctgatttttagaattttcagctgttctgctctggtttctccccatctttgtggtttatctacctttggttcttgatgatggtgatgtacagatggggttttggtgtggatgtcttttctgtttgttagttttccttctaacagtcaggaccctcagctgcaggtctgttggagtttgctggaggtccactccagtccctgtttgcctgggtattaccagtggaggctgcagaacagcaaatattacagaacagcaaatgttgctgcctgattcttcctctggaagcttcatctcagaggggcacccagctgtatgaggtgtcagttggcccctactgggaggtgtcccccagttaggctactcgggggtcacggacccacttgaggaggcagtctgtccattctcagatctcaaactctctgctgggagaaccactactctcttcaaagctgtcagacagggatgtttaagtctgcagaagtttctgctgccttttgttcagctatgccctgcccccagaggtggagtctacagaggcaggcaggtctccttgagctgtggtgggctccacccagtttgagcttcctggtcgctttgtttacctactcaagtctcagcaatggcagacgcccctcccccagctttgctgccgccttgcagttcggtctcagactactgtgctagcagttcaatctcagactgctgtactagcagtgagcaaggctctgtgggcatgggaccctctgagccatgtgcaggatataatctcctggtgtgccgtttgctaagaccattggaaaagtgcaatattagggtgggagtgtcccgattttccgggtacatctgtcatggcttcccttggctaggaaagggaattccctgaccccttacacttcccgggtgaggcaatatcccgccttgcttcggctcactctccgtgggctgcacccactgtctgacaagccccggtgagatgaacccagtacctcagctggaaatgcagaaaccacccatcttctgctttgctcatgctgggaactgtggactggagctgttcctattcggccatcttgaaacctcccctctctcacgatcacaaggtcccacaataggccgtctgcaggctgaggagcaagaaaagccagtctgaattccaaaactgaagaaattggagtctgatgttcaagggcaggaaacatccagtgccaaagaaagatgtagaatattcaacattcttaaagaaaataattttcaacctagaatttcatatccagccaaactaagctttataacaaaggagaagtaaaatcctttacaaacaagcaaatgctgaggaattttgtcaacaccaggcctgccttacaagaggtcctgaagaaaacactaaatatggaaaggaaaaaccagtaacagctactgcaaaaacataccaaattgtaaacaccatcaacactataaagaaactgcatcaactaatgggcaaaatagccagctagcatcataatgacaggatcaaattcacacataacaatattaaccttaaatgtaaatgggctaaatgccccaattaaaagacacagactgggaaattgaataaagagtcaagacccattggtttgctgtgttcagaagacccatctcagggtgaaaagacatacatgggctcaaaataaagaaatgaaggaatatttaccaagcaaatggaaagaaaaaaaaagcagcggttgcaatcttagtctttgatgaaacagactttaaaccatcaaagatcaaaagagacaaaggagggcattacctaatggtaaaagtatcaatgcaacaagaagatctgactgtcctacttatatatgcacccaatacaggagcacccagattaataaagcaagttcttagagacctacaaagagacttagacttccacacaaaaatagtgggagactttaacaccccacagccaatattagatcgacgtgacagaaaattaacaaggatattcaggacgtgaattcagctctggaccaagctgacctaatagacatctacagaactcgacaccacaaatcaacagaatatacattcttctcagcaccacattgcacttattctaaaattgaccacataattggaagtaaaacacttctcagcaaatgccgtagaatggaaatcataacaaacagtctctcagaccaaagtgcaatcaaactagaactcaggattaataaactcactcaaaaccacacaactatatggaaactgaacaacctgctcctgaattactactgggtaaataacaaaattaaggcagaagtagataagttcttagaaaccaaagagaacaaagacacaatgtgccagaatctctggtacacagctaaagccatgtttagagggaaatttatagcactaaatgcccacaggagaaagcgggaaagatctaaaatcaacaccctaacatcacaattcaaagaaccagagaagcaagagcaaacaaatacaaaagctagcagaagacaagaaataactaagatcagagcagaactgaaggggataaagacacgaaaaccctttaaaaaattaataaatccaagagctggttttttgaaaagattaacaaaatacatagaagcctagccagactaataaagaagaaaatagagaagaatcaaatagacacaataaagaataataaaggggatatcaccaatgatgccacagaaatacaaactaccatcagagaatactttaaacacctctatgcaaataaaatagaaaatctaaaagaaatggataaattcctggacacatacaccctcccaagactaaaccaggaagaagtcaaatccctgaatagaccaataacaagttctgaaatcgaggcagtaattaatagcttaccaaccaaaaaaagcccagaccagagggattaacagtcaaatcctaacagaggtacaaagaagagctagtactattccttctgaaactattccacacaatagaaaaagagggactcctgcctaactcattttatgaggccagcatcattctgataccaaaacctggcagagacacaacaagaaaagaaaatttcaggccaacatccctgatgaacatcaatgtgaaaatcctcaataaaatactggcaaactgaatccagcagcacatcaaaaagcttatccaccatgatcaagttggcttcatccctgggatgcaaggctggttcaacatattcaaatcaataaacataatccatcacataaacagaaccaatgacaaaaaccgtatgattatcgcaatagacgcagaaaaggcctttgataaaattcaatacccaatcatgctaaaaactcttaataaactaggtattgatggagcatgtctcaaaataataagagctacttatgacaaatgcatagccaatatcatactgaatgagcagaagctggaagcattccctttgaaaaccagcacaagacaaggatgccctctctcaccactcctattcaacatagtattggaaattctgtccagggcaatcaggcaagagaaagaaataaaggtattcaagtgggaagagagggagtcaaattatttctctttgcagatgacatgattgtatatttagaaaactctatcatctcagcccaaaatctccttaagctgataagcaacttcagcaaagtctcaggatacaaaatcaatgtgcaaaaatcacaagcattcctatacaccaataagagacacagagccaaatcctgagtgaattcccattcacaattgctacaaagagaataaaatatacctaggaatccaacttacaagggatgtgaaggacctcttcaaggagaactacaaaccactgctcaaggaaataagataggacacaaacaaatggaaaaacattccatgctaatggattggaagaatcaatattgtgaaaattgccatactgcccaaagtgatttatagattcaatgttatccccatcaagctaccattgatttcttcacataattagaaaaaactactttcaatttcatatggaatagaaaaagggcctgtatatccaagacaacctaagcaaaaagaacaaagctggaggcatcatgctatctgacttcaaaatatactacaaggctacagtaacaaaaacagcatggtatggtactggtaccaaaacagatatatagaccaatagaacagaacagaggcctcagaaataacaccacacatctacaactattggatctttgacaaactggacaaaaataagcaatggggaaaggattccctatttaataaatggtgttgggaaaactggctagccatatgcagaaaactgaaactggatcccttccttacaccttatacacaaattaactcaagatagattaaagaattaaatgtaagacctaaaaccataaaaaccctagaagacactttgggaggccgaggtggatggatcacgaggtcaggagatcgagaccatcttggctaacacagtgaaagcccatctctactaaaaatacaaaaaattagctgggtgtggtcgtgggcacctgtagtcccagctacttgggaggctgaggcaggagaatggcatgagctgaggaggttgagcttgcagcaagccaagattgtgccactgcactccagcctgggcaacagagtgagactccatcaaaaaaacaaaaacaaaaacaaaaaatcaaaccctagaagaaaacataggcaataccattcaggacataggcatgggagaagacttcatgactaaaacagcaaaaccaatggcaacaaaagccaaaatttacaaatcagatctaattaaaataaagagcttctgcacagcaaaaaactctcatcagagtgaaaaagcaacctatggagaaaaattctgtggtctagccatctgacaaagggctaatgtttagaatgtacaagcaacttaaacaaatgtacaagaaaaaaaaaacaaccccatcaaaaagtgggcaaaggatatgaacagacacttctgacaggaagacctttatgtggctgacaaacatgaaaaaagctcatcatcactgttaattagagaaatgcaaatcgaaaccacaatgagataccatctcatgcccgttagaatggcgatcattaaaaagtcaggaaacaacagatgctgaagaggatgtgtggagaaagaggaacacatttacactgttggtgggagtgtaaattagttcaaccattgtggaagacagtgcggtgattcctcaaggatctagaaccagaagtaccatttgacccagcaatcccattactgggtatatacccaaaggattataaatcattctacaataaagacacatgcacacgtatgtttattgtagcactattcacaatagcaaagacttggaaccaactgaaatgcccatcaatgatagactggataaagaaaatgtggcacatatacactgtggaatactatgcagccataaaacaggatgagttcatgtcttttgcagggacatggatgaagctggaaaccatcattctcagcaaactaacacaagaacagaaaaccaaacaccatatgttctcactcataagtgtgagttgaacaatgagaacacatggacacaggaaggggaacatcacacacaggggcctgttggggagttgaggctaggggagggattggattaggagaaatacctaatgtagatgatgggttgctgggtgcagcaaaccaccatgacacgtgtatacctatgtaacaaacccacacattctacacatgtatctcagaacttaaagtataataataataagatacagaactgcagaatgaataagaactcaccaaccatctgctgccttcaggagactcatttaagacataaggactcacataaacttaaagtaaatgggtggaaataataataagtggtgtcactgatgtggaggtagattataaaactcttatcatatgctggtggaagatcaaaatgataaaacgaattaaaaaatcagtcagatggtttcttaaaaagttccatcaatatgcctctatcttacaaacctgcaattctattcctgaatctttatcccaaggaaatgaaaaagtaagtccacaaagagttctatatgaatatttataggagctttatttattataattcaaactgtaaaaataatttcaatgttcatcaataacaaaatgaaaaaataatttgcaacctactggtacacttgaatactattcagcactgagtatcttaaatagcatggatggagctcaaaaatatactcaggaaagaagccatgtatattctgtatgagttcatttacatgagatcatttacatttcctccaaaagaggaaaaactaatttctgttgaaagaaaccaatgtatttgcctctggcagtggtaagggggtagcacagattaattgggtagggactcaagagagtttctggggtcacagaaatgttccgtgtggtgatgggagtttgggctccacaggtataggtgttgatccaaaatcatcaaaaaaacaacattgcagatctgtgcatctcactctgtgggaaagtatatctcaactgtaaaaagggcagaaattgcttttaaacgctcagccttttagcacatccagttgcttggagaaccagcttactcaaatgggggtctaggctggagactaggtcacaggcatagagtctctaaactttcccatggcacataatacgtttcaggttttctcagagagctgcaggttagtaatctgaggattctgacaagttgggtcaacgttcctaggaggcatgaatgggagtgcattctctaagatccctccaccccagggtccttgctttctgtgcctcttactccattgttttctgactcctctgtagccactcgacctcttcagatcccattgtctacccagccatcgccctttatgacttgggtcccactgttctttcatctcatcctccattccctcagtttcggagtggctgccgctagcagaggatggactgagagcaggagaggtggtcctgcccaggaacccatcctagagaaatggcatcctgtctgggagctagttttttagggcaggttttataagtcttgtaaagccagacacacttgatctacctggtatgttatttacagtaatactattttcataattgcttttcactctaaaagtagagccttttagctacactgtgagtaaataaaggggctggcctgggaatggtatcatgttggatgttgtttcttccctgaagtaatatatatcagttacaatttacatgttactgcagagtcctagagagagacacagagaatgagacagataccaatacatttttatgtgcattaaaaaaatctaaggccaggcgcagtggctcacacctgtaatcccagcactttgggaggccgaggtgggtggatcacgaggtcaggagattgagaccatcctggctaacacggtgaaaccctgtctctactaaaaatacaaaaaattagccaggcgtggtggcgggcgcctgtagtcccagctactcaggagactgaggcaggagaatggcttgaacccaggaggcagaccttgcagtgagccgagattgcgccactgcactccagtctgggcgacagagcgagactccgtcacaaaaaaaaaaaaaaatctaaaatgcactcttcaaaatctatgtcatttattctggaggaatgcagttggcagaaggaggaagatattccgaatttttcttgtatacatttatgtatgatctcagtttttttatggatcatagaccaattttgatattttaaaataaaaattataatctatcttggaaatttacatggttctttagaacttgaggaccgtttttgcttttcggaatattattgtacctaaaatgggaatattacaacgtcactttttaacactttgttataacaaagtttagacagcgctgggtgcccctgaattttttcccgcctcttgtgacctgtgttgttttggaatttgcagtggcctgaccgagaactactgcaggaatccagattctgggaaacaaccctggtgttacacaaccgatccgtgtgtgaggtgggagtactgcaatctgacacaatgctcagaaacagaatcaggtgtcctagagactcccactgttgttccagttccaagcatggaggctcattctgaagcaggtaagaagtctgtggccagatatctacacatttgaacattgggatgaaaagagatggaaaatctgactgatgcagaagccttccatgctacacagaaacttgagggtatggcaggtggaaagaagcctcagcactctctctggtggagcaatttttggcgcaacgtgcgtgggcggtgacttcaggaatggtgcaaacccacctgggcacttgacttaccactcactttgttatgaaaggggttatctcggtgttccagacaaaattccaattctaacatcaggccaaatttgtgccaaatttcacactagtgagtgtttccaggcatttattaaaatggacagtgttcattgcaatcttcagcattgcagttgctgaggtatgtggccgctgagtttgtcatcctggggaaacctaatatgatgatatttattccatctaatcctggggctatttggcagtaaataccacagaatacactatttctctggcttatttcagtcttaggtaggctctgcacacctatgcttggaaggcaggaatttcttggtgttcttgtgccttcttctcatggaacgtgcatctttggtgtgtgttgagaggaagggtagtagacttctgctttgttgcaatgcaggatgctggaacaagaggattccctgtctctactgtaagggaataagattttagcctccatccttctctaagaagcaatgtgtctttgcctccaagtactagatgcaggaccatgaactgccccgtccaccagaagcttaaggctttggcttttcaggagcaatcatctagggaactgtgcagggttttcatgtctgtcccctactgacagccaatcaccatacagcctgcataacctaatccatcatcgtctggtttcctgcctcattgttttcatgaacaaccagtagagagccatacgaaagagcttgcacatgagtctttgttccaattgtaagagcactgataggtccttttcccaccaggttttgaatataaaatttctaagaacttattaaaatattagaatgttattaatctattgtttttgcttcagcatgtccttctgcttgtgagtatactaaagagaacagtcataattctgaaactactgtcctgtttgtgtcataaattgcttcacatgtttctgcatactagtagttactcagcttgattttgtctattttcagcaccaactgagcaaacccctgtggtccggcagtgctaccatggtaatggccagagttatcgaggcacattctccaccactgtcacaggaaggacatgtcaatcttggtcatccatgacaccacaccggcatcagaggaccccagaaaactacccaaatgagtatgtctttgatgttacttgtaagaggagcaacagccaacttaagttcctcctagaagagccttgcttcaagctaacttgttaggacaaatttcccttagacccagaaggtgtgtcaaaatgtccagacaactttgcttttgatcaaagagtctgagagaataggtattttaggcttgctatcttttctaatagtctgatggaagcagaaggctacatggagctgatgaggtctttttaatataaagctcaagagatcaaatgatcaaatacttagagtgccattctacaaggctcataaaagatcaatgcactctttcacccatgcaattctatcattctaacctcccttctctgaaatgaaggctttttgccatttttgtcatgggtcacaagtaaataattcacatgtatatgagtatatatataaccaggtgtgtttattcagactagtatgtatatatatacatatatatgttcatataagttagtattcatatatatgttcatatatatatgttcatacagactagtattcatatatatatacatatatatatacacacacatatatatatatatatatatgttctagggaaacatgcaaggtttttatgtctgtccctgactgatgaccaaataccctatagcctgcacagctgcaagctgtatagccatacaatttgcaggacacacacacatacacacacacacacacacacacacacactaacatataatataatataatataatataatataatataatataatataatataattaatatatataaacctgtgtgaacacactgggttctaagctccagttttctgaagggatatgggttgccaggagaggaagagcaaaagcaagaatgtagatgagaattaggaagtaaacagatatggagattaaaatgggcaggtacatggacaaaaaaccaggtctgacaaaaactggctttctgccataaatgactataaaagatattaaaaaacactttccacatgttggacaagagacagtacaggactgagataatttagaaaaggaaatgaatgagcgcaactccgtaactattatgactttcttcctggagaaccttcctggactgaagggcaaggaattggagccaaagccaaccacagcagtcttgctgaactgaggaaagagactggagtttgggatagctaagaaaatgtgtattttctatgctaggtaataatgagaaagaatttgtggtgaaaaggagctgaaggaatatgcatggaagtctaatataaactgcatatgcacagggagaaattctacaaagtgggacagagaaccactactggggaaaggacaaattcagggaaacagtgagctcaatggtgacgccagagctcacgtagcactgggggataccggggttctgatcagcccgaggagagacacctcattgaacatctcgggcattcagtagagaccccagaaaagtcatactttaggagtaggatttatgccttcttagaataaagactaccccagaaacaccctagtaaagcttaaaaaccaagtctaaaaggacccaaatgatctccaagtaaattaactgcctgacagaagaaaactcaaccatcactggaggtaaataacatgattacagtgctctgtaatgttgcattcacaaggagtgacatcatttaaaaatttatgaggcaggaaaaagcaattagtgtgatccataactaggagaaaaaccagtcaatacaaatagaccaagaaatagtagaaacgatggaattgacaaagaaattaaaactgtatatatgataattgtgttcaaagatttaaagaaaacatgaacatgagggaaacaaatgcagaatataaaaaaaagcaaatgcgtaaaacaaccaaatggaaattaaagaactacaaaaaagtataaccttaataaaatactcactggatggccttaatattagtttatacattacagaagaaaaagtgaaccagaagataactcaatgaaagccatacaatctgtaagacacacacacacgcacacgcgcgcgcgcgcacacacacacacacacagagagagagagagagagaaagagagagagagaaaggctgaaaaaaataaatagaaccttaaggatatcagtgaaaatagcaaaagatttaatatatgggtaaagcaagtcacagaaggacgggaaggagatattgggacagaaaaaaatactcaaagcaatgatggctgaagactttacacgtatgaagaaaatgataaactcacagtcaagaagctcaatgaatcagaaatagtatttttaaaagcaaaactctatgatttacttgggtacattatagataaatcgtccaacatcaaagataacaaggataatcttataagccagaggaaaacaatatcatttacatagagggacagtaatgaaagtgaccgatgccttctccttggaaacaatggcataacatctttaaagtgataaagagaaataaaaacagatcaacctaggacgacatgtccagccaaaacaaacaaataaacaaaaaaaccctttaaaataaacgtgatgtaaatacgtattctgccacctccagaggaaacaagcaaaaaaacaaaagaatgtttccaaggcaggcttctgtattaaaagattttaaggaaagttattcaggtagaagaaaaataataccagatgggaactttaatccatactaagtaatgaagagccctggaaatggcaaatggcaatgtcaatataaaatactcttatttatctaatttttaaatgtatttaaaggacaatttgtgatattaattaaaataataggaatatattgttgtttcaacgtatgtagtagtaaaattcataaaaacagtagcacaaataatgcagatgataactggaagtatactgttaatgagttttttgcattatccatgaagttatataatattaatagatggttgaatgtgatagtttaaggtgggatattataaatcctaggacaaccaaaaaaatttaaactgagaggaatggatagtaagaggaatagtccttttatgcaaaagaaggaagaaaaagaggaataaagaatataaaagatatggtgtaaacagaaaatacatagcattattgtagacacaaactgaactaccttatgagtatattaaatataaaaggattaagcattacaaataaaaggcagagattgtaaattgaataaaaaccacagctaagtgtgttctttttagaataaatactctttaagtgtaaagatctactttaaacaccaaaatatgaaaaaggatatataccatgaaaacctgaatcataaataagctggagtggtgattaatggatgcaggcactcctaaagactaataagtgaatgtggtcaaattgaagaaacaaaagtatatacgtgctcaatgtgcaaaaactttttctgtatacatgctatgatcctttggaaaattaaagttttaaagcaatatcactgacaatagtatcaaaaccaaaaaatatttagtgataaatttcacacactatgctcaaggactatacaccttgcactagaaaacaatgttgaggaaagaattaaaagatctaaatatacaccatgcttatagattaaaagactccatatcagttctcgtgaaattgatctttggatgaaacccacacccaagcactattgcaacagtccttttttggaaaaaaaaattggaggacttatataccttaatataaagacttataaaagtacaggaatcaagacatgtggtattggcctggccccttggctcatgcctgttaccccaacattttgggaggctgagtctggaggatggcttgagcccagatgttcaagaccagccttagcaacagagtgagaccctctctctacaaaaaataaacaattagatcgatgtgatgacttgcacatgtagtttcagctactcggaatgctgaggtgagaggattgcttgactcaggaggtctagccatgagtgagcattgatcatgcctctgcattccagcctggatgatggaatgagacactgtctcaaaaaaaaaaaaaaaaaaggatatgtgttattggccaaaaaagtatgcaaacctaaaaagggatggcccaccaccagacccacatacatatatggtaaatggattttccgtatagatggcaaagcaattcaatggagacaaaaatgttttacaaaatcattctgaaccatttggatatccatgatacaaaacaaaagcagaacttgacttttgcttttcatctcaaattattttgatatctcttccacctaagtgtcagagctaaaactgaacctgaaatatgaaagttccatgaaaaaatataaaatcttcacaaccttggagaaggcaaacttttttgaggcaggagtctgtaaacactcactataaaataaaacaaattataatgtgggctttcatgaaaactcatgcttaccaaaagtcattgttaagaaaataaataggcaagtaacacatgagaagaaaaatgctctctgtccatatatctgacaaatggcttgtgtccagaatataggaacatttctcccactcactaaacagaggacaaacaactaatgggcaacagattgaataggcatttcttggggatagatagatgtacacatagccaataagcacctgaaaaaatgtccagtatctcagccatgaaaaataaagagttataatcatcatgagatgtcaccaaacacccaatggacatggatattattaagaagacaccacagtaactgatgtcactgatgtagagcaaggatgtgaaactctctcatatgctggtgaaagtgcaaaatgatacaaccacttttgaaatcagtctgatagtttctccaaaagttcaataaatgcacttttaccctacaaacctgcaatcctgtttgtgaatatttaccccacagaaatggaaacataagtccacgaagacatctccaagaatattcatagcagctttattttttataaccccaaactgtagacaatttcaatgtcaatcaataagaaaatgaataaataatttgtgaactagtcatacaatggcatactgttcagcaataaaagggagcatgtttttgatactctcaaatagtatggaagatgctcaaaaatattacattaaagaaagatgccagataacaaaaatgaacattatgtatgagtctattgatgtaaggttccagaaaggtaaaactaatttctggtgaaagaaaccaatatcatttgcctctggccatgggaagagagtagcagagattgattgagcagtaaaacgaagtttttttctggggtgatgtaaatgtcctgtattgtgattgaagtgtgagttacacaagtgtacatgttcatcagaagtcatcaaactacatctaagatctgtgcatttgactatacatgaaaatatacctcagttgaaaatagatcaataacctccctcatatactatacttgctaacacagccagctgcttggagaaccagcttgctggaatggagaatctgggcttgagactgggtcacatgtatagagtctctacagagacaatgttgcattcccacggtacataatacatttcaaggtttctcagacagccacatgtcatgaatgtgaggattctgagaggttggagcaacattcctgggaggaacgaaggggagcacattctccaagatcccccaccaccggggtcctcaccggctgtgcttttttttttttttttcttgacagagtctcgctctgtcgccaggcaggagtgtaatggcccaatctcggctgattgcagcctccaactccagggttcaagagattctcctgcctcagcttcatgagtagctgggactacagatgtgcgccactgcgcccagctaatttttgtatttttagtagagacggggttttgccatgttggccaagatggtctcgctctgttgacctcgtgatccacccgccttggcttcccaaagtgctgggattacaggcgtgagccaaagcacccagcctgtgcctctcacttactcaattgtttttctgaaccctccatagctggtggaccttttcagatcccatagtctagccagccctctcactttatgccttgggtcccactgttccttcatctcatcccccttctgtcagtcccgcagtggctgtggccagtagaggatggactgagagtaggagaggaggttctgcccaggaacccatcctagagaaacagcatcctgcctgggacctagtcttccaggtcagcttttataagtcttttagactcaaactcacttgacccacctgaagtggtattgacaataatgctattttcatggttgtttttcactgtaaatgcagagccttttagctacacgactagtacagagagtaagggaggctggcctgggaatgatatcatcttggatggcatttcctccttggagaaatatatgttagttccaactcacatgttactatacagtcctgtagaaagagatacagagagttagacaggtatagacgcatttgtatatgcataacaatctataagacacacatcaaaatccgtataccggttcctctaggggtatgtgcttggcagaaggtagaaggagggtattctggttcctttcttttgcacatttatgtatgatctcagtttttatatggagcattgatagggtttggctatgtccccacccaaaatctcatcttgacttgtaatctctataatcctgataatccccatgtgtcaagggcaggaccaggtggaggtaactggatcatgggggcagtttctcccaggctgttctcatgacagtgagagagtctcctgagatctgatggttttgtaagtgtctggcatttcccctacttgcacttactctgtcctgccgcctgtgaagaaggtgcctgtttctcccttgccttctgccatgactgtaaatttccagaggcctccccagcaatgtggaactgtgagtcaattaaaactcttttctttgtaacttacccagtctgtctcgggtatttcctcatagcaatgtgagaacgggctaatacaagcatatactacttttgatattttaaaataaaaattatcatctatctttgaaaggcatgcacaaatgggaagttgaggaacatttgtgttgtggcaattgtatgatacctttaatgggaatatttcaaagacacttgttaagactttgttagaacaaaatgtagagggtgctggatgtccctgaatattcttccgcctcctgtaacttgtattgctttggaatttccagtggcctgacaatgaactactgcaggaatccagatgccgatacaggcccttggtgttttaccatggaccccagcatcaggtgggagtactgcaacctgacgcgatgctcagacacagaagggactgtggtcgctcctccgactgtcatccaggttccaagcctagggcctccttctgaacaaggtaagaagtctgtgtcttaccttgtctagcacatacctctctatgtgcttggacaacgggatgaaaagacatgaaaaaccacactgatgcagaagcctttagtgctacacgggagctcgagtgttggttgaggttctgccatgaccaaggaagtctcagtgccgtccctgggaaagccagagctgtgatttttggcacaacttgtgggagtagtgactttaggactggcgcaaaacctccagggtgctcaacttaaccactcaccttattctaaaatgggttatttcagtgtcccagtcaaattcctattctaacatgctgtcaactgtgtgattatttccaagccaataagcatttccagtaatttcttaaaatagtgttcattgcagtcttcagcgttgtggctcctgagggatgtggcccctgattctgtcgtcctagagaagcctgacatgactgcattgattctgtatcgtcctgggtctatgtggctgcctggctgtctgtaatcatctgttttatttttatttttttctacagactgtatgtttgggaatgggaaaggataccggggcaagaaggcaaccactgttactgggacgccatgccaggaatgggctgcccaggagccccatagacacagcacgttcattccagggacaaataaatgggcaggtctggaaaaaaatgtaagccactttgatttggactctttttccctttgctgacaaatcttttcaaacagaagaggggcagaggaaaatactggaaagacttcaggaggctaagcgtaattagccttagcatggaaagtgcaagcagcacaggccagcaaagccccacgcgtgtgggggttctcaggcctcttctcttttgacatttctttactgtttccattgttgggtgctgtttctcgtttctagtgcttgtcctctaagccaggggtccccactccagtactggtactggtactggtactggaactggtaattatctgtggcctgttaggaactgggctgcacagcaggaggtgagcttcgggggagcaaacaaagcttcatctgtattttctgctgcttcccatcactctcatagctgcctgagctctgccagctgtcagatcagaggcagcattagattatcatagcacaaaccctattgtgaactgcacatgtgaggaatctagattgcatgctccttatgagaatctaatgcctgatgatctgtcatgcttccatcacccccagatgggaccacctacttgcaggaaaattagctcagggctcccactgattttaccttatggtgagatgcacatttatttcattatatattacaatgtaataataattgaaataaagtgcacgataaatggaaggtacttgagtcatcctttaaccatcgccccctcaccccaggtgcacagaaaaattgccttttatgaaactggtctctggtgccaaaaaagttggggaaccacactgctctgggttctagtagtcagagatgccctctatgaggcttaagtcagatttttctagaaaagatttggatgggccatcaggtcaccatgagacttcccttagcctcatgcattctctgtgatggtttactttggggcctatgaatagggaagactgagatataggaaaaaccaaagtgtctgtgttcccccactctcacacccatgtaacataacacttctcacaccagatatggggggatttctcctcacaccccaagcgagtctccagcagataccagctgggtgtcctacaatgtaactcggtcctgacactctatctggagacagtgtcagatcccacaagttaaggctcagtcctacaagactgccccactgcagatgccaatcccaagttgcaggctgtgacctgtacttctgcccagctggataaagatctgtttttctatatgaccctccatgggtttgattactttgctagagtggctcacagaactcagggaaacacgttacttttatttacccatttattataaaagatattaaaaaggatcctggtgaacagccaggtggaagagatgcacagggcaaggcacgtgggaaggggctcagagcctctatgccctctccagtgcaccagtccccagtaccctaagtgttcagcaacccagaagctctccaagtgcagtcttgttgggtttttatggaggcttcattacagaggcacagttgattacatcattggccatcggtgatcggctcaccttcggcccctcttccctccctggaggttggagggtggggctgaacagttccaaccctcaagtcacatggttggttcccttggcaaccagcccctggggctatccaggaacccaccaagagttgcttcattgcagctcccttcacccaggaaactccaagggatttaggagctctgtgttaagaactggggggcagagacccaatatacatttcttattctatcacaatatcacaggaagctaaggatgatactgcctttgtgtgtcttggctgtggatggtgcataatgcatggaagtaagcatttctgaatcaacagcaaacaggctttatcaggtagaagacccctcagcgccccagggacaaagctcatcaatgatgtcccactgtcctctgaggctctagctctaagacctccagtgggtcaagctcctggagaagtggcacattctccaaagacccttcagggtcaccacaccctggttaagggtgtggcctcataactccttttgactatgactgatggcttacagcatagaaagaaataactttgtcaaaaaatataataatgatagaaaggaagaaggaacgctcccttttgtcttctaagaatagatgtgaaatgtgtgtgccttagaatatcttctccctctcctgctccacgtgagctggagcttacatgcctgcttgttttcagtactgccgtaaccctgatggtgacatcaatggtccctggtgctacacaatgaatccaagaaaactttttgactactgtgatatccctctctgtggtaagttgccttctgttttggtaaggaaactgcttccttaatatggatttggaaaaaaaaaagcaaaaaaaacagaaaatggcttttgagctgagtgcttctggggaggagatggctgccctctccaccagagcctgcttttcatcatggccaccttgaacctgccctactattggccccatttgttaggaaaacacccgcccctcccaccacacacacataaataaaataaatgtcaaattcccaaagggcaaacttagaggtgatctaatcagcccgggatagtcccaccgaacccttctttgtctagcgtgggatgcatgaaaaacaaatttagagtcattatgatgaaaaactgtcctcttctgcagctgagaagaaaaaaaaaatacgagcagcaggaaacagctaagcatgtaatgcacattgtaaacctcagatggccatcctaggaaatcaatgaagggtagtgcagctctttagccccagatggcctttctcgtaagattactactcatgagtcccattagcgacattgcttagagactgcttgttaggttccttcctcattgctctgagactcttattgggagtatgaggcttggatcaggggaaggggaattgacattagatcttaaatgattggggtaacaaatccatgggggaaaaaaagccacttgtacttgttccctattttcttcctgctgaccaatcaacttgtctgtccgagttacagaacaccaccctggacttttcttttgtgtaatttggttgcttgtggttgggtctgccatgtgaagggaccttgagctgggggaagaaggttggcctccaagtccactgaagaccagcatcctgagattgcctggggaggtggtacagggcagtgatgaagatcatgggagccacactgcccatcgtcacatttgggccactcctggggagagcaagagggaagaaggagaggttagggtgataggaaagattctacttggccaatattattataatgtggcattgtggtctctggatttagtgtgagttgatagctgacttttttctcgagtgggtgcttttgttctattttgtcggtgctattgcagaagcatcttggtggttcctctacctcaaagtctcttgatggggtcagttccagttctccgcttctggccccatctagtacacgccactgcctctcactgcctgggctctctatccttgacaggctgccttgaatttaagcccagtctgacttacctgcctcaaacacccacagtagtgcctgggactcatgcacctttgactcccatggaagggaagtgcagtagcttcccaggtgcaattctgctgtcctcacccacattgaggatgtatgagaatcaggttcttagagattggagaaagaaggaagaatgggaacaagatttcttccaatggactgtgaggttccccaccttactttgatgtaagacaagtgaggttaaccccaagcctggtgaggagggttcccatcagacacttggaaatcctgaggactgtttcctgcagaaggatgtggttggtgggatattcaggtttgactcatgattgagaaagttagagcctctggttggagaaagagtttaataactatttcatttccaccaacacattcagtacgaataataaataagtaaaaataaatagaaacattcagttttattttgaatagtaggagtagggtataatttctgtagttactcttttagtacaatgatgcatgtttactgtatgtaaggcatactagcagaaattgagctcagcactagaaaagatgattgcattccatgccatgcttcttttttacaaaagacttctatagatagattctcaaaacaacccacagcaaatgaaaagttatttggaaaactcaggttccagattcactggagtgtagaatctctggttggttggggaggaatttcctcttgcagttgttattaataattatatgaataattattaactatattaatatttatagttttgaagaccttgaagggctggagacaacagagaagcatttttgaacaccctctgtagcccctgcactgttgtaggcattgatgggtggtaccaaagatgggacactttccctacctccagagaccttgtgggcttgctgcagagagaaggcagggaggaggaaaagaagaatagaggcacatgtgtgtaaattacccccacagcagtcagttagtcatgggaggctccccagaagaactgtcctgaagctggctgagagaaggcaacatttcaacataggacagttatccttgctacataaaatcacatacacacatgcacatatgtccacacacagagactcacatgcaaaagaatcctttgtgcctttcagtaaactttacatggtttagaaagaacttatatttccttgaaaggagagtgtcctttgttgtttactaccactttttaaacttagaaagaaaaatctaaagagtgtttatgattttaccatttaatttcacctttgagatgtgaaaaactagtgcttggaattcgtcctgaattaaacgacacaattgctaacttggactcaaatgcgacttcttttcccaccttgtgccacagcatcctcttcatttgattgtgggaagcctcaagtggagccgaagaaatgtcctggaagcattgtaggggggtgtgtggcccacccacattcctggccctggcaagtcagtctcagaacaaggtaagaacaggcccagaaaccatctatactgtccttccatgtaagccccacaaaacccttctacatttacacagaacccacacagctgatgcatcaatacctgcctctctgttttctgaaggaggaaaaaatatagaaaaattaaaaaaagttatattattataggttctctacttggaaaatagccaaaatacaaatctttttcttgatctgggcagttccatcaaaatctgtaggcacagtgatttgcaccaagttccaatacttttggaaaatattgaagatgctctgagggtttctatggatatccattgtctcactgtcagatgaaaagaaagggaagtttttagaaatgtgacactttgcagtgagggaggacaagagcaaacttacctacagtctatcacaggcacagatttttttttacacttttgtgaatcattgaattcaatgccgaggctattcatctattcacaaacacatgaacaaattatgggttgtgatccccataaatgaagagtaatcagtccgaacccacagaacctggacattttgggtatcgtttcagtggaacatgcaattcgtaagttcagtttgcttgggtgtctcttaggaagaacacataggacacagacccatctgcctgcatgttttgcttcctcatctcctttctacaccagggcacctgtgctcaattgctgttctcctctaaagagacttccttctgtaagtttgtgaaatgccatcgacaaacctgatcgcatcgcatttcactctgctgttgagttgatttttctttactttatcgtttgtaacttcttgctctacagagctttcaccttccacatatttcagattcattctttcctaaactgtgtggtggtctatgtcctcactgactatcaacatactgccatcatgcacttcctatctctattcctcttcgttgcaatctggctccaagtggctcacaccattattctgatctatcaactgcctacacagtcctagaaagtaagtgagtcaagaaacatcccccaaaagtaaacttttcaggtaagatcagaagaccctcatgagtcactgctgctcaggatcgtatctggctccttgaagagtgaccttgcatagatcttgtcataaaaaatgaaagagaccttgggaaggtcttgggctggtcacttttgtcagagtccagggctgtggggtgaaagccacagctatagagcttcattctggagtcacttagctttgctctcctggggacaggctgtgcctattcttgcctcaggcatcaaaaaaagtggcacagatgggcccttctgaaaaatctcactactggagcacagctcgaagtttctactatcctgacgttgggcggtagtcctttgctttgggaatatgaacatgatcaaaactgagtgaacttgtcttcctggctttctgtacaatgaagtagaacaaaccatccaatttgaccaaagccttggcatgttttctttctaggtttggaaagcacttctgtggaggcaccttaatatccccagagtgggtgctgactgctgctcactgcttgaagaagtacgtttaagggaaaactgacatggggtcttatcttcaagacttttttcctccctctcttcctccatcccttctttcttcccaccctccccttccttcctccccacctctcttccttttctggaaggaacactaggaaccagggaatgcatgcagaatcctgaggcagaatttccagggcaattggatgagagaggagggaagtgtttctagagggaatctgcagagggaagacccagtgcaagtgattttttggacctgtataaaccgcaggacagagctgttcactaccagaggcatcaatctgtattgcattgctctagagcaatatctgaggctgaataatttataaagaaaagagtttaattggcacatgtttctgcaggctttacaggaagcaggatgctgtcatctcctctgcttctgtgtgggcctaaggaagattacaatcatggtggagggcaaagtgggagcaggcatgtcacatggccagagcaggagcaagagacagagagagatggggtgggggtgctgcacaataccaaatgaccagactttgcaagaactaagagtgagagctcactgatcaccatgaagatgtggcccaagccattcaagagggatgcacctctatgatccaaacccctttcacaggccatagctccatcactggggactacagttgaacacgagatttaggtggggacaaatatacaaactatatcacagtctctgatgaaacagattgagaacagaccttaactgtcagtttccagcaaattgtgaattttgtttcttgccactcataagtcactgattctgggtggccgagggtgtcagagggacagcgccaagttcatggcacagaggatacctgaaggggctggaccatatttttctcttgacatcctcatcttttctaggtcctcaaggccttcatcctacaaggtcatcctgggtgcacaccaagaagtgaacctcgaatctcatgttcaggaaatagaagtgtctaggctgttcttggagcccacacaagcagatattgccttgctaaagctaagcaggtactcgctcacctgtggtcttcaccccacgctggtgaagatatttgctttatgtctgggttttatgggccatggccactgcatggcagtggggaggaactgtctatcacatgaaaggctcaagggctttggggacagcatcaatcttcaaccccagccctgccacatgttagttgtgctctttaaaaaggcagaaggattcgtttcctcacgtggaaaaagagataccctgttacccgtaaaacttacttaatgttcaccagttcatccacattcatgatcagggaaaggttgttattccaggctaactattctcctttcataataatatgctggagagaatcaaatgagattgcatttcaaagcgcttgaaaaaccaccatatcgagccatgcttagtgtgggcgcctctaatcactgctattcaggaggctgacgaggaagaattgcttgagcccaggacttcaaggctgtaggcagctatgattgtgccactgcactccaggctgggtgacagatcaagaccctgtctcaacaaaagaaaagaaaacaaaacaaatgaacagaaatattccacaatgtcaaaaaaaaaaaaaacccacacaacatacaatttacaaatgcaaataataatattattgttgtcttctttgattttctctttcctggtgaaattttgttttattaagcctgacaaagtgatacctttgcttacatcacttaaagttagtctatttggacctaggtgacagtacaatcagctaagaaacagtatttgtaggagaggcaggtttgggacaggtgacaaggcatgtggggtgctcgctgtgctggtggctctggaaggcagggtgtcaatgcagacagggatgagcatggcctggttgggaaggcatggggcaggcaggagcctgagctgctctcctgggcctggtcacaagcccatggcagcttctctgggtctgtgaactgaggggtgatgtcctggaatcctctgacactctaggaaggagagaagggcctttctggctcagcctttataaacagtagctgatctccctcttgctccccagggtcctccccaccatcccagcaaatgtgcaaatacaagatctctgctcctcatggtcctcagagagctggggtgttctgatggcttgaacaagtcacttaggaaatgtggggttttggaggcattctctgataggctgatacgttttgagtttagagttcccaccgcacatccccacacccctagagtctagggcatttagtgctccatgagggaacctgtagagtgaggacatctgcatcacaggctgggccttctagtgtccagaagcagaaagtgtgtctgcttcaaagttggtgctaatgatgatttttggtcagaatacggcatttctcatttccattcctttatccccttgaacttactaaagtagaatcaggtctaaaaaccagagttctaatctttaagagtccctgggattctaaggtatatgaatgtccttggaaaacaataccatttagttcatgcaaggtgcttatttcccatcctctttcatttgatgtctagcattttactgcattcttaccaccacggtttagtaacattcacgaggaggaagtggaggatccagatggagcaacttgctctgggcacacaaggcatttgcaattttataccctcttgatgatgtctcagccagacattctgcccagtcatcaatgccctcttcaattaatatgaaaggacacacttggcatgagattccaatcgtgcacagaatatacatgagaagtgtgcctttgtcatccctactttcaaaggctaaggccaccctcagtttcttgcatgcaactgatgcctttcaaatgaaaccttacatctgtgtagtccataggcaaccacaggcaaatgtgagggtgaaacgctgtgttctacattgttctgtgtcagtgaagcaaggcagtgccagctcagagggctctggggcttcaaggcagggatgcctggttgtaggtactgccacttccagctgggcagtgaaacataactgctaatactttccttacaggcctgccgtcatcactgacaaagtaatgccagcttgtctgccatccccagactacatggtcaccgccaggactgaatgttacatcactggctggggagaaacccaaggtgagatcaattccattgcccacgtaacaaattgtttttgaccttcagtgcatgttacaaaatgagcattttggagatagttgtacaaattcctacccatgaatgtggtctacccactcctgactttgcctggacacctgtctatgtctccataatcagtcttcaagggacttgggcaaggggagcggtgccatttccttgagtctctctcttttttgttttcagaatcttttaattttttttgtaatgattgtatgtttcccttacaacaaaaacaaacaccagtagaggtctttgagtctcttaatcataatttcagcattcatattgcttccccaggtaagtggggttttgacccagccctcaagttaagggtgttagattatttttcatgtgaaattagacagactgcgtttctaaacatggtgcaaaacagtaacgacaaaagttgtaattaaactattcttcttcccaaatacccacatgtctaatgtgtgtgtgagggtgttaggcaggggacctgaagctgggggagaggcagacagttcccatggccccaagtctaggatggcatttggtattggttgatgggtgagagcaagagagggaatatttttgtgcatgatgtggtatcagcacctgtactacattttatggattccttcttctctttgcggtatgccctgacaataattatatccgtcagccttacccccttggcagtaggaaaactgaaactgtcttaaagtctcagctctactttctcagaggtgcaggcaagggcactgggagtctggggccctggaaaactgttctgactctgccacttgccagatagacctgaactagacacgttacctctttgtaccacttggctctaatcccttatctgtaaaaccagcattttcaaatggtgctttgcacatcagccttttgcataagctttgatttgataaaatgttttttgtgtttttaaaaagattaaaaaccacaggtttagataatttcaaagtaggcttccctttttctgtcattttcctattatttttaaaacctcacctccttgactccttgttccctttttctgcactgctgagtctgggagcactgaggccaggtaaaaggaaacttggcaaatgaggggcacctatgggtgtgggaggctgctcctggtgtttgcatattttaaaatttaaatgctacaaaccactgtgagttaggtattattgttcctattttaccattgaggaagctggggctcagagaaggtggagggtggtacagacaaacctgaattggaaccctggctcctgcctatgggctgtcaggacttagaaaagtcgtgagctctcgctgattgtttcctcagctgatgtgggctgcagggctgttatgggggaaataataagaaagtgcatcaagtgctgagcacatcctaagcactccatcatggcagctcctactactaataaagaatagaattatatctaacatgattctttcttgcaagtgacagaaaatccaactcaaattggattaagcaaaacaagggaaattcttagtgagctgcaaagttttcaggctcacatgatggccccaaatcccaggtcctcccaatcatggagtaggcactatttgggggcacaaaggtgacattcccatggctgcagatgctgtggtgctgtggctgtaccgggaaagaataagaaaggccactctcccaattatgtgaacaatagtctgcccactctgagaagtcaaacttgggtcacagtcctgcccctgaacccatcactgactggctctgacctgcaccaattgttccatgttggaggtgaaggcaagaccccactaatacccataaggggcaaaagttagatagatccttcaagaggattatgggaggtagggcaaaaagctgctgggcagccagaaagcaaacagagcctctatgatacctcaactgatgaaagcatgaagctaaaatcataaggatctgggtgtgagttctggctctcccatcttccatgtgacattgggcagttatttaatctcttttagcctccgctttctcatcttacatatgagataattgtgaggattaagattacacataatcatcatcatcaccgtccaccactaccaccatcatccccatcaacatcatcgccaccactatcatcattcttactggcactaccatcaccatcaccaccattccaccaccatcaccaatatcatcactgtcaacatcattaccaccatcaccatcaccaccaccatcatcattactaccactaccactactaccaccatcaccatcaccaccattccaccaccatcaccaatatcatcactctcaacatcatcaccatcaccatcaccaccaccatcatcatcattactaccactaccactactaccaccatcaccatcaccactgtcccactactatcagcatgacatcaccatcaccaccaccatcatcattaccaccgctactaccaacatcaccatcaccacaattctactgccatcaccattaacattaccaccaccatcatcactatcaccatcaccaccatcatcaccactgccattatcactgccaccatcatcactatcctctatatttcctcatctgtattatcattactaccaccatcactatcaccaccatcgtcaccatcataatcaccatcaacaccatctccaataccaccatcactgtaaccatcatcaccaccaccatgatcactatcaccatcatcacaatgatcactgtaaccatcattactacccaccaccatcaccactactccaccaccatcaccattatcattaccatcaccattatcaccaccatcatcatcaccagcaccaccatcatcaccagcaccaccatcaccatcaccatcattaacaccatcactatcaccattggtttaatcatcaccaccatcatcataaataaacatcacataaccagggtgtagctgggtgttgaccccagagcccactcactgtttcctctctcccacccccatccacacatttctaaccaccatcctgcactgggctcccagtctcctctggtctcacccacatgtccactgagaaaaggattttcagaacaccaactagaccaggaggagccacatacataactcaggcctgcttatcaactttctacatgttaataatgacatcagatcaatgggtgttctcagcttctcagaaggaggtcaaaattctccccctctccccttcatgtgtccagaccttcccggatttggatgtaccaagtgcagagtggtgttgaggccaaggggctcatccatgtaagtctcatctgcaatcactgggctgatcccgtggccctgtctccagggcgccatcagagagggcttcaatcctcaggttacctgtggcccaccctgccctcagaggtgccatctctacattggccacgagatggcagcacatactcatagactgcattaatttcccagcaactcctggtgggttttccctcttatcaggatgtttgccttgctcagagagcaaatctgagagcagtgacacctaacttaactttcagcaaaatattttgagaagggtgcccctttacacatctgtgcagtccaggtgatgcatcccatgcccaatgctcggtagtcaggaggagcttcctccatgcagctctgcggaagagactcttccacgctgctcatgtaaactccagattcggtgtcagttttctgacaccgaagacaatgatctaagtgcagtcaagggctttggggaaagcaggagagagtgcctcagttctagcctgtgccatgcttgcaaagttttgcaaaattctaatgagagctgggcttgcaacattggaaacttggattatttgtgagagcactgagaaatccctgggcatgtccatctggaaaaacagcatttcctctggcactttagcagaggttctgtttcaatttggcgaaggaaattaagcagtttttcacaaaagaagaactacaacgaggagaattgtccctagtatttcttctccctaattgtcaaggaagtgtaaattagaaaatgaatcaggacaatttccacctactatgttagctaatattttaaaaattgaatatcacaagggtgaggcaaagtaattgttttccagtgacattttccactgtcacacccttttagagaataatttggcaatgttactgtgagatagaaatatgtctatataattatgggaactgagacttcagaaagtaataaggaataagaatgaaatttatgaacaaacatgtggaaggttggaagcaagagtggggccaacacgcatggggaggaagcatttgggcagcgactccgcagacccagactcaagctgagctatacaacctccttacgcctcagtttcctcaactgaagaacaggaatgacaagtgcctgtttcataggaccgttgtgaggattaagtgagatataccacattatgagcttgtgcctggaaaggttgattcttagtaaatgatgactattcttttttattgcaataaaatttatacaacatagagttactattttaaccatttttgcaggtaccactgagtggcattcagtacattcacaatggtgtgcaaccgtcaccatatttccaggacatttttctcatccccaaaggaaacctcatgcccattaagcagtcactcctcattaaaatattagttatgaagactgtagcatttttttaaaaactcatgatataacattgattgaaaaaatcagtataggaaattgtgcattatgatgtaatagtaaaagaagcatataaaaatctgaaaaaagtatataaaaagaatagcaattgtatttctcagactctctttacattgtaaaaatcattttgatagcttcaaaagaaaagcaaaaagtacacaaacaacaaccaaccccaaagcagcatgacaaagcccagattgttgaatccaggtcttgggaacataaaatcttatatgacatttgcactttaatgggtcagagagtccagtggcattgggagctgccttgtgttctgcagcctcacggacagacaggaggtccagctccactgctctgttcttctggaatttcctcgtgaacaagctttggcctcagtaaccatttctttcatctttttaaacacaggtacctttgggactggccttctcaaggaagcccagctccttgttattgagaatgaagtgtgcaatcactataagtatatttgtgctgagcatttggccagaggcactgacagttgccaggtaagaaaagatcaatagatcaaagtcttgtgctctcccgtctcagtctcagtcccttagacgtcagtcccaaagtggcaaattcaggaaggttttgtcagtggaagaccccagtctaagtgttgctcagaaactccccagatctgtccctgaatgcatattcagatcatctaaggagacgtcttggggcttgagttccagatccatagcaagggagccgtaagtgccataactacctcaggccactcaccttcctggtgtgtgctggtcaccagtgactgaagtggtggcttttccagtagagaggaaggtagagggtacaggaccgagacaaattacacacacttaacaatgatgtccaggctagcccagtctaaaggaaacaccaagttaggaagcaatgcatgcaggattcacaagggattattttttttcccaggaaaaaactaagtgatgtggttttgttgaatagactttgctaagtacttaagcactgcagatgcttgagtaatatgctcataagttcctttctgatttgaattactgggaaaatgtacatatggataagagaaggatggcatcccatattaaaaggttggcagcttaaagctcacatgaattttcccctacctctgtttagggtgacagtggagggcctctggtttgcttcgagaaggacaaatacattttacaaggagtcacttcttggggtcttggctgtgcacgccccaataagcctggtgtctatgctcgtgtttcaaggtttgttacttggattgagggaatgatgagaaataattaattggacgggagacagagtgaagcatcaacctacttagaagctgaaacgtgggtaaggatttagcatgctggaaataatagacagcaatcaaacgaagacactgttcccagctaccagctatgccaaaccttggcatttttggtatttttgtgtataagcttttaaggtctgactgacaaattctgtattaaggtgtcatagctatgacatttgttaaaaataaactctgcacttattttgatttgaattaattttggttttggtcttcaaaattttcatgctcttttcatcccatctatttttatttttattttttagactttacgtcctggggtacatgtgcagaatgtgcaggtttgttacatagatgtacacgtgccatggtagtttgctgcacccatcaacctgtcatctaattcggtatttcttttagttctatccctcccctagccctccaccccttgacaggcccaggtgtgtgatgttgccctccctgtgtccatgtgttctcattgttcaactcacacttatgagtgagaacatgccgtgtttgtttttctgttcttgtgttagtttgctgagaatgatagtttccagcttcatccatgtccctgcaaaggacatgaactcatccttttttatggctgcatagaattccatggtgtatatgtgccacattttatccaatctaacattgatgggcaattgggttggttccaactctttgctattgtgaatagtgccacaataaacatacgtgtgcatgtgttttcatagcagaatgatttataatcctctgggtatatacccagtaatgggattgcagggtcaaatggtgtttctggtgctagatctttgaggaatcaccacactgtcttccacaatggttgaactaatttatgctcccaccaacaatatcaaggcattcctatttctccacatcctctccagcatctgttgtttcctgactttttaatgatcgccattctaactggcatgagatggtatctcattgtggttttgatttgcatttctctaatgatcagtgatgatgagcttttctcatatgtttgttggctgcataaatgccttttttggagaagcatctgttcatatcctttgcccactttttgatggtgttgtttttttctggtaaatttgtttaagttctttgtagattctggatattagccttttgtcagatggatagatggcaaaaattttatcctattatgtaggttgcctgttcactccgatgatagtttcttttgctgtgcagaagctctttggtttaattagatctcatttgtctattttggcttttgttaccattgcttttagtgttttagtcatgaagtcttctcccatgctatgtcctgaatggtattgcctaagttttcttccagggtttttatggttttaggttttgcatttaagtctttaatccatcttgagttaatttttgtataagtaatgcccttctttgtctcttttgatctttgttggcttaaagtatattttatcagagactagaattgcaatccctgcttttttttttctttttgctttccttttgcttggtaaatattcttccatccctttattttgagcctatgtatgtctgcacatgagataggtttcctgaatacagcacaccaatgggtcttgactctttattcaatttgccagtctgtgtcttttaattgggggcatttagtccatttacatttaaggttaatattgttatgtgtgaatttgatcctgtcattatgatgctagcgggttattttgcccattagttgatgcagtttcttcatagtgtggatggcctttacaatttggtagtttttgcagtggctggtaccaattgttcctttccatgtttagtgcttcgttcaggagctcttgtgaggcaggccttgtggtgacaaaatctttcagcatttgcttgtctgtaaaggattttatttctcctttgcttatgaagcttagtttcgctgggtatgaaattctgggttgaaaattattttcttttagaatgttgaatattggcccccactctcttcgggcttgttgggtttctgcagagagatccactgttagtctgattggcttccctttccgggtaacccaacctttctctctggctgcccttagaaatttttccttcatttcaaccttggtgaatctgacgattatgtcttgaggtggctcttctcgaggagtatctttgtggtgttctctgtatttcctgaatttgaatgttggtctgtcttgctaggttggggaagctctccttgataatatcctgaagagtgttttccaacttggttctattctccccatcactttcaggtacatcaatcaaatgtagatttggtcttttcacatagtcccatatttcttggagcctttgtttattccttttcattctttatcctctattcttgtcttcttgctttatttcattaagttgatcttcaatctctgatatcctttcttttgcttgatcgatttggctattgatacttgtatatgcttcacaaagttcttatgctgtgtttttcagtcagatcaggtcatttatgttcttctctaaactggttattctacttagcaattcatgtaaccttttttcaaggttcttagcttctttgcattgggttagaacatgctgctttagctcggaggattttgttattatacaccttatataatagcctgatataactataagatttttttgtaagcaccatcgtaaccacaaagcaaaaacctaaagtagatatacaaaagataaaaaggaatcaaagcataccactagagaaaatcacttaatcacaaataaagatacgaagagtggaataaaggaacgaagggtctacaaaacaaccagaaagcaattaacaaaatggtgatagcagatcttacctataaataattatcttgaatggaaatggattaaattttccaataaaaagacatacagtggccaaatagattaaaaaataagatccaactatatgatgcctataacacactcacttcacctgtaaggactcaaacagactgaaagtaaagggatggaaaaaatattctatgcaaatggaaacaagaagatagaggggtagttatacagattgagtatcactaatccaaacatctgaaatctgaaatactccaaaattaaaaatgtttaagtgccaacatgatgttcaaaggaaatgttcttcggagcattttggatttttgtgtttagggatgcaaaaacagtaaatatataatttgtattagtccattctcacactgctataaagaatactacaaagagactgagtaattataaaggaaagatgtttaattaactcagagttccacaggcttaacaggaagcatggctaaggaggccacaggaaacttataatcatggcggaagatgaaggagaagcaggcaccttcttcacaaggtggcaggacggagtgtgagtgtgtgaaggaggaactgtcaaacacttataaaaccatcagatcttgtgggaactcactcactctcacaagaacagcatagggaaaaccgcccccatgatccaatcccctcccactgggctcctcccttgacacatggggatcatgagggttacaattcacgatgagatttgggtgggacacagccaaaccatatcataatgcaaacattgcaaaaacaattcaaaattcaaaacatttctggtttcaggcattttggataagggaaactcaactcaacatgaggtaaagcagactttaagtcaaaaactgtaaaaagagacgaagaagaatgtaataataaggagatcagttcattacaaatatatagcaattataaatatatattaatatatatacccaaaattgtagtacctacatatagtaactaaaacaaacattaatagatctcacaggagagctacactgtaatataatcatagtagcacacttgaatagctccactttcactaatggacagatcatccagacagagaatcaatatggaaacacgagacttaaactacactttagccaagtagacctaacagaaatatatagaacattccatccaacagcagtagaatacacattattctcaagtgcacagggaatattctccagaatagatcatatgttaggtcacaaaactagtcaaaaaatgtaagaagattgaaatcatatcaggttttttttttagatcataatcgtatgaaactagaaatcaataatgggggaatattggaaaatccacaaatagatagaaattaatcaatatgctcctgaacaatcaatgagtcgaagaagatattaaaagaggaaattttaaaaaatcaagacatgagttcatgtcctttgcagggacatgaatgaagctggaaaccatcattctcagcaaactatcataaggacagaaatccaaacaccgcatgttctcactcataggtaggaattgaacaatgagaacacttggccacagggcggggaacatcacacaccagggcttgtcagggggtgggaagctggtgaagggatagcattaggagaaatatctaatgtaaatgacgagttgatgggtgcagcaaaccaacacggcacatgtatacctatgtaacaaacctgcacgttgtgcacatgtaccccagaacttaaagtataataataaaaaaagaaatatttgtttttgatttatatgccaatcagacaaaatgtgaaaagccctactgaaattaagtatcaccatgaaagataaattctggataattttttcaagttttaacaatgtagctttaattggagaaagctatcatttggaatgagttaatctatcctatactaaaataagtcacttgctttaaaacataataaatatgattttgaattgaaaacaaaaacaactcaagacaaaggaaaatggacacactaacataccaataatttatagtatgcagcaaaagtggttttaagagggaagcttttaccaataaacacttccattaaaaaagaagatctcaaataagcaacctaagattacacctcaacaaactagacaaagaactaactaacccaaaagttagtagaaggaaagaaataataaagatcacatcagaaatagtaaagactaaaaaactgataccaaaaagaaataaaactactagttggttttcaataaaataacaaaattgaccaacttttagctagattaagaaaaacagagaatactcaaataaaaccagaaagaggagacattacaatagatactacagaagtacaaacgatcataagagactactatgaataattacatgccaacaaattggataacttagaagaaatggatgaattcctagagcaaaaaacctacaaagactgactcagaaagaaatagaaaatctgaacagaccaataatgtgtacatgattgtatcagtaataacaagtctcccatcaatgaaaaggccaggacctaatggcttcactgctgaagcataccaaacattacaaagactaatatcaaccctcctcaaactcttcttaaaaactaaaaagaaggaatgctttcacattcattttatgaggatagcattacactgatactaaacacagaaaaataatacgctaataaaagaacattacaggcaatatccctgataaacatatgtgcaaaaatccgcaacaaaatactagaaaactgaatccagtagcactttaaaaagatcattcaccatgatcaagtgcgatttgtttcacgaatgcaagaatagttcaacttacacaaataaataaatgaaaggatggatgataaaaatgtgtatctatatatatatgttttatacacacacacacacacacacacacacacacacacagaggaatattattcagccttaatgaagaagaaaatcctgcctttgcatcaacctggaggacattataataagtgaaataagccagacacagaaaggcaaatactgtgtgatctcgcttacatatggaatctaagaaagtcaaattcctagaaatagagagtagcttagtgattgccagagccgtggaagggggaaatggagagatgttgatcaaaggatacaactgtatagctttgcaagataaataggttctggagatctaatgtgcagaatggtgactagagttaataatactgtattgcatacttgaaatttgctaaaagagttgatcttaagtgtcctcaccatatacacaaaagtattatgtgaggtggtgaatattttaattagcttatgataataatttcacagtgtacatctatattaaggcattacattgtacatcttaaatatatataatttttatttgtgaagtgtacctcaataaaactggaaaaaataattgaaaagtaatgaaaaaaattaaaagctattatgtgtcaaatgacattatcaagaaagtgaaaagcaacctactgatgaagcaaacctattgacaaaggcctggtgtccagaatatattaagatctctaggctgggagcagtggctcacacctgtaatcccagcacttggggaggccaaggtgggaggatcacttgagcctgggagttcgacactgcagtgagctatgattgggccactgccctccaggctgcgtgacagagtgagactgccatctcttaacccacttcttatttagaaaaagaaaatatgtagcttgctgcctgcatagtattcttggggcaaatgggaaatgagttaaaaaaaaaaaaaagaactcttacaactcaacaataaaaagaaaaacaagaacgtgaatagacattttttccaaaaaagatatacaaataggcaataagtacatgaaatgatggtcaacatcattagtcattaagaaaatgccaataaaatcacaatgaaataagacttcatatccattaaaatgtctataatttaaaaaatggaaaataacaagcatttgtgaggatgtggagaaattagaatcctgtatattgctggtgggaatgtacagggaaaatggtttggccactgtggaaaacaatttgacagttccttaaaatgctaaacatagaattaccatgtgatctaacaattttactcttaggtgtatatatacaagaattgaaaacaagtgcccaaacagataccttgcatgagaatgttcatagcagcactgttacaacagccacacccaaatgtcaatcaatagatgaggggataaacaaattgtggtttatacagctacaaaaaggaatgaagtactggtatccgctacatggctgaaacttgaaagcaagggctgggatggggtcatggaaagtaccagcttattgggtactgcattgtgctttggggtcatgaaaatgttttggaactggatggaggtggtggttgccaatgtgaacatactaaatacaacgcattgttcactataagactgctacttttcttatgagaatttcacttcaattaaaaaataccttccatgtatcctttctaaggatgatactagaatatttgctttggcaaaatgaggaagtaactttttttaaaaaggaagatgtgggatccatgaaacgggatcaaatatcagagaggaaagggggtcttctggatgacagtccatggagatcccacaactgcacagcaggccggctgtgcacccaggccacaccagagcagagccggtggttcccgaggagctctctggaagaaaaacgctagatggcctgattggtttgggggcatattgaaaaggtatataactgagaatttggagtggaattaggaaacagacataaaagcttacagaaaagaaaataatgaattctagggagaaatataaaaggatactacaggcctcagttacataaacactgaatatttacttaaccaaaattacaatataattacataattattttaggtacatatggcaaaaggatgtgtgggtgtatgtagtatgtacggtgtgtgaagtgtatgtgtgtggtatgtggacggtatgtgtatgctgtgtatgccaataaaatcacaatgaaataagacttcatatccattaaaatgtctataatttaaatgtctataattttaaaaatggaaaacacttctcatatggcaggagcaggagcaagggtgggggaggtaccacacacacttaaacaaccagatctcctgagaactcactatcaggagaacagcacctggagaaggtgctaaaccattcatgagttactgccctatgagccaatcacctcccatcagaccccgcctccacactaaggattacaatttgacttgaaatttgggcatgaacacagatcgaaaccatatcaataggtaatgactaaaactgaaaaaagaagtaccacagtcagaaagttatttagagagctgaaggtaaatgccaataggatcagttgaaagaattggaggtggccgggtgcggtggctcaggcctgtaatcccagcactttgggaggcggaggtgggtggatcgccctgaggtcaggagtttgagaccagcctggccaacatggtgaaacccagtctctactaaaaatacaaaaattagccaggcctggtggtggacgccgtagtcccagctactcaagaggctgaggcaggagaatcgcttgaaccagggaggtgaaggttgcagtgaaccgagatcgtgccactgcactccagcctgggtgacagagcaaaactccatctcaaaaataaatgaaataaagaattggaagtgtttgcctctggagagaaggaaacgcagtaattctgtaaaaacagaactttttactttttttctttttttttttttttttgagacagagtctccttctgtcacccaggctggagtgcagtggtgcagtcttggctcaccgcaacctctgcctcttgggttcaagcaattcccgtgcctcagcctcccaagtagctaggattacagatatgggctgctatatccagctaatttttttttatttttattagagatgaagtttcaccatgttggccaatctggtctcaagctcctggactcatgatcctcctgcctcggccttccaaattgctatgattacaggtgtgagccaccatgcctggacagaactttttgactctttaaactatgtgcatatataaagctgatttaaaaaaaaccaagtaaaataattttaaaatgttccaaaacagattggatgggtacacacttcatcatgagtggttgagggagactgggttagagatgaggaaattccagggactggggaaaagttaaaatgacaaactgttcacaattgttaactgcaggttgtgggaaagttggtaagttgctacagtgtttgttccctctgtaggtttgcatatatttaacatttcttaaattagcataataatgaactgtgtaatcagctgtagagttgagggtgtggagctggcacaggacagctgagctactggtttaaaataaatgacatttaaaaaaatggctatttgtagaattaacagatataagacaccctgatcaagggatgataagaaaggactccagggctctgtctcagctgtcttggcaacacctggaagacatgggcctctgcaaggtctcatactttcaggaggtgttgatgaaggatatggacagatctgaagctctgggcactgcatggtctgagaagagaagctccggaaacgcgggagctgagtgcagatgcagaagggctgtcatccagcagaggggtaggtgacaactggcctagcgagtgacccttatcatggctacatttgttgatcactttctttgtatgaggcactgctgtgattgcattaaatttccacttacctaaatccaacgttgtgcacttgtgaatttctactcttacaaaaaacacaacggcaacaacctcaaaccagtaatctagtcaaaaaagcaattcccaaggcatgacattcagattcatcagcactcacagagactacagtgattgctgataacgccaacttaatacctggccaacagcatggatcctgacctccacttttcttgtgtgtttacagaaccacaaaaaggtgcagtgttttca

SEQ ID NO: 3 - DNA, 138001 bp, Homo sapiens
ctctcccaaattgtcaaagaagtataaattagaaaatgaatcaggacaatttcaacctgttagattagctaatatttaaaaattgaacactcatacaagtgtggtgaagtgattgttttctagtgacattttacactgtcataaccttctagaaaataaattggcagtgttattgggagacagaaatatgtctatataatttatgggaacttaggctcagaaaatattaaggaataagaatgaactttatgaacaaagatgtggagggttggaagcaagaggggggccaacgcgcacggggaggaagcatttgggcagtgactccgcagacccaggctcaggttgaactagacaacctccttacacctcagtttccttaactgtagagcaggagtgatggaactgcctgtttcataggactgttgtgaggatgaagtgagatacaccacattataagcttgtgcctggaaaggataatgcttagtaaatgatgactattcttttttattgcaataaaatgtacacagcgtaagagttactattttaaccatttttgcagggtaccaccaagtggcatttagtacattcacagtggtgtgcaaccatcatcatatttccagaatattttcctcatccccaaaggaaacctcatgctcattaatcagtagctctcctttaaaatattagttatgaagatcatagcactatacaaaactcattatgtaatgttgagtgaaaaaatcagggtgtgaaattttgtgatatgatgtaattagtgaaagaagcatacaaaaagtctgaaaatataaaaacaatagcaattgcatttctcagactctacatttaaacattattctttatggttttaaaagcaaagaaaaaggtaaagaaacaacaaccaaccgcaaagcaccatgacaaagctcagattgttaaatccaggtttttggaacatagactcttatatgacgtttacactctccagggttcagagagtctggcagcattgggagctgccttgtgttctacagcctcacggacagacaggaggtccatcaccactgctctgttcttctggagtttccttgtgaacatgttgtggacgtagttaccatttctttcatctttttaaacacaggtacctttggggctggctttctcaaggaagcccagctccctgtgattgagaatgaagtgtgcaatcgctatgagtttctgaatggaagagtcaaatccactgagctctgtgctgggcatttggctggaggcattgacagttgcaaggtaagaaaagatcaagagaccaaagttagtcttgtgctctcctgtctcagtctcagtcccttagacttgagtcccaaagtagcgaattcaagtaggatttaatcaatggaagaccccagtctaagtgttgctcagaaactccctagatctgtcccaaatgtatattcagatcatccaaggggacttcttggggcttgagttccagatcagcagcaagggagccataagtgccataactacctcagaccactcaccctcctggggtgtcccggtggccagggactaaagtggtgatttttctggtagggaaggaggtagagggtacaggacagagactaactgcacacaatatctgagactggagctcagatattgctgatgatcagagttggcgtgtctccccaattgatttacaactggggcttggatactgttttaaacgggaggagcctcctaaccatcttgacacaaccactgacgtgactacactagagatagactctttccacttaattctaccactcttgctttacttcatgagaacgaaaatgtaagattgcaccatgaattcatttgcggaaagattgatactatgcttttattttattttattttattttattttattttattttattttattgagactctcaccccggttgaagtgcactgacgtgattttggctcactgcaacttccacctcctgggttcaagtgaatactccagcctccctagtagctgggattacaggtgcccaccaccacgcctggctaatttttgtatttttagtagagatggggtttcaccacattggcctggctggtctcaaactcctgaccttgtgatccacctgtcttggcctcccaaagtgctgggattacagagttgagccaccgcactcgaccctatgttttatttttaaaaatatttatttatttatttaagccacaactactagaataggaaggattgatattttattaattttatttggtatttattatttttttttctttcctgagacattcttgctctgtcacccaggctggagtgcagtggcacattcttggctcactgcaacctccatctcctgtgttcaagcaattctagtgcctcagcctacttagtagctgggatgactggcatgtgcctccacacccagctaatttttgtattttttgtagagacagggttttggcatgttgcccaggcttgtctcaaactcctggcctcaggtgatccatctgccgtggcctcccaaaatgctgggattataggcatgagccaccaccccctcctggaaggattgatatcttataacataatttataattacagaaaacatgtgagttcactaggaataaataaattttgaagataataaaagattttcacttatgttgtcatttcggcacagtttggtataggatgtggagatgttaacatttatacctagcttgctcgtaaactaagacctgaaagggttgtgtctatcagctgcacccctgggtagcgacacaacctcgggaaggcctcagccccctcctcgtacagcactgcctgttggaaagcttgagggaggctatggatgtgcagcacttggcagagggtctggtcatggaagttaccagcaaatatgagctacttttatgattttattttatccaaaagaaagagaatgaaagaagaggggaggaaacaagactaatcaggaaagatgaaggtctaggggtgagggaaggagtaaggagacataaaggcaatgtggagcagctgaggggggaaatggctttcaccacttcccagcatctattgacattgcactctcaaatattttataagactctatattcaaggtaatgtttgaaccctgctgagccagtggcatgggtctctgagagaatcattaacttaatttgactatctggtttgtgggtgcgtttactctcatgtaagtcaacaatgtcctgggattgggacacactttctgggcactgctggccagtcccaaaatggaacataaggaagtggttcttctacttcttttatttctgaaatcaggtaagacatagtttttttaaattataagaattattttttctcccacaatgtagtaaaaatacatatgccatggctttatgtgcaattcatttaatttttgattcatgaaattcccagttcaaaatcttgtatatgattgaaaaattcttaaaaaaataagtttaatttccccgtgaagactgtcacggtgctggaatgaatgggcagaaaaaataatggttgatttttctaatctaaaagagtgtgcctacatgatggccagtctggctgaaaaataaatagccattgtagctaactatgcaaaggatggctaagctcttcgcttggttctcagtttcattaatttatatcatctctgttcaggtgccatgctcccctcactagcaagttgaaacaatgaaataactctttgaatatgtttggttccttgacctgttcatggagtgggactcagcatttctctctttgttatggcctgagtaaggctttccatcggtatacatttgcttcttatccctggagaaattatacacatccatttgccagatgatatacgcatataatgattcaacaaatactcagggtatttgttgagtgggttaggtccccacatttttatacatacatacacacatacacaccgtgtgtgattgtgaatgtaagtgtgtgtcctttacaaatactagcttatttagctcatggtataggtagggtagcatagtcatccccattttataaacaaagaaatctagacttaggaaaatcatgttatttgtctcgtgaccaaattcccaaatcaaggaaataaagaaacctggatttaagccagatttccaagaaaaaatctagggctcttctcactttttcatctttgttccaacatttgaaaaaataaatctaaacacattccaatgtaactgaagagcaggttaattgtttgccacttgcagaatccaattaagaagagagaagtctggtataaagaaagtgatttgcttccaaagctagcttaggggaagaaatgcagcagtcctgccgtactacttcactttaggagcagaaagtggcacttttaaaaggcaacagaggaggcgagcaaggattcaggggtccatgctagcttgggcaccttatccaccaggtagttgagcagttgcctgctggtgcctttgtgagcagggtgttgtcccttgaggcaaatctctggagggtgagagttttgtagtgggcatgctttggtttataaatcacctgtgaactcaggagttccatcttgaagcacatacatagttagatgaacttgccctgcagggagagtctgatgaaagggaggtagatgcttgcaatttaatctataaattaccagataaaattttacaagttgactttaaagtcaaacacatttgaatttagtggaagccattcaagaaaatatcaaagaaaatacagagcaggagaagattaagcaaagagttttttggggaaattggtgtctatgtctgtgtgtgtagggagtgcaggggatatgaatattctatttcagcccatggaaactaggatgtagatcactgtgaacttattcagcaggctacacccaaaggctagaacaaacttctctgccacaggattaacatatgttttaatcgacctggggggcacattctctgataagctcttttggaaagccaggctttctgtggacgtgttatctttccaatgtgtgctggaatgcccggggagaggaaaaagtttcttttacagccatgctcagtgagaagcggagaaacatcttctattcacaaattgctaagtcttttacacatgcaaatatgcatacacattcacacaccacagtgaggaagaaattctcacaccattaataaaatacatttacttcagtagcaatatacatctacattttgcctataatataaaagtatttttcctattaaaagatttgtttaatgtttcttcaccaacaaataaaccctattaaatccccattgccatatgagccctggaggtgaatcagagaaacaaaaggattgtggaaaaatcatcaggttaaaaaaagaaaaattgattctgttttgggatatttcctagcaacatgagctggggaggggatctcagcagtgatgctctatgaagcataataaaatgacacagttacaggtaacttagttaaagggggaaataaatggaagtttcctctttttgaatatcaattgtagcctgctctgctacatttcaaaaacactcttcaaaatgtttaactgaactcactgtaggaagcaccttattaatttattgtgtgttttgaagtcacactgtgagctatagaatttacccaagcacaactcttcctggaaaagagagttcaaatgagaaacagtgcggggtgaagacatggatatgggcctaaaatatctatttctcaatgatattttgatatatctatcaagtgctttttagtggattaggttcagaatgcatcagccaatgcctgttcaataatccagttttccagcatagagcatattaaattgaggaaggacaaagtcacagaggtggggagcaggtggactgtggccaaggactttgcatgaaacagtgagcgtgcatcctcctccttgccctgccctcatggtctgtgtactctcaggaggtcaggacaggcctttctgagaatgagaatctgttcatctgcctttctactggatacttgtcatcggcatacaaacacatgttctctgcagtgtgtcatctttcagaacctcccctgaccctgtattccctagaagtctcgctgctttcagagccaggcttctctcctgctgccacccccactgctcttctagtcactctttaacccactccatctgcatgtggcccccaccacacccctcaaagtggtcaaggttgtcctgttgcttaattccatggaagcttggctatcttcattttattagcctcttttggcctctcaccctgtgaaaatcactacattttgtgccagagatggagctggcatctccaggcttggaagagggctgctgaagctcagccaggtgtcctaaggagcctcaggacaggggatgctcagtagccttgcaatgggaacacagctgagccccacttggccaccctttgccacaaccaggcagaaagcagcttttgaacagatttgttgcctcagatttgatctcaaagaaaaatcgtgggcagtattggtcccaggttctgcttttttacaatttcctctgaaatctggatgcctatcaacaccttggaaaaactgaattctccccaactaatagtggtgtgtcactgtagtaagcctagtacaaaaatggccttctttgtggaggagcttcatatcctccattttttttttgcttaatttttgcccaagatgagaacataatttagttcactttttatttattcccaacatcatccatgcaccaacatttttgtaactaaaggagggaccattcagaagatgcttatcaactgtcaaagtgacagtgttacaaccaatgcacatattgtaagaaatcaaacaatggcctccaaggttcatttctacacagggattagcagatcaacatcaatcttggcaacacagttgccactgatggtgtcttattttttttatcatgacatggcaatcaagagcaaacatgatttattcttatttaagattttatggttagactaggcagatagctagatatgagcaggaggtggaagcccctgagagaatggaggtctggagaatctgaaaccccagagattacccaagtcctgcatgctagacatgagtggaggagggggaatacctaggtagaaaagaatgccccttaagatgcccagcagtcgctcactgtgcagttaacttttcagaatgctgctagatacatgctgatagggagggaagagggcaaaggagaaattcctaagagatacacggttgcagttagtatacatctgagtgctatacaaccttctttgggtggtggcaagaagcaatgcagccattacgtagaattcatatcaaacacctgtatcacaggtgttaaagaaacaagaaacattgtacttcttgtattcttaataatgatttgcaatattgtctttagtatcactgcaaacctctataaatatgatttttaaaaagtatttctttaggttggaattacttctacgcattgacttatcttcctgggtttcattagccgtacccgttgtactttcttccttaccactgtttatctcaaactcttgagattaaagtatgggctcaggagggagcgaggagcttcaggactctcacggacctccagcacagtgtagctgccttatggaaaagtggccacactgttttctgcactggtccctgcccctactattcctcactgggcagagcacagccaccctggccctgcctgaacattttagtcagtgttggctctgtgcttctctggggaggaaatccaagagacaacccacagcccctctgccatttcagctgcagcagtaccaccgttaatgcccttgggcttgagaaagaagggacctggccacttccctgacacctccagcacacagcagggaaagaattccagtttctctttcttgtgagctttcacctgctactcttcaccaggcaaggctcctggcttgggcccacagtgcaggcacctcgaactcagttgaacatttccactggctgcactctgtgtttttgtggggtgaagctcccagaggtgactgaaagtccttctgccactaacactgcagtcatactgcccttgctgtacttggactagggaaggaaaaaagatcctgagtgctttactcacaccccagtgtgccccagccaccctatggaaaagaggccagtgtgtcatccctgcaagcaccctgaggcccctgcccctgctgcccccaagctgtagagccagaatataaagctggcagaaaaatgtaaaaaggctagactggcttagcctcccagcctacatctttctcctgtgctggatccttcctgctcttgaacatcggactccaagttcttcagctgtgggacttggactgtcttccttgctcctcagattgcaggtggcctattatgggaccttgtaatcttgtgagttaataccacttaataagctcccctttgtgtgagtatatctatatctatagatagatataggtatactcactatatatacacatatatacatatactctctctctctctctctcatatatatatatatataatctcctattagttctgtccctctagagaaccccgactaatacagattttcataccagaagtggttcttgaggaacagaatattaaggatggaattctttcattggttttgggacttctggtgttggctgattaatatgattagaccaaaaaatgctaaggactctacttctaatagtatggagaacactgatagtacttggcctgaattgtttagagagttatgcaaaataaatgcatttgacactactgattcatcacttatgagaggcaaggagtttagtgactctatacataatacctttgactatatgtggagaaccaaggaacataatgaagttggttgattgctcctaagttctctggagaaagagatgaaagaaaatgatgatctcaggggatctgtctcccaccttcagaagcagatactgagccacaaatctgctaagattgccctgaatgagagttttaactcctgtagagaaagagttgaaattgtgaaaaaacagagacaagctgttatcatgcgagtagctgatctgcaacaagaggtgcatgcacagccttgccaggtgtttactgttaaagtgagggcattgactggaaaaaaatgggaccctggaacttggagtggggatgtgtgggagaaccctgatgaagctgaggacactgagtttgtgaactctgatgaaacttttttgccagaagaaacagtttccccatccccagtagtggtaacatcccctccctgacccgtgctgccattagcctttccacctttgtctgaggatgtaaaccctgcactgcttgaggcaacagtgatggccttccctgaggcagctgccaggcaagataatgttgattctcctcaagaggcacccctaatgcccctgaatgcttctagacctataactaggctaaattccttgcgggccccagaggtgaggttcagagtgtgacccatgaggaggtgcattatactctaaaagaactgcttaagctttctaatttatattggcagaaatctggagaacaggcatgggaatggatattaagggtaagggataatggtggaagggacatagagttggatcaagctgaatttattggtttggccctactaagtagggattctgcatttaatgttgcagctcggggacttagaaaaggttctgatagggccgggagcagtggctcacgcctgtaatcccagcaccttgggaggcgggggcgggcagatcacgagatcaggagattgagacaattctggctaaaatggtgaaaccccatctctgctaaaaatacaaaaattagctgggcatggtgatgcgtaactgtaatctcatctacttgggaggctgaggcaagagaactgcttgaacctgtgaggcagagattgcagtgagccaagatcgccccactgcattccagcctggtaacagagcaagactccatttccaaaaaaaaaaaaaaaaaagttataatagtttatttgcttggttagctgaaatatggattaaaagatggtccaatgttagtgagctggaaatgccttggtttaatgtagaggaagtgatccaaaggcttagggagattaggatggtggagtggattagtcactttagacctactcatcccagctgggagggtccagaagatacacccttggccgaagctttgtgaaatagatttgtgagagcagcacctgtatttttgaagagcccgtaattgctcttctctgtatgtcagatctaacagtaggaaccacagtcactcaactacaaaatttaaatacaatgggaataattggatcctgaggtggcaggggccaagtgttggcactgaaccatcaaaggcaaggtgggcataactaccataatagacagcagaggcaaagcagccatcagaatagtctgactcatgtagagctctggcattggctaattaatcatggtgttcctagaagtgaaattgatgggaaacctactgtattcctacttgatttatataaacaaaaaactgccaggtagaatggactaaagactaatctgaattataaaaacagagaatcatgggccctcaatcaatttccagactcgaacctgttacagttccagaacccactgaatgaaggggaggctggatccccttgaggaaggacaccactaggctactgacaacttatgctgttactctttctcccatccttccctaaggagacctctggccttttaccagggtaactgtgtgtactggagaaagggaagtaatgagacatttcagaaagtactggacactggctctgagctgacgttgattccagggtacccaaaacgttattgtggttccccagttaaagtaggggcttatggaggttaggtaattaatggagttttagctcatttctgacttacagtggttccagtgggtccctggacttatcctctggtcattttcccagtgccaaaatgcataatttgtatagacatacttattagctggcagaaatgccacattggctccctgactggtaggatgagggctattatggtgggaaaggccaaacagaagccattagagctgtctctacctagaaaaataaaaaaatcaaaaacaatatcccatccctggagggactgaagtgattagtgtcaccatcaaggacttgaaagacgcaggggtggtgattcccaccacatccctgttcaactctcccatttgacctgtgcagaggacagatggatcttggaaaatgatggtggattattttaagcttaaccaagtggtgactccaattgcagctgctctaccagttgtggttttgttgcttgagcaaattaacacatctcctggtgcctggtatgcagccattggcttggcaagtggctttttctccattcctgtccataagacccaccagaagcaatttgccttcagctgacaaggccagcattatacctttaccaccctacctcaggggtgtatcaactctccagctttgtgtcataatcttatttggagagaccttgctcgcttttcacttccacgagatataacactggtccattacattcatgacattatgatgattggatacagtgagcaagaagtagcaaacacactgaacttattggtgagacatttgtatgccagaggatgggaaataaatccagctaaaatttagggactttctacctcggtaaaatttctagggttccagtggcatgagacctatggagatattccttctaaggtgaagcataacttgctgcgtttggcccctcttacaaccaagaaagaggcacaatgcctggtgggcctatttggattttggaggcaacacattcctcgtttgggtgtgttactctggcccatttatcgagtgacctgaaaggctgccagatttaagtgcagtctagaacaaaagaaggctctgaaacaggtccaggctgctgtgaaagctgctctgccatttgggccacatgaccccgcagatccaatggtgcttgaggtgtcagtggcagatagggatgctgtttggagcctttggcaggcccccataggtgaatcacagtggagacctctaggattttggagcaaggccctgccacttctgcagataactactctccttttgagagacagctattggtctgttattgggctttggtggtaactgaacgtttgactgtgggtcataaagtcaccatgctacctgaacctgcctatcatgaactggttgctttctgacccatctagccatgaagtgggtcagcacagcggcatttcatcatcaaattgaagtggtgtgtatgtgatcgggcttgagcaggtcctgaaggcacaagtaagttacataaggaagtggctcaaatgcccatgttctccactcatgccaccctgccttccctcccccagcctgcaccaatggcctcatggggagttccctatgatcagttgacagaggaagggaagactaaggactggttcatagatggttctgcacgatatgcaggcaccacccgaaagtggacagctgcagcactatatccactttctaaatgcatgtgtacacttgtgctaagaaaatatctttattttatttcctttatttttcctttatcatgtgaccttagatttatggacttcacatcagcatttaagcatttaagtgttgttcatatcagcatttaaatattgttaaccttatgtaataacttttggtttggggattggtgcgtttctggttgtatgaggatagttgtattatattaggcataattatgaccttattattgtctttatttgaagattatgtatgatttcaggatgtgtgtatgggttcaagttgacaaggagttggacttgtgatggttaatactgtcaacttgattggattgaaagatgcaaagtattaatctcggttatgtctgtgagggtgtggcaaaaggagattaacatttgagtcagtgggctgggaaggcagacccacccttaatctgggtacacaccatctaatcaagttccagtgtggccagattgtaaagcagggagaaaaatgtgaaaagactagactgaattagcttcccagcctacatctttctcctgtgccaaatgcttcctgctcttgaacatcggactccaagttcttcagcgttgggagttggactggctttcttgctcctcagcttgcagagggcctgttgtggaaccttgtgatccgctgagttaatactacttaataagatcccctttatatacatataatatattatattatatataatatatataatatatattatatataatatatataatatattatatattatatataatatatattatatattatatataatatatattatatataatatatattatatattatatattatatataatatatattatatataatatatataaaatatatatatatcctattagttctgtccctctagagaaccctgactaatacaatttatgtcattaatctcatttattgatttgtatacattgaaccaaccttatatcccaggaataaaacctacttgattgtggtggattagctttttgatgtactcttggattcaattgctggtattttattgagaatttttgcatctgtgttcatcaaggatattggcttgaagttttctttttttgttgttccatatcagaatgatgacgacctcatagaatgagttagtctgtcctcttttatcttttggaattgtttcaggaggcttgatatcagctcttctttatatgactggtatactttggctaggaatctctctggtccaggggtttttctggtgtaggtttttaattactgattcaacttcagaactcattactcattattgagttctaaaactcactttcatgtactcttcaaaagactgtcttcttctgttgttgagcggggtgttctctcaaggtcgtttaggtgaaggtggttgctggtgttcttctgtatccttactgcttgtctttctctttttttattgactactgaggattaatggtgatgtgtccaactttaactctagattagtctatttctcttttagattgtaactctgttttatatattttgaagctctgttgttaggcatgtgtatttggattgttaggtcttcttgatgatgacctttatcattatgtaatgtttcttcttatctctggaagtattcgttgttctgaagtctatttgtgctgatatgaatacagccttcacagctctattttcactagtatttgtatatctttttctcagcttttaaattgagatgttcagaccatttgcattaaagtagttgttaataggattaaatttaaatctaccattaagttggttatttctctttgtcccatttaaactttgttccttttttcatatttttctgccttcatttatattgagtttatctccacgacttacttattaaattaatttttaatggttttagtattttccacaatgtttataatatatactttgattttttcacattccaccttcaaatgacagaattatactggatatatagaaatcttacatcattgcacttctccttcctccctctcaaaatgttgtgctattgctctttgtaatagaggcttacttctattatgttatagctctcataatacattgacactatttttaccctgaataatcagttgttttttaaagtgattatgactacaaatattttgaataatttctttattttaccatttctggtgctccttatcttttacagtagatcccaatttccatctggagtcacattctttctgtgaaaaacaacctttagcatttcttatagcacgggactgctgttgctgttgtctttcagcttttctttgtctgaagaagtctttattttgccttcagtttttaaaagtgattttgctgagtatagatactgggttgagagtttcattccttgtatcattttaacaatgatgttccattatattccgttttgaatagtttctgactagaaatctgatctttgtttctttgtattcaatagttcctttttctctgactgcctttaagatattctcatctttgtttttcaacagtttgactataatttgtttattattaactttttgtatttattctgcttgaggtttcctgagctccttggatttgcagattgttgatttttattgtttttgtaaaattcatagccattatctattctactgttttgttttttttttcacttctctctctctgtattcttctttttggactgtaagtattcaaatgttagatcattcatattgcttcataaaccttatatgcttcttctgcttttttttttttgtcaggaactctttttttgtatctgtgttggtttggataagttctagtagactatgttcaagtttatggattattttgttagttgtgtctaattgactcctcagtgcattcagagaattcttcatctctgatattataaatctcttcctagcattttcatgttactcttttctatagtttccatctctttgctgaaattctccccctatccatggatattgtccacctttaccacaagattctttaacatattaacataggtatcatacaaacccaaactgatagtttccagatggtgtcttttctgagtctgtctgtcttgattgctttattatttaacagtgacttatcttccctcttcagcttttggtgtgtcttgtaattgtttaatcaaacactgggtatcataaatggaggaacagtagagattgcagtaaatattatttatgctttgaaatgggcacccatcttctgttgaaaatatgttttgtggtcaattgagtcaacctagtaactggttgaactgaatttggcatttgtgcttgttgcttttatcttaaatgcaccacaggtttaaattcctccagtgatgggttgctgctatcttttgcttagagtggggcctggggtgtggaagaattttctcagtgttcctatctattattagattttagcagtcactgcatgcctgcactacagaggggatatcttcatacacataatctaaccccattgaaactgctgtttcttcttaatgaatgctcaatctttggtggaaataaacaaatgctgtatctcctggagccacttcagtcttagtcaggttctgcagggctttgaagggaatgcattctcagtattcttgtgccttatttggatggaacttgaacctgtggtgggtttggagagaaagagtagcagacgtctgctatgttgcaatgcaggatgctgggcacaagaaaatttccagtctctcctccaaggaaataagatttgatcatctacctatccctgagaagtgaagggctttgcctgcggtgctagatgcaaaaccatttttctccccccattgcccagaaacttaaggctttggcttttctgagcagtggtctagggaattgtgcaaggttttcatatttgaccctgacagcccatcaccacctacagcttgcagtgccaaatgtatctccctctgatctctcctgtcctgtggtcctcatgaacattaagaagagatttctaaaaaagagcttgcacatgagcatagtttctggtgagaagaattctgatatgttaacttcctctaaacttttaaataaaatatttctaagaattaaataaagttctagaatgatatgaatctattcctttggttttttgcacgtctgtctgcctgctaatcaagagaagagaatggtcgtaattctcagagactttttcctgtttgtgtcataaatgacttcacatttttttctgttctaagaactattcagcttgatttcttctgttttaattttagcagcacctgagcaaagccatgtggtccaggattgctaccatggtgatggacagagttatcgaggcacgtactccaccactgtcacaggaaggacctgccaagcttggtcatctatgacaccacatcaacataataggaccacagaaaactacccaaatgcgtatgtcattaatcttacagtaagcaaaacaaggtccaagtaaaatttgtcttagaaaaggtgtgcgtcaagctaacttcttatgattaaatttttctcacacatagaatgcatggcaaaatgtctgagaaacattactttgagcaaagagtatgatagaagagaaatgttaagctggctctctttcctgagagtttgataaaatcaggagaatatctggcggtggtgaggccacaataatggaaaatcagaatgtttagacagagtcagcttcaacaacactcactaaaggtcaatgtgatctttaccccttgaaattctataattctaatctccaattcctgaagtgaaggttgtgttggccttttctgtcttggctcacaagtaaatgatatgtgcatatctatggaaaggcgaatctatctttttctatatctatgtctattccaacgggtagaaacaccctgggtcctgagcaccagtggtctgaaggaatacgggttgccaggaagagagaagcaaaggcaggaaggcagatgaaagtaagaaatgagacagatgctaaacaataaaaagtgcgggaagatagacagaagctggggtctgaccacaccatggccagtctttcacacataagtgactaccaaagacaagaaaaaatgatttccgcttgttggacaatagatggtagaggaccaagggaattgcgagagagagaacaatgagatcaactcaacagatgcactggttttcttcctggagacccttcctgcactgaagggcaggagatggagcccaaaaaaaactgtagccatcttgctgaacagaggagggacattggagtttgggattattcaggtggctaggattttctaggcctgctaacaatgagaacagatttgtggaggaaaggagttctagaaatatgcatagaaatctcctcgagtcattggctaaacatgaagctgcatgtacacagaaaatagatccacaagaaagtagggcaaagaacatctacggaagagcagcaactacaatggaacagtgagctcaataaacatgacagagctcaaatagcactaagggatattggagtttggaccacacagaggagagagacttcactgaacatcttgggcattcagtagagacccaggaaaagccatactttaggagtagaattagtatattcttagaataaaggcagctccacacaaacaatagcaaaactgaaaaggaagtctccaagcatcagaatgatgtccaagtcaatgaactgcctctgagaggaaaactcaaccatctttagaggtaaacatcaaagtcaagtggctcagctatgcagtatccacagtgtgaggcctaaatataaaacttgactacacatagaaaccttttagtgtgacccacaagcaggaggaaaatcagccaatacaaacagacccagaagagacagaaatgattagaatggcataaaaatttgacatatcactatataataattgagttctaggatttaagaaaacatgaatatagaatgcaacagacaccttatccagagacagtaagagtataaagagccaaatcgaagaactactaagagatatgtcttaaatgaaaaaattactagatggcctccccatctagttagacatttcagaagaaaataccaaatgaaaaataattgcatagaacctacagaaccagatacacacatacaaaacacacgcatgcatacacacacactcaaacatgtataagcttacaaacacacacacacatccacaaatgctgaaaaatgaaatcaaccgagccacacagacataaaggaaaacataaaaagatttcctacatgtgggaagcaagtcacagaaagggggaaggagattggaacagaaatatatactgaaagcaaggatggctgaaaattttccaaatataaagaagattaaaaaatcacggactcaagaagctcaatggatcagaaaaataatttctaaaatgacaattataggatgccactgggtacatagcagttcaactgtcagagggcaaagacataatacacagaaaaatctcgtaaggaacgggaaaaacaaaaagctgtgtcttgctagaggaacagtgatacaagtgactaatgtgttcccatcagaaacactgcaacctggacacaaaagaataacattaaagtaataaacgtaagaaagaagagctcaactgagaaggctacatccagcaataaaatgccttgaagttcatccatgttggaggaatgcacattgtgcactcccctaaacaaagaaaccggaaactgtaagactttggaatcagcaggcttatgtaacaaaagaggtgaccctaaggaattaaggagaagaagaatagaacaagaagggaactttctgcagcctatataatgaagaacctagcaattggcaaatgtagatgaaaatgctacatgttttcttgatcaaacgtttatatctttttaaatgagagttgacgagttgaagcaaaatgataccaatatatttaactttaccatatgtagaagtaaaaatttgaacatgtagcataaatcatgtagggattaattggaagtgtaccactgtaagtttcttacctcatgcacgatagtatgtaatactaataaaaggttaatgtgtgggttcaaagggatattgcaaatcctagagcaatcacaaagtttttaactctgaggtttgttgtataataacaatattttatgtattcaaaagagggaagccaaggaagaaaaaaaagtctttaaagagctctggctcttagtacatccagttgctcattgaatgagcttcctggaatggagggtctgggactgagactaggccacatgtgtagagccactagagacacaatgttggatccccatggcccataatacatttcccattttctcaggcagccacaggtcatgaatgtgaggatactgagaggttggagcaacgttcttgggaggcataaggaagagcgaatgcttcaagatccccgcagcccaaactcctcagctgctttgcctcctaattcattgttttttgctcctccatagctgtccgacctcttcagatctcttagtcttcctgccatcttcctttatgccatgggacccactgttctttcaactcatcccccagttctggagtggctgtggacagcagaggatagactgagagcaggagagaaggtcctgcccaggaacccattctagagatactgcattctgcctgggagcaagttttccagggcagctttgagaagtcttgcagaaacaaacctacttgaccgacatgatatgggaatgacagacagtaatactatttgcacaatgcttttccatgggaaaggtagagccttttcactaggttttgagtacatggagtgtgagagttgacctggaaaggttatcctccttgatgccatgttttctctgaagaactacatgttcgttgcaactcccacattagaatatgaagtcctaccgagagagatacggagactagacagatacagatgcatttgcatgtgaatacacaatcccacaatacagacgtcaaaacccataccagttattccagagagatggattgggcagaaggcagaaggagaatactctgatcgtttttcggccacgtgtgtgtgttatctcagtgtttctaagaagcgtttgctactttagattttttatttaaaaaaaatagtaataatctattaagtatgagagatgtgcagagaggattagtgatcgagagccatttttgctggtggcaatcatatggtacttttaatgggaatattagaaaggcaccggtaatgaccttgttgcagcacaaaggagagagtgtggggtgcccctgcatgttgtcccacctcttgtgacgtgtatcgttttggaatttccagtggcttgatcatgaactactgcaggaatccagatgctgtggcagctccttattgttatacgagggatcccggtgtcaggtgggagtactgcaacctgacgcaatgctcagacgcagaagggactgccgtcgcgcctccgactgttaccccggttccaagcctagaggctccttccgaacaaggtaaggagtctgtggccagacatctacacgcttcgatgctgggatgaaaagccatggaaattcccactgatgcagccgccttcaatggtaaacggatgctcgagtgttgcctgagttctaccatgtaggaggaagcctccgtgcactctctgggggagccagcggagtgatttctggtgcaacgtggttgggctttgtctttaggatgggcacaaaccctccagggggatcgacttcaaaattcaccttgttgtaaaacgggctacctcagtgtcccagccaaaatttttattgtaacatgctgtcaggtgtgtcactctttccaagccagtaagcttttccggggatttcttcaagtagccagcattcagagcaatcttcagcattgcagattctgagaaatgtggctctggagcctgtcaccctcgagaaacctaagagggctgcattgattccatgtggccctgggtctatggagcagtacatgagctcccagtgctctaaggctcttcagccctaggctttgaagggagtgatttctcagtattcttaaacctctttctgatgacacttgtacctgtgaggggtctagagagaaagagtagtagactcctactttactacaattcaggatgcagggcatgagaggattccctctctcctccaagggaagaagcttttggcgtgcacacatccctgagaagcaaagtgtctttgtcttcagtcagatacataggaccgttttctgccccatggcccggaagccaaaggccttggctttcatgatcaacggtctagggaaacatgcaaaatttccatgtctgtcccaaactctgcccccgacagccaattaccacctgcagcccgcattgccaaatgcggtgccgtttgcatgaagattcagtagagtttcctagaaaggtgctacctcgtgagctcactttccaatgaggaatctgatctgttgtgtttctctaaggtgtcaggtgaaatatttccaagaacttactacagttctagaatgggaggaatctgttgctttggtgtttgtttgttggtcggttttctcacatccatctgcctatggataaggaaaagagaacggtcgtaattctcatagactcctttctggttgtgtcacaaatggcttcacatgtttctctatgctcagagatactcagcttgatttcccgtgttttcatttcagcaccgactgagcaaaggcctggggtgcaggagtgctaccatggtaatggacagagttatcgaggcacatactccaccactgtcacaggaagaacctgccaagcttggtcatctatgacaccacactcgcatagtcggaccccagaatactacccaaatgcgtatgtctttgttctttaccataagagaagaaagggccaagtgaagtttctgttacaagagatgtgtctcaagctgagttctccgaactcaacttgtgacagatgcagatggcgtagcaaaatgtctcaggatgattgccttggagctaagggtctgagagaagggaaatgttaagctccctctccttcctcctagttctattgagcagaagggaaatctggaggtgaggagatcacattatgaagaaagtcagaatgacaaaggaccagacacttagattacccttccacaacaccaactaaacgtcaatggagactttccagttggaattccgttattctggcttccacttcctgaagggaaggttgcgtttgccttttctctctgggttcaagaggaaagaataggtgcttatttatggacaggtgaattgatctgtttctatatctacgtatattccgattgtcagaaaaacactcgttcctaagtaccagtggcctgaagggatacaggttcccagcaagagaagatccaaggaaggaaggcagatgagagtcagcacagagagggatgctgaaaagtaaaagggatgggtggatggagagaagcccgggtctgaccacccaatggccaatattttggccacaagcgactaccagagacatggaaaaatggtttctacatgtgggacaacagatggtagaggacctagagaattgagagaggggcaatgatgggctccactccgcagatgccttggctttcttcctggatacccttcctgcactgaatagcaaggagatggagcccaagcagactgtagccatcttgctgaatggaggagagggattggagtttgggatgactgtggtagctgaaatttttctaggtctgctagaaataagaactggtttgtgtggaggaaaagagctctacaaatacgcatagaagtctcctccagtcgttggcctgacatgacgctgcctgtgcacaggaaatggttccacgagaaagtgtggcaaagaacatttactgagaaacagcaagtacaagagcacaggaagctcaataaagaagagagagatcacatagcactctgggatactggagttcttcccagctagaccagagagtcctcacggagcacattgccaattcagtggagaccccagaacagccgtaatttaaaggtacacttagtatattactagaataaagtcagctgcagacaaccccttgcacagctggaaagcaagtgtccaagcatcaaatcggtttccaatcaatgaagtgcctgtgagaggaaatctcaactctctttagaagtaaacaacaaagtcgattgcctcagctatgcggtatccgcagagtgagtcctaaatttaaaatctgactacatgtagaaaagcgtttcgtgtgacccatgaccaggaaataaatcgggtaatacaaacaggctcaggaatgagagaaatgattagaattgcgtgaaaatttgacatatcagtatgataactgatttcaaatatttaaaaaaacaacatgcaagaaagcagatatcatatcaagagaaattaacagtacagaatagccaaattaaattaaagaggtagtataaaaaaagtatgtcttaattgaaaaaaattactgtatggccggctgatcaatttagacgtttcagaggaaaacattacccaacacacaattctagagaacctacagaatgagctacacacacacacacacacacacacacacacactgaaaacacacccatactcacacacacgcagaaactcacaagttctaacacacacagacacgcgcacccctgaagaaacagtgaaatataaaattaagcgagcctcacagacatgtaggaaaatatgaaaagatttcctgcatgtgggaagcaagtcacagtaaagagcaagggagtttataatagaaacaaataccagaatcaaggatggctgataacttttcaattacgaagaacattaaaaaaaatcacagaatcgtgaaactcaagggatcatatagggaatttcggaaaaaaaacccaacctgtatgatgtacttttgtacatcacagttcgaaggtaacaaggcaaagatgtaataagaagaaacctgtcacgagaaactggaggaaaaagagctgtgtcttcctacaagtacactgatacaaattgccaatgtgttcacctcagaaacactggaagccagataccagggaatattgttaaaatgataatcaggaacaaaaagagatcaaccgggaatgctgaatccagcaataaaatgccttgaaggtcatccatgtcggataaatgcatattgtgcactgccccaaagaaagaaaccggaaactgtaagaattggaaatcagcaggcttatgtaacaagagaggtgacccgaaggaattaggtagaagaagaattgaacaagaaaggaactttctgcagcccacgtaatgaagaatccagcaattggcaaatgtagatagatgtaaatgcaaaatattttcttgatcaaatttctatatctttgtaaatgagagttgactacttgaaacaaaatgatagcaagatatttaacttcagcatatgtagaggtaagaatttgaaatggtagcataaatcacgaagggattaattcgaagtgtaccgttgtaagtttctttacctcatgcacgatggtgtgtcatattaataaaagggtactgtgcgggttcgaagggatattgcaaatcctagagcaatcacaaaggtttgaactctgaggtttttggtataataagaatagtccatgcattcaaaagagggaagccaaggaagaactagaagtctttcaagagctcaggctcttatacatccagttgctcattgaaccagcttcctggaatggagggtctggggttgagactaggccacaagtctagagtctctagagagacagtgttggaaccccatggcccataatacatttcccattttctcaggcagccagaggtcatgaatgtgaggatactgggaggttggagcaacgttcttgggaggcataaggaagagcgaatgcttcaagatccccgcagcccaaactactcgcctgctttgccccctaatgcatttttctctgctgctccgtagctgtccgacctcttcagatctcttagtccaccctgccgtcttcctttatgccatgggtcccactgttctttcaactcatccccctttccctcagtcccggagtagctgcggccagcagagggtagactgagagcaggagagaaggacctgcctaggaaccccttctagagatactgcatcctgcctgggagcaagttttccagggcagctttgagaagtcttggagaaacaaacctactaaacctgacagacagtaatactatttgcacaatgcttttctgtgggaaaggtagagccttttcactacgtattgagtacatagagtgtgagggttgacctggaacggctatcctcctggatgacgtgtgttttctgaagaactacatgttcgttgcaactcccacattagaatatgaagtcctaccgagagagatacggagactagacagatacagatgcatttgcatgtgaatacacaatcccacaatacagacgtcaaaacccataccagttattccagagagatggattgggcagaaggcagaaggagaatactctgatcgtttttcggccacgtgtgtgtgttatctcagtgtttctaagaagcgtttgctactttagattttttatttaaaaaaatagtaataatctattaagtatgagagatgtgcagagaggattagtgatcgagagccatttttgctggtggcaatcatatggtacttttaatgggaatattagaaaggcaccggtaatgaccttgttgcagcacaaaggagagagtgtggggtgcccctgcatgttgtcccacctcttgtgacgtgtatcgttttggaatttccagtggcttgatcatgaactactgcaggaatccagatgctgtggcagctccttattgttatacgagggatcccggtgtcaggtgggagtactgcaacctgacgcaatgctcagacgcagaagggactgccgtcgcgcctccgactgttaccccggttccaagcctagaggctccttccgaacaaggtaaggagtctgtggccagacatctacacgcttcgatgctgggatgaaaagccatggaaattcccactgatgcagccgccttcaatggtaaacggatgctcgagtgttgcctgagttctaccatgtaggaggaagcctccgtgcactctctgggggagccagcggagtgatttctggtgcaacgtggttgggctttgtctttaggatgggcacaaaccctccagggggatcgacttcaaaattcaccttgttgtaaaacgggctacctcagtgtcccagccaaaatttttattgtaacatgctgtcaggtgtgtcactctttccaagccagtaagcttttccggggatttcttcaagtagccagcattcagagcaatcttcagcattgcagattctgagaaatgtggctctggagcctgtcaccctcgagaaacctaagagggctgcattgattccatgtggccctgggtctatggagcagtacatgagctcccagtgctctaaggctcttcagccctaggctttgaagggagtgatttctcagtattcttaaacctctttctgatgacacttgtacctgtgaggggtctagagagaaagagtagtagactcctactttactacaattcaggatgcagggcatgagaggattccctctctcctccaagggaagaagcttttggcgtgcacacatccctgagaagcaaagtgtctttgtcttcagtcagatacataggaccgttttctgccccatggcccggaagccaaaggccttggctttcatgatcaacggtctagggaaacatgcaaaatttccatgtctgtcccaaactctgcccccgacagccaattaccacctgcagcccgcattgccaaatgcggtgccgtttgcatgaagattcagtagagtttcctagaaaggtgctacctcgtgagctcactttccaatgaggaatctgatctgttgtgtttctctaaggtgtcaggtgaaatatttccaagaacttactacagttctagaatgggaggaatctgttgctttggtgtttgtttgttggtcggttttctcacatccatctgcctatggataaggaaaagagaacggtcgtaattctcatagactcctttctggttgtgtcacaaatggcttcacatgtttctctatgctcagagatactcagcttgatttcccgtgttttcatttcagcaccgactgagcaaaggcctggggtgcaggagtgctaccatggtaatggacagagttatcgaggcacatactccaccactgtcacaggaagaacctgccaagcttggtcatctatgacaccacactcgcatagtcggaccccagaatactacccaaatgcgtatgtctttgttctttaccataagagaagaaagggccaagtgaagtttctgttacaagagatgtgtctcaagctgagttctccgaactcaacttgtgacagatgcagatggcgtagcaaaatgtctcaggatgattgccttggagctaagggtctgagagaagggaaatgttaagctccctctccttcctcctagttctattgagcagaagggaaatctggaggtgaggagatcacattatgaagaaagtcagaatgacaaaggaccagacacttagattacccttccacaacaccaactaaacgtcaatggagactttccagttggaattccgttattctggcttccacttcctgaagggaaggttgcgtttgccttttctctctgggttcaagaggaaagaataggtgcttatttatggacaggtgaattgatctgtttctatatctacgtatattccgattgtcagaaaaacactcgttcctaagtaccagtggcctgaagggatacaggttcccagcaagagaagatccaaggaaggaaggcagatgagagtcagcacagagagggatgctgaaaagtaaaagggatgggtggatggagagaagcccgggtctgaccacccaatggccaatattttggccacaagcgactaccagagacatggaaaaatggtttctacatgtgggacaacagatggtagaggacctagagaattgagagaggggcaatgatgggctccactccgcagatgccttggctttcttcctggatacccttcctgcactgaatagcaaggagatggagcccaagcagactgtagccatcttgctgaatggaggagagggattggagtttgggatgactgtggtagctgaaatttttctaggtctgctagaaataagaactggtttgtggaggaaaagagctctacaaatacgcatagaagtctcctccagtcgttggcctgacatgacgctgcctgtgcacaggaaatggttccacgagaaagtgtggcaaagaacatttactgagaaacagcaagtacaagagcacaggaagctcaataaagaagagagagatcacatagcactctgggatactggagttcttcccagctagaccagagagtcctcacggagcacattgccaattcagtggagaccccagaacagccgtaatttaaaggtacacttagtatattactagaataaagtcagctgcagacaaccccttgcacagctggaaagcaagtgtccaagcatcaaatcggtttccaatcaatgaagtgcctgtgagaggaaatctcaactctctttagaagtaaacaacaaagtcgattgcctcagctatgcggtatccgcagagtgagtcctaaatttaaaatctgactacatgtagaaaagcgtttcgtgtgacccatgaccaggaaataaatcgggtaatacaaacaggctcaggaatgagagaaatgattagaattgcgtgaaaatttgacatatcagtatgataactgatttcaaatatttaaaaaaacaacatgcaagaaagcagatatcatatcaagagaaattaacagtacagaatagccaaattaaattaaagagctagtataaaaaaagtatgtcttaattgaaaaaaattactgtatggccggctgatcaatttagacgtttcagaggaaaacattacccaacacacaattctagagaacctacagaatgagctacacacacacacacacacacacacacaaactgaaaacacacccatactcacacacacgcagaaactcacaagttctaacacacacagacacgcgcacccctgaagaaacagtgaaatataaaattaagcgagcctcacagacatgtaggaaaatatgaaaagatttcctgcatgtgggaagcaagtcacagtaaagagcaagggagtttggaatagaaacaaataccggaatcaaggatggctgataacttttcaattacgaagaacattaaaaaaaatcacagaatcgtgaaactcaagggatcacatagggaatttcggaaaaaaaacccaacctgtatgatgtacttttgtacatcacagttcgaaggtaacaaggcaaagatataataagaagaaacctgtcacgagaaactggaggaaaaagagctgtgtcttcctacaagtacactgatacaaattgccaatgtgttcacctcagaaacactggaagccagataccagggaatattgttaaaatgataatcaggaacaaaaagagatcaaccgggaatgctgaatccagcaataaaatgccttgaagatcatccatgtcggataaatgcatattgtgcactgccccaaagaaagaaaccggaaactgtaagaattggaaatcagcaggcttatgtaacaagagaggtgacccgaaggaattaggtagaagaagaattgaacaagaaaggaactttctgcagcccacgtaatgaagaatccagcaattggcaaatgtagatagatgtaaatgcaaaatattttcttgatcaaatttctatatctttgtaaatgagagttgactacttgaaacaaaatgatagcaagatatttaacttcagcatatgtagaggtaagaatttgaaatggtagcataaatcacgaagggattaattcgaagtgtaccgttgtaagtttctttacctcatgcacgatggtgtgtcatattaataaaagggtactgtgcgggttcgaagggatattgcaaatcctagagcaatcacaaaggtttgaactctgaggtttttggtataataagaatagtccatgcattcaaaagagggaagccaaggaagaactagaagtctttcaagagctcaggctcttatacatccagttgctcattgaaccagcttcctggaatggagggtctggggttgagactaggccacaagtctagagtctctagagagacagtgttggaaccccatggcccataatacatttcccattttctcaggcagccagaggtcatgaatgtgaggatactgggaggttggagcaacgttcttgggaggcataaggaagagcgaatgcttcaagatccccgcagcccaaactactcgcctgctttgccccctaatgcatttttctctgctgctccgtagctgtccgacctcttcagatctcttagtccaccctgccgtcttcctttatgccatgggtcccactgttctttcaactcatccccctttccctcagtcccggagtagctgcggccagcagagggtagactgagagcaggagagaaggacctgcctaggaaccccttctagagatactgcatcctgcctgggagcaagttttccagggcagctttgagaagtcttggagaaacaaacctactaaacctgacagacagtaatactatttgcacaatgcttttctgtgggaaaggtagagccttttcactacgtattgagtacatagagtgtgagggttgacctggaacggctatcctcctggatgacgtgtgttttctgaagaactacatgttcgttgcaactcccacattagaatatgaagtcctaccgagagagatacggagactagacagatacagatgcatttgcatgtgaatacacaatcccacaatacagacgtcaaaacccataccagttattccagagagatggattgggtaggaggcagaaggagaatactctgatcgtttttcggccacgtgtgtgtgttatctcagtgtttctaagaagcgtttgctactttagattttttatttaaaaaaaatagtaataatctattaagtatgagagatgtgcagagaggattagtgatcgagagccatttttgctggtggcaatcatatggtacttttaatgggaatattagaaaggcaccggtaatgaccttgttgcagcacaaaggagagagtgtggggtgcccctgcatgttgtcccacctcttgtgacgtgtatcgttttggaatttccagtggcttgatcatgaactactgcaggaatccagatgctgtggcagctccttattgttatacgagggatcccggtgtcaggtgggagtactgcaacctgacgcaatgctcagacgcagaagggactgccgtcgcgcctccgactgttaccccggttccaagcctagaggctccttccgaacaaggtaaggagtctgtggccagacatctacacgcttcgatgctgggatgaaaagccatggaaattcccactgatgcagccgccttcaatggtaaacggatgctcgagtgttgccggagttctgccatgttgggggaagcctccgtgtactctctgggggagccagcggagtgatttctggtgcaacttgggtgggctttgtctttagaatgggcacaaaccttccagggtgatgggcttcacaactcacctccttctaaaatgggctatctcagtgtcttagccaaaatttttattgtaacgtgctgtcaggtgtgtgattctttctgtcgcagtaagcttttctggggatttcttcaagtagccagcagtcagtgcaatcttcagcattgcagatttcaaaaaatgtggctctggagcctgtcatcctcgagaaacctaacagggctgcattaattccatatggtcctgggtctatggagcagtatatgagctcccaatgctctaaggctcttcagtcctaggctttgaagggagtgatttctcagtgttcttaaacctctttctgatggcacttgtacctgtgaggggtctagagagaaaggttagtagacttctcctttactgcaattcaggatgcagggcatgagaagattccctccctcctccaagggaagaaggttttggcgtgcacacatccttgagaagcaaagtgtctttgccttcagtcagatatataggatcgttttctgccccatggcctggaagccagaggccttggctttcatgatcaacgatctagggaaacatgcaaaatttccatgtctttcccctcctctgccctcgacagccaattaccacctgcatcctgcattgccaaatgcagtgccctttgtatgaacattcagtagagtttcatagaaaggtgctacttcgtgagcgcactttgcagtgagaaggagtctgttctgttctgtttttctaaggatttcaggtgaaatatttcctagaacttactacagttctagattggtaggaatctgtaggtttgctgtatgttttttggttggttttctcccatccatctgcctacaggtaagggaaagataacgttcgtaattctcatagactcctttctggttgtgtcataaatggcttcacatatttcgttattctcagagatactcagtttatttcttgtgttttcatttcagcaccgactgagcagaggcctggggtgcaggagtgctaccacggtaatggacagagttatcgaggcacatactccaccactgtcactggaagaacctgccaagcttggtcatctatgacaccacactcgcatagtcggaccccagaatactacccaaatgcgtatgtctttgttctttaccataagagaagaaagggccaagtgaagtttctgttacaagagatgtgtctcaagctgagttctccgaactcaacttgtgacagatgcagatggcgtagcaaaatgtctcaggatgattgccttggagctaagggtctgagagaagggaaatgttaagctccctctccttcctcctagttctattgagcagaagggaaatctggaggtgaggagatcacattatgaagaaagtcagaatgacaaaggaccagacacttagattacccttccacaacaccaactaaacgtcaatggagactttccagttggaattccgttattctggcttccacttcctgaagggaaggttgcgtttgccttttctctctgggttcaagaggaaagaataggtgcttatttatggacaggtgaattgatctgtttctatatctacgtatattccgattgtcagaaaaacactcgttcctaagtaccagtggcctgaagggatacaggttcccagcaagagaagatccaaggaaggaaggcagatgagagccagcacagagagggatgctgaaaagtaaaagggatgggtggatggagagaagcccgggtctgaccacccaatggccaatattttggccacaagcgactaccagagacatggaaaaatggtttctacatgtgggacaacagatggtagaggacctagagaattgagagaggggcaatgatgggctccactccgcagatgccttggctttcttcctggatacccttcctgcactgaatagcaaggagatggagcccaagcagactgtagccatcttgctgaatggaggagagggattggagtttgggatgactgtggtagctgaaatttttctaggtctgctagaaataagaactggtttgtggaggaaaagagctctacaaatacgcatagaagtctcctccagtcgttggcctgacatgacgctgcctgtgcacaggaaatggttccacgagaaagtgtggcaaagaacatttactgagaaacagcaagtacaagagcacaggaagctcaataaagaagagagagatcacatagcactctgggatactggagttcttcccagctagaccagagagtcctcacggagcacattgccaattcagtggagaccccagaacagccgtaatttaaaggtacacttagtatattactagaataaagtcagctgcagacaaccccttgcacagctggaaagcaagtgtccaagcatcaaatcggtttccaatcaatgaagtgcctgtgggaggaaatctcaactctctttagaagtaaacaacaaagtcgattgcctcagctatgcggtatccgcagagtgagtcctaaatttaaaatctgactacatgtagaaaagcgtttcgtgtgacccatgaccaggaaataaatcgggtaatacaaacaggctcaggaatgagagaaatgattagaattgcgtgaaaatttgacatatcagtatgataactgatttcaaatatttaaaaaaacaacatgcaagaaagcagatatcatatcaagagaaattaacagtacagaatagccaaattaaattaaagagctagtataaaaaaagtatgtcttaattgaaaaaaattactgtatggccggctgatcaaattagacgtttcagaggaaaacattacccaacacacaattctagagaacctacagaatgagctacacacacacacacacacacacacacacacactgaaaacacacccatactcacacacacgcagaaactcacaagttctaacacacacagacacgcgcacccctgaagaaacagtgaaatataaaattaagcgagcctcacagacatgtaggaaaatatgaaaagatttcctgcatgtgggaagcaagtcacagtaaagagcaagggagtttggaatagaaacaaataccggaatcaaggatggctgataacttttcaattacgaagaacattaaaaaaaatcacagaatcgtgaaactcaagggatcatatagggaatttcggaaaaaaaacccaacctgtatgatgtacttttgtacatcacagttcgaaggtaacaaggcaaagatataataagaagaaacctgtcacgagaaactggaggaaaaagagctgtgtcttcctacaagtacactgatacaaattgccaatgtgttcacctcagaaacactggaagccagataccagggaatattgttaaaatgataatcaggaacaaaaagagatcaaccgggaatgctgaatccagcaataaaatgccttgaagatcatccatgtcggataaatgcatattgtgcactgccccaaagaaagaaaccggaaactgtcagaattggaaatcagcaggcttatgtaacaagagaggtgacccgaaggaattaggtagaagaagaattgaacaagaaaggaactttctgcagcccacgtaatgaagaatccagcaattggcaaatgtagatagatgtaaatgcaaaatattttcttgatcaaatttctatatctttgtaaatgagagttgactacttgaaacaaaatgatagcaagatatttaacttcagcatatgtagaggtaagaatttgaaatggtagcataaatcacgaagggattaattcgaagtgtaccgttgtaagtttctttacctcatgcacgatggtgtgtcatattaataaaagggtactgtgcgggttcgaagggatattgcaaatcctagagcaatcacaaaggtttgaactctgaggtttttggtataataagaatagtccatgcattcaaaagagggaagccaaggaagaactagaagtctttcaagagctcaggctcttatacatccagttgctcattgaaccagcttcctggaatggagggtctggggttgagactaggccacaagtctagagtctctagagagacagtgttggaaccccatggcccataatacatttcccattttctcaggcagccagaggtcatgaatgtgaggatactgggaggttggagcaacgttcttgggaggcataaggaagagcgaatgcttcaagatccccgcagcccaaactactcgcctgctttgccccctaatgcatttttctctgctgctccgtagctgtccgacctcttcagatctcttagtccaccctgccgtcttcctttatgccatgggtcccattgttctttcaactcatccccctttccctcagtcccggagtagctgcggccagcagagggtagactgagagcaggagagaaggacctgcctaggaaccccttctagagatactgcatcctgcctgggagcaagttttccagggcagctttgagaagtcttggagaaacaaacctactaaacctgacagacagtaatactatttgcacaatgcttttctgtgggaaaggtagagccttttcactacgtattgagtacatagagtgtgagggttgacctggaacggctatcctcctggatgacgtgcgttttctgaagaactacatgttcgttgcaactcccacattagaatatgaagtcctaccgagagagatacggagactagacagatacagatgcatttgcatgtgaatacacaatcccacaatacagacgtcaaaacccataccagttattccagagagatggattgggcagaaggcagaaggagaatactctgatcgtttttcggccacgtgtgtgtgttatctcagtgtttctaagaagcgtttgctactttagattttttatttaaaaaaaatagtaataatctattaagtatgagagatgtgcagagaggattagtgatcgagagccatttttgctggtggcaatcatatggtacttttaatgggaatattagaaaggcaccggtaatgaccttgttgcagcacaaaggagagagtgtggggtgcccctgcatgttgtcccacctcttgtgacgtgtatcgttttggaatttccagtggcttgatcatgaactactgcaggaatccagatgctgtggcagctccttattgttatacgagggatcccggtgtcaggtgggagtactgcaacctgacgcaatgctcagacgcagaagggactgccgtcgcgcctccgactgttaccccggttccaagcctagaggctccttccgaacaaggtaaggagtctgtggccagacatctacacgcttcgatgctgggatgaaaagccatggaaattcccactgatgcagccgccttcaatggtaaacggatgctcgagtgttgcctgagttctaccatgtaggaggaagcctccgtgcactctctgggggagccagcggagtgatttctggtgcaacgtggttgggctttgtctttaggatgggcacaaaccctccagggggatcgacttcaaaattcaccttgttgtaaaacgggctacctcagtgtcccagccaaaatttttattgtaacatgctgtcaggtgtgtcactctttccaagccagtaagcttttccggggatttcttcaagtagccagcattcagagcaatcttcagcattgcagattctgagaaatgtggctctggagcctgtcaccctcgagaaacctaagagggctgcattgattccatgtggccctgggtctatggagcagtacatgagctcccagtgctctaaggctcttcagccctaggctttgaagggagtgatttctcagtattcttaaacctctttctgatgacacttgtacctgtgaggggtctagagagaaagagtagtagactcctactttactacaattcaggatgcagggcatgagaggattccctctctcctccaagggaagaagcttttggcgtgcacacatccctgagaagcaaagtgtctttgtcttcagtcagatacataggaccgttttctgccccatggcccggaagccaaaggccttggctttcatgatcaacggtctagggaaacatgcaaaatttccatgtctgtcccaaactctgcccccgacagccaattaccacctgcagcccgcattgccaaatgcggtgccgtttgcatgaagattcagtagagtttcctagaaaggtgctacctcgtgagctcactttccaatgaggaatctgatctgttgtgtttctctaaggtgtcaggtgaaatatttccaagaacttactacagttctagaatgggaggaatctgttgctttggtgtttgtttgttggtcggttttctcacatccatctgcctatggataaggaaaagagaacggtcgtaattctcatagactcctttctggttgtgtcacaaatggcttcacatgtttctctatgctcagagatactcagcttgatttcccgtgttttcatttcagcaccgactgagcaaaggcctggggtgcaggagtgctaccatggtaatggacagagttatcgaggcacatactccaccactgtcacaggaagaacctgccaagcttggtcatctatgacaccacactcgcatagtcggaccccagaatactacccaaatgcgtatgtctttgttctttaccataagagaagaaagggccaagtgaagtttctgttacaagagatgtgtctcaagctgagttctccgaactcaacttgtgacagatgcagatggcgtagcaaaatgtctcaggatgattgccttggagctaagggtctgagagaagggaaatgttaagctccctctccttcctcctagttctattgagcagaagggaaatctggaggtgaggagatcacattatgaagaaagtcagaatgacaaaggaccagacacttagattacccttccacaacaccaactaaacgtcaatggagactttccagttggaattccgttattctggcttccacttcctgaagggaaggttgcgtttgccttttctctctgggttcaagaggaaagaataggtgcttatttatggacaggtgaattgatctgtttctatatctacgtatattccgattgtcagaaaaacactcgttcctaagtaccagtggcctgaagggatacaggttcccagcaagagaagatccaaggaaggaaggcagatgagagtcagcacagagagggatgctgaaaagtaaaagggatgggtggatggagagaagcccgggtctgaccacccaatggccaatattttggccacaagcgactaccagagacatggaaaaatggtttctacatgtgggacaacagatggtagaggacctagagaattgagagaggggcaatgatgggctccactccgcagatgccttggctttcttcctggatacccttcctgcactgaatagcaaggagatggagcccaagcagactgtagccatcttgctgaatggaggagagggattggagtttgggatgactgtggtagctgaaatttttctaggtctgctagaaataagaactggtttgtggaggaaaagagctctacaaatacgcatagaagtctcctccagtcgttggcctgacatgacgctgcctgtgcacaggaaatggttccacgagaaagtgtggcaaagaacatttactgagaaacagcaagtacaagagcacaggaagctcaataaagaagagagagatcacatagcactctgggatactggagttcttcccagctagaccagagagtcctcacggagcacattgccaattcagtggagaccccagaacagccgtaatttaaaggtacacttagtatattactagaataaagtcagctgcagacaaccccttgcacagctggaaagcaagtgtccaagcatcaaatcggtttccaatcaatgaagtgcctgtgagaggaaatctcaactctctttagaagtaaacaacaaagtcgattgcctcagctatgcggtatccgcagagtgagtcctaaatttaaaatctgactacatgtagaaaagcgtttcgtgtgacccatgaccaggaaataaatcgggtaatacaaacaggctcaggaatgagagaaatgattagaattgcgtgaaaatttgaaatatcagtatgataactgatttcaaatatttaaaaaaacaacatgcaagaaagcagatatcatatcaagagaaattaacagtacagaatagccaaattaaattaaagagctagtataaaaaaagtatgtcttaattgaaaaaaattactgtatggccggctgatcaatttagacgtttcagaggaaaacattacccaacacacaattctagagaacctacagaatgagctacacacacacacacacacacacacacaaactgaaaacacacccatactcacacacacgcagaaactcacaagttctaacacacacagacacgcgcacccctgaagaaacagtgaaatataaaattaagcgagcctcacagacatgtaggaaaatatgaaaagatttcctgcatgtgggaagcaagtcacagtaaagagcaagggagtttggaatagaaacaaataccagaatcaaggatggctgataacttttcaattacgaagaacattaaaaaaaatcacagaatcgtgaaactcaagggatcacatagggaatttcggaaaaaaaacccaacctgtatgatgtacttttgtacatcacagttcgaaggtaacaaggcaaagatataataagaagaaacctgtcacgagaaactggaggaaaaagagctgtgtcttcctacaagtacactgatacaaattgccaatgtgttcacctcagaaacactggaagccagataccagggaatattgttaaaatgataatcaggaacaaaaagagatcaaccgggaatgctgaatccagcaataaaatgccttgaagatcatccatgtcggataaatgcatattgtgcactgccccaaagaaagaaaccggaaactgtaagaattggaaatcagcaggcttatgtaacaagagaggtgacccgaaggaattaggtagaagaagaattgaacaagaaaggaactttctgcagcccacgtaatgaagaatccagcaattggcaaatgtagatagatgtaaatgcaaaatattttcttgatcaaatttctatatctttgtaaatgagagttgactacttgaaacaaaatgatagcaagatatttaacttcagcatatgtagaggtaagaatttgaaatggtagcataaatcacgaagggattaattcgaagtgtaccgttgtaagtttctttacctcatgcacgatggtgtgtcatattaataaaagggtactgtgcgggttcgaagggatattgcaaatcctagagcaatcacaaaggtttgaactctgaggtttttggtataataagaatagtccatgcattcaaaagagggaagccaaggaagaactagaagtctttcaagagctcaggctcttatacatccagttgctcattgaaccagcttcctggaatggagggtctggggttgagactaggccacaagtctagagtctctagagagacagtgttggaaccccatggcccataatacatttcccattttctcaggcagccagaggtcatgaatgtgaggatactgggaggttggagcaacgttcttgggaggcataaggaagagcgaatgcttcaagatccccgcagcccaaactactcgcctgctttgccccctaatgcatttttctctgctgctccgtagctgtccgacctcttcagatctcttagtccaccctgccgtcttcctttatgccatgggtcccactgttctttcaactcatccccctttccctcagtcccggagtagctgcggccagcagagggtagactgagagcaggagagaaggacctgcctaggaaccccttctagagatactgcatcctgcctgggagcaagttttccagggcagctttgagaagtcttggagaaacaaacctactaaacctgacagacagtaatactatttgcacaatgcttttctgtgggaaaggtagagccttttcactacgtattgagtacatagagtgtgagggttgacctggaacggctatcctcctggatgacgtgtgttttctgaagaactacatgttcgttgcaactcccacattagaatatgaagtcctaccgagagagatacggagactagacagatacagatgcatttgcatgtgaatacacaatcccacaatacagacgtcaaaacccataccagttattccagagagatggattgggcagaaggcagaaggagaatactctgatcgtttttcggccacgtgtgtgtgttatctcagtgtttctaagaagcgtttgctactttagattttttatttaaaaaaaatagtaataatctattaagtatgagagatgtgcagagaggattagtgatcgagagccatttttgctggtggcaatcatatggtacttttaatgggaatattagaaaggcaccggtaatgaccttgttgcagcacaaaggagagagtgtggggtgcccctgcatgttgtcccacctcttgtgacgtgtatcgttttggaatttccagtggcttgatcatgaactactgcaggaatccagatgctgtggcagctccttattgttatacgagggatcccggtgtcaggtgggagtactgcaacctgacgcaatgctcagacgcagaagggactgccgtcgcgcctccgactgttaccccggttccaagcctagaggctccttccgaacaaggtaaggagtctgtggccagacatctacacgcttcgatgctgggatgaaaagccatggaaattcccactgatgcagccgccttcaatggtaaacggatgctcgagtgttgcctgagttctaccatgtaggaggaagcctccgtgcactctctgggggagccagcggagtgatttctggtgcaacgtggttgggctttgtctttaggatgggcacaaaccctccagggggatcgacttcaaaattcaccttgttgtaaaacgggctacctcagtgtcccagccaaaatttttattgtaacatgctgtcaggtgtgtcactctttccaagccagtaagcttttccggggatttcttcaagtagccagcattcagagcaatcttcagcattgcagattctgagaaatgtggctctggagcctgtcaccctcgagaaacctaagagggctgcattgattccatgtggccctgggtctatggagcagtacatgagctcccagtgctctaaggctcttcagccctaggctttgaagggagtgatttctcagtattcttaaacctctttctgatgacacttgtacctgtgaggggtctagagagaaagagtagtagactcctactttactacaattcaggatgcagggcatgagaggattccctctctcctccaagggaagaagcttttggcgtgcacacatccctgagaagcaaagtgtctttgtcttcagtcagatacataggaccgttttctgccccatggcccggaagccaaaggccttggctttcatgatcaacggtctagggaaacatgcaaaatttccatgtctgtcccaaactcttcccccgacagccaattaccacctgcagcccgcattgccaaatgcggtgccgtttgcatgaagattcagtagagtttcctagaaaggtgctacctcgtgagctcactttccaatgaggaatctgatctgttgtgtttctctaaggtgtcaggtgaaatatttccaagaacttactacagttctagaatgggaggaatctgttgctttggtgtttgtttgttggtcggttttctcacatccatctgcctatggataaggaaaagagaacggtcgtaattctcatagactcctttctggttgtgtcacaaatggcttcacatgtttctctatgctcagagatactcagcttgatttcccgtgttttcatttcagcaccgactgagcaaaggcctggggtgcaggagtgctaccatggtaatggacagagttatcgaggcacatactccaccactgtcacaggaagaacctgccaagcttggtcatctatgacaccacactcgcatagtcggaccccagaatactacccaaatgcgtatgtctttgttctttaccataagagaagaaagggccaagtgaagtttctgttacaagagatgtgtctcaagctgagttctccgaactcaacttgtgacagatgcagatggcgtagcaaaatgtctcaggatgattgccttggagctaagggtctgagagaagggaaatgttaagctccctctccttcctcctagttctattgagcagaagggaaatctggaggtgagaagatcacattatgaagaaagtcagaatgacaaaggaccagacacttagattacccttccacaacaccaactaaacgtcaatggagactttccagttggaattccgttattctggcttccacttcctgaagggaaggttgcgtttgccttttctctctgggttcaagaggaaagaataggtgcttatttatggacaggtgaattgatctgtttctatatctacgtatattccgattgtcagaaaaacactcgttcctaagtaccagtggcctgaagggatacaggttcccagcaagagaagatccaaggaaggaaggcagatgagagtcagcacagagagggatgctgaaaagtaaaagggatgggtggatggagagaagcccgggtctgaccacccaatggccaatattttggccacaagcgactaccagagacatggaaaaatggtttctacatgtgggacaacagatggtagaggacctagagaattgagagaggggcaatgatgggctccactccgcagatgccttggctttcttcctggatacccttcctgcactgaatagcaaggagatggagcccaagcagactgtagccatcttgctgaatggaggagagggattggagtttgggatgactgtggtagctgaaatttttctaggtctgctagaaataagaactggtttgtgtggaggaaaagagctctacaaatacgcatagaagtctcctccagtcgttggcctgacatgacgctgcctgtgcacaggaaatggttccacgagaaagtgtggcaaagaacatttactgagaaacagcaagtacaagagcacaggaagctcaataaagaagagagagatcacatagcactctgggatactggagttcttcccagctagaccagagagtcctcacggagcacattgccaattcagtggagaccccagaacagccgtaatttaaaggtacacttagtatattactagaataaagtcagctgcagacaaccccttgcacagctggaaagcaagtgtccaagcatcaaatcggtttccaatcaatgaagtgcctgtgagaggaaatctcaactctctttagaagtaaacaacaaagtcgattgcctcagctatgcggtatccgcagagtgagtcctaaatttaaaatctgactacatgtagaaaagcgtttcgtgtgacccatgaccaggaaataaatcgggtaatacaaacaggctcaggaatgagagaaatgattagaattgcgtgaaaatttgacatatcagtatgataactgatttcaaatatttaaaaaaacaacatgcaagaaagcagatatcatatcaagagaaattaacagtacagaatagccaaattaaattaaagaggtagtataaaaaaagtatgtcttaattgaaaaaaattactgtatggccggctgatcaatttagacgtttcagaggaaaacattacccaacacacaattctagagaacctacagaatgagctacacacacacacacacacacacacacaaactgaaaacacacccatactcacacacacgcagaaactcacaagttctaacacacacagacacgcgcacccctgaagaaacagtgaaatataaaattaagcgagcctcacagacatgtaggaaaatatgaaaagatttcctgcatgtgggaagcaagtcacagtaaagagcaagggagtttggaatagaaacaaataccggaatcaaggatggctgataacttttcaattacgaagaacattaaaaaaaatcacagaatcgtgaaactcaagggatcacatagggaatttcggaaaaaaaacccaacctgtatgatgtacttttgtacatcacagttcgaaggtaacaaggcaaagatataataagaagaaacctgtcacgagaaactggaggaaaaagagctgtgtcttcctacaagtacactgatacaaattgccaatgtgttcacctcagaaacactggaagccagataccagggaatattgttaaaatgataatcaggaacaaaaagagatcaaccgggaatgctgaatccagcaataaaatgccttgaaggtcatccatgtcggataaatgcatattgtgcactgccccaaagaaagaaaccggaaactgtaagaattggaaatcagcaggcttatgtaacaagagaggtgacccgaaggaattaggtagaagaagaattgaacaagaaaggaactttctgcagcccacgtaatgaagaatccagcaattggcaaatgtagatagatgtaaatgcaaaatattttcttgatcaaatttctatatctttgtaaatgagagttgactacttgaaacaaaatgatagcaagatatttaacttcagcatatgtagaggtaagaatttgaaatggtagcataaatcacgaagggattaattcgaagtgtaccgttgtaagtttctttacctcatgcacgatggtgtgtcatattaataaaagggtactgtgcgggttcgaagggatattgcaaatcctagagcaatcacaaaggtttgaactctgaggtttttggtataataagaatagtccatgcattcaaaagagggaagccaaggaagaactagaagtctttcaagagctcaggctcttatacatccagttgctcattgaaccagcttcctggaatggagggtctggggttgagactaggccacaagtctagagtctctagagagacagtgttggaaccccatggcccataatacatttcccattttctcaggcagccagaggtcatgaatgtgaggatactgggaggttggagcaacgttcttgggaggcataaggaagagcgaatgcttcaagatccccgcagcccaaactactcgcctgctttgccccctaatgcatttttctctgctgctccgtagctgtccgacctcttcagatctcttagtccaccctgccgtcttcctttatgccatgggtcccactgttctttcaactcatccccctttccctcagtcccggagtagctgcggccagcagagggtagactgagagcaggagagaaggacctgcctaggaaccccttctagagatactgcatcctgcctgggagcaagttttccagggcagctttgagaagtcttggagaaacaaacctactaaacctgacagacagtaatactatttgcacaatgcttttctgtgggaaaggtagagccttttcactacgtattgagtacatagagtgtgagggttgacctggaacggctatcctcctggatgacgtgcgttttctgaagaactacatgttcgttgcaactcccacattagaatatgaagtcctaccgagagagatacggagactagacagatacagatgcatttgcatgtgaatacacaatcccacaatacagacgtcaaaacccataccagttattccagagagatggattgggcagaaggcagaaggagaatactctgatcgtttttcggccacgtgtgtgtgttatctcagtgtttctaagaagcgtttgctactttagattttttatttaaaaaaaatagtaataatctattaagtatgagagatgtgcagagaggattagtgatcgagagccatttttgctggtggcaatcatatggtacttttaatgggaatattagaaaggcaccggtaatgaccttgttgcagcacaaaggagagagtgtggggtgcccctgcatgttgtcccacctcttgtgacgtgtatcgttttggaatttccagtggcttgatcatgaactactgcaggaatccagatgctgtggcagctccttattgttatacgagggatcccggtgtcaggtgggagtactgcaacctgacgcaatgctcagacgcagaagggactgccgtcgcgcctccgactgttaccccggttccaagcctagaggctccttccgaacaaggtaaggagtctgtggccagacatctacacgcttcgatgctgggatgaaaagccatggaaattcccactgatgcagccgccttcaatggtaaacggatgctcgagtgttgcctgagttctaccatgtaggaggaagcctccgtgcactctctgggggagccagcggagtgatttctggtgcaacgtggttgggctttgtctttaggatgggcacaaaccctccagggggatcgacttcaaaattcaccttgttgtaaaacgggctacctcagtgtcccagccaaaatttttattgtaacatgctgtcaggtgtgtcactctttccaagccagtaagcttttccggggatttcttcaagtagccagcattcagagcaatcttcagcattgcagattctgagaaatgtggctctggagcctgtcaccctcgagaaacctaagagggctgcattgattccatgtggccctgggtctatggagcagtacatgagctcccagtgctctaaggctcttcagccctaggctttgaagggagtgatttctcagtattcttaaacctctttctgatgacacttgtacctgtgaggggtctagagagaaagagtagtagactcctactttactacaattcaggatgcagggcatgagaggattccctctctcctccaagggaagaagcttttggcgtgcacacatccctgagaagcaaagtgtctttgtcttcagtcagatacataggaccgttttctgccccatggcccggaagccaaaggccttggctttcatgatcaacggtctagggaaacatgcaaaatttccatgtctgtcccaaactctgcccccgacagccaattaccacctgcagcccgcattgccaaatgcggtgccgtttgcatgaagattcagtagagtttcctagaaaggtgctacctcgtgagctcactttccaatgaggaatctgatctgttgtgtttctctaaggtgtcaggtgaaatatttccaagaacttactacagttctagaatgggaggaatctgttgctttggtgtttgtttgttggtcggttttctcacatccatctgcctatggataaggaaaagagaacggtcgtaattctcatagactcctttctggttgtgtcacaaatggcttcacatgtttctctatgctcagagatactcagcttgatttcccgtgttttcatttcagcaccgactgagcaaaggcctggggtgcaggagtgctaccatggtaatggacagagttatcgaggcacatactccaccactgtcacaggaagaacctgccaagcttggtcatctatgacaccacactcgcatagtcggaccccagaatactacccaaatgcgtatgtctttgttctttaccataagagaagaaagggccaagtgaagtttctgttacaagagatgtgtctcaagctgagttctccgaactcaacttgtgacagatgcagatggcgtagcaaaatgtctcaggatgattgccttggagctaagggtctgagagaagggaaatgttaagctccctctccttcctcctagttctattgagcagaagggaaatctggaggtgaggagatcacattatgaagaaagtcagaatgacaaaggaccagacacttagattacccttccacaacaccaactaaacgtcaatggagactttccagttggaattccgttattctggcttccacttcctgaagggaaggttgcgtttgccttttctctctgggttcaagaggaaagaataggtgcttatttatggacaggtgaattgatctgtttctatatctacgtatattccgattgtcagaaaaacactcgttcctaagtaccagtggcctgaagggatacaggttcccagcaagagaagatccaaggaaggaaggcagatgagagtcagcacagagagggatgctgaaaagtaaaagggatgggtggatggagagaagcccgggtctgaccacccaatggccaatattttggccacaagcgactaccagagacatggaaaaatggtttctacatgtgggacaacagatggtagaggacctagagaattgagagaggggcaatgatgggctccactccgcagatgccttggctttcttcctggatacccttcctgcactgaatagcaaggagatggagcccaagcagactgtagccatcttgctgaatggaggagagggattggagtttgggatgactgtggtagctgaaatttttctaggtctgctagaaataagaactggtttgtgtggaggaaaagagctctacaaatacgcatagaagtctcctccagtcgttggcctgacatgacgctgcctgtgcacaggaaatggttccacgagaaagtgtggcaaagaacatttactgagaaacagcaagtacaagagcacaggaagctcaataaagaagagagagatcacatagcactctgggatactggagttcttcccagctagaccagagagtcctcacggagcacattgccaattcagtggagaccccagaacagccgtaatttaaaggtacacttagaatattactagaataaagtcagctgcagacaaccccttgcacagctggaaagcaagtgtccaagcatcaaatcggtttccaatcaatgaagtgcctgtgagaggaaatctcaactctctttagaagtaaacaacaaagtcgattgcctcagctatgcggtatccgcagagtgagtcctaaatttaaaatctgactacatgtagaaaagcgtttcgtgtgacccatgaccaggaaataaatcgggtaatacaaacaggctcaggaatgagagaaatgattagaattgcgtgaaaatttgacatatcagtatgataactgatttcaaatatttaaaaaaacaacatgcaagaaagcagatatcatatcaagagaaattaacagtacagaatagccaaattaaattaaagagctagtataaaaaaagtatgtcttaattgaaaaaaattactgtatggccggctgatcaaattagacgtttcagaggaaaacattacccaacacacaattttagagaacctacagaatgagctacacacacacacacacacacacacacacacacaaactgaaaacacacccatactcacacacacgcagaaactcacaagttctaacacacacagacacgcgcacccctgaagaaacagtgaaatataaaattaagcgagcctcacagacatgtaggaaaatatgaaaagatttcctgcatgtgggaagcaagtcacagtaaagagcaagggagtttataatagaaacaaataccagaatcaaggatggctgataacttttcaattacgaagaacattaaaaaaaatcacagaatcgtgaaactcaagggatcatatagggaatttcggaaaaaaaacccaacctgtatgatgtacttttgtacatcacagttcgaaggtaacaaggcaaagatgtaataagaagaaacctgtcacgagaaactggaggaaaaagagctgtgtcttcctacaagtacactgatacaaattgccaatgtgttcacctcagaaacactggaagccagataccagggaatattgttaaaatgataatcaggaacaaaaagagatcaaccgggaatgctgaatccagcaataaaatgccttgaaggtcatccatgtcggataaatgcatattgtgcactgccccaaagaaagaaaccggaaactgtaagaattggaaatcagcaggcttatgtaacaagagaggtgacccgaaggaattaggtagaagaagaattgaacaagaaaggaactttctgcagcccacgtaatgaagaatccagcaattggcaaatgtagatagatgtaaatgcaaaatattttcttgatcaaatttctatatctttgtaaatgagagttgactacttgaaacaaaatgatagcaagatatttaacttcagcatatgtagaggtaagaatttgaaatggtagcataaatcacgaagggattaattcgaagtgtaccgttgtaagtttctttacctcatgcacgatggtgtgtcatattaataaaagggtactgtgcgggttcgaagggatattgcaaatcctagagcaatcacaaaggtttgaactctgaggtttttggtataataagaatagtccatgcattcaaaagagggaagccaaggaagaactagaagtctttcaagagctcaggctcttatacatccagttgctcattgaaccagcttcctggaatggagggtctggggttgagactaggccacaagtctagagtctctagagagacagtgttggaaccccatggcccataatacatttcccattttctcaggcagccagaggtcatgaatgtgaggatactgggaggttggagcaacgttcttgggaggcataaggaagagcgaatgcttcaagatccccgcagcccaaactactcgcctgctttgccccctaatgcatttttctctgctgctccgtagctgtccgacctcttcagatctcttagtccaccctgccgtcttcctttatgccatgggtcccactgttctttcaactcatccccctttccctcagtcccggagtagctgcggccagcagagggtagactgagagcaggagagaaggacctgcctaggaaccccttctagagatactgcatcctgcctgggagcaagttttccagggcagctttgagaagtcttggagaaacaaacctactaaacctgacagacagtaatactatttgcacaatgcttttctgtgggaaaggtagagccttttcactacgtattgagtacatagagtgtgagggttgacctggaacggctatcctcctggatgacgtgcgttttctgaagaactacatgttcgttgcaactcccacattagaatatgaagtcctaccgagagagatacggagactagacagatacagatgcatttgcatgtgaatacacaatcccacaatacagacgtcaaaacccataccagttattccagagagatggattgggcagaaggcagaaggagaatactctgatcgtttttcggccacgtgtgtgtgttatctcagtgtttctaagaagcgtttgctactttagattttttatttaaaaaaaatagtaataatctattaagtatgagagatgtgcagagacgattagtgatcgagagccatttttgctggtggcaatcatatggtacttttaatgggaatattagaaaggcaccggtaatgaccttgttgcagcacaaaggagagagtgtggggtgcccctgcatgttgtcccacctcttgtgacgtgtatcgttttggaatttccagtggcttgatcatgaactactgcaggaatccagatgctgtggcagctccttattgttatacgagggatcccggtgtcaggtgggagtactgcaacctgacgcaatgctcagacgcagaagggactgccgtcgcgcctccgactgttaccccggttccaagcctagaggctccttccgaacaaggtaaggagtctgtggccagacatctacacgcttcgatgctgggatgaaaagccatggaaattcccactgatgcagccgccttcaatggtaaacggatgctcgagtgttgcctgagttctaccatgtaggaggaagcctccgtgcactctctgggggagccagcggagtgatttctggtgcaacgtggttgggctttgtctttaggatgggcacaaaccctccagggggatcgacttcaaaattcaccttgttgtaaaacgggctacctcagtgtcccagccaaaatttttattgtaacatgctgtcaggtgtgtcactctttccaagccagtaagcttttccggggatttcttcaagtagccagcattcagagcaatcttcagcattgcagattctgagaaatgtggctctggagcctgtcatcctcgagaaacctaacagggctgcattaattccatatggtcctgggtctatggagcagtatatgagctcccaatgctctaaggctcttcagtcctaggctttgaagggagtgatttctcagtgttcttaaacctctttctgatggcacttgtacctgtgaggggtctagagagaaaggttagtagacttctcctttactgcaattcaggatgcagggcatgagaagattccctccctcctccaagggaagaaggttttggcgtgcacacatccttgagaagcaaagtgtctttgccttcagtcagatatataggatcgttttctgccccatggcctggaagccagaggccttggctttcatgatcaacgatctagggaaacatgcaaaatttccatgtctttcccctcctctgccctcgacagccaattaccacctgcatcctgcattgccaaatgcagtgccctttgtatgaacattcagtagagtttcatagaaaggtgctacttcgtgagcgcactttgcagtgagaaggagtctgttctgttctgtttttctaaggatttcaggtgaaatatttcctagaacttactacagttctagattggtaggaatctgtaggtttgctgtatgttttttggttggttttctcccatccatctgcctacaggtaagggaaagataacgttcataattctcatagactcctttctggttgtgtcataaatggcttcacatatttcgttattctcagagatactcagtttatttcttgtgttttcatttcagcaccgactgagcagaggcctggggtgcaggagtgctaccacggtaatggacagagttatcgaggcacatactccaccactgtcactggaagaacctgccaagcttggtcatctatgacaccacactcgcatagtcggaccccagaatactacccaaatgcgtatgtctttgttctttaccataagagaataaagggccaactgaagtttctgtgacaagagacatgcttcaagctgagttctccgaactcaacttgtgtcagattcagatggtgtagcaaaatgtctcaggatgatttccttggagctaagggtctgagagaagagaaatgttaagctgcctcaccttcctcctagttttgtggagcagaagggaaatgaggaggcgaggagatcaccttatgaagaaagtcagaatgacgaaccaccaaacacttagattacccttgcccaacacccactaagcgtcaatgaagactttccagttggaattccgttattctgacttccaattcctgaagggaagattgtgtttgccttttctgtctgggctcatgaggaaagtttatgtgcttacttatggacaggtgaattgatctgtttctatttctacctgtattccaatagggagaaaatctcttggtcctaagtaccagtggcctgaaaggatagaggttcccagcaagagaagatccaaggaaggaaggcagatgagagtcagcacagagagggatgctgaaaagtaaaagggatgggtagatggatagaagccctggtctgaccaccccatggccaatcatttggccataatcaacaaccaaagacatggaaaaatggtttctacatgtgggacaacagatggtagaggacctagagaattgagagagggccaatgatgagctcaactccatagatgccttggctttcttcctggatacccttcctgcactgaatagcaaggagatggagctcaagcagcctgtagccatctagctgagcagaggagagggattggagtttgggatgactctggtattttctaggtccgctacaaataagaactggtttgtggaggaaaggagctctacaaatacgcatagaagtctcctccagtagttggcctcacatgacactgcatgtgcacagaaaatggttctacagaaagtgtggcaaagaacatttactgagaaacagcaactacaagagaacagcaagctcaattaagaagatagagatcacatagcactctgtgttattggagttcttaccagctagatgagagagtgctcacggaacacattgccaattcagtggagaccccagaacagccataatttcaaagtacaattagtatattactagaataaaggcagctgcagacaaccccttgcacagctgaaaagcaagtgtccaagcatcaaatgggtttccaatcaatgaagtgcctgtgagaggaaatctcaactctcttcagaagtaaacaacaaagtcaattgcctcagctatgcggtatccccagagtgagtcctaaattaaaaatttgactacgtgtagaaaagaatttcgtgtgatccatgaccagaaaataaatcaggcaatacaaacaggctcagaaatgacatcgataattagaattgcatgaaaatttgacatatcagtatgataactgatttcagatatttaaaaaaagtgcaacaaagcaggtatcatatcaagacaaattaatagtatagaatagccaaatcaaattaaagaactattatacaaaaagtatgtcttaaatgaagaaattactgtatgtccgcctgaaaaatttagatgtttcagaagaaaaaattaaccaaaaacaattctgcagaacctacagaatgagccacacacacacacattcaaaacacacccatacacacacacatgcaaaaactcacaagttctaacacacacacaaacacacacacacatgcacatccctaaagaaatagggaaatataaaattaaccgaccctcagagacatgcaggaaaatataagaagatttcctgcatgtgggaagcaagtcacagtaaagagcaagggagtttggagtagatacaaataccggaatcacggatggctgataacttttcaattatgaagaacgttagaaaaatcacagattcatgaaactaaagggatcaaataggaaatttcgagaaaaaaaactacatgatgcacttctctacatcacagttcaaaggtaacaaggcaaggatataagaagaagaaacatctcacgagaaactggagaaaaaagagctgtgtcttcctagagtacagtgatacaaattgctaatgcgttcacctcagaaacactggaagccagataccagggaatattattaaaatgataatgaggaacaagaagagatcaaccgagaatgctgaatccagcaataaaatgccttgaagatcatccatgttggataaatgcatattgtgcactgcccaaaacaaagaaactggaaagtgtaagactttggaatcagcaggcttatgtagcaacagaggtgacccgaaagaattaggtataagaagaatagaagaattgcatgaaaatttgacatatgactaagataactatttcaaatatttaaaaaaagatgaatatgtaataaaacagataaaatatcaaaagaaagtaacagtattgactagccaaatcaaattaaagacttagtgtaaaaagctatgtcttaaaagaaaaaattactggatggctgcctgatcaatttagacatttctgaataggaaactaaccaaaaatcaattctacagaaccaactacacacatatatacacatacaacacacccatacacacccacgcaaaaactcacaagttcacacacacacacacacacacacaaccctcaagaaatagtgaaatagaaaaccaaccgaacctcacagacatgttgcaaaataggaaaagatttcctgcatatgggaagcaagtcacagaaaagagaacgggagattggaaacagaaacaaataccggaatcaaggatggccgaaaacttttcattgatcaagaatattaacaaaatcgcaaaaacacgaaattcaatgcatcaaataggcgtttcgaaaaaaagaaaaaatctggtatgatgcacttttgtacttcacattttcacggtaagaagacaaagatataataacaagaaacttcttatgagaaactggggaaaaacaagctgtttcttgctagaagaacagtgatacaaattgctaatgcattctcgtcaaaaacactggaagccagataccgggaatgttattaatgtggtaaacaggaacaagaagagatcaaccaagaatgctaaatccagcaataaaatgccttgaagatcatccatgctgcataaatgtatgttgtgcactgccccaaacaaagaaaccggaaactgtaagaatttggaatcagcaggctgatgtaacaagagaggtgacccaaaggaattaggtagaagaagaatagtacaagaagggaactttctgcagcccatgtaatgaagaacccagcaattggcaaatgtagatgtaaatgcaaaatattttcttgaccaaatttctatatatttttaaatgagcgttgactactggaaacaaaatgatagcaatatatttaattttagcatatgtagaggtaagaatttgaacaagtagcgtaaatcatgtagggaataattagaagtgtaccattgtaagtttcttacctcatgcacaatggtatgtaatattaataaaatgttactgtgtgggttcaaggagatattgcaaatcctagagcaatcacaaagttttgaactctgaggtatattgtataataagaatattccatgtattcaaaagagagaagccaaggaagaaagaaatttgtcacgagtttgggctcttagtacatcctgtagctcattgaaccagcttcctggaatggagggtctgggattgacactaggccacatgtatagagtctctagagagacagtgtttcatccccatggcccgtaatacatttcccattttctcaggcagccacaggtcatgaatgtgaggatagagagaggttggagcaacgttcttgggaggcataaggaagagcaaatgcttcaagatccccgcagcccaaactcctacctgctttgccccctaatgcagtgttcctccgtagctgtccgacctcttcagatctcttagtctaccctgccatcttcctttatgccatgggtcccactgttctttcaactcatccccctttccctcagtgcagagtagctgcggccagcagagggtagactgagagcaggagagaaggtcctgcccaggaacccattctagagatgctgcattctgcctgggagcaagttttccagggcagctttgagaagtcttgcagaaacaaacctatttgacccacatgatatgggaatgacagaaagtaatacaatttgcacagtgcttttccatgggaaaagtagagccttttcgcgaggttttgagtacatagagagtgaaggttgacctggaaaggttatcctcctggatcccatgttttttctgaagaactacctgttagttgcaacttgcacattagaatatgaagtcctaccgagagagatacggagaactagataaatacagatacttttgtatgtgaataaacgattccacaatacacacatcaaaatccataccagttattccagagagatggattgggcagaaggcagaaggagaatactctgatcgttttttgcccacgtgtatgtattatctcagtgtttctaagaagcgtttgctactttagatttttttttataataataatcttttaagtatgagaaatgtgcagacaggattagtgattgagagccatttgtgcttgtggcaatcatatggtacttttatgggaatattagaaaggcactggtaatgaccttgttgcagcacaaaggagagggtgtggggtgcccctgcatattgtcccacctcttgtgacgtgtatcgttttggaatttccagtggcttgatcatgaactactgcaggaatccagatcctgtggcagccccttattgttatacgagggatcccagtgtcaggtgggagtactgcaacctgacacaatgctcagacgcagaagggactgccgtcgcgcctccaactattaccccgattccaagcctagaggctccttctgaacaaggtaaggagcctgtggccagaaacctacacgtttcgatgctgggatgaaaagccatggaaattcccactgatgcagcagcctccaatggtaaacggatgctcgagtgttgactgagttctgtcatgtaggaggaagcctccgtgcactctctgggggagccagcggattgatttctggtacaacgttgggtgggctgtgtctttagaattggcacaaaccctccagggtgatcgacttcacaactcacctcgttgaaaaatgggctatctcagtgtcttagccaaaatttttattgtaacatgctgtcagatgtgtgactctttccaagccagtaagcttttcctgggacttcttcaattagccagcattcagtgcaatcttcagcattgcagattcagagaaatgtggctctggagcctgtcacccttgagaaacagggctaacagggttgcattaattccaaatcaccctggttctatggagcagtacatgaactcccaatgatctatgtttcaggacttcctcagtcataggtgggctctgcagccctaggtttttaagtgagtgactgccccgtgttctggtggcagttgtacctgtgagcggtctggatagaaagagtcggagacttctgtattattgcaactcaggatgtgggtcatgagaggatttcatctctcctgcaggggagtaagctgttcgcctccacccatccctgataactgaagtgtctttgtctgcagtcctagacgaaggactgttgtctctcccatggcccagaagctgaagaccttgccttttgttatgaaacgttcattgttttcatgtctgtccgtttctctgcccctaacacccaatcaccatgtatggcctgtacccccaaatgcatcgtgctttgctgtttgctgccccatagtcctcatgaacattcagtagaaattcccataaatgtgcttgcacgtgagcacagtttccattgagaagccctctcatttgtcctttttttctaagcttttatgtgaaatatttctaagaacttactacagttctaaagtgttaggaatttgtttctttggtgtttttgtttgttggttggttgttgcttttctcaagtccatctgcctacaaataaagaaacaagaatgttacttgtcatattctcctgaggtcataattctcagagacttttttctggtttgtgccataagtggcttcacatgtttgtctcttcttggaaacactcagtttgatttcttttcttttcatttcagcaccaactgagcaaaggcctggggtgcaggagtgctaccacggaaatggacagagttatcaaggcacatacttcattactgtcacaggaagaacctgccaagcttggtcatctatgacaccacactcgcatagtcggaccccagcatactacccaaatgcgtatgtctattttctttaccataagtgaaggaagggtcagtggaaatttctgttagtagagtcatgcttcaagctgagtgttcaggactcaagttgtctcagatgaacagtgcatagcaaaatgtctcaggaacattgtctttgagcaaagagtctaagagaagacaaatgttaatctggctctccttcctcctagtttaatggagcagaaaggtatctggaggcaaggatatcacattaagaaacaagtcaagatgacaaatgatgaaactcttagagtacccttccacaacacccactaaggttcaatgcagccttttctccttggaattctattaaactaaactccaattcctgaagtgaaggttctgttggggttttctgttttggcttacaaggaaagtatatatgtatatctatggagaggcaaatctatctctttctatatctacgtctattccaatatgtagaaacacagtcggttctgaccaccagtggtctgaagggatactggttgttagagaataaaaatggcaggaaggcagatgagagtcagcaaagagagagatcctgtaaagtaaaagggtggatagatggacagaagcccaggtctgaccagcccatggccaggctttaggccataagtgacaccaaagacatggaaaaatggtttctacatgttggacaacagacagtagtggaccaaaagaatagtgacagggggaacaatgagatcaactccatagataccttggctttcttcctggaggcccttcttgcactgaagagcaaggtgatggagcccagatggactgtagccatcttcctgaatgcaggagagagattggaatttgggactactgtggtagctaggattttataggcctgctgagaatgagaatggatttgtggatgaaaggagctccaggggcacgcatagtagtctcctcgaatctttggctaaacatgacgttgcatgtgcccagaaaaaggttccacaagaaagtagagaaaagaatatatcctgaggaatagcaactgcgattgaacagtgagctcaataaagaggacagagccctcatagcattctgggatactggagttctgaccagctggaggagagacctcactgaacctcttgggaatacagtagagactccagaaaagtcatactttaggagtagaattagtaaatttctagaaaaaaaggcagctctagacaaaccctggcaaaactgaaaagcaagtctccaagcattaaaatcatttccaagtcaattaactgcctgggagaggaaaaccctctttagaggtaaacaacaaagtcaagtggctcagctatgtggtgttcacagtgtgagttctaaatttaaaacttgactacacatagagaagcttttagtatgaaccatgaccaggtgaaaaatcagtcaatacaaatagacctagaaatgacagaaatgattagaatggcaaaaaatttgacatatcaatatgtcaactgagttttaggttttaagaaaacatgaatacggaatgaagcagataccatatcaagagacagtaacagtatagaagagccaaattaaattaaagaactagtataagaaggtatgtcttaaatgaaaaaattactggatgtattcccaatggagtgagatgtttcagaagtaaaaactaactgaaaaacaattttataccacctacagaaccagctacacatacacaaatgacacacacatatacacacatactcacacatgcacaggcttagaaacatgcacgcacacacacacacacacacacacacacctccacaaatactaaaaaatgaaatccactgatcctcacagacaggcgggaaaatataaaaagatttcctgcatgtgggtaggaagtcacagaaggagaggaaggagagattgctacaggaacaaatactggaagcaaggatagctaaaaacttttcaaataagaagaatattaaaaaccacagattcaagaagctgaatgaatcagacagggaatttccaaaaaaaaaaaaaaaaaaactgtatgattcacttttgtacatcaccgttcaacagtcagaaggcaaagatataataacaagaaacatctcatgagaaactggaggaaaaagagctgtgtcttgctagaagaacagtgatacaaattgctaatgcattctcatcagaaacactggaacccagttaacaggggatatcattaaaatgataaactagaaaaaaaagagatcaaatgagaatgctacatccagcaataaaatgccttgaagatcatccatgttggataaatgcatattgtgcactgccccaaataaataaaccaaaaactaataatttggaatcagcaggcttgtgtaacaagagatgttgcccaaagaaaattagctagaagaagaatagttcaagaggagaactttctgcagcccacgtaatgaagaacccagcaaatggcaaatgtagatgtaaatgcaaaatattttcttgatcaaatttctatatctttttaaatgagagttgactacttgaagcaaaatgatagcaatatatttaactttagcatatgtagaggtaaaaatttgaacatatagactaaatcatgtggggaataattggaagtgtaccattgtaagtttcttaccttatccacgatggtatgtaatattaatgaaaggttgaatttgtgggtccaaagggatattgtaaatcctaaagcaatcataaaattttgaattctgagggatattatataataagaattttccatgtatccaaaagagggaagccaaggaagaaaaagaagtctttcaagtactcaagctctgagcacatccagttgctcattgaaccagcttcctggaatggagggtctgggcttgagactaggtcacatgtgtagagtctctagagagacagtgttggatccccatggcccataatacatttcccgttttcccaggcagccacaggtcacgaatgggaggattctgagaggttggagcaatgttcttaggaggcataaggaggagtgaatgctctgagatttccccagcctgaggtcctccatagctgcccgacctcttcagacctcatagtctgcccagctgtctccctttatgccatgagtgccactgttctttcaactcatcccccattccctcagtcccggaattgctgtggccagcagaggatggactgagagcaggagaggaagtcctgaccaggaacccatcctagagatactgcatcctgcctgaaagctaggtttccagggcagctttgagaagtcttgcagaaagaaacccacttgacccacctgatacggtatcgacagacaggaatactttttgtgcaatggttttacatgctgaacatagagccttttggctacattttgagtacattgaatgagactgctggcctgggaaggatatcatgctggatgccatttttttctctggagaactatgtgttagttccaactcgcacattactatatgaagtcctacacagagagatacggagagctagacagatagagatacttttgtatgtgcataaccaattccacaatacacacgtcaaaatccataccagttattccagagagatggattgggcagaaggcagaaggaggatattctgatccctttttggccacatgtatgtataatctcagtgtttctaggaagtgtgtgctgcattagattttttttctttaaaaaaagtgataatatattaagtatgagaaatgtgcagagaggattagagattgagagccatttgtcattgtggcaattgtatggtatctcttttgggaatatttcaaaggcaccagtaatgaccttgttgtagcaaaatatacagtgttcctgcatatgtacccattttttgtgatgtgtattcttttggaatttccagtggcttgatcaagaactactgccgaaatccagatcctgtggcagccccttggtgttatacaacagatcccagtgtcaggtgggagtactgcaacctgacacgatgctcagatgcagaatggactgccttcgtccctccgaatgttattctggctccaagcctagaggctttttttgaacaaggtaagaagttgtgccagacatttacctgcttggatgctgggatgaaaagccatggatacccccactgacgcacaacccttcagtgctacactggttctcgtgtgttggttctgggtctgccatgtgggaggaagccttagcgcactctctgggggagccagaggtgtgatttttggtgcaacctgtgcgagctgtgtctttaggatgggcggaaaccattctgggtgctcgacttcaccactcccctcattgtaaaaggggctatctcattgtcctagacaaaattcttattgtaatatgctgtcagatgtgtgtgtctttccaagccagtaaacttttccagggatttcttcaagtagacagcattcagtgcaatcttcagcattgcagattccgagaaatgtggctctagatcctgttatccttgagaaacctaactgggttgcattaattccatatctccctgggtctgtggagtagtacatgagctcccgaagctctatctctcaggtctttttcagtccgaggcaggttgtgcagttcttagctttgaagggagtgattttttcgtgtgcttttgcctctttctgatggaacttgtacctgcggggggtctggagaaaaagagtagtagacttttgctttattgcaatgcattatgctgggcacgagaggattccctatcttattgtaggtgataagcttttggcctccactcatccctgagaagtgaagtgttgttgcctacagttttagctgcaggactgttgtctgccccatcaccaggagtttaatgctttcttttttgagcaatcatctagggacacatgcaaggtttttatatgtccttgcctcctccccaaaaaaccattttaatgcttggagacttgcttttcagctttgccaaatgcatcaccctttcttctatgctgttccatgtcgtcatgaacactctgtagagattcctagaaatgagcttccatgttagtggagtttccgatgagaagcaatctgatatttcttttccactaagttttacatgaaatatttctaagaacttactacagttctagaatggtaggcatctcttactttcgtgtttgtttgtgtgttttctcatgtccatttgcctattaataaagaatagagaatggttgtaaatctcagtgactcttttttggtttatgtcataaatggcttcctgtatttttctgttctaggaaataataagcttgatgtcttctgttttaatttcagcactgactgaggaaacccccggggtacaggactgctactaccattatggacagagttaccgaggcacatactccaccactgtcacaggaagaacttgccaagcttggtcatctatgacaccacaccagcatagtcggaccccagaaaactacccaaatgcgtacgtctttgttctttaccataagcgaaggaagggccaatggaagtttctgttagaagagtcatgcttcaaggtgactgctcaggactcaacttggctcagatgcagaggaacatttcctgtgagcaaaagttcttagagaagactttgtttttttgagacagagtcttgctttgttgcccaggctggagtgcagtggcatgatctcggctcactgcaagctccgcctcccgggttcacaccattctcctgcttcagcctctctagcagctgggactacaggcacccaccaccacacccggctaattttttgtatttttagtagagacagggtttcactgttctagccaggatggtcttggtctcctgacctcgtgatccgcctgcctcagcctcccaaagtgctgggattacaggcgtgagccaccgtgcctggctgagaagacattttttaagctggctctccttcctcctagttttatggaagcagaaggatatatggagttgagaagatcttattaataaaacagccgggatgacaaatgaccaaagagttagagtatccttctacaacatcggctgagggttaatacaaccttttcaccttggaattctatcattctaagctctagtccctgaagtgaatgttgtgttggccttttgcatcttgggtcacagggaattgatacttgcacatctatggagaggcaaatctttttctatctacttctttttcaatgggtacaaacacacttggtcctgagcaccagtggtctgaagagatacggtctgcccagaggagaagaacaaaggcaggaaagcagatgagagtcagcaaaggggcgatgctgaaaagtaaaaggggcgggtagatggacagaagccatgatctggccattctatggccagtctttcggccataagtgactaccaaagacacggcaaaacggtttccacatgttgaacaacagatgctagaggaccaagagtattgcaagagggagaaaatgagatcaacccatcaatgccttggctttcttcaaggagacccttcctgcactgaagagcaaggagatggagcccaagctgactgtagccatgttgctgaacagaggagagtgattggactttgggattactcaggtagttaggattttctagccatgctaagagtaagaatggacttgtggaggataggagctccaggcatagaagtctcctcaagtgttagtctaaacataaagcagcacttgcatagaagattttccacaagaaaatatggcaaaaaaacaccatatattgaggaacaacaactacaagggaacagtgagcttaataaaggtgacagagctcacatagtgctctggaatattggagttttgaccagctagagagaagagacctcattgaaaatcttgggcattcagtagagacctcagaaaagtcagactttatgagtagactttgtatattcctagaataaaggcagctccagaaaaaacctagcaaagctgaaaagcaaatctccaagcattaaaatggtgtcctagtcaattaactgccttctagaagaaaactcaacactctttacaggtgaacaacaaagttaagttgctgagctatgcaatatccacagtgtgagtcctaaatttataactttactacacataaaaaagcatttagtgtgaaccataaccaggaaaataatcagtcaataaaaatagaaccaggaatgatagaaatgatttaaatggcatgagaatttgacatattagtatcataactgcattgctggatttaagaaaacataaacatggaacgtaacagatatcatatcaagggaaagtaaaaggataaaagagtcaaatcaaattaaaggactattaaaaggtatatcttaaatgaaaaattcactggatggtctcccaatcaggttagttgtttccagggaaaaaattaactgaaaaataattcaatagaatctacagaaatagctgcacatatatacacacaatggcacacgtgcacacacccacacccacacaggtgtgaatcctagagccacacgagcattgaaacatagagaagtaaaaattgttcattgaggaatatgtagcaatgctcaatgtgttttaccctaataagagcttttgtgatgtatgattgaaaaactgacacaactgaagagagaaatagataagcccacactctgagttagagatttccttgattctctcactatggttataaatctttcccaaacacaacaggctagaacaaatatgcagaaaattagacatagtatctttgttctcaataaaaacgtcgacctatttaacattataccgaactaccgagtacacattaaagtgtgcatggagcattcactgaggtgtactctacacatgaccttccagcaagtctccatagatttaaaagaattaaagtcatacagagtgtgtcactttattctcccagaataaagtgagatatgaataatgagaagtttgccagcttctcaaatatttgggagtcatacggtgcatttcaaaatactctttgggacaaagaaaacatcactaaggaatttagaaaagttttgaactgagtaagaatataacacaatttatccaaacttaggagatgcagtgaatgtctttaggcttttacataattttagatgctcttagggaaaaacagaagcatgtaataatcaagatttcaaactgcaattctcaaagtgtagtctagagaaacctgaggacctttgagtaccttcagagacagtccatgaggttaaaggactttgctacgtgaaaagtaagatgctattggccctttttactttcattttccaacaagagaagaggggagttttccagcagttacataatatgtaatggcatcatgtctctgatggctaagaaaatgggcaattgttgactttgtgtgttaaaaaaattctcagtgttggtttcttatactataaatattcatcttgtgttttgaaaaagaaaagctctttggaatcccctatgaacaaagactttgacagttgttgatctaagaccacagcttaaatatctacacaagaaaaaaaaaaaaagcaaataagagccaaggaaagcagatggaaggaagtagtccaaaccagtgacattcagtgaacaagaaaagagaccaacaagggagtaaactcttgaaacagaaagttgattctttgaaaagatccatatgattgaacacagtctggctaaacaaatgacagaccaatgagggtgcacaaccatcaccatctggagtaacagaggagaggtgccattactatagcatcttccagttctgaaagctgaaaagaagattttgagaacaattgtatgtgaataaattcaggaatgttaatcatgtgggccaattcctgaggaagacaacaaatcagcaaaccagatgctgaatagttagtgtagtcctgtagagagacatacagagaggctgacagagaaatatttgtatgtgcataaaacaatctacaagacacacttcaaaatcaatctcagttaatctggaggaacatatttcacagaaggtggaaggagggtattctgatcctcttgtacattgtacaacattgtacaatgtacagagtataattgtacaagtacaattgaagttgtacaagtacaagtgcaacttgcacaatgtacagagtaaacattgatgtttactctcaattttcttatggagcacagatgactttggatgtgttacaatatgaatgataatttgtctttgagatgttcgcagttgtttagaagttgaggaccatttgtgcatattatgggacctttagtgaaaatatttcaaagtctctttttacactttgttacagcaaaatgtagagggcgctaagtgcccttgaatcttctcccatctctggtgacctgtgttgttttgaaatttgcagtggcctgaccaggaactactgcaggaatccagatgctgagattcgcccttggtgttacaccatggatcccagtgtcaggtgggagtactgcaacctgacacaatgcctggtgacagaatcaagtgtccttgcaactctcacggtggtcccagatccaagcacagaggcttcttctgaagaaggtaggaagtctatggccagacaaccacaccctaggacgttgggatgaaaagagttgcaaaatcttagtgatatagaagccttccatgctcacacaattccaagtagaatgtggactcagggtcagccactgggaaggaacactcagcgccttctctgggagaaccagagctgtgatgtttggtaccctgtgaaagggtggtatctataggaagggtgcagaccctctagggcactggacttaccactcccctggttattcaaaggatcattttagtgtcttagccagaagaatattctaacattttgccaaatttgtgaagatttaccaagctcatgataagcctttcatggtatttcttcaagtagtcagtgttcattgcatctttggctttgcggtttcggaggaatgcggtttttgagtctgtcatccttgagaaacctaatatgacttttcttagttccatatacttctgggtccaggtagcagtacatagccaacaaatgctccatcgttctggcctatctccatcttaagccagtcctgcacaactaggctttgatgggagggatctctcagtgttcttgcccctccttctcatggaacatatatctgtgttggtctctgagaagaagagtagtggatatctactttgttgcaatgcagaatcctgggccaaagataccagccatccctccaagggaataaaattttggccagtagccctctctgagagacaatttgtctttgcctacgagtcctagatgcaggaccgcttcctgccccatcttcaagaagctgaaggctttggctttggaggatcagcagtctagggaaatgtgtgacggtttcatgtctgtccccactgacagtcaatcaccacctacaacctgcacagcctgatgcatagcagtctagtttcctgccttattctcaggaacacccagaagatgtctatattaaagagcatgcacatgagtgcaattttgactgataggcactctgatctttcctttggtgcctgtgttttaaaggaaatctttctaagaactcgttaaagttctagaatgctatgaatctttgggttttattattggtatgtccatctgcctgctagtacagaacagagcatggtagtctttctcagagacaatgatcctgtttcagtcacagatttcttctgatgcttctgtgttctagaaattactcagcttgatttctcctctttgaatttcagcaccaacggagcaaagccccggggtccaggattgctaccatggtgatggacagagttatcgaggctcattctctaccactgtcacaggaaggacatgtcagtcttggtcctctatgacaccacactggcatcagaggacaacagaatattatccaaatgggtacaaccttgagttttcttcaaagacagacagcagcccccttacatttctcttggaagggccatgcttccaactaacttcttatgacaaatttatctcagatctggaatgttgggtagaatgtctcaggcttctttcttcaggcacagtgtctgaaaggagagaaatgtcaggccagctctcttttctcatagttgacagaagcaggaggatatttgaaggtggtgagttctcatgaatagaaagctcaggacacatggccacgtgcttagaaatagcaccattccacaatgcccactaaagaccaatgcaatagttcaaccagggatttctgtcattctaatctccaagtcctgaagtgaaggttgtattagccatgttcatcttgggcaacaaataaaggatatctatgttgacatccagatcttccaatcactttctcctctaacctgtacctgggttctgagaacaaggtatctgaagagctatgtgttgccagcacatgaggggcaaaagtaggaaggcagctgagagtcaggaagtataaagattctgaagagttacacatgcaggaagatggacagaaacccagttcagaccacgtcagcgtttctgccatgaaggactatcaaatacataggaaaagtgttttcataggttggacaacagacatgacaggcctgagaaaattcagaaagggaatcaaaggagatcaaccttatcatgtccctggcatccttccttgagacccttgaagggcaagcagatggagcccagctgaccacagcagtcttgcttaactgaggagagagactggagtttgtgatgcctcaggcatctgacgtattctaggctggctaagaatgagaggggatttgtggaggaaaggagctccaagaatacacaccgaagtcttctcaaggctttggctaaatacaaagctgcgtatgcacaaggagagttttcacaaagaaagaacaataaagaaaagctactggggaaagaacaactgcaagggaacagtgagctcaatggagatgctagagctcacatagcactgggggatatttgagttctgaccactcagaggagagacacctcactgaacatcttgggcattcagtagaggtcaaagaaagccataatttgggagtaggatcttcggattcctagaaataaggtgactccagaaacactccagcaacccttcttccaagccagtctaaaaggatccaaatgatttccaagtaaattaactgccttccagaaaaaagtaaactcaaccctccttagaggtaaggaacgaatacaagtttctcagttatatgacatccccagagtgcaacttgcatttaaaaatttactagacacaaaagaagttttcactgtgatccataactgggagaaaaatcactcaacacaaataggcccagaaataatagaaattatggcattggcaagaacatttaaaatgcacctctgagaactgtgtttcaggaaaatgtcagcaaaagctgaccatgagagaaatgaatgcataatatcagaaaagaaaagaattgaagagccaaatggaaatttaaaaactgagaaaagttatatctgtaatgaggaattcactggatggccttataaccagtttagatattatggtaggaaaaggtgaacgagaaaatgattcaattaaagctagacaaaccacaagacagacagacagacacaaatacacatacacacaatgactgaaccaattaatcaacagagcctcaaggacatctaggaaaacatccacacatttaatatatgtgttaggcaagtcacagaaagagaggaaaaagataatgtgacagaagttatacttgaagccatgacggctgacaaatttccaaacatacagaaaatgagaaattcatagtcatgaagctcaatgactcaggtatagatttttaaagagcaaaactctgatttactggggtacatcatagttaaattgtctgatttcaaagctaagaagaaaaaaagggggttcctatgaacaaacattttgacagttgatctaagaccacagcttaaatatctaggcaaggaaaagcaaataagacacaaggaaaggggatggatggaaatagtccaaaccaatgacattcagtgaacaagaaaatagaccaacaaaggagtaaatccatgaaacagaaagttggttctttgaaaagattcatgtgattgaccacagtctggctgaacagatgacagaccaaggagggagtacaaccatcaccatttgaagtaacaggggagaggagccattgctataccatactccaggtctgaaagctgacaagaagatatcaagaaaaactgtatgtgaataaattcatgaatgtagatcatgtggatcaattccttaggtaaacaacaaatcagcaaaccagatactgaatagattgggtactcctatagaaagacatacagatagccagacagagaaacatttgtacgtgcataaaacaatctacaagactcacttcaaaatctctcagttaatccaaagtaacatatttggcagaaggtggaaggagggtattctgatcctttcttgtacacattgatgttttctctcggttttcttatggagtatagacgagtttggatgtgttacaataagaatgataatctgtctttgaaatgttcacagttgtttagaagttgaggacgatttgtgattgttacaggacctttagtgagaatatttcaaagtcactttttaccactttgttacaacaaaatgtagaggatgtctggtgcccttgtatcttctcccatctctggtgaactgtattgttttgtaatttgcagtggcctgaccaggaactactgcaggaatccagatgctgagattagtccttggtgttataccatggatcccaatgtcagatgggagtactgcaacctgacacaatgtccagtgacagaatcaagtgtccttgcgacgtccacggctgtttctgaacaaggtaagaagtctctggccagacaaccacacccttggacgttgggataaaaagagttgcaaaatcttagtgatacagaagccttccatgctgcacgggaatctgaatgtggactcagggtcagccaatgggaaggaagcctcagcgccttctctgggggaaccagggctgagatttttggcaccccgtgacagggtggtgtctttaggaagcgtgcagaccttctagggcactggatttaccactcccctggttattcaatagattatttcagtgtcctagtgaaaatggatattctaacatcctgccaaatttgtgatgatttaccaagctcatcatgagcctttcctggtatttcttcaagtagacagtactcattgcaaacttcagctttacagtttcagaggaatgtggtttttgagtctgtcatccttgagaaacctgatatgactttacttagttccatatcctcctgggtctaggtaacagtacatagccagcaaatgctctatctccctgtctaccttaatcttaggcaggtgctgcacacctaggctttgatggaagggatttcttagtgttcttgcccctccttctcatggaacacgtatctgtgttgctgtttgtgaagaagagtagtggatgtctactttgttgcaatgcaggatcctgggcccaagatttcccgccgtccctccaagggaataaaattttggccagtacccctctctgagagacaatgtgtctttgcctggaagtcctagatggaggaccacttcctgccccatcttccagaaacttaaggctttggctttggaggatcagtgctctggagaaatgtgtgacggtttcatgtctgcccccactgacaaccaccacctacagcctgcaccgcctgatgcatggcactctggtctcctgccttgttctcaggaacacccaaaagagatctttgccaaagaacaggcacatgagtgcaattttgactgataggcactctgatctgtcctttggtgcccaggttttaaagaaaatctttctaaaaactcattgaagttccagaatgctatgaatctttgagctttgttattggcatgtccatctgcctactaatgtagaacagagcatggtcgtcattttcagagatgatgtcctgtttctatcatggattttttttctcatgcttctgtgttctggaaattactcagtttgttttctcctctttgaatttcagcaccaacggagcaaagccccacagtccaggactgctaccatggtgatggacagagttatcgaggctcattctccaccactgttacaggaaggacatgtcagtcttggtcctctatgacaccacactggcatcagagaaccacagaatactacccaaatgggtatgtctttgagttttctcccaagagaaacagccacccacttaaatttctcctggaagagccatgcttccagctaacttcttatgacccaatttctctcagacccagaatgttggacagaatgtctcaggcttcttgctttgggcacagggtctgagaggagagaaatgtcaggccagctctcttttctcatagttgatagaagtaggaggatacttggaggtggtgaggtctcatgaatagaaagctcagaagaacatatgaccatgtgcttagaaatagcaccattccacaatgcccactaaagaccagtgaaatagttcaaccagggaattctgtcattctaatctccaagccctggagtgaaggttgtgtttgccatgtttgtcttgggtaacaagtgaaggatatctatattgacttcgagatcttccgatcactttctcctctaacctgtataaacacattgggttctgagaacaaggtgtctgaaaagctatgtgttgccagcccatgaggggcaaaaggaggaaggcagctgagagtcaggaagtatagagatgctgaagagttacacattcaggaagatggacagaaacccatgtctggctatgccagcctttctgccatgaaggactatcaaatacatgagaaaacagttttcacaggttggacaacagatatggtaggcttgagagaactgagaaagggaatcaaaggagatcaacttcatcattaacctgtcttccttcctggacacagtgttggattgaaggacaagcagatggagcccagctgaccacagcagtcttgcttaactgaggagagagactggagtctgcgatgcctcaggcagctgatgtgttctaggctggctaagaatgagaagggatttgtggaagaaaggagctccaggaatacacacagaagtctcctcaaggctttggctaaatacaaagctgcgtatgcacagggagagttttcataaagaaagaacaacaaagaaaagctacttgggaaagaacaactgcaggggaacagtaagctcaatggagatgccagagctcacatagcactgggggatatttgaattctgaccactcagaggagaaacacctcactacattttgggcattcagtagagaccaaagaaagctgtattttgggattgggatcatcttattcctagaatcaaggtgactccagaaaaactccaacaacccttcttccaagccagtctaaaaggatccaaatgatctccaagtaaattaactgcattccacaagaaaaaaaaaactcaaccccccttagaggcaagggacaaatacaagttgctcagttatatggcattcctattgcgttacttctatttaaaaatttaatagagacacaagaagctttcactgtgatacataactgggagaaaaaatcactcaacacaaacaggcccagaaattatagaattgatgacattggtgagaacatttaaaatgcacctctgagaactgtgtttcaggaaaatgtcagcaaaagctgaccatgagagaaacaaaagcagaatagcaagagaaaagaaaagaaccggagagccaaatgaaaattaaagaactgagaaaaggtacatctctaatgaagaactcactggatggccttatcatcactttagacattacggtaggaaaggtgacctagaaaataattcaataggagctacacaaatcacaggacagacagacagaccaacagacagaaacacacacacacacacacacacacacacacacacacacacacacacacaaagactgaacctattaatcaacagagcctcaagggcatctaggaaaaatccacacatttaatatatgtgttaggcaagtcacagaaggagaagaaaaagatatcatgacagacattatacttgaagcgatgatggctcgcaacacgccaaatatacagaaaacaagaaactcatagtcaagaagctaaatgactcaggtatagaattttaaagagcaaaactctatgatttactgggatatatcatagttaagttgcctcaattcaaagctaaaaagaaaaaaagggggttcctatgaacaacagctttgacagctgttgatctaagaccacagcttaaatatctaggcaaggaaaagcaaataaggcacaaggaaagaggatggaaggaaatagtccaaaccaatgacattcagtggaaaagaaaatagaccaacaaaggagtaaatccatgaaacagaaagttaggttctttgaaaagtctatatgattggccaaagtctggctaaacagatgacagaccaaggagggagcatatccatcaccatcatgagtaacaggagagagatgccattgctatagcatcctccaggtgtgaaagctgagaagtagatattgagatcaactgtatgtaaataaattcatgaatgtagatcatgtggatggattgcttaggtaaataacaaatcagcaaatcaaacactgaatagatcatgcagttttatagagacttacagacagcctgacagataaacatttgtatgtacgtgaaacaatctccaagacacacttcaaaatccctctcggttaatccaaaggaatgtatttggcagaaggtagaaggagggtattctgatcctttctggtacacattgatgttttctctcagttttcttataaagcatagattactttgaatgtgttacaataagaatcataagctgtctttgaaatgttgacagttgtttagaagttgaggaccatttgtgagtgttatgggactttagtgagaatatttcaaatttgcttgtttacactttgttacaagaaaacatagagggtgccaggtggtgctgtatcttctccaatctctggtgacctgtattgttttggaatttgcagtggcctgaccaggaactactgcaggaatccagatgctgagattcgcccttggtgttataccatggatcccagtgtcagatgggagtactgcaacctgacgcaatgtccagtgatggaatcaactctcctcacaactcccacggtggtcccagttccaagcacagagcttccttctgaagaaggtaagaagcctgcagtcagacaaccataccctcggacattgggataaaaagatttgcaaaatctttgtgatgcagaaaacttccatgctgcacaggaagtcgaaggtgaagtcatggacagccaatgggaaggaagcttcagtgccttctctggggggaccagagctgggatgttgagtgccttgtgagggatggtgtctttaaaaggggcacagaccctctaggacactggatttatcacttccctgttatcaaacgaatcatattagtgtcctagccaagatggatattctaacatcctgccaaacttgtgaagatataccaagctcctaagcctgtccagccctttcttcaagtaggcagtgtttattgcagtcttcagctttaccattttgaaggaatgccatttttgaggctgttgttcttgagaaacctaacatgtcttcattagatccgtattgtcctgagactttgaagcagtacatagccaccaaattgtttatctccccagcctaccttcatcttgggcatgccttccacacctaggatttgagggaagggatttctcagtgttctcatccctgcttctcatggaacatttatctccgttgttttttgagaagaagagtagtggatgtcagctttcttgtaatgagggatcctgggcccaagattccctgtctcccctcctaggctataaaattttggcctgtactccttctccctgagaggcaatgtgtctttacctacaagtcctagatgcaagatccttttctgccccacaccccagaatctgaaggcttttgctttggaggagcagtggtctagtgtgcaagggtttcatgtataccccccactaacagccaatcaccacctatagcctgaacagcttgatgcatggcaccctggtctcctgccttgttctcatgaacacccagaagaggtgtaagcaaaagaccattcacatgagtgtaattttgaagtataggcactctgatctgttttttgtttgtttctttgtttgtttgttttccagggttgaattaaaatatttatgactacttattaaatttctagaatcctataagtctatttgtatttttattctacatttcaatttgcatgctaatatagaagagtgtaaattgttaatcctcagattattccactttgtgtgtcataatttttttcacatttcccttttctaggcaatactgagcttgattttctcttttaatttcagcaccaactgaaaacagcactggggtccaggactgctaccgaggtgatggacagagttatcgaggcacactctccaccactatcacaggaagaacatgtcagtcttggtcgtctatgacaccacattggcatcggaggatcccattatactatccaaatgcgtatgtctatcatgttagccataaaaggaacaatagtcaactaaaatttctcttagctggcccatgctacaagctcacttcctaggtccaaatttctcatagactcagagtttgtagcaaaatgtctcaggaaacttacttttgagcaaaaggtctgaatgaagagaagttttaggattgctatctttcataacaatttgatggaagcagcaggatatatggaggtggtgaagtctcattaatgtaaagctaaggagatcaaatgaccaaatgctgagacaaagtatcattccacaatgcccactaaaggtccatgcagtctttcaaccatgcaattctatcattctatcctccattccctgaagtgaaatttgtgtttgccatttttgacacgaatcagaagtaacaaattcaggctgggtgcagtggctcaggcctgtgatcccaacactttgggaggacaagacgggcagatcaccagaggtcaggagttcaagaccagcctggctaacatggcaaaaccccatctctacgaaaaattaaaaaattagccggtcatggtggtgggtacctgtaattccaactacttgggaggctgaggcaggagaaacacttgagcctgggattcagagtttgctgtgagccgagaacatgccactgcactccagcctgggtgacagagcaagactcaatctcaaaaaaaaaaaaaaagaagaagaagaagaaaagaagaagaggaagaagaagaagaggaagaagaagaagaagaagaagaggaagaggaagaggaggaggaggaggaggaggaagaagaagaagaagaagaagaagaagaagaagaagaagaagaagaagaagaagaagaagaagaagaaaatagaaatgagtgcatatatttatatatgagtactagcctgtatgaacacactgggttctaagcaccagttttctgaagggatatgggttgtcaggcagagtaaaagcaggaatgcagatgagagtcaggaagtaaacagatgtggtgattaaaatgggcaggtacatggacaaaaaaatgcatgtctgacaaaaactggcctcttgccataagtgagtatgaataatatggaaaaactgtttgcacatgttgaacagcagacagtacaacctgagatagtttagaaagggaaacaaataagatcaaccccataattacccttcctagacttaagggcaaagagttttaaccaaagcattccacagcagtcttgctaaactggggagagagactggagttttgtttactaataaaaccgagattttctaggttaggtaataatgagaaagtatttgtggagaaaaggagctccaggaatacacacagaagtctcttcaagtctctggctgaacagaaagctgtgtatgcacagaaagagtttccagagagaaaggagaacaaagaacagctactggggaaagaacaactgctggggaacagtgagctcaatgaagatgccagagctcacatagcactgggaggtatttgagctctgaccagcctgaggagagacacttcattgaacatcttgggcattcagcaaagaccccaaaaaaccatacttcaggagtagaattaatgcattcctagaataaagtctactccagaaacaccctagaaaagcttagaaaccaagtctaaaaagatccaaatgatctccaagtaaattaattgcctgtcagaagaaaacaacctcttcagaggtaaacaacaaaattaaattgctcaattatatagtatgcacaatgtgtggcatacatttaaaaatttgctaaacatacaaaaagcatttagtgtgacccataaccaggagaaaaatcagtcaatacaaatagacccaaaaatgataaaaataacagaattggcaaggagatttaaaatgtatgtatcataattgtgttcaaggatttaaagaaagcgtggacaagaaataaataaatggataatatcaacagaaagaaaaattgtaaaaggaccaaatggagagtcaagaactgaaaaaaaagacatctctttaatgagaaaatcactacatggccttataatcatattagatagtacagatgataaagctaactagaaaatattagggtggtgcaaaccatagcacgcttatacaaagcctgagaagataaacagagcctcaaggacatctatgaaaatatcaaaatatttaatatttgtttaaagcaagtcacagaggaagggaaagagatattggaacagaaaaaatacttgaagcagtgatggctgatgactttctaaatatggaaaaaatgataaactcacatagtcaagaagctcaatggatcagatataggattttaaaaagtaaagctgtatgatttatttggacacatcataattaaattgtccataatcaaagatagaaagtaaaatcttatttgaagcccaagggaaaaaacatacctttacatagagtaacagtgacacaaatgactgatgccttctcatcagaaacaacacaaatcagaaacaatagaataacacctttagagtggtaagaagaaaaaaagatcaaatcagaaacaacaaaataacacgtttagagtggtaaggaggaaaacaagatcaaatcagaaacaatggaataacacctttagagtgtaagaaagaaaaaaagatcaaatcaggaacaacagaataacgccttcagagtggtaagaaggaaaacaagataaaatcagaaacaatgaaataacacctttagagtagtaagaagaagaaaagatcaggtcagaaaaaatggaataatatgctaagaagaaaaaaaaagatcaagtcagaaacaatggaataacacctttagagtgaaaagaaggaaaaaaacccagcaagcttaaacgctatgcacagcaaacaattccactgaaaatgaatgttacgtaagtacatattctgtcctcctaaaaacaaagaacaaataaaagaatgtttcatcagcaggattatgtaataaaagatgtgaaagaatgctatgtaagtagaagaaaaataataccatatgggaattggcatcaaaaccacaaaatactatcaaaacaaaaaaactttattgataaatttaacacaatatgcaaaagaactataccatgtatactacataacattggtgagaagaaaattagaagatctaaataaagacacatcatgcttatagattaaaaaatccaatgtcacttttcacaaaactgatctttagtttcaacccacacccaagcagaattcctgcagtcttttcttgaaaacctaacagaatgtatatgctagaatcaccaagacaatctttaaaaagaataaaaaacttggaataaaatcacaagtttgtgggatagatgcatatggtaatatggaaattctcataaagacacagtaatcaagacatgtggtattggctgggacgcttggctgtaatcctaacactttgggaggccaagatgagaggattgcctgagatgaggagttgcagacaagcctgggcaacatagcaagaccctcatctctacaaatatttaaaaaaattagccaggtttggtgccatgtgcctgtagtcccagctattcaggaagctgaggtgggaggatcactggagcccatgaggtggaggctgaaatgagccatgattgtgctactgaactttagcctgggagacagattaaaaccttccctctctctctcaaacaaacaaacaaaaaatacatagtattgggcaaaacatatgcaaacaaaaacagaaaagggtcagcataaatttacatatatggtcaatttattttcaatacaggtagcaaagcaatttaatgaggaaatttttttccaaaattggtctgaaacaactggatagccatagaaaaaaactataacaaatgtgacgcttgaatcctactgtatgactcaaattaaattaatttgagatagctcttagacctcaatgtaacagctaattctgaggctgaaatataagactgctatgaaaaagtatagtatcttataaccttggagaaggaaaaattttttgagggaagaaccagaaaacactaactgtaaaagaaaacaaatgataatgtggacattcattgaataaaaacttatgctcaccaaatatgactgttaagaaaataaataagtaagtaacacactggaagaaaaacactctcatccatatatctgacaaatggcctgtatccagagtatagaaacatttctcccactcactaatcagaggacaaacaacctaatcaaaatgggcaacaggcttgaatagtcatttcttaggagaagatgcacacagagccaacaatcacctgaaaaagtgcacaacatcttagccatcaaaaatcaagagttataaccctcataagatgacactgaacatccagtgtacatggatatcattaagaagacacaataataagtggtgtcaccgatttggagctagaatgtgccactctctcatatgctggtggaagttcaaaatcatacaacaaattaaaaaatcagtctgatgctttcttataaagttcgataaatatgcatctatcctacaaacctgtaattctattcttgaatatttaccccccaaaatgaaaacataagtccacaaaaatctatataaatattcatagcagctttatgttttataaactcaaaataaaaactatttcaatgttttcatcaaaagaaaatgaaaactatttaaatggtttcatcaaaagaaaatgaaaaaagaatttccagtatatttatacaaaggaatactattcatcaacaaggaacaagttactgatagtctcagaagcatgaacaaacctcaaaaatatattaaggaaagaagccagacgtcaaagtgtatagtctgtatgagtccattcatgtgagtttatagaaaacacaatttatggtgaaagaaaccaatagcatttgacactggccgtgggaagagggtagcagagattgattgagcagccacacaagggagtttctggggtggtgaaaatgttctgcattgtgagggcagtgtgggctacacaagtatatgtatttatcaaatctcatccagctacatttaagatctgtgcatctcactctatgtgaaaatatactcaactgaaaaacagagcaggtatctgtttcaggtgctacatcacttgatacgtccagttgtgttaaaaaccactgcctaacatcctcaaatgggggatctgggcttgagactaggtcacatgtgtagagtctctacagagaccgtgttggattcccatgctccataatacgttccaagttttctcagacagccacaggtcatgaatgtgaggattctgagaggttggagcaacgttcttgggaggcataatggggaaggcattctccaagattcctccagcctggggtcttcacctgctgtgcctcttactgcattgttttctgactcatccatagccacttgaccccttcagatcccatagtctacctagccgtctccctttatgccttgggtcccgctgttctttcaactcatcacccattccttcagtcccagagtggctgcagccagcagaggatggactgagagcaggagaggaggtcgtgcccatgaacccatcctagagaagcagcatcctgcctgggagctagttttccagggaagcttttataagtcctgtagacccaaacccacttgctctaccagatacagtatttatagtaatactattttcatgattattttatattgcaaatgtagagcatttatgctacactatgagtaaatagagtaagggggctggcatgggaattatataatcttggatgccacttcttccttggggaaatgtatttgagttccaacttacatattactatatagtcttatagagagagagacaaagagctagacagacagagatatctttgtatgtgcattaaaaaatctaagatacatatttcaaaatctgtgtcatttattctggaggaaagtatttggcagaaggtgaaaggaagatattctgatcctttcttgtacagacatgtattatctcagttttcatagagagcatatactacttttgatgttttaaaacaaaaattataatctgtgatgtgtccacagttgtttaaaagttgaagctgaagaccatttgtgcttgtggcaatattattgtggtataatgggaatatttcaaaggcacttgttaacactttgttacagcaaaatgtagagggcgctaagtgcccttgaatattctcccatctctggtgacctgtgttgttttgaaatttgcagtggcctgaccaggaactactgcaggaatccagatgctgagattcgcccttggtgttacaccatggatcccagtgtcaggtgggagtactgcaacctgacacgatgtccagtgacagaatcgagtgtcctcacaactcccacagtggccccggttccaagcacagaggctccttctgaacaaggtaagaaatttgtggttagacatctatatactgggatgaaaaaccatggaaaatcttactgatgcagaagccttcagtggtacactggagggttggttgagggtctgcaatgtggaggaaagcctcagcgccctctctgggggatccagaactgtgatttttggcacgctgtgaggaggcagtgtctttaggaagggcacggtgtctttaggaagggcacagacccgccagggcactggacttaccactcccctggttattaaatgggtcatttcagtgtcctagccaaaatggatattctaacagcctgccaaatatgtgaagatttccaagccaataagcctttccagtgatttaaagtagacttttttcattgcaatctacagtttgcagtttcttaagaacatggcctttgagtatgatatcctagagaaacctaaggagactgcattatttttctattgtcctggggctgcatagcaggaggtaaccaacgaatgctgtctctccctggcctatctcagtctttcacaggctctgttcacctcagctttgaagttagaaatttctaggtgttcttgcctcttcttctcatgaaacctgcattggcagtgagtctacagaagaagaggaagagaattctgctttgttacaattcaggactctgggcactagaagattccctatctctcctccaagggaataagttgtttgtctctaaccctccttgagaaacaatgagtctttgcctgcactcctaaatgtaggatgatttcctgcccaaattttcaaaagattaagccttttgccttggtatgagcaatggtctagggaaatgcgcaagggtcttgtgtcggcccctgactgaccaccagtcacctcctacagcctgcaccaaggaatgcattgcattctggtcttctgccctgtggttctcatgaaaaccagcagagattcatatgatggagctgcacatgaatgtaatttccaatgtccagcattctcctctgttctttatctttagatttaaaaataatgtttctatgaacttattaaaattctagaatactatgaatctactgggtcttttcacatccttttgctactagtagaaaaaagaatagtaataattttcagaggctactgtccagtatgtgacataaattgtctcccatgtttctctgctcatgcaattactgagtatgatttattttattttaatttcagcaccacctgagaaaagccctgtggtccaggattgctaccatggtgatggacggagttatcgaggcatatcctccaccactgtcacaggaaggacctgtcaatcttggtcatctatgataccacactggcatcagaggaccccagaaaactacccaaatgcgtatgtatttgattaaaaccataagaggagcaacagccaactcaaatattggttagaagacccatgctttaagctcacttcctagggacaaatttctcttagactcacattttggcaaaatgtctcaggacctttgcttttgagcaaagagtctaagagaagagaaattttaggcctgctatttttcctaatagttttatggaaggagtagaatatacggaagtggcgaagtcatattaatgtaaagctcagaagataaatgaccaaagcttaaacacagcaccattccacaatgcccactaaaaatcaatgtcatctttcactcgtgcaattctgtcattctaaatttcaattcccgaaggtttgtttgccatttttgtcatgggtaataagtaaaaaaaaaaaaattaagatgtgtatatatatatatatatatatatatatacacacacacacacacacacaaacatctgaatatttatatatatgtctgaatatttatatacttgtgtataaaacttatatttaaatttttgcataaatttatatatttttaatatttcattaaaaattatattgtttcactatgtatgtctgagtatttttatatattttaatataacattttaaatatttatatataaatattcaggtatgtaactgaatattcatttacacacacaaatatatgtgtgcatgtgtgtatatatatatatacccatatatatatatatatatatatatacatatatatatatatatatatatgtatatatatatatatatatatatatacacacacacacacacacacatacatacaggtataaacacactgggcctgaagcaccagtggtctgaaaggacatgtgttgccaggacttgaagagcaaaagcaggaaggcggatgagagtcaggaggtacacaaacgctgaaaagtaaaatggacaagtacatggacaaaaagcaggtataagcataacagccttttggaagtaaatgactataaaatatatgaaaatactgttttcacaagttgcacaacagatagtagtgtattgagataatttagaacagaaaacaaatgtgatcaaccccataagtgtgctgtatttcatcatggattgaaggaaaaagagatggagcccaagaagaccacagcagtcttgatgaactgagagacaccagagtttgggattacaaaggcagctgggattttctacacttggtaataatgagaaagaatttgtggagataaagagctacagtcatgtacctagaagtcacctcagtgtaatataaatctgcatatgcacagggagtgattccacaatgaaagtaggacaaagaacagctactggggaaagaataactacaagggaacaatgagttcaatggagatggcagagctcacaaagcactgggggatatttgagttcttaccagctagaaaagagacctcattgcaaatcttgggcattcagtagagaccccagaaaagccactctttggaaacagagttgatgtattttaagagcaaaatctactccacaaaaatcctagcaaaattgaaaagcaagtcagaaagaccaaaatcctctcaacataaattagttgcccatcagaagaaagcttaacctcttcataggtaaacaataaaatcaaattgctcagttatctggcatccacaatatgtgacataaatttaaaaatttactagacatacaagaagcatttagtgtgatccataaccaggagaaaaatcattcaatacaaatagacccagaaatgacagaaatgatagaattagcaaaaacatttaaaatatacatatgatcatttgatcttgtgatcagatatcacaagagaagaaagagatacttgaacagaaaaaatgcctgaagcaatgatggctgaaaactttccaaatatgaagaaaaaaaagctcacagattcaagaaaactaatcaatcagaaatatgattttgaaaagtaaaaatgtatgatttactttggcaaatcttcttggttaaattgtctaaaatcaaagaaagctaggaaaattttataagccagaggaaaaaagattgtttatataaaggaacagttacacaaatgactgatgccttctcatcagaaacaatgaaagtcagaaacaataaagtaacatctttaaagtaatagaagaaaaacccaagaggtgagggatcgtggcagacaggaggcaggactagattgcagctctggacagagcagcatgcagaggctcatattgtgaattttagccccatattgactgcaagaacagaccagcaatcctgagaggacccacagaccgtgtgaaggaagcagactgctcctgcaggataagggagacaccccaaatactgtgagttccccaactgcagaagtggaaaagggaggccttactccctcaaacacaccccacaactggagaagctgaaagtctgtttgcaggagaagttcccaactttacctgggcctcagtaaatttagagagctgagccaagcaaaatataggggtagaggaagcagcagagaagacctcagagcttgctggatccccaagcagctcattcctgcctggcaccacagagatccatcagaagtgtggccaaaggaacagagggtaaaactccacatggaggactgctctacctgaactttctaacaatttgaacagggggagaagcctcctggccagaacttgggggagggcatgaatctggtttgcagacttcacaggtgggggaaggactaaagcccttttctttcacagctgggaggtggaaagcctcaggcaagttttcaagcctgactttccccccacctggaaacagacttggagctgttgcggggttgggggcatggtgggagtaagaccagcccttcagtttgcatgggtgctgggtgaggcctgtgactgacagcttccctccacttccccgacaactcagatgactcagcagaggcagccataatcctcctaggtacacaactccagtgacctgggaacttcacccccacaccatacagaagcttcagtaagacgtgcccaaggaaagtctgagctcagacacgcctagtcccacccccaactgatggtccttccctacccaccctggtagcagaagacaaagagcatataatctttggagttctagggcccacccacctctagtccctctccacactagtatagctgatgcaggaggccaaccagcacaaaaatagagcattaaaccaccaaagctaggaacccctatggagtccattgcaccctcctccacctccaccagaacaggcactggtatccacagctgagagacccatagatggttcacatcacaggactctgtacagacagtccccagtaccagcccagagctgggtagacttgctaggtggcaagacccagaagacaggcaataatcactgcagttcagctcacaggaagccacatccataggaaaagagggagagtactacatcaagggaacaccccatgggataaaaacatctgaacaacagccttcagccctaccttccctctgacacagtctacccaaatgagaaggaaccagaaaaccaaccctggtaatatgacaaaacaaggctcatcacactcccagttcaccagcaatggatccaaaccaagaagaaatccctgatttacctgaaagagaattcaggaggttagttattaagctaatcagggagggaccagagaaaggcaaagcccaatgcaaggaaatccaaaaaaaaaaaggtataagaagtaaaaggtgaaatattcaacaaaatagatagcttaataaaaaaacaataaaaaattcagtagactttggacacacctttggaaatgtgacatgctctggaaagtctcagcaatagaactgaacaagtagaaaaaataaattcagagctcaaagacaaggacttcaaattaacccaatccaacaaagacaaagaataaaggataagaaaatatgaacaaagccttcaagatgtctgggattatgttaaatgaccaaatataagaataatcgtggctcctgaggaaaaagacaatactaaaagcttggaaaacatatttgggggaataactggggaaaacttacctggccttgctggacacctagacatgcaaatacaagaaacacaaagaacatgtaaatacaagcagcacaaagaacacctgggaaattcatcacaaaaagatcttagcctaggcacattctcatcaggttatgcaaagttaagacgaaggcaagaatcttaagagctgtgagacagaagcaccaggtaatgtataaaggaaaccctatcagattaacagccagtttttcagcaggaactgtacaagctataaaggattggagccctatcatagcctcctcaaacaaaacaattatcagtcaagaattttgtatccagcgaaagtaagcatcatatatgaaggaaagatacagtcgtttttggacaaacaaatgctaagagaattcaccattaccaagtcaccactagaagaactgctaaaaggagctctaaatcttgaaacaaatcctagaaacacatgaaaacagaatctctttaaagcataaatcacacaggacctataaaacaaaagtacaagttaaaaaacaaaaacaaaaaacaaaaccaaagtacggaggcaataaagaatatgatgaatgcagtggcacctcacatttcaatgctaaaattgaatctaaatggcctaaatgctccacttaaaggatacaaaaagagttggtggctggcaagatggctgaataggaacagctccagtctgccgctccccgtgagatcaacacatagggtgggtcatttctgcatttccaaccaaggtacccggctcatctcattgggactggttagacagtgggtgcagcccacagagggtgacctgaagcagggtggggtgtcacctcacctgggaagtggaaggggtcagggaactccctcccctagccaaaggaagccgtgagggactgtgccgtgaagaccagtgcattctggcacaaatactatgcttttcccacggtctttgcaacctgaagaccaggagattcccttgggtgcctacaccaccagggccctggatttcaagcccaaaactgggctggcatttgggcagacactaagctagctgcaggagttttttttcataccccagtggtccctggaatgccagcaagacagaaccattcacccccgtgaagaaagggctgaagccagggagctaagtggtctttctcagtggatcccacccccatggagcccagcaagctaagctccactggcttgaaattcttgctgccagcacagcagtctgaagttgacctgggacgctcaagcttggtgggaggaggggtatccacaaatactggggcttgagtaggaggttttcccctcacagtgtaagcaaaaccgctaggaagtttgaactgggcagggtgcactgcagcttggcaaagccattgtagcaagagtgcctctctagattcctcctctctgggcagggcatctctgaaagaaaggcagcagccccagtcagaagcttatagataaaactcccatctccctgggacagagcaactggaggaaggggtggctgtgagtgcagctccagcagacttagtttcctgcctgccagctctgaaaagagcaccagatcccccaacacagcactagagctctgataagggacagactgcctcctcaagtgggtcctggtttcagaagataataagaaactcctctgagctaaaggagcatgttctaacacaatgcaaggaagctaagaaccttgaaaaaggtcagaggaattgctaactacagtaagcagtttagagaagaacataaatgaccttagggagctgaaaaacacagcacgagaacttcatgacacatacacaagtatcaatagcaaaatcgatcaagtggaagaaaggatatcagagattgaaaatcaacttaatgaagtaaagcgtgaaaacaagattaaggaataaagaatgaaaaggaatgaacaaatcctccaagtatgggactatgtgaaaagattgaacctacgtttgattggtgtacctgaaagtgatgggagaatggaaccaagttggaaaacactcttcaggatattatccaggagaacttccccaacctagcaagacaggccaacattcaaattaaggaaatacagagaataccacattcaaattcaggaaatacagagaacaccacaaagatactcctcaagaagagcaacctgaagacacataatcgtcagattcaccaaggttgaaatgaaggaaaaaaatgttgagggcagccagagagaaagtttgggttacccacaaagggaaccccatcagactaacagtggatcttcctgcagaaactctacaagccagaagagagtgggaggccaatattcaacattcttttttactattattatactttaagttctagggtacatgtgcacaaggtgcaggtttgttacatatgtatacatgtgccatgttggtgtgctgcacccattaactcttcatttacattaggtatatctcctaatactatccctccccactccccccatcccatgacaggccccggtgtgtgatgttccccactctgtgtccatgtactctcattgttcaattcccacctatgagtgagaacattcggtgtttggatttctgtccttgtgatagtttgctgagaatgatggtttccagcttcatccacatccctacaaaggacatgaagtcatccttctttatggctgcatagtattccatggtgtatatgtgccacattttcttaatccagtctaccattgatggacgtttgtgttggttccaagtctttgctattgtgaatagtgccgcaataaacatatgtgtgcatgtgtctttatagcagcatgatttataatcctttagatatatatccagtaattgtatggctgtgtcaaatggtatttctagttctaaatccttgaggaatcaccgcactgtcttccacaatggttgaactagtttacagtcccaccaccagtgtaaaaatgttcctatttctccacatcctctctagcatctgttgtttcctgactttttaatgatcaccattctaactggtatgagatggtatctcattgtggttttgatttgcatttctctgatggccagtgatggtgagcactttttcatgtgtctcttgactgcataaaagttttcttttgagaattgtctgttaatatcctttgccaactttttgatggggttgtttgattttttttcttgtaaatttgtttatgttctttgtagattctggatattagccctttgtcagatgggtagattgtaaaaattttctcccattctgtagcttgcctgttcattctgagggtagtttcttttgctgtgcagaagctctttagtttaattagatcccattggtcaattttggcttttgttgctattgcttttggtgatttagtcatgaagtccttgcccatgcctatgtcctgaatggtattgcttaggttttcttctagggtttatatggttttaggtctaacatttaagtctttaatccatcttgaattaatttttatataaggtgtaaggaagggatccagtttcagctttctacatatggctaggcagttttcccagcaccatgtattaaatagggaaacctttccctatttcttgtttttgtcaggtttgtcatagatcagatggttgtagatgtgtggtattatttctgagggctctgttctgttccattggtctatatctctgttttggtaccagtaccatgctgttttggttactgtagccttgtaatgtagtttgaagtcaggcagagtgatgcctccagctttgcttttttggcttaggattgtcttggcaatgcatgctcttttttgttccatatgaactttaaagtagttttttccaattctgtgaagaaagtcattggtagcttgatggggatggcattgaatctataaattaccttaggcagtatggccattttcacaatattgattcttcctatccatgagcatggaatgttcttccatttgtttgtgtcctcttttatttcattaagcagtggtttgtagttctccttgaagaggtccttcccatcccttgtaagttggattcctaggtattttattctctttgaagcaattgtgaatgggagttcatccatgtccctacaaaggacatgaagtcatgtatgggaatgcttgtgatttttgcacattgattttgtatcttgagactttgctgaagttgcttatcagcttaaggagattttggtctgagaagatggggttttctaaatatacaatcatgtcatctgcaaacagggacaatttaacttcctcttttcctaactgaataccctttatttccttctcctgcctaattgccctggccagaacttccaacactatgttgaataggagtggtgagagagggcatccctgtcttgtgccagttttcaaagggaatgcttccagtttttgcccattcagtatgatattggctatgggtttgtcataaatagctcttattattttgagatatgtcccatcaatacatagtttattgagagttcagcatggagagctgttgaattttgtcaaaggccttttctgcatctattgagataatcatgtggtttttgtctttggttctgtttatatgatggattacatttattgatttgcatatgttgaaccagccttgcatcccagggataaagccaacttgatcatggtggataagctttttgatgtgctgctggattcggtttgccagtattttattgaggatttttgcatcaatgttcatcatggatgttggtctaaaattctcatttttgttgtgtctctgccaggatttggtatcaggatgatgctggcctcataaaatgagttagggaggattccctctttttctatgattggaatagtttcagaagaattggtaccagctcctctttgtatctgtggtagaattcggctatgaatctctcctggactttttttggttggtaggctcttaattattgcctcaatttcagagcctgttattggtctattcaaggattcaatttctttctggtttagtcttggtagggtgtatgtgtccaggaatttttccatttcttctagattttctagtttatttgcacagaggtgtttataatattctctgatggtagtttgtatttctgtgggattggtagtgatatcccctttatcattttttattgcatctatttgattcttctctcttttcttctttattagtcttgctagtggtctatcaattttgttgatcttttcaaaaaaccagctcctggattcattgatgttttgaaggtttttttgtgtctctatctccttcagttctgctctggtcttagttatttcttgccttctgctagctttttaatgtgtttgctcttgcttctctagttcttttaatggtgatgttagggtgtcaattttagatctttcctgctttctcttgtgggcatttagtgctgtaaatctccccctacacactgctttaaatgtgtcccagagattctggtatgttgtgtctttgttgtcattggtttcaaagaatatctttatttctgccttcatttcgttacatacccagtagtcactcaggtgcaggttgttcagtttccatatagttgagcagtttttaatgagtttcttaatcctgagtcctagtttgattgcactgtggtctgagagacagtttgttataatttctgttcttttacatttgctgaggaatgcctcacttccaactatctggtcaatttcagaataagtgcgatgtggtgctgagaagaatgtatattctgttgatttggggtggagagttctgtagatgtctattaggtctgcttggtgcagagctgagttcaattcctggatatccatgttaactttctgtctcattgatctgtctaatgttgacagtggggtgttaaagtctcccattattattgtgtgggagtctaagtctctttgtaggtctctaaggacttgctttatgaatctaggtgctcctgtattgggtgcatatatatttaggatagttagctcttcttgttaaattggtccctttaccattatgtaatggccttctttgtctcttttgatctttgttagtttaaagtctgttttatcagagactaggattgcaacccctgctttttttgttgttttccatttgcttggtagatcttcctccatccctttattttgagcctatgtgtgtctctgcacgtgagatgtgtcttcagaatacagcacactgatggatcttgactctttatccaattttccagtctgtgtcttttaattggagcatttagcccatttacatttaaggttaatatttttatgtgtgaatttgatcctgtcatcatgatgttcgctggttattttgctcattagttgatgcagtttcttcctagcatcgatggtttttacaatttggcatgtttgtgcagtggctgataccgattgtttctttccatgtttagtgcttccttcaggagctcttgtaaggcaggcctggtggtgacaaaatctctcagcatttgcttgtctgtaaaggattttatttctccttcacttatgaagcttagtttggctggatatgatattctcagttgaaaattcttttctttaagaatgttgaatattggctgccactctcttctggcttgtagagtttctgctgagagatctgctgttagtctgatgggcttccctttgtgggtaacccgacctttctggtgaatctgacaattatgtgtcttggagttactcttctcgaggagtatttttgtggcattctctgtatttcctgaatttgaatgttggcctgcctttgtaggttggggaagttctcctggataatatcctgaagagtgttttccaacttggttccattctcctcgtcactttcaggtacaccaagcagatgtagatttggtcttttcacatagtcccatatttattggaggctttgttcatttctttttactcctttttttctctaaacttctcttctcgcttcatttcattcatttgatctttaatcactgataccctttcttccacttgattgaatcaactactgaaacttgttcatgtgtcacgtagttctcgtgccatggttttcagctccattagatcatttaaggtcttctctatgctgtttattttagtctgccattcatctaaactttttcaaggtttttagcttctttgcaatgggttcgaacatccttctttagctcggagaaatttgttattacagatcgtctgaagccttcttctctcaactcatcaaagtcattctctgtccagctttgttctgttgctcgtgaggagctgcgttccttcggaggagaagaggcaccctgatttttagaattttcagctgttctgctctggtttctccccatctttgtggtttatctacctttggttcttgatgatggtgatgtacagatggggttttggtgtggatgtcttttctgtttgttagttttccttctaacagtcaggaccctcagctgcaggtctgttggagtttgctggaggtccactccagtccctgtttgcctgggtattaccagtggaggctgcagaacagcaaatattacagaacagcaaatgttgctgcctgattcttcctctggaagcttcatctcagaggggcacccagctgtatgaggtgtcagttggcccctactgggaggtgtcccccagttaggctactcgggggtcacggacccacttgaggaggcagtctgtccattctcagatctcaaactctctgctgggagaaccactactctcttcaaagctgtcagacagggatgtttaagtctgcagaagtttctgctgccttttgttcagctatgccctgcccccagaggtggagtctacagaggcaggcaggtctccttgagctgtggtgggctccacccagtttgagcttcctggtcgctttgtttacctactcaagtctcagcaatggcagacgcccctcccccagctttgctgccgccttgcagttcggtctcagactactgtgctagcagttcaatctcagactgctgtactagcagtgagcaaggctctgtgggcatgggaccctctgagccatgtgcaggatataatctcctggtgtgccgtttgctaagaccattggaaaagtgcaatattagggtgggagtgtcccgattttccgggtacatctgtcatggcttcccttggctaggaaagggaattccctgaccccttacacttcccgggtgaggcaatatcccgccttgcttcggctcactctccgtgggctgcacccactgtctgacaagccccggtgagatgaacccagtacctcagctggaaatgcagaaaccacccatcttctgctttgctcatgctgggaactgtggactggagctgttcctattcggccatcttgaaacctcccctctctcacgatcacaaggtcccacaataggccgtctgcaggctgaggagcaagaaaagccagtctgaattccaaaactgaagaaattggagtctgatgttcaagggcaggaaacatccagtgccaaagaaagatgtagaatattcaacattcttaaagaaaataattttcaacctagaatttcatatccagccaaactaagctttataacaaaggagaagtaaaatcctttacaaacaagcaaatgctgaggaattttgtcaacaccaggcctgccttacaagaggtcctgaagaaaacactaaatatggaaaggaaaaaccagtaacagctactgcaaaaacataccaaattgtaaacaccatcaacactataaagaaactgcatcaactaatgggcaaaatagccagctagcatcataatgacaggatcaaattcacacataacaatattaaccttaaatgtaaatgggctaaatgccccaattaaaagacacagactgggaaattgaataaagagtcaagacccattggtttgctgtgttcagaagacccatctcagggtgaaaagacatacatgggctcaaaataaagaaatgaaggaatatttaccaagcaaatggaaagaaaaaaaaagcagcggttgcaatcttagtctttgatgaaacagactttaaaccatcaaagatcaaaagagacaaaggagggcattacctaatggtaaaagtatcaatgcaacaagaagatctgactgtcctacttatatatgcacccaatacaggagcacccagattaataaagcaagttcttagagacctacaaagagacttagacttccacacaaaaatagtgggagactttaacaccccacagccaatattagatcgacgtgacagaaaattaacaaggatattcaggacgtgaattcagctctggaccaagctgacctaatagacatctacagaactcgacaccacaaatcaacagaatatacattcttctcagcaccacattgcacttattctaaaattgaccacataattggaagtaaaacacttctcagcaaatgccgtagaatggaaatcataacaaacagtctctcagaccaaagtgcaatcaaactagaactcaggattaataaactcactcaaaaccacacaactatatggaaactgaacaacctgctcctgaattactactgggtaaataacaaaattaaggcagaagtagataagttcttagaaaccaaagagaacaaagacacaatgtgccagaatctctggtacacagctaaagccatgtttagagggaaatttatagcactaaatgcccacaggagaaagcgggaaagatctaaaatcaacaccctaacatcacaattcaaagaaccagagaagcaagagcaaacaaatacaaaagctagcagaagacaagaaataactaagatcagagcagaactgaaggggataaagacacgaaaaccctttaaaaaattaataaatccaagagctggttttttgaaaagattaacaaaatacatagaagcctagccagactaataaagaagaaaatagagaagaatcaaatagacacaataaagaataataaaggggatatcaccaatgatgccacagaaatacaaactaccatcagagaatactttaaacacctctatgcaaataaaatagaaaatctaaaagaaatggataaattcctggacacatacaccctcccaagactaaaccaggaagaagtcaaatccctgaatagaccaataacaagttctgaaatcgaggcagtaattaatagcttaccaaccaaaaaaagcccagaccagagggattaacagtcaaatcctaacagaggtacaaagaagagctagtactattccttctgaaactattccacacaatagaaaaagagggactcctgcctaactcattttatgaggccagcatcattctgataccaaaacctggcagagacacaacaagaaaagaaaatttcaggccaacatccctgatgaacatcaatgtgaaaatcctcaataaaatactggcaaactgaatccagcagcacatcaaaaagcttatccaccatgatcaagttggcttcatccctgggatgcaaggctggttcaacatattcaaatcaataaacataatccatcacataaacagaaccaatgacaaaaaccgtatgattatcgcaatagacgcagaaaaggcctttgataaaattcaatacccaatcatgctaaaaactcttaataaactaggtattgatggagcatgtctcaaaataataagagctacttatgacaaatgcatagccaatatcatactgaatgagcagaagctggaagcattccctttgaaaaccagcacaagacaaggatgccctctctcaccactcctattcaacatagtattggaaattctgtccagggcaatcaggcaagagaaagaaataaaggtattcaagtgggaagagagggagtcaaattatttctctttgcagatgacatgattgtatatttagaaaactctatcatctcagcccaaaatctccttaagctgataagcaacttcagcaaagtctcaggatacaaaatcaatgtgcaaaaatcacaagcattcctatacaccaataagagacacagagccaaatcctgagtgaattcccattcacaattgctacaaagagaataaaatatacctaggaatccaacttacaagggatgtgaaggacctcttcaaggagaactacaaaccactgctcaaggaaataagataggacacaaacaaatggaaaaacattccatgctaatggattggaagaatcaatattgtgaaaattgccatactgcccaaagtgatttatagattcaatgttatccccatcaagctaccattgatttcttcacataattagaaaaaactactttcaatttcatatggaatagaaaaagggcctgtatatccaagacaacctaagcaaaaagaacaaagctggaggcatcatgctatctgacttcaaaatatactacaaggctacagtaacaaaaacagcatggtatggtactggtaccaaaacagatatatagaccaatagaacagaacagaggcctcagaaataacaccacacatctacaactattggatctttgacaaactggacaaaaataagcaatggggaaaggattccctatttaataaatggtgttgggaaaactggctagccatatgcagaaaactgaaactggatcccttccttacaccttatacacaaattaactcaagatagattaaagaattaaatgtaagacctaaaaccataaaaaccctagaagacactttgggaggccgaggtggatggatcacgaggtcaggagatcgagaccatcttggctaacacagtgaaagcccatctctactaaaaatacaaaaaattagctgggtgtggtcgtgggcacctgtagtcccagctacttgggaggctgaggcaggagaatggcatgagctgaggaggttgagcttgcagcaagccaagattgtgccactgcactccagcctgggcaacagagtgagactccatcaaaaaaacaaaaacaaaaacaaaaaatcaaaccctagaagaaaacataggcaataccattcaggacataggcatgggagaagacttcatgactaaaacagcaaaaccaatggcaacaaaagccaaaatttacaaatcagatctaattaaaataaagagcttctgcacagcaaaaaactctcatcagagtgaaaaagcaacctatggagaaaaattctgtggtctagccatctgacaaagggctaatgtttagaatgtacaagcaacttaaacaaatgtacaagaaaaaaaaaacaaccccatcaaaaagtgggcaaaggatatgaacagacacttctgacaggaagacctttatgtggctgacaaacatgaaaaaagctcatcatcactgttaattagagaaatgcaaatcgaaaccacaatgagataccatctcatgcccgttagaatggcgatcattaaaaagtcaggaaacaacagatgctgaagaggatgtgtggagaaagaggaacacatttacactgttggtgggagtgtaaattagttcaaccattgtggaagacagtgcggtgattcctcaaggatctagaaccagaagtaccatttgacccagcaatcccattactgggtatatacccaaaggattataaatcattctacaataaagacacatgcacacgtatgtttattgtagcactattcacaatagcaaagacttggaaccaactgaaatgcccatcaatgatagactggataaagaaaatgtggcacatatacactgtggaatactatgcagccataaaacaggatgagttcatgtcttttgcagggacatggatgaagctggaaaccatcattctcagcaaactaacacaagaacagaaaaccaaacaccatatgttctcactcataagtgtgagttgaacaatgagaacacatggacacaggaaggggaacatcacacacaggggcctgttggggagttgaggctaggggagggattggattaggagaaatacctaatgtagatgatgggttgctgggtgcagcaaaccaccatgacacgtgtatacctatgtaacaaacccacacattctacacatgtatctcagaacttaaagtataataataataagatacagaactgcagaatgaataagaactcaccaaccatctgctgccttcaggagactcatttaagacataaggactcacataaacttaaagtaaatgggtggaaataataataagtggtgtcactgatgtggaggtagattataaaactcttatcatatgctggtggaagatcaaaatgataaaacgaattaaaaaatcagtcagatggtttcttaaaaagttccatcaatatgcctctatcttacaaacctgcaattctattcctgaatctttatcccaaggaaatgaaaaagtaagtccacaaagagttctatatgaatatttataggagctttatttattataattcaaactgtaaaaataatttcaatgttcatcaataacaaaatgaaaaaataatttgcaacctactggtacacttgaatactattcagcactgagtatcttaaatagcatggatggagctcaaaaatatactcaggaaagaagccatgtatattctgtatgagttcatttacatgagatcatttacatttcctccaaaagaggaaaaactaatttctgttgaaagaaaccaatgtatttgcctctggcagtggtaagggggtagcacagattaattgggtagggactcaagagagtttctggggtcacagaaatgttccgtgtggtgatgggagtttgggctccacaggtataggtgttgatccaaaatcatcaaaaaaacaacattgcagatctgtgcatctcactctgtgggaaagtatatctcaactgtaaaaagggcagaaattgcttttaaacgctcagccttttagcacatccagttgcttggagaaccagcttactcaaatgggggtctaggctggagactaggtcacaggcatagagtctctaaactttcccatggcacataatacgtttcaggttttctcagagagctgcaggttagtaatctgaggattctgacaagttgggtcaacgttcctaggaggcatgaatgggagtgcattctctaagatccctccaccccagggtccttgctttctgtgcctcttactccattgttttctgactcctctgtagccactcgacctcttcagatcccattgtctacccagccatcgccctttatgacttgggtcccactgttctttcatctcatcctccattccctcagtttcggagtggctgccgctagcagaggatggactgagagcaggagaggtggtcctgcccaggaacccatcctagagaaatggcatcctgtctgggagctagttttttagggcaggttttataagtcttgtaaagccagacacacttgatctacctggtatgttatttacagtaatactattttcataattgcttttcactctaaaagtagagccttttagctacactgtgagtaaataaaggggctggcctgggaatggtatcatgttggatgttgtttcttccctgaagtaatatatatcagttacaatttacatgttactgcagagtcctagagagagacacagagaatgagacagataccaatacatttttatgtgcattaaaaaaatctaaggccaggcgcagtggctcacacctgtaatcccagcactttgggaggccgaggtgggtggatcacgaggtcaggagattgagaccatcctggctaacacggtgaaaccctgtctctactaaaaatacaaaaaattagccaggcgtggtggcgggcgcctgtagtcccagctactcaggagactgaggcaggagaatggcttgaacccaggaggcagaccttgcagtgagccgagattgcgccactgcactccagtctgggcgacagagcgagactccgtcacaaaaaaaaaaaaaaatctaaaatgcactcttcaaaatctatgtcatttattctggaggaatgcagttggcagaaggaggaagatattccgaatttttcttgtatacatttatgtatgatctcagtttttttatggatcatagaccaattttgatattttaaaataaaaattataatctatcttggaaatttacatggttctttagaacttgaggaccgtttttgcttttcggaatattattgtacctaaaatgggaatattacaacgtcactttttaacactttgttataacaaagtttagacagcgctgggtgcccctgaattttttcccgcctcttgtgacctgtgttgttttggaatttgcagtggcctgaccgagaactactgcaggaatccagattctgggaaacaaccctggtgttacacaaccgatccgtgtgtgaggtgggagtactgcaatctgacacaatgctcagaaacagaatcaggtgtcctagagactcccactgttgttccagttccaagcatggaggctcattctgaagcaggtaagaagtctgtggccagatatctacacatttgaacattgggatgaaaagagatggaaaatctgactgatgcagaagccttccatgctacacagaaacttgagggtatggcaggtggaaagaagcctcagcactctctctggtggagcaatttttggcgcaacgtgcgtgggcggtgacttcaggaatggtgcaaacccacctgggcacttgacttaccactcactttgttatgaaaggggttatctcggtgttccagacaaaattccaattctaacatcaggccaaatttgtgccaaatttcacactagtgagtgtttccaggcatttattaaaatggacagtgttcattgcaatcttcagcattgcagttgctgaggtatgtggccgctgagtttgtcatcctggggaaacctaatatgatgatatttattccatctaatcctggggctatttggcagtaaataccacagaatacactatttctctggcttatttcagtcttaggtaggctctgcacacctatgcttggaaggcaggaatttcttggtgttcttgtgccttcttctcatggaacgtgcatctttggtgtgtgttgagaggaagggtagtagacttctgctttgttgcaatgcaggatgctggaacaagaggattccctgtctctactgtaagggaataagattttagcctccatccttctctaagaagcaatgtgtctttgcctccaagtactagatgcaggaccatgaactgccccgtccaccagaagcttaaggctttggcttttcaggagcaatcatctagggaactgtgcagggttttcatgtctgtcccctactgacagccaatcaccatacagcctgcataacctaatccatcatcgtctggtttcctgcctcattgttttcatgaacaaccagtagagagccatacgaaagagcttgcacatgagtctttgttccaattgtaagagcactgataggtccttttcccaccaggttttgaatataaaatttctaagaacttattaaaatattagaatgttattaatctattgtttttgcttcagcatgtccttctgcttgtgagtatactaaagagaacagtcataattctgaaactactgtcctgtttgtgtcataaattgcttcacatgtttctgcatactagtagttactcagcttgattttgtctattttcagcaccaactgagcaaacccctgtggtccggcagtgctaccatggtaatggccagagttatcgaggcacattctccaccactgtcacaggaaggacatgtcaatcttggtcatccatgacaccacaccggcatcagaggaccccagaaaactacccaaatgagtatgtctttgatgttacttgtaagaggagcaacagccaacttaagttcctcctagaagagccttgcttcaagctaacttgttaggacaaatttcccttagacccagaaggtgtgtcaaaatgtccagacaactttgcttttgatcaaagagtctgagagaataggtattttaggcttgctatcttttctaatagtctgatggaagcagaaggctacatggagctgatgaggtctttttaatataaagctcaagagatcaaatgatcaaatacttagagtgccattctacaaggctcataaaagatcaatgcactctttcacccatgcaattctatcattctaacctcccttctctgaaatgaaggctttttgccatttttgtcatgggtcacaagtaaataattcacatgtatatgagtatatatataaccaggtgtgtttattcagactagtatgtatatatatacatatatatgttcatataagttagtattcatatatatgttcatatatatatgttcatacagactagtattcatatatatatacatatatatatacacacacatatatatatatatatatatgttctagggaaacatgcaaggtttttatgtctgtccctgactgatgaccaaataccctatagcctgcacagctgcaagctgtatagccatacaatttgcaggacacacacacatacacacacacacacacacacacacacactaacatataatataatataatataatataatataatataatataatataatataattaatatatataaacctgtgtgaacacactgggttctaagctccagttttctgaagggatatgggttgccaggagaggaagagcaaaagcaagaatgtagatgagaattaggaagtaaacagatatggagattaaaatgggcaggtacatggacaaaaaaccaggtctgacaaaaactggctttctgccataaatgactataaaagatattaaaaaacactttccacatgttggacaagagacagtacaggactgagataatttagaaaaggaaatgaatgagcgcaactccgtaactattatgactttcttcctggagaaccttcctggactgaagggcaaggaattggagccaaagccaaccacagcagtcttgctgaactgaggaaagagactggagtttgggatagctaagaaaatgtgtattttctatgctaggtaataatgagaaagaatttgtggtgaaaaggagctgaaggaatatgcatggaagtctaatataaactgcatatgcacagggagaaattctacaaagtgggacagagaaccactactggggaaaggacaaattcagggaaacagtgagctcaatggtgacgccagagctcacgtagcactgggggataccggggttctgatcagcccgaggagagacacctcattgaacatctcgggcattcagtagagaccccagaaaagtcatactttaggagtaggatttatgccttcttagaataaagactaccccagaaacaccctagtaaagcttaaaaaccaagtctaaaaggacccaaatgatctccaagtaaattaactgcctgacagaagaaaactcaaccatcactggaggtaaataacatgattacagtgctctgtaatgttgcattcacaaggagtgacatcatttaaaaatttatgaggcaggaaaaagcaattagtgtgatccataactaggagaaaaaccagtcaatacaaatagaccaagaaatagtagaaacgatggaattgacaaagaaattaaaactgtatatatgataattgtgttcaaagatttaaagaaaacatgaacatgagggaaacaaatgcagaatataaaaaaaagcaaatgcgtaaaacaaccaaatggaaattaaagaactacaaaaaagtataaccttaataaaatactcactggatggccttaatattagtttatacattacagaagaaaaagtgaaccagaagataactcaatgaaagccatacaatctgtaagacacacacacacgcacacgcgcgcgcgcgcacacacacacacacacagagagagagagagagagaaagagagagagagaaaggctgaaaaaaataaatagaaccttaaggatatcagtgaaaatagcaaaagatttaatatatgggtaaagcaagtcacagaaggacgggaaggagatattgggacagaaaaaaatactcaaagcaatgatggctgaagactttacacgtatgaagaaaatgataaactcacagtcaagaagctcaatgaatcagaaatagtatttttaaaagcaaaactctatgatttacttgggtacattatagataaatcgtccaacatcaaagataacaaggataatcttataagccagaggaaaacaatatcatttacatagagggacagtaatgaaagtgaccgatgccttctccttggaaacaatggcataacatctttaaagtgataaagagaaataaaaacagatcaacctaggacgacatgtccagccaaaacaaacaaataaacaaaaaaaccctttaaaataaacgtgatgtaaatacgtattctgccacctccagaggaaacaagcaaaaaaacaaaagaatgtttccaaggcaggcttctgtattaaaagattttaaggaaagttattcaggtagaagaaaaataataccagatgggaactttaatccatactaagtaatgaagagccctggaaatggcaaatggcaatgtcaatataaaatactcttatttatctaatttttaaatgtatttaaaggacaatttgtgatattaattaaaataataggaatatattgttgtttcaacgtatgtagtagtaaaattcataaaaacagtagcacaaataatgcagatgataactggaagtatactgttaatgagttttttgcattatccatgaagttatataatattaatagatggttgaatgtgatagtttaaggtgggatattataaatcctaggacaaccaaaaaaatttaaactgagaggaatggatagtaagaggaatagtccttttatgcaaaagaaggaagaaaaagaggaataaagaatataaaagatatggtgtaaacagaaaatacatagcattattgtagacacaaactgaactaccttatgagtatattaaatataaaaggattaagcattacaaataaaaggcagagattgtaaattgaataaaaaccacagctaagtgtgttctttttagaataaatactctttaagtgtaaagatctactttaaacaccaaaatatgaaaaaggatatataccatgaaaacctgaatcataaataagctggagtggtgattaatggatgcaggcactcctaaagactaataagtgaatgtggtcaaattgaagaaacaaaagtatatacgtgctcaatgtgcaaaaactttttctgtatacatgctatgatcctttggaaaattaaagttttaaagcaatatcactgacaatagtatcaaaaccaaaaaatatttagtgataaatttcacacactatgctcaaggactatacaccttgcactagaaaacaatgttgaggaaagaattaaaagatctaaatatacaccatgcttatagattaaaagactccatatcagttctcgtgaaattgatctttggatgaaacccacacccaagcactattgcaacagtccttttttggaaaaaaaaattggaggacttatataccttaatataaagacttataaaagtacaggaatcaagacatgtggtattggcctggccccttggctcatgcctgttaccccaacattttgggaggctgagtctggaggatggcttgagcccagatgttcaagaccagccttagcaacagagtgagaccctctctctacaaaaaataaacaattagatcgatgtgatgacttgcacatgtagtttcagctactcggaatgctgaggtgagaggattgcttgactcaggaggtctagccatgagtgagcattgatcatgcctctgcattccagcctggatgatggaatgagacactgtctcaaaaaaaaaaaaaaaaaaggatatgtgttattggccaaaaaagtatgcaaacctaaaaagggatggcccaccaccagacccacatacatatatggtaaatggattttccgtatagatggcaaagcaattcaatggagacaaaaatgttttacaaaatcattctgaaccatttggatatccatgatacaaaacaaaagcagaacttgacttttgcttttcatctcaaattattttgatatctcttccacctaagtgtcagagctaaaactgaacctgaaatatgaaagttccatgaaaaaatataaaatcttcacaaccttggagaaggcaaacttttttgaggcaggagtctgtaaacactcactataaaataaaacaaattataatgtgggctttcatgaaaactcatgcttaccaaaagtcattgttaagaaaataaataggcaagtaacacatgagaagaaaaatgctctctgtccatatatctgacaaatggcttgtgtccagaatataggaacatttctcccactcactaaacagaggacaaacaactaatgggcaacagattgaataggcatttcttggggatagatagatgtacacatagccaataagcacctgaaaaaatgtccagtatctcagccatgaaaaataaagagttataatcatcatgagatgtcaccaaacacccaatggacatggatattattaagaagacaccacagtaactgatgtcactgatgtagagcaaggatgtgaaactctctcatatgctggtgaaagtgcaaaatgatacaaccacttttgaaatcagtctgatagtttctccaaaagttcaataaatgcacttttaccctacaaacctgcaatcctgtttgtgaatatttaccccacagaaatggaaacataagtccacgaagacatctccaagaatattcatagcagctttattttttataaccccaaactgtagacaatttcaatgtcaatcaataagaaaatgaataaataatttgtgaactagtcatacaatggcatactgttcagcaataaaagggagcatgtttttgatactctcaaatagtatggaagatgctcaaaaatattacattaaagaaagatgccagataacaaaaatgaacattatgtatgagtctattgatgtaaggttccagaaaggtaaaactaatttctggtgaaagaaaccaatatcatttgcctctggccatgggaagagagtagcagagattgattgagcagtaaaacgaagtttttttctggggtgatgtaaatgtcctgtattgtgattgaagtgtgagttacacaagtgtacatgttcatcagaagtcatcaaactacatctaagatctgtgcatttgactatacatgaaaatatacctcagttgaaaatagatcaataacctccctcatatactatacttgctaacacagccagctgcttggagaaccagcttgctggaatggagaatctgggcttgagactgggtcacatgtatagagtctctacagagacaatgttgcattcccacggtacataatacatttcaaggtttctcagacagccacatgtcatgaatgtgaggattctgagaggttggagcaacattcctgggaggaacgaaggggagcacattctccaagatcccccaccaccggggtcctcaccggctgtgcttttttttttttttttcttgacagagtctcgctctgtcgccaggcaggagtgtaatggcccaatctcggctgattgcagcctccaactccagggttcaagagattctcctgcctcagcttcatgagtagctgggactacagatgtgcgccactgcgcccagctaatttttgtatttttagtagagacggggttttgccatgttggccaagatggtctcgctctgttgacctcgtgatccacccgccttggcttcccaaagtgctgggattacaggcgtgagccaaagcacccagcctgtgcctctcacttactcaattgtttttctgaaccctccatagctggtggaccttttcagatcccatagtctagccagccctctcactttatgccttgggtcccactgttccttcatctcatcccccttctgtcagtcccgcagtggctgtggccagtagaggatggactgagagtaggagaggaggttctgcccaggaacccatcctagagaaacagcatcctgcctgggacctagtcttccaggtcagcttttataagtcttttagactcaaactcacttgacccacctgaagtggtattgacaataatgctattttcatggttgtttttcactgtaaatgcagagccttttagctacacgactagtacagagagtaagggaggctggcctgggaatgatatcatcttggatggcatttcctccttggagaaatatatgttagttccaactcacatgttactatacagtcctgtagaaagagatacagagagttagacaggtatagacgcatttgtatatgcataacaatctataagacacacatcaaaatccgtataccggttcctctaggggtatgtgcttggcagaaggtagaaggagggtattctggttcctttcttttgcacatttatgtatgatctcagtttttatatggagcattgatagggtttggctatgtccccacccaaaatctcatcttgacttgtaatctctataatcctgataatccccatgtgtcaagggcaggaccaggtggaggtaactggatcatgggggcagtttctcccaggctgttctcatgacagtgagagagtctcctgagatctgatggttttgtaagtgtctggcatttcccctacttgcacttactctgtcctgccgcctgtgaagaaggtgcctgtttctcccttgccttctgccatgactgtaaatttccagaggcctccccagcaatgtggaactgtgagtcaattaaaactcttttctttgtaacttacccagtctgtctcgggtatttcctcatagcaatgtgagaacgggctaatacaagcatatactacttttgatattttaaaataaaaattatcatctatctttgaaaggcatgcacaaatgggaagttgaggaacatttgtgttgtggcaattgtatgatacctttaatgggaatatttcaaagacacttgttaagactttgttagaacaaaatgtagagggtgctggatgtccctgaatattcttccgcctcctgtaacttgtattgctttggaatttccagtggcctgacaatgaactactgcaggaatccagatgccgatacaggcccttggtgttttaccatggaccccagcatcaggtgggagtactgcaacctgacgcgatgctcagacacagaagggactgtggtcgctcctccgactgtcatccaggttccaagcctagggcctccttctgaacaaggtaagaagtctgtgtcttaccttgtctagcacatacctctctatgtgcttggacaacgggatgaaaagacatgaaaaaccacactgatgcagaagcctttagtgctacacgggagctcgagtgttggttgaggttctgccatgaccaaggaagtctcagtgccgtccctgggaaagccagagctgtgatttttggcacaacttgtgggagtagtgactttaggactggcgcaaaacctccagggtgctcaacttaaccactcaccttattctaaaatgggttatttcagtgtcccagtcaaattcctattctaacatgctgtcaactgtgtgattatttccaagccaataagcatttccagtaatttcttaaaatagtgttcattgcagtcttcagcgttgtggctcctgagggatgtggcccctgattctgtcgtcctagagaagcctgacatgactgcattgattctgtatcgtcctgggtctatgtggctgcctggctgtctgtaatcatctgttttatttttatttttttctacagactgtatgtttgggaatgggaaaggataccggggcaagaaggcaaccactgttactgggacgccatgccaggaatgggctgcccaggagccccatagacacagcacgttcattccagggacaaataaatgggcaggtctggaaaaaaatgtaagccactttgatttggactctttttccctttgctgacaaatcttttcaaacagaagaggggcagaggaaaatactggaaagacttcaggaggctaagcgtaattagccttagcatggaaagtgcaagcagcacaggccagcaaagccccacgcgtgtgggggttctcaggcctcttctcttttgacatttctttactgtttccattgttgggtgctgtttctcgtttctagtgcttgtcctctaagccaggggtccccactccagtactggtactggtactggtactggaactggtaattatctgtggcctgttaggaactgggctgcacagcaggaggtgagcttcgggggagcaaacaaagcttcatctgtattttctgctgcttcccatcactctcatagctgcctgagctctgccagctgtcagatcagaggcagcattagattatcatagcacaaaccctattgtgaactgcacatgtgaggaatctagattgcatgctccttatgagaatctaatgcctgatgatctgtcatgcttccatcacccccagatgggaccacctacttgcaggaaaattagctcagggctcccactgattttaccttatggtgagatgcacatttatttcattatatattacaatgtaataataattgaaataaagtgcacgataaatggaaggtacttgagtcatcctttaaccatcgccccctcaccccaggtgcacagaaaaattgccttttatgaaactggtctctggtgccaaaaaagttggggaaccacactgctctgggttctagtagtcagagatgccctctatgaggcttaagtcagatttttctagaaaagatttggatgggccatcaggtcaccatgagacttcccttagcctcatgcattctctgtgatggtttactttggggcctatgaatagggaagactgagatataggaaaaaccaaagtgtctgtgttcccccactctcacacccatgtaacataacacttctcacaccagatatggggggatttctcctcacaccccaagcgagtctccagcagataccagctgggtgtcctacaatgtaactcggtcctgacactctatctggagacagtgtcagatcccacaagttaaggctcagtcctacaagactgccccactgcagatgccaatcccaagttgcaggctgtgacctgtacttctgcccagctggataaagatctgtttttctatatgaccctccatgggtttgattactttgctagagtggctcacagaactcagggaaacacgttacttttatttacccatttattataaaagatattaaaaaggatcctggtgaacagccaggtggaagagatgcacagggcaaggcacgtgggaaggggctcagagcctctatgccctctccagtgcaccagtccccagtaccctaagtgttcagcaacccagaagctctccaagtgcagtcttgttgggtttttatggaggcttcattacagaggcacagttgattacatcattggccatcggtgatcggctcaccttcggcccctcttccctccctggaggttggagggtggggctgaacagttccaaccctcaagtcacatggttggttcccttggcaaccagcccctggggctatccaggaacccaccaagagttgcttcattgcagctcccttcacccaggaaactccaagggatttaggagctctgtgttaagaactggggggcagagacccaatatacatttcttattctatcacaatatcacaggaagctaaggatgatactgcctttgtgtgtcttggctgtggatggtgcataatgcatggaagtaagcatttctgaatcaacagcaaacaggctttatcaggtagaagacccctcagcgccccagggacaaagctcatcaatgatgtcccactgtcctctgaggctctagctctaagacctccagtgggtcaagctcctggagaagtggcacattctccaaagacccttcagggtcaccacaccctggttaagggtgtggcctcataactccttttgactatgactgatggcttacagcatagaaagaaataactttgtcaaaaaatataataatgatagaaaggaagaaggaacgctcccttttgtcttctaagaatagatgtgaaatgtgtgtgccttagaatatcttctccctctcctgctccacgtgagctggagcttacatgcctgcttgttttcagtactgccgtaaccctgatggtgacatcaatggtccctggtgctacacaatgaatccaagaaaactttttgactactgtgatatccctctctgtggtaagttgccttctgttttggtaaggaaactgcttccttaatatggatttggaaaaaaaaaagcaaaaaaaacagaaaatggcttttgagctgagtgcttctggggaggagatggctgccctctccaccagagcctgcttttcatcatggccaccttgaacctgccctactattggccccatttgttaggaaaacacccgcccctcccaccacacacacataaataaaataaatgtcaaattcccaaagggcaaacttagaggtgatctaatcagcccgggatagtcccaccgaacccttctttgtctagcgtgggatgcatgaaaaacaaatttagagtcattatgatgaaaaactgtcctcttctgcagctgagaagaaaaaaaaaatacgagcagcaggaaacagctaagcatgtaatgcacattgtaaacctcagatggccatcctaggaaatcaatgaagggtagtgcagctctttagccccagatggcctttctcgtaagattactactcatgagtcccattagcgacattgcttagagactgcttgttaggttccttcctcattgctctgagactcttattgggagtatgaggcttggatcaggggaaggggaattgacattagatcttaaatgattggggtaacaaatccatgggggaaaaaaagccacttgtacttgttccctattttcttcctgctgaccaatcaacttgtctgtccgagttacagaacaccaccctggacttttcttttgtgtaatttggttgcttgtggttgggtctgccatgtgaagggaccttgagctgggggaagaaggttggcctccaagtccactgaagaccagcatcctgagattgcctggggaggtggtacagggcagtgatgaagatcatgggagccacactgcccatcgtcacatttgggccactcctggggagagcaagagggaagaaggagaggttagggtgataggaaagattctacttggccaatattattataatgtggcattgtggtctctggatttagtgtgagttgatagctgacttttttctcgagtgggtgcttttgttctattttgtcggtgctattgcagaagcatcttggtggttcctctacctcaaagtctcttgatggggtcagttccagttctccgcttctggccccatctagtacacgccactgcctctcactgcctgggctctctatccttgacaggctgccttgaatttaagcccagtctgacttacctgcctcaaacacccacagtagtgcctgggactcatgcacctttgactcccatggaagggaagtgcagtagcttcccaggtgcaattctgctgtcctcacccacattgaggatgtatgagaatcaggttcttagagattggagaaagaaggaagaatgggaacaagatttcttccaatggactgtgaggttccccaccttactttgatgtaagacaagtgaggttaaccccaagcctggtgaggagggttcccatcagacacttggaaatcctgaggactgtttcctgcagaaggatgtggttggtgggatattcaggtttgactcatgattgagaaagttagagcctctggttggagaaagagtttaataactatttcatttccaccaacacattcagtacgaataataaataagtaaaaataaatagaaacattcagttttattttgaatagtaggagtagggtataatttctgtagttactcttttagtacaatgatgcatgtttactgtatgtaaggcatactagcagaaattgagctcagcactagaaaagatgattgcattccatgccatgcttcttttttacaaaagacttctatagatagattctcaaaacaacccacagcaaatgaaaagttatttggaaaactcaggttccagattcactggagtgtagaatctctggttggttggggaggaatttcctcttgcagttgttattaataattatatgaataattattaactatattaatatttatagttttgaagaccttgaagggctggagacaacagagaagcatttttgaacaccctctgtagcccctgcactgttgtaggcattgatgggtggtaccaaagatgggacactttccctacctccagagaccttgtgggcttgctgcagagagaaggcagggaggaggaaaagaagaatagaggcacatgtgtgtaaattacccccacagcagtcagttagtcatgggaggctccccagaagaactgtcctgaagctggctgagagaaggcaacatttcaacataggacagttatccttgctacataaaatcacatacacacatgcacatatgtccacacacagagactcacatgcaaaagaatcctttgtgcctttcagtaaactttacatggtttagaaagaacttatatttccttgaaaggagagtgtcctttgttgtttactaccactttttaaacttagaaagaaaaatctaaagagtgtttatgattttaccatttaatttcacctttgagatgtgaaaaactagtgcttggaattcgtcctgaattaaacgacacaattgctaacttggactcaaatgcgacttcttttcccaccttgtgccacagcatcctcttcatttgattgtgggaagcctcaagtggagccgaagaaatgtcctggaagcattgtaggggggtgtgtggcccacccacattcctggccctggcaagtcagtctcagaacaaggtaagaacaggcccagaaaccatctatactgtccttccatgtaagccccacaaaacccttctacatttacacagaacccacacagctgatgcatcaatacctgcctctctgttttctgaaggaggaaaaaatatagaaaaattaaaaaaagttatattattataggttctctacttggaaaatagccaaaatacaaatctttttcttgatctgggcagttccatcaaaatctgtaggcacagtgatttgcaccaagttccaatacttttggaaaatattgaagatgctctgagggtttctatggatatccattgtctcactgtcagatgaaaagaaagggaagtttttagaaatgtgacactttgcagtgagggaggacaagagcaaacttacctacagtctatcacaggcacagatttttttttacacttttgtgaatcattgaattcaatgccgaggctattcatctattcacaaacacatgaacaaattatgggttgtgatccccataaatgaagagtaatcagtccgaacccacagaacctggacattttgggtatcgtttcagtggaacatgcaattcgtaagttcagtttgcttgggtgtctcttaggaagaacacataggacacagacccatctgcctgcatgttttgcttcctcatctcctttctacaccagggcacctgtgctcaattgctgttctcctctaaagagacttccttctgtaagtttgtgaaatgccatcgacaaacctgatcgcatcgcatttcactctgctgttgagttgatttttctttactttatcgtttgtaacttcttgctctacagagctttcaccttccacatatttcagattcattctttcctaaactgtgtggtggtctatgtcctcactgactatcaacatactgccatcatgcacttcctatctctattcctcttcgttgcaatctggctccaagtggctcacaccattattctgatctatcaactgcctacacagtcctagaaagtaagtgagtcaagaaacatcccccaaaagtaaacttttcaggtaagatcagaagaccctcatgagtcactgctgctcaggatcgtatctggctccttgaagagtgaccttgcatagatcttgtcataaaaaatgaaagagaccttgggaaggtcttgggctggtcacttttgtcagagtccagggctgtggggtgaaagccacagctatagagcttcattctggagtcacttagctttgctctcctggggacaggctgtgcctattcttgcctcaggcatcaaaaaaagtggcacagatgggcccttctgaaaaatctcactactggagcacagctcgaagtttctactatcctgacgttgggcggtagtcctttgctttgggaatatgaacatgatcaaaactgagtgaacttgtcttcctggctttctgtacaatgaagtagaacaaaccatccaatttgaccaaagccttggcatgttttctttctaggtttggaaagcacttctgtggaggcaccttaatatccccagagtgggtgctgactgctgctcactgcttgaagaagtacgtttaagggaaaactgacatggggtcttatcttcaagacttttttcctccctctcttcctccatcccttctttcttcccaccctccccttccttcctccccacctctcttccttttctggaaggaacactaggaaccagggaatgcatgcagaatcctgaggcagaatttccagggcaattggatgagagaggagggaagtgtttctagagggaatctgcagagggaagacccagtgcaagtgattttttggacctgtataaaccgcaggacagagctgttcactaccagaggcatcaatctgtattgcattgctctagagcaatatctgaggctgaataatttataaagaaaagagtttaattggcacatgtttctgcaggctttacaggaagcaggatgctgtcatctcctctgcttctgtgtgggcctaaggaagattacaatcatggtggagggcaaagtgggagcaggcatgtcacatggccagagcaggagcaagagacagagagagatggggtgggggtgctgcacaataccaaatgaccagactttgcaagaactaagagtgagagctcactgatcaccatgaagatgtggcccaagccattcaagagggatgcacctctatgatccaaacccctttcacaggccatagctccatcactggggactacagttgaacacgagatttaggtggggacaaatatacaaactatatcacagtctctgatgaaacagattgagaacagaccttaactgtcagtttccagcaaattgtgaattttgtttcttgccactcataagtcactgattctgggtggccgagggtgtcagagggacagcgccaagttcatggcacagaggatacctgaaggggctggaccatatttttctcttgacatcctcatcttttctaggtcctcaaggccttcatcctacaaggtcatcctgggtgcacaccaagaagtgaacctcgaatctcatgttcaggaaatagaagtgtctaggctgttcttggagcccacacaagcagatattgccttgctaaagctaagcaggtactcgctcacctgtggtcttcaccccacgctggtgaagatatttgctttatgtctgggttttatgggccatggccactgcatggcagtggggaggaactgtctatcacatgaaaggctcaagggctttggggacagcatcaatcttcaaccccagccctgccacatgttagttgtgctctttaaaaaggcagaaggattcgtttcctcacgtggaaaaagagataccctgttacccgtaaaacttacttaatgttcaccagttcatccacattcatgatcagggaaaggttgttattccaggctaactattctcctttcataataatatgctggagagaatcaaatgagattgcatttcaaagcgcttgaaaaaccaccatatcgagccatgcttagtgtgggcgcctctaatcactgctattcaggaggctgacgaggaagaattgcttgagcccaggacttcaaggctgtaggcagctatgattgtgccactgcactccaggctgggtgacagatcaagaccctgtctcaacaaaagaaaagaaaacaaaacaaatgaacagaaatattccacaatgtcaaaaaaaaaaaaaacccacacaacatacaatttacaaatgcaaataataatattattgttgtcttctttgattttctctttcctggtgaaattttgttttattaagcctgacaaagtgatacctttgcttacatcacttaaagttagtctatttggacctaggtgacagtacaatcagctaagaaacagtatttgtaggagaggcaggtttgggacaggtgacaaggcatgtggggtgctcgctgtgctggtggctctggaaggcagggtgtcaatgcagacagggatgagcatggcctggttgggaaggcatggggcaggcaggagcctgagctgctctcctgggcctggtcacaagcccatggcagcttctctgggtctgtgaactgaggggtgatgtcctggaatcctctgacactctaggaaggagagaagggcctttctggctcagcctttataaacagtagctgatctccctcttgctccccagggtcctccccaccatcccagcaaatgtgcaaatacaagatctctgctcctcatggtcctcagagagctggggtgttctgatggcttgaacaagtcacttaggaaatgtggggttttggaggcattctctgataggctgatacgttttgagtttagagttcccaccgcacatccccacacccctagagtctagggcatttagtgctccatgagggaacctgtagagtgaggacatctgcatcacaggctgggccttctagtgtccagaagcagaaagtgtgtctgcttcaaagttggtgctaatgatgatttttggtcagaatacggcatttctcatttccattcctttatccccttgaacttactaaagtagaatcaggtctaaaaaccagagttctaatctttaagagtccctgggattctaaggtatatgaatgtccttggaaaacaataccatttagttcatgcaaggtgcttatttcccatcctctttcatttgatgtctagcattttactgcattcttaccaccacggtttagtaacattcacgaggaggaagtggaggatccagatggagcaacttgctctgggcacacaaggcatttgcaattttataccctcttgatgatgtctcagccagacattctgcccagtcatcaatgccctcttcaattaatatgaaaggacacacttggcatgagattccaatcgtgcacagaatatacatgagaagtgtgcctttgtcatccctactttcaaaggctaaggccaccctcagtttcttgcatgcaactgatgcctttcaaatgaaaccttacatctgtgtagtccataggcaaccacaggcaaatgtgagggtgaaacgctgtgttctacattgttctgtgtcagtgaagcaaggcagtgccagctcagagggctctggggcttcaaggcagggatgcctggttgtaggtactgccacttccagctgggcagtgaaacataactgctaatactttccttacaggcctgccgtcatcactgacaaagtaatgccagcttgtctgccatccccagactacatggtcaccgccaggactgaatgttacatcactggctggggagaaacccaaggtgagatcaattccattgcccacgtaacaaattgtttttgaccttcagtgcatgttacaaaatgagcattttggagatagttgtacaaattcctacccatgaatgtggtctacccactcctgactttgcctggacacctgtctatgtctccataatcagtcttcaagggacttgggcaaggggagcggtgccatttccttgagtctctctcttttttgttttcagaatcttttaattttttttgtaatgattgtatgtttcccttacaacaaaaacaaacaccagtagaggtctttgagtctcttaatcataatttcagcattcatattgcttccccaggtaagtggggttttgacccagccctcaagttaagggtgttagattatttttcatgtgaaattagacagactgcgtttctaaacatggtgcaaaacagtaacgacaaaagttgtaattaaactattcttcttcccaaatacccacatgtctaatgtgtgtgtgagggtgttaggcaggggacctgaagctgggggagaggcagacagttcccatggccccaagtctaggatggcatttggtattggttgatgggtgagagcaagagagggaatatttttgtgcatgatgtggtatcagcacctgtactacattttatggattccttcttctctttgcggtatgccctgacaataattatatccgtcagccttacccccttggcagtaggaaaactgaaactgtcttaaagtctcagctctactttctcagaggtgcaggcaagggcactgggagtctggggccctggaaaactgttctgactctgccacttgccagatagacctgaactagacacgttacctctttgtaccacttggctctaatcccttatctgtaaaaccagcattttcaaatggtgctttgcacatcagccttttgcataagctttgatttgataaaatgttttttgtgtttttaaaaagattaaaaaccacaggtttagataatttcaaagtaggcttccctttttctgtcattttcctattatttttaaaacctcacctccttgactccttgttccctttttctgcactgctgagtctgggagcactgaggccaggtaaaaggaaacttggcaaatgaggggcacctatgggtgtgggaggctgctcctggtgtttgcatattttaaaatttaaatgctacaaaccactgtgagttaggtattattgttcctattttaccattgaggaagctggggctcagagaaggtggagggtggtacagacaaacctgaattggaaccctggctcctgcctatgggctgtcaggacttagaaaagtcgtgagctctcgctgattgtttcctcagctgatgtgggctgcagggctgttatgggggaaataataagaaagtgcatcaagtgctgagcacatcctaagcactccatcatggcagctcctactactaataaagaatagaattatatctaacatgattctttcttgcaagtgacagaaaatccaactcaaattggattaagcaaaacaagggaaattcttagtgagctgcaaagttttcaggctcacatgatggccccaaatcccaggtcctcccaatcatggagtaggcactatttgggggcacaaaggtgacattcccatggctgcagatgctgtggtgctgtggctgtaccgggaaagaataagaaaggccactctcccaattatgtgaacaatagtctgcccactctgagaagtcaaacttgggtcacagtcctgcccctgaacccatcactgactggctctgacctgcaccaattgttccatgttggaggtgaaggcaagaccccactaatacccataaggggcaaaagttagatagatccttcaagaggattatgggaggtagggcaaaaagctgctgggcagccagaaagcaaacagagcctctatgatacctcaactgatgaaagcatgaagctaaaatcataaggatctgggtgtgagttctggctctcccatcttccatgtgacattgggcagttatttaatctcttttagcctccgctttctcatcttacatatgagataattgtgaggattaagattacacataatcatcatcatcaccgtccaccactaccaccatcatccccatcaacatcatcgccaccactatcatcattcttactggcactaccatcaccatcaccaccattccaccaccatcaccaatatcatcactgtcaacatcattaccaccatcaccatcaccaccaccatcatcattactaccactaccactactaccaccatcaccatcaccaccattccaccaccatcaccaatatcatcactctcaacatcatcaccatcaccatcaccaccaccatcatcatcattactaccactaccactactaccaccatcaccatcaccactgtcccactactatcagcatgacatcaccatcaccaccaccatcatcattaccaccgctactaccaacatcaccatcaccacaattctactgccatcaccattaacattaccaccaccatcatcactatcaccatcaccaccatcatcaccactgccattatcactgccaccatcatcactatcctctatatttcctcatctgtattatcattactaccaccatcactatcaccaccatcgtcaccatcataatcaccatcaacaccatctccaataccaccatcactgtaaccatcatcaccaccaccatgatcactatcaccatcatcacaatgatcactgtaaccatcattactacccaccaccatcaccactactccaccaccatcaccattatcattaccatcaccattatcaccaccatcatcatcaccagcaccaccatcatcaccagcaccaccatcaccatcaccatcattaacaccatcactatcaccattggtttaatcatcaccaccatcatcataaataaacatcacataaccagggtgtagctgggtgttgaccccagagcccactcactgtttcctctctcccacccccatccacacatttctaaccaccatcctgcactgggctcccagtctcctctggtctcacccacatgtccactgagaaaaggattttcagaacaccaactagaccaggaggagccacatacataactcaggcctgcttatcaactttctacatgttaataatgacatcagatcaatgggtgttctcagcttctcagaaggaggtcaaaattctccccctctccccttcatgtgtccagaccttcccggatttggatgtaccaagtgcagagtggtgttgaggccaaggggctcatccatgtaagtctcatctgcaatcactgggctgatcccgtggccctgtctccagggcgccatcagagagggcttcaatcctcaggttacctgtggcccaccctgccctcagaggtgccatctctacattggccacgagatggcagcacatactcatagactgcattaatttcccagcaactcctggtgggttttccctcttatcaggatgtttgccttgctcagagagcaaatctgagagcagtgacacctaacttaactttcagcaaaatattttgagaagggtgcccctttacacatctgtgcagtccaggtgatgcatcccatgcccaatgctcggtagtcaggaggagcttcctccatgcagctctgcggaagagactcttccacgctgctcatgtaaactccagattcggtgtcagttttctgacaccgaagacaatgatctaagtgcagtcaagggctttggggaaagcaggagagagtgcctcagttctagcctgtgccatgcttgcaaagttttgcaaaattctaatgagagctgggcttgcaacattggaaacttggattatttgtgagagcactgagaaatccctgggcatgtccatctggaaaaacagcatttcctctggcactttagcagaggttctgtttcaatttggcgaaggaaattaagcagtttttcacaaaagaagaactacaacgaggagaattgtccctagtatttcttctccctaattgtcaaggaagtgtaaattagaaaatgaatcaggacaatttccacctactatgttagctaatattttaaaaattgaatatcacaagggtgaggcaaagtaattgttttccagtgacattttccactgtcacacccttttagagaataatttggcaatgttactgtgagatagaaatatgtctatataattatgggaactgagacttcagaaagtaataaggaataagaatgaaatttatgaacaaacatgtggaaggttggaagcaagagtggggccaacacgcatggggaggaagcatttgggcagcgactccgcagacccagactcaagctgagctatacaacctccttacgcctcagtttcctcaactgaagaacaggaatgacaagtgcctgtttcataggaccgttgtgaggattaagtgagatataccacattatgagcttgtgcctggaaaggttgattcttagtaaatgatgactattcttttttattgcaataaaatttatacaacatagagttactattttaaccatttttgcaggtaccactgagtggcattcagtacattcacaatggtgtgcaaccgtcaccatatttccaggacatttttctcatccccaaaggaaacctcatgcccattaagcagtcactcctcattaaaatattagttatgaagactgtagcatttttttaaaaactcatgatataacattgattgaaaaaatcagtataggaaattgtgcattatgatgtaatagtaaaagaagcatataaaaatctgaaaaaagtatataaaaagaatagcaattgtatttctcagactctctttacattgtaaaaatcattttgatagcttcaaaagaaaagcaaaaagtacacaaacaacaaccaaccccaaagcagcatgacaaagcccagattgttgaatccaggtcttgggaacataaaatcttatatgacatttgcactttaatgggtcagagagtccagtggcattgggagctgccttgtgttctgcagcctcacggacagacaggaggtccagctccactgctctgttcttctggaatttcctcgtgaacaagctttggcctcagtaaccatttctttcatctttttaaacacaggtacctttgggactggccttctcaaggaagcccagctccttgttattgagaatgaagtgtgcaatcactataagtatatttgtgctgagcatttggccagaggcactgacagttgccaggtaagaaaagatcaatagatcaaagtcttgtgctctcccgtctcagtctcagtcccttagacgtcagtcccaaagtggcaaattcaggaaggttttgtcagtggaagaccccagtctaagtgttgctcagaaactccccagatctgtccctgaatgcatattcagatcatctaaggagacgtcttggggcttgagttccagatccatagcaagggagccgtaagtgccataactacctcaggccactcaccttcctggtgtgtgctggtcaccagtgactgaagtggtggcttttccagtagagaggaaggtagagggtacaggaccgagacaaattacacacacttaacaatgatgtccaggctagcccagtctaaaggaaacaccaagttaggaagcaatgcatgcaggattcacaagggattattttttttcccaggaaaaaactaagtgatgtggttttgttgaatagactttgctaagtacttaagcactgcagatgcttgagtaatatgctcataagttcctttctgatttgaattactgggaaaatgtacatatggataagagaaggatggcatcccatattaaaaggttggcagcttaaagctcacatgaattttcccctacctctgtttagggtgacagtggagggcctctggtttgcttcgagaaggacaaatacattttacaaggagtcacttcttggggtcttggctgtgcacgccccaataagcctggtgtctatgctcgtgtttcaaggtttgttacttggattgagggaatgatgagaaataattaattggacgggagacagagtgaagcatcaacctacttagaagctgaaacgtgggtaaggatttagcatgctggaaataatagacagcaatcaaacgaagacactgttcccagctaccagctatgccaaaccttggcatttttggtatttttgtgtataagcttttaaggtctgactgacaaattctgtattaaggtgtcatagctatgacatttgttaaaaataaactctgcacttattttgatttgaattaattttggttttggtcttcaaaattttcatgctcttttcatcccatctatttttatttttattttttagactttacgtcctggggtacatgtgcagaatgtgcaggtttgttacatagatgtacacgtgccatggtagtttgctgcacccatcaacctgtcatctaattcggtatttcttttagttctatccctcccctagccctccaccccttgacaggcccaggtgtgtgatgttgccctccctgtgtccatgtgttctcattgttcaactcacacttatgagtgagaacatgccgtgtttgtttttctgttcttgtgttagtttgctgagaatgatagtttccagcttcatccatgtccctgcaaaggacatgaactcatccttttttatggctgcatagaattccatggtgtatatgtgccacattttatccaatctaacattgatgggcaattgggttggttccaactctttgctattgtgaatagtgccacaataaacatacgtgtgcatgtgttttcatagcagaatgatttataatcctctgggtatatacccagtaatgggattgcagggtcaaatggtgtttctggtgctagatctttgaggaatcaccacactgtcttccacaatggttgaactaatttatgctcccaccaacaatatcaaggcattcctatttctccacatcctctccagcatctgttgtttcctgactttttaatgatcgccattctaactggcatgagatggtatctcattgtggttttgatttgcatttctctaatgatcagtgatgatgagcttttctcatatgtttgttggctgcataaatgccttttttggagaagcatctgttcatatcctttgcccactttttgatggtgttgtttttttctggtaaatttgtttaagttctttgtagattctggatattagccttttgtcagatggatagatggcaaaaattttatcctattatgtaggttgcctgttcactccgatgatagtttcttttgctgtgcagaagctctttggtttaattagatctcatttgtctattttggcttttgttaccattgcttttagtgttttagtcatgaagtcttctcccatgctatgtcctgaatggtattgcctaagttttcttccagggtttttatggttttaggttttgcatttaagtctttaatccatcttgagttaatttttgtataagtaatgcccttctttgtctcttttgatctttgttggcttaaagtatattttatcagagactagaattgcaatccctgcttttttttttctttttgctttccttttgcttggtaaatattcttccatccctttattttgagcctatgtatgtctgcacatgagataggtttcctgaatacagcacaccaatgggtcttgactctttattcaatttgccagtctgtgtcttttaattgggggcatttagtccatttacatttaaggttaatattgttatgtgtgaatttgatcctgtcattatgatgctagcgggttattttgcccattagttgatgcagtttcttcatagtgtggatggcctttacaatttggtagtttttgcagtggctggtaccaattgttcctttccatgtttagtgcttcgttcaggagctcttgtgaggcaggccttgtggtgacaaaatctttcagcatttgcttgtctgtaaaggattttatttctcctttgcttatgaagcttagtttcgctgggtatgaaattctgggttgaaaattattttcttttagaatgttgaatattggcccccactctcttcgggcttgttgggtttctgcagagagatccactgttagtctgattggcttccctttccgggtaacccaacctttctctctggctgcccttagaaatttttccttcatttcaaccttggtgaatctgacgattatgtcttgaggtggctcttct

SEQ ID NO: 4 - DNA, 13938 bp, Homo sapiens
ctgggattgggacacactttctggacactgctggccagtcccaaaatggaacataaggaagtggttcttctacttcttttatttctgaaatcagcagcacctgagcaaagccatgtggtccaggattgctaccatggtgatggacagagttatcgaggcacgtactccaccactgtcacaggaaggacctgccaagcttggtcatctatgacaccacatcaacataataggaccacagaaaactacccaaatgctggcttgatcatgaactactgcaggaatccagatgctgtggcagctccttattgttatacgagggatcccggtgtcaggtgggagtactgcaacctgacgcaatgctcagacgcagaagggactgccgtcgcgcctccgactgttaccccggttccaagcctagaggctccttccgaacaagcaccgactgagcaaaggcctggggtgcaggagtgctaccatggtaatggacagagttatcgaggcacatactccaccactgtcacaggaagaacctgccaagcttggtcatctatgacaccacactcgcatagtcggaccccagaatactacccaaatgctggcttgatcatgaactactgcaggaatccagatgctgtggcagctccttattgttatacgagggatcccggtgtcaggtgggagtactgcaacctgacgcaatgctcagacgcagaagggactgccgtcgcgcctccgactgttaccccggttccaagcctagaggctccttccgaacaagcaccgactgagcaaaggcctggggtgcaggagtgctaccatggtaatggacagagttatcgaggcacatactccaccactgtcacaggaagaacctgccaagcttggtcatctatgacaccacactcgcatagtcggaccccagaatactacccaaatgctggcttgatcatgaactactgcaggaatccagatgctgtggcagctccttattgttatacgagggatcccggtgtcaggtgggagtactgcaacctgacgcaatgctcagacgcagaagggactgccgtcgcgcctccgactgttaccccggttccaagcctagaggctccttccgaacaagcaccgactgagcaaaggcctggggtgcaggagtgctaccatggtaatggacagagttatcgaggcacatactccaccactgtcacaggaagaacctgccaagcttggtcatctatgacaccacactcgcatagtcggaccccagaatactacccaaatgctggcttgatcatgaactactgcaggaatccagatgctgtggcagctccttattgttatacgagggatcccggtgtcaggtgggagtactgcaacctgacgcaatgctcagacgcagaagggactgccgtcgcgcctccgactgttaccccggttccaagcctagaggctccttccgaacaagcaccgactgagcaaaggcctggggtgcaggagtgctaccatggtaatggacagagttatcgaggcacatactccaccactgtcacaggaagaacctgccaagcttggtcatctatgacaccacactcgcatagtcggaccccagaatactacccaaatgctggcttgatcatgaactactgcaggaatccagatgctgtggcagctccttattgttatacgagggatcccggtgtcaggtgggagtactgcaacctgacgcaatgctcagacgcagaagggactgccgtcgcgcctccgactgttaccccggttccaagcctagaggctccttccgaacaagcaccgactgagcaaaggcctggggtgcaggagtgctaccatggtaatggacagagttatcgaggcacatactccaccactgtcacaggaagaacctgccaagcttggtcatctatgacaccacactcgcatagtcggaccccagaatactacccaaatgctggcttgatcatgaactactgcaggaatccagatgctgtggcagctccttattgttatacgagggatcccggtgtcaggtgggagtactgcaacctgacgcaatgctcagacgcagaagggactgccgtcgcgcctccgactgttaccccggttccaagcctagaggctccttccgaacaagcaccgactgagcaaaggcctggggtgcaggagtgctaccatggtaatggacagagttatcgaggcacatactccaccactgtcacaggaagaacctgccaagcttggtcatctatgacaccacactcgcatagtcggaccccagaatactacccaaatgctggcttgatcatgaactactgcaggaatccagatgctgtggcagctccttattgttatacgagggatcccggtgtcaggtgggagtactgcaacctgacgcaatgctcagacgcagaagggactgccgtcgcgcctccgactgttaccccggttccaagcctagaggctccttccgaacaagcaccgactgagcaaaggcctggggtgcaggagtgctaccatggtaatggacagagttatcgaggcacatactccaccactgtcacaggaagaacctgccaagcttggtcatctatgacaccacactcgcatagtcggaccccagaatactacccaaatgctggcttgatcatgaactactgcaggaatccagatgctgtggcagctccttattgttatacgagggatcccggtgtcaggtgggagtactgcaacctgacgcaatgctcagacgcagaagggactgccgtcgcgcctccgactgttaccccggttccaagcctagaggctccttccgaacaagcaccgactgagcaaaggcctggggtgcaggagtgctaccatggtaatggacagagttatcgaggcacatactccaccactgtcacaggaagaacctgccaagcttggtcatctatgacaccacactcgcatagtcggaccccagaatactacccaaatgctggcttgatcatgaactactgcaggaatccagatgctgtggcagctccttattgttatacgagggatcccggtgtcaggtgggagtactgcaacctgacgcaatgctcagacgcagaagggactgccgtcgcgcctccgactgttaccccggttccaagcctagaggctccttccgaacaagcaccgactgagcaaaggcctggggtgcaggagtgctaccatggtaatggacagagttatcgaggcacatactccaccactgtcacaggaagaacctgccaagcttggtcatctatgacaccacactcgcatagtcggaccccagaatactacccaaatgctggcttgatcatgaactactgcaggaatccagatgctgtggcagctccttattgttatacgagggatcccggtgtcaggtgggagtactgcaacctgacgcaatgctcagacgcagaagggactgccgtcgcgcctccgactgttaccccggttccaagcctagaggctccttccgaacaagcaccgactgagcaaaggcctggggtgcaggagtgctaccatggtaatggacagagttatcgaggcacatactccaccactgtcacaggaagaacctgccaagcttggtcatctatgacaccacactcgcatagtcggaccccagaatactacccaaatgctggcttgatcatgaactactgcaggaatccagatgctgtggcagctccttattgttatacgagggatcccggtgtcaggtgggagtactgcaacctgacgcaatgctcagacgcagaagggactgccgtcgcgcctccgactgttaccccggttccaagcctagaggctccttccgaacaagcaccgactgagcaaaggcctggggtgcaggagtgctaccatggtaatggacagagttatcgaggcacatactccaccactgtcacaggaagaacctgccaagcttggtcatctatgacaccacactcgcatagtcggaccccagaatactacccaaatgctggcttgatcatgaactactgcaggaatccagatgctgtggcagctccttattgttatacgagggatcccggtgtcaggtgggagtactgcaacctgacgcaatgctcagacgcagaagggactgccgtcgcgcctccgactgttaccccggttccaagcctagaggctccttccgaacaagcaccgactgagcaaaggcctggggtgcaggagtgctaccatggtaatggacagagttatcgaggcacatactccaccactgtcacaggaagaacctgccaagcttggtcatctatgacaccacactcgcatagtcggaccccagaatactacccaaatgctggcttgatcatgaactactgcaggaatccagatgctgtggcagctccttattgttatacgagggatcccggtgtcaggtgggagtactgcaacctgacgcaatgctcagacgcagaagggactgccgtcgcgcctccgactgttaccccggttccaagcctagaggctccttccgaacaagcaccgactgagcaaaggcctggggtgcaggagtgctaccatggtaatggacagagttatcgaggcacatactccaccactgtcacaggaagaacctgccaagcttggtcatctatgacaccacactcgcatagtcggaccccagaatactacccaaatgctggcttgatcatgaactactgcaggaatccagatgctgtggcagctccttattgttatacgagggatcccggtgtcaggtgggagtactgcaacctgacgcaatgctcagacgcagaagggactgccgtcgcgcctccgactgttaccccggttccaagcctagaggctccttccgaacaagcaccgactgagcaaaggcctggggtgcaggagtgctaccatggtaatggacagagttatcgaggcacatactccaccactgtcacaggaagaacctgccaagcttggtcatctatgacaccacactcgcatagtcggaccccagaatactacccaaatgctggcttgatcatgaactactgcaggaatccagatgctgtggcagctccttattgttatacgagggatcccggtgtcaggtgggagtactgcaacctgacgcaatgctcagacgcagaagggactgccgtcgcgcctccgactgttaccccggttccaagcctagaggctccttccgaacaagcaccgactgagcaaaggcctggggtgcaggagtgctaccatggtaatggacagagttatcgaggcacatactccaccactgtcacaggaagaacctgccaagcttggtcatctatgacaccacactcgcatagtcggaccccagaatactacccaaatgctggcttgatcatgaactactgcaggaatccagatgctgtggcagctccttattgttatacgagggatcccggtgtcaggtgggagtactgcaacctgacgcaatgctcagacgcagaagggactgccgtcgcgcctccgactgttaccccggttccaagcctagaggctccttccgaacaagcaccgactgagcaaaggcctggggtgcaggagtgctaccatggtaatggacagagttatcgaggcacatactccaccactgtcacaggaagaacctgccaagcttggtcatctatgacaccacactcgcatagtcggaccccagaatactacccaaatgctggcttgatcatgaactactgcaggaatccagatgctgtggcagctccttattgttatacgagggatcccggtgtcaggtgggagtactgcaacctgacgcaatgctcagacgcagaagggactgccgtcgcgcctccgactgttaccccggttccaagcctagaggctccttccgaacaagcaccgactgagcaaaggcctggggtgcaggagtgctaccatggtaatggacagagttatcgaggcacatactccaccactgtcacaggaagaacctgccaagcttggtcatctatgacaccacactcgcatagtcggaccccagaatactacccaaatgctggcttgatcatgaactactgcaggaatccagatgctgtggcagctccttattgttatacgagggatcccggtgtcaggtgggagtactgcaacctgacgcaatgctcagacgcagaagggactgccgtcgcgcctccgactgttaccccggttccaagcctagaggctccttccgaacaagcaccgactgagcaaaggcctggggtgcaggagtgctaccatggtaatggacagagttatcgaggcacatactccaccactgtcacaggaagaacctgccaagcttggtcatctatgacaccacactcgcatagtcggaccccagaatactacccaaatgctggcttgatcatgaactactgcaggaatccagatgctgtggcagctccttattgttatacgagggatcccggtgtcaggtgggagtactgcaacctgacgcaatgctcagacgcagaagggactgccgtcgcgcctccgactgttaccccggttccaagcctagaggctccttccgaacaagcaccgactgagcaaaggcctggggtgcaggagtgctaccatggtaatggacagagttatcgaggcacatactccaccactgtcacaggaagaacctgccaagcttggtcatctatgacaccacactcgcatagtcggaccccagaatactacccaaatgctggcttgatcatgaactactgcaggaatccagatgctgtggcagctccttattgttatacgagggatcccggtgtcaggtgggagtactgcaacctgacgcaatgctcagacgcagaagggactgccgtcgcgcctccgactgttaccccggttccaagcctagaggctccttccgaacaagcaccgactgagcaaaggcctggggtgcaggagtgctaccatggtaatggacagagttatcgaggcacatactccaccactgtcacaggaagaacctgccaagcttggtcatctatgacaccacactcgcatagtcggaccccagaatactacccaaatgctggcttgatcatgaactactgcaggaatccagatgctgtggcagctccttattgttatacgagggatcccggtgtcaggtgggagtactgcaacctgacgcaatgctcagacgcagaagggactgccgtcgcgcctccgactgttaccccggttccaagcctagaggctccttccgaacaagcaccgactgagcaaaggcctggggtgcaggagtgctaccatggtaatggacagagttatcgaggcacatactccaccactgtcacaggaagaacctgccaagcttggtcatctatgacaccacactcgcatagtcggaccccagaatactacccaaatgctggcttgatcatgaactactgcaggaatccagatgctgtggcagctccttattgttatacgagggatcccggtgtcaggtgggagtactgcaacctgacgcaatgctcagacgcagaagggactgccgtcgcgcctccgactgttaccccggttccaagcctagaggctccttccgaacaagcaccgactgagcaaaggcctggggtgcaggagtgctaccatggtaatggacagagttatcgaggcacatactccaccactgtcacaggaagaacctgccaagcttggtcatctatgacaccacactcgcatagtcggaccccagaatactacccaaatgctggcttgatcatgaactactgcaggaatccagatgctgtggcagctccttattgttatacgagggatcccggtgtcaggtgggagtactgcaacctgacgcaatgctcagacgcagaagggactgccgtcgcgcctccgactgttaccccggttccaagcctagaggctccttccgaacaagcaccgactgagcagaggcctggggtgcaggagtgctaccacggtaatggacagagttatcgaggcacatactccaccactgtcactggaagaacctgccaagcttggtcatctatgacaccacactcgcatagtcggaccccagaatactacccaaatgctggcttgatcatgaactactgcaggaatccagatgctgtggcagctccttattgttatacgagggatcccggtgtcaggtgggagtactgcaacctgacgcaatgctcagacgcagaagggactgccgtcgcgcctccgactgttaccccggttccaagcctagaggctccttccgaacaagcaccgactgagcaaaggcctggggtgcaggagtgctaccatggtaatggacagagttatcgaggcacatactccaccactgtcacaggaagaacctgccaagcttggtcatctatgacaccacactcgcatagtcggaccccagaatactacccaaatgctggcttgatcatgaactactgcaggaatccagatgctgtggcagctccttattgttatacgagggatcccggtgtcaggtgggagtactgcaacctgacgcaatgctcagacgcagaagggactgccgtcgcgcctccgactgttaccccggttccaagcctagaggctccttccgaacaagcaccgactgagcaaaggcctggggtgcaggagtgctaccatggtaatggacagagttatcgaggcacatactccaccactgtcacaggaagaacctgccaagcttggtcatctatgacaccacactcgcatagtcggaccccagaatactacccaaatgctggcttgatcatgaactactgcaggaatccagatgctgtggcagctccttattgttatacgagggatcccggtgtcaggtgggagtactgcaacctgacgcaatgctcagacgcagaagggactgccgtcgcgcctccgactgttaccccggttccaagcctagaggctccttccgaacaagcaccgactgagcagaggcctggggtgcaggagtgctaccacggtaatggacagagttatcgaggcacatactccaccactgtcactggaagaacctgccaagcttggtcatctatgacaccacactcgcatagtcggaccccagaatactacccaaatgctggcttgatcatgaactactgcaggaatccagatgctgtggcagctccttattgttatacgagggatcccggtgtcaggtgggagtactgcaacctgacgcaatgctcagacgcagaagggactgccgtcgcgcctccgactgttaccccggttccaagcctagaggctccttccgaacaagcaccgactgagcagaggcctggggtgcaggagtgctaccacggtaatggacagagttatcgaggcacatactccaccactgtcactggaagaacctgccaagcttggtcatctatgacaccacactcgcatagtcggaccccagaatactacccaaatgctggcttgatcatgaactactgcaggaatccagatgctgtggcagctccttattgttatacgagggatcccggtgtcaggtgggagtactgcaacctgacgcaatgctcagacgcagaagggactgccgtcgcgcctccgactgttaccccggttccaagcctagaggctccttccgaacaagcaccgactgagcagaggcctggggtgcaggagtgctaccacggtaatggacagagttatcgaggcacatactccaccactgtcactggaagaacctgccaagcttggtcatctatgacaccacactcgcatagtcggaccccagaatactacccaaatgctggcttgatcatgaactactgcaggaatccagatgctgtggcagctccttattgttatacgagggatcccggtgtcaggtgggagtactgcaacctgacgcaatgctcagacgcagaagggactgccgtcgcgcctccgactgttaccccggttccaagcctagaggctccttccgaacaagcaccgactgagcagaggcctggggtgcaggagtgctaccacggtaatggacagagttatcgaggcacatactccaccactgtcactggaagaacctgccaagcttggtcatctatgacaccacactcgcatagtcggaccccagaatactacccaaatgctggcttgatcatgaactactgcaggaatccagatcctgtggcagccccttattgttatacgagggatcccagtgtcaggtgggagtactgcaacctgacacaatgctcagacgcagaagggactgccgtcgcgcctccaactattaccccgattccaagcctagaggctccttctgaacaagcaccaactgagcaaaggcctggggtgcaggagtgctaccacggaaatggacagagttatcaaggcacatacttcattactgtcacaggaagaacctgccaagcttggtcatctatgacaccacactcgcatagtcggaccccagcatactacccaaatgctggcttgatcaagaactactgccgaaatccagatcctgtggcagccccttggtgttatacaacagatcccagtgtcaggtgggagtactgcaacctgacacgatgctcagatgcagaatggactgccttcgtccctccgaatgttattctggctccaagcctagaggctttttttgaacaagcactgactgaggaaacccccggggtacaggactgctactaccattatggacagagttaccgaggcacatactccaccactgtcacaggaagaacttgccaagcttggtcatctatgacaccacaccagcatagtcggaccccagaaaactacccaaatgctggcctgaccaggaactactgcaggaatccagatgctgagattcgcccttggtgttacaccatggatcccagtgtcaggtgggagtactgcaacctgacacaatgcctggtgacagaatcaagtgtccttgcaactctcacggtggtcccagatccaagcacagaggcttcttctgaagaagcaccaacggagcaaagccccggggtccaggattgctaccatggtgatggacagagttatcgaggctcattctctaccactgtcacaggaaggacatgtcagtcttggtcctctatgacaccacactggcatcagaggacaacagaatattatccaaatggtggcctgaccaggaactactgcaggaatccagatgctgagattagtccttggtgttataccatggatcccaatgtcagatgggagtactgcaacctgacacaatgtccagtgacagaatcaagtgtccttgcgacgtccacggctgtttctgaacaagcaccaacggagcaaagccccacagtccaggactgctaccatggtgatggacagagttatcgaggctcattctccaccactgttacaggaaggacatgtcagtcttggtcctctatgacaccacactggcatcagagaaccacagaatactacccaaatggtggcctgaccaggaactactgcaggaatccagatgctgagattcgcccttggtgttataccatggatcccagtgtcagatgggagtactgcaacctgacgcaatgtccagtgatggaatcaactctcctcacaactcccacggtggtcccagttccaagcacagagcttccttctgaagaagcaccaactgaaaacagcactggggtccaggactgctaccgaggtgatggacagagttatcgaggcacactctccaccactatcacaggaagaacatgtcagtcttggtcgtctatgacaccacattggcatcggaggatcccattatactatccaaatgctggcctgaccaggaactactgcaggaatccagatgctgagattcgcccttggtgttacaccatggatcccagtgtcaggtgggagtactgcaacctgacacgatgtccagtgacagaatcgagtgtcctcacaactcccacagtggccccggttccaagcacagaggctccttctgaacaagcaccacctgagaaaagccctgtggtccaggattgctaccatggtgatggacggagttatcgaggcatatcctccaccactgtcacaggaaggacctgtcaatcttggtcatctatgataccacactggcatcagaggaccccagaaaactacccaaatgctggcctgaccgagaactactgcaggaatccagattctgggaaacaaccctggtgttacacaaccgatccgtgtgtgaggtgggagtactgcaatctgacacaatgctcagaaacagaatcaggtgtcctagagactcccactgttgttccagttccaagcatggaggctcattctgaagcagcaccaactgagcaaacccctgtggtccggcagtgctaccatggtaatggccagagttatcgaggcacattctccaccactgtcacaggaaggacatgtcaatcttggtcatccatgacaccacaccggcatcagaggaccccagaaaactacccaaatgatggcctgacaatgaactactgcaggaatccagatgccgatacaggcccttggtgttttaccatggaccccagcatcaggtgggagtactgcaacctgacgcgatgctcagacacagaagggactgtggtcgctcctccgactgtcatccaggttccaagcctagggcctccttctgaacaagactgtatgtttgggaatgggaaaggataccggggcaagaaggcaaccactgttactgggacgccatgccaggaatgggctgcccaggagccccatagacacagcacgttcattccagggacaaataaatgggcaggtctggaaaaaaattactgccgtaaccctgatggtgacatcaatggtccctggtgctacacaatgaatccaagaaaactttttgactactgtgatatccctctctgtgcatcctcttcatttgattgtgggaagcctcaagtggagccgaagaaatgtcctggaagcattgtaggggggtgtgtggcccacccacattcctggccctggcaagtcagtctcagaacaaggtttggaaagcacttctgtggaggcaccttaatatccccagagtgggtgctgactgctgctcactgcttgaagaagtcctcaaggccttcatcctacaaggtcatcctgggtgcacaccaagaagtgaacctcgaatctcatgttcaggaaatagaagtgtctaggctgttcttggagcccacacaagcagatattgccttgctaaagctaagcaggcctgccgtcatcactgacaaagtaatgccagcttgtctgccatccccagactacatggtcaccgccaggactgaatgttacatcactggctggggagaaacccaaggtacctttgggactggccttctcaaggaagcccagctccttgttattgagaatgaagtgtgcaatcactataagtatatttgtgctgagcatttggccagaggcactgacagttgccagggtgacagtggagggcctctggtttgcttcgagaaggacaaatacattttacaaggagtcacttcttggggtcttggctgtgcacgccccaataagcctggtgtctatgctcgtgtttcaaggtttgttacttggattgagggaatgatgagaaataattaattggacgggagacagagtgaagcatcaacctacttagaagctgaaacgtgggtaaggatttagcatgctggaaataatagacagcaatcaaacgaagacactgttcccagctaccagctatgccaaaccttggcatttttggtatttttgtgtataagcttttaaggtctgactgacaaattctgtattaaggtgtcatagctatgacatttgttaaaaataaactctgcacttattttgatttga

SEQ ID NO: 5 - DNA, 533 bp, Homo sapiens
tgctcagttcatccctagaggcagctgctccaggaacagaggtgccatgcagccccgggtactccttgttgttgccctcctggcgctcctggcctctgcccgagcttcagaggccgaggatgcctcccttctcagcttcatgcagggttacatgaagcacgccaccaagaccgccaaggatgcactgagcagcgtgcaggagtcccaggtggcccagcaggccaggggctgggtgaccgatggcttcagttccctgaaagactactggagcaccgttaaggacaagttctctgagttctgggatttggaccctgaggtcagaccaacttcagccgtggctgcctgagacctcaataccccaagtccacctgcctatccatcctgcgagctccttgggtcctgcaatctccagggctgcccctgtaggttgcttaaaagggacagtattctcagtgctctcctaccccacctcatgcctggcccccctccaggcatgctggcctcccaataaagctggacaagaagctgctatg

SEQ ID NO: 6 - DNA, 3964 bp, Homo sapiens
ctactccaggctgtgttcagggcttggggctggtggagggaggggcctgaaattccagtgtgaaaggctgagatgggcccgaggcccctggcctatgtccaagccatttcccctctcaccagcctctccctggggagccagtcagctaggaaggaatgagggctccccaggcccacccccagttcctgagctcatctgggctgcagggctggcgggacagcagcgtggactcagtctcctagggatttcccaactctcccgcccgcttgctgcatctggacaccctgcctcaggccctcatctccactggtcagcaggtgacctttgcccagcgccctgggtcctcagtgcctgctgccctggagatgatataaaacaggtcagaaccctcctgcctgtctgctcagttcatccctagaggcagctgctccaggtaatgccctctggggaggggaaagaggaggggaggaggatgaagaggggcaagaggagctccctgcccagcccagccagcaagcctggagaagcacttgctagagctaaggaagcctcggagctggacgggtgccccccacccctcatcataacctgaagaacatggaggcccgggaggggtgtcacttgcccaaagctacacagggggtggggctggaagtggctccaagtgcaggttcccccctcattcttcaggcttagggctggaggaagccttagacagcccagtcctaccccagacagggaaactgaggcctggagagggccagaaatcacccaaagacacacagcatgttggctggactggacggagatcagtccagaccgcaggtgccttgatgttcagtctggtgggttttctgctccatcccacccacctccctttgggcctcgatccctcgcccctcaccagtcccccttctgagagcccgtattagcagggagccggcccctactccttctggcagacccagctaaggttctaccttaggggccacgccacctccccagggaggggtccagaggcatggggacctggggtgcccctcacaggacacttccttgcaggaacagaggtgccatgcagccccgggtactccttgttgttgccctcctggcgctcctggcctctgcccgtaagcacttggtgggactgggctgggggcagggtggaggcaacttggggatcccagtcccaatgggtggtcaagcaggagcccagggctcgtccagaggccgatccaccccactcagccctgctctttcctcaggagcttcagaggccgaggatgcctcccttctcagcttcatgcagggttacatgaagcacgccaccaagaccgccaaggatgcactgagcagcgtgcaggagtcccaggtggcccagcaggccaggtacacccgctggcctccctccccatcccccctgccagctgcctccattcccacccgcccctgccctggtgagatcccaacaatggaatggaggtgctccagcctcccctgggcctgtgcctcttcagcctcctctttcctcacagggcctttgtcaggctgctgcgggagagatgacagagttgagactgcattcctcccaggtccctcctttctccccggagcagtcctagggcgtgccgttttagccctcatttccattttcctttcctttccctttctttctctttctatttctttctttctttctttctttctttctttctttctttctttctttctttctttctttctttctttcctttctttctttcctttctttctttcctttctttctttctttcctttctttctctttctttctttctttcctttttctttctttccctctcttcctttctctctttctttcttcttcttttttttttaatggagtctccctctgtcacctaggctggagtgcagtggtgccatctcggctcactgcaacctccgtctcccgggttcaacccattctcctgcctcagcctcccaagtagctgggattacaggcacgcgccaccacacccagctaatttttgtatttttagcagagatggggtttcaccatgttggccaggttggtcttgaattcctgacctcaggggatcctcctgcctcggcctcccaaagtgctgggattacaggcatgagccactgcgcctggccccattttccttttctgaaggtctggctagagcagtggtcctcagcctttttggcaccagggaccagttttgtggtggacaatttttccatgggccagcggggatggttttgggatgaagctgttccacctcagatcatcaggcattagattctcataaggagccctccacctagatccctggcatgtgcagttcacaatagggttcacactcctatgagaatgtaaggccacttgatctgacaggaggcggagctcaggcggtattgctcactcacccaccactcacttcgtgctgtgcagcccggctcctaacagtccatggaccagtacctatctatgacttgggggttggggacccctgggctaggggtttgccttgggaggccccacctgacccaattcaagcccgtgagtgcttctgctttgttctaagacctggggccagtgtgagcagaagtgtgtccttcctctcccatcctgcccctgcccatcagtactctcctctcccctactcccttctccacctcaccctgactggcattagctggcatagcagaggtgttcataaacattcttagtccccagaaccggctttggggtaggtgttattttctcactttgcagatgagaaaattgaggctcagagcgattaggtgacctgccccagatcacacaactaatcaatcctccaatgactttccaaatgagaggctgcctccctctgtcctaccctgctcagagccaccaggttgtgcaactccaggcggtgctgtttgcacagaaaacaatgacagccttgacctttcacatctccccaccctgtcactttgtgcctcaggcccaggggcataaacatctgaggtgacctggagatggcagggtttgacttgtgctggggttcctgcaaggatatctcttctcccagggtggcagctgtgggggattcctgcctgaggtctcagggctgtcgtccagtgaagttgagagggtggtgtggtcctgactggtgtcgtccagtggggacatgggtgtgggtcccatggttgcctacagaggagttctcatgccctgctctgttgcttcccctgactgatttaggggctgggtgaccgatggcttcagttccctgaaagactactggagcaccgttaaggacaagttctctgagttctgggatttggaccctgaggtcagaccaacttcagccgtggctgcctgagacctcaataccccaagtccacctgcctatccatcctgcgagctccttgggtcctgcaatctccagggctgcccctgtaggttgcttaaaagggacagtattctcagtgctctcctaccccacctcatgcctggcccccctccaggcatgctggcctcccaataaagctggacaagaagctgctatgagtgggccgtcgcaagtgtgccatctgtgtctgggcatgggaaagggccgaggctgttctgtgggtgggcactggacagactccaggtcaggcaggcatggaggccagcgctctatccaccttctggtagctgggcagtctctgggcctcagtttcttcatctctaaggtaggaatcaccctccgtaccctgccttccttgacagctttgtgcggaaggtcaaacaggacaataagtttgctgatactttgataaactgttaggtgctgcacaacatgacttgagtgtgtgccccatgccagccactatgcctggcacttaagttgtcatcagagttgagactgtgtgtgtttactcaaaactgtggagctgacctcccctatccaggccccctagccct

SEQ ID NO: 7 - DNA, 20 bp, Artificial sequence
  Synthetic oligonucleotide
tgctccgttggtgcttgttc

SEQ ID NO: 8 - DNA, 20 bp, Artificial sequence
  Synthetic oligonucleotide
tcttcctgtgacagtggtgg

SEQ ID NO: 9 - DNA, 20 bp, Artificial sequence
  Synthetic oligonucleotide
ttcttcctgtgacagtggtg

SEQ ID NO: 10 - DNA, 20 bp, Artificial sequence
  Synthetic oligonucleotide
ggttcttcctgtgacagtgg

SEQ ID NO: 11 - DNA, 20 bp, Artificial sequence
  Synthetic oligonucleotide
cgactatgcgagtgtggtgt

SEQ ID NO: 12 - DNA, 20 bp, Artificial sequence
  Synthetic oligonucleotide
ccgactatgcgagtgtggtg

SEQ ID NO: 13 - DNA, 20 bp, Artificial sequence
  Synthetic oligonucleotide
agcttcttgtccagctttat